European Patent Application EP 4 541 896 A1, published April 23, 2025. Title: Ｇタンパク質共役型受容体の解析方法. Applicant: 花王株式会社. The sequence listing filed with the application follows.

SEQUENCE LISTING (317 sequences)

SEQ ID NO: 1 - protein, 353 aa, Homo sapiens
MVGDTLKLLSPLMTRYFFLLFYSTDSSDLNENQHPLDFDEMAFGKVKSGISFLIQTGVGILGNSFLLCFYNLILFTGHKLRPTDLILSQLALANSMVLFFKGIPQTMAAFGLKYLLNDTGCKFVFYYHRVGTRVSLSTICLLNGFQAIKLNPSICRWMEIKIRSPRFIDFCCLLCWAPHVLMNASVLLLVNGPLNSKNSSAKNNYGYCSYKASKRFSSLHAVLYFSPDFMSLGFMVWASGSMVFFLYRHKQQVQHNHSNRLSCRPSQEARATHTIMVLVSSFFVFYSVHSFLTIWTTVVANPGQWIVTNSVLVASCFPARSPFVLIMSDTHISQFCFACRTRKTLFPNLVVMP

SEQ ID NO: 2 - protein, 395 aa, Homo sapiens
MTHTLYPTPFALYPINISAAWHLGPLPVSCFVSNKYQCSLAFGATTGLRVLVVVVPQTQLSFLSSLCLVSLFLHSLVSAHGEKPTKPVGLDPTLFQVVVGILGNFSLLYYYMFLYFRGYKPRSTDLILRHLTVADSLVILSKRIPETMATFGLKHFDNYFGCKFLLYAHRVGRGVSIGSTCLLSVFQVITINPRNSRWAEMKVKAPTYIGLSNILCWAFHMLVNAIFPIYTTGKWSNNNITKKGDLGYCSAPLSDEVTKSVYAALTSFHDVLCLGLMLWASSSIVLVLYRHKQQVQHICRNNLYPNSSPGNRAIQSILALVSTFALCYALSFITYVYLALFDNSSWWLVNTAALIIACFPTISPFVLMCRDPSRSRLCSICCRRNRRFFHDFRKM

SEQ ID NO: 3 - protein, 301 aa, Homo sapiens
MASRYVAVGMILSQTVVGVLGSFSVLLHYLSFYCTGCRLRSTDLIVKHLIVANFLALRCKGVPQTMAAFGVRYFLNALGCKLVFYLHRVGRGVSIGTTCLLSVFQVITVSSRKSRWAKLKEKAPKHVGFSVLLCWIVCMLVNIIFPMYVTGKWNYTNITVNEDLGYCSGGGNNKIAQTLRAMLLSFPDVLCLGLMLWVSSSMVCILHRHKQRVQHIDRSNLSPRASPENRATQSILILVSTFVSSYTLSCLFQVCMALLDNPNSLLVNTSALMSVCFPTLSPFVLMSCDPSVYRFCFAWKR

SEQ ID NO: 4 - protein, 357 aa, Homo sapiens
MLKLVIIENMAEIMLFSLDLLLFSTDILCFNFPSKMIKLPGFITIQIFFYPQASFGISANTILLLFHIFTFVFSHRSKSIDMIISHLSLIHILLLFTQAILVSLDFFGSQNTQDDLRYKVIVFLNKVMRGLSICTPCLLSVLQAIISPSIFSLAKLKHPSASHILGFFLFSWVLNMFIGVIFCCTLRLPPVKRGQSSVCHTALFLFAHELHPQETVFHTNDFEGCHLYRVHGPLKRLHGDYFIQTIRGYLSAFTQPACPRVSPVKRASQAILLLVSFVFTYWVDFTFSFSGGVTWINDSLLVWLQVIVANSYAAISPLMLIYADNQIFKTLQMLWFKYLSPPKLMLKFNRQCGSTKK

SEQ ID NO: 5 - protein, 841 aa, Homo sapiens
MLLCTARLVGLQLLISCCWAFACHSTESSPDFTLPGDYLLAGLFPLHSGCLQVRHRPEVTLCDRSCSFNEHGYHLFQAMRLGVEEINNSTALLPNITLGYQLYDVCSDSANVYATLRVLSLPGQHHIELQGDLLHYSPTVLAVIGPDSTNRAATTAALLSPFLVPMISYAASSETLSVKRQYPSFLRTIPNDKYQVETMVLLLQKFGWTWISLVGSSDDYGQLGVQALENQATGQGICIAFKDIMPFSAQVGDERMQCLMRHLAQAGATVVVVFSSRQLARVFFESVVLTNLTGKVWVASEAWALSRHITGVPGIQRIGMVLGVAIQKRAVPGLKAFEEAYARADKKAPRPCHKGSWCSSNQLCRECQAFMAHTMPKLKAFSMSSAYNAYRAVYAVAHGLHQLLGCASGACSRGRVYPWQLLEQIHKVHFLLHKDTVAFNDNRDPLSSYNIIAWDWNGPKWTFTVLGSSTWSPVQLNINETKIQWHGKDNQVPKSVCSSDCLEGHQRVVTGFHHCCFECVPCGAGTFLNKSDLYRCQPCGKEEWAPEGSQTCFPRTVVFLALREHTSWVLLAANTLLLLLLLGTAGLFAWHLDTPVVRSAGGRLCFLMLGSLAAGSGSLYGFFGEPTRPACLLRQALFALGFTIFLSCLTVRSFQLIIIFKFSTKVPTFYHAWVQNHGAGLFVMISSAAQLLICLTWLVVWTPLPAREYQRFPHLVMLECTETNSLGFILAFLYNGLLSISAFACSYLGKDLPENYNEAKCVTFSLLFNFVSWIAFFTTASVYDGKYLPAANMMAGLSSLSSGFGGYFLPKCYVILCRPDLNSTEHFQASIQDYTRRCGST

SEQ ID NO: 6 - protein, 839 aa, Homo sapiens
MGPRAKTISSLFFLLWVLAEPAENSDFYLPGDYLLGGLFSLHANMKGIVHLNFLQVPMCKEYEVKVIGYNLMQAMRFAVEEINNDSSLLPGVLLGYEIVDVCYISNNVQPVLYFLAHEDNLLPIQEDYSNYISRVVAVIGPDNSESVMTVANFLSLFLLPQITYSAISDELRDKVRFPALLRTTPSADHHIEAMVQLMLHFRWNWIIVLVSSDTYGRDNGQLLGERVARRDICIAFQETLPTLQPNQNMTSEERQRLVTIVDKLQQSTARVVVVFSPDLTLYHFFNEVLRQNFTGAVWIASESWAIDPVLHNLTELRHLGTFLGITIQSVPIPGFSEFREWGPQAGPPPLSRTSQSYTCNQECDNCLNATLSFNTILRLSGERVVYSVYSAVYAVAHALHSLLGCDKSTCTKRVVYPWQLLEEIWKVNFTLLDHQIFFDPQGDVALHLEIVQWQWDRSQNPFQSVASYYPLQRQLKNIQDISWHTINNTIPMSMCSKRCQSGQKKKPVGIHVCCFECIDCLPGTFLNHTEDEYECQACPNNEWSYQSETSCFKRQLVFLEWHEAPTIAVALLAALGFLSTLAILVIFWRHFQTPIVRSAGGPMCFLMLTLLLVAYMVVPVYVGPPKVSTCLCRQALFPLCFTICISCIAVRSFQIVCAFKMASRFPRAYSYWVRYQGPYVSMAFITVLKMVIVVIGMLATGLSPTTRTDPDDPKITIVSCNPNYRNSLLFNTSLDLLLSVVGFSFAYMGKELPTNYNEAKFITLSMTFYFTSSVSLCTFMSAYSGVLVTIVDLLVTVLNLLAISLGYFGPKCYMILFYPERNTPAYFNSMIQGYTMRRD

SEQ ID NO: 7 - protein, 852 aa, Homo sapiens
MLGPAVLGLSLWALLHPGTGAPLCLSQQLRMKGDYVLGGLFPLGEAEEAGLRSRTRPSSPVCTRFSSNGLLWALAMKMAVEEINNKSDLLPGLRLGYDLFDTCSEPVVAMKPSLMFLAKAGSRDIAAYCNYTQYQPRVLAVIGPHSSELAMVTGKFFSFFLMPQVSYGASMELLSARETFPSFFRTVPSDRVQLTAAAELLQEFGWNWVAALGSDDEYGRQGLSIFSALAAARGICIAHEGLVPLPRADDSRLGKVQDVLHQVNQSSVQVVLLFASVHAAHALFNYSISSRLSPKVWVASEAWLTSDLVMGLPGMAQMGTVLGFLQRGAQLHEFPQYVKTHLALATDPAFCSALGEREQGLEEDVVGQRCPQCDCITLQNVSAGLNHHQTFSVYAAVYSVAQALHNTLQCNASGCPAQDPVKPWQLLENMYNLTFHVGGLPLRFDSSGNVDMEYDLKLWVWQGSVPRLHDVGRFNGSLRTERLKIRWHTSDNQKPVSRCSRQCQEGQVRRVKGFHSCCYDCVDCEAGSYRQNPDDIACTFCGQDEWSPERSTRCFRRRSRFLAWGEPAVLLLLLLLSLALGLVLAALGLFVHHRDSPLVQASGGPLACFGLVCLGLVCLSVLLFPGQPSPARCLAQQPLSHLPLTGCLSTLFLQAAEIFVESELPLSWADRLSGCLRGPWAWLVVLLAMLVEVALCTWYLVAFPPEVVTDWHMLPTEALVHCRTRSWVSFGLAHATNATLAFLCFLGTFLVRSQPGCYNRARGLTFAMLAYFITWVSFVPLLANVQVVLRPAVQMGALLLCVLGILAAFHLPRCYLLMRQPGLNTPEFFLGGGPGDAQGQNDGNTGNQGKHE

SEQ ID NO: 8 - protein, 309 aa, Homo sapiens
MFSPADNIFIILITGEFILGILGNGYIALVNWIDWIKKKKISTVDYILTNLVIARICLISVMVVNGIVIVLNPDVYTKNKQQIVIFTFWTFANYLNMWITTCLNVFYFLKIASSSHPLFLWLKWKIDMVVHWILLGCFAISLLVSLIAAIVLSCDYRFHAIAKHKRNITEMFHVSKIPYFEPLTLFNLFAIVPFIVSLISFFLLVRSLWRHTKQIKLYATGSRDPSTEVHVRAIKTMTSFIFFFFLYYISSILMTFSYLMTKYKLAVEFGEIAAILYPLGHSLILIVLNNKLRQTFVRMLTCRKIACMI

SEQ ID NO: 9 - protein, 291 aa, Homo sapiens
MIPIQLTVFFMIIYVLESLTIIVQSSLIVAVLGREWLQVRRLMPVDMILISLGISRFCLQWASMLNNFCSYFNLNYVLCNLTITWEFFNILTFWLNSLLTVFYCIKVSSFTHHIFLWLRWRILRLFPWILLGSLMITCVTIIPSAIGNYIQIQLLTMEHLPRNSTVTDKLENFHQYQFQAHTVALVIPFILFLASTIFLMASLTKQIQHHSTGHCNPSMKARFTALRSLAVLFIVFTSYFLTILITIIGTLFDKRCWLWVWEAFVYAFILMHSTSLMLSSPTLKRILKGKC

SEQ ID NO: 10 - protein, 333 aa, Homo sapiens
MLTLTRIRTVSYEVRSTFLFISVLEFAVGFLTNAFVFLVNFWDVVKRQALSNSDCVLLCLSISRLFLHGLLFLSAIQLTHFQKLSEPLNHSYQAIIMLWMIANQANLWLAACLSLLYCSKLIRFSHTFLICLASWVSRKISQMLLGIILCSCICTVLCVWCFFSRPHFTVTTVLFMNNNTRLNWQIKDLNLFYSFLFCYLWSVPPFLLFLVSSGMLTVSLGRHMRTMKVYTRNSRDPSLEAHIKALKSLVSFFCFFVISSCAAFISVPLLILWRDKIGVMVCVGIMAACPSGHAAILISGNAKLRRAVMTILLWAQSSLKVRADHKADSRTLC

SEQ ID NO: 11 - protein, 314 aa, Homo sapiens
MATELDKIFLILAIAEFIISMLGNVFIGLVNCSEGIKNQKVFSADFILTCLAISTIGQLLVILFDSFLVGLASHLYTTYRLGKTVIMLWHMTNHLTTWLATCLSIFYFFKIAHFPHSLFLWLRWRMNGMIVMLLILSLFLLIFDSLVLEIFIDISLNIIDKSNLTLYLDESKTLYDKLSILKTLLSLTSFIPFSLFLTSLLFLFLSLVRHTRNLKLSSLGSRDSSTEAHRRAMKMVMSFLFLFIVHFFSLQVANWIFFMLWNNKCIKFVMLALNAFPSCHSFILILGNSKLQQTAVRLLWHLRNYTKTPNPLPL

SEQ ID NO: 12 - protein, 299 aa, Homo sapiens
MITFLPIIFSILVVVTFVIGNFANGFIALVNSTEWVKRQKISFADQIVTALAVSRVGLLWVLLLNWYSTVLNPAFYSVELRTTAYNIWAVTGHFSNWPATSLSIFYLLKIANFSNLIFLRLKRRVKSVILVVLLGPLLFLACHLFVVNMNQIVWTKEYEGNMTWKIKLRRAMYLSDTTVTMLANLVPFTVTLISFLLLVCSLCKHLKKMQLHGKGSQDPSTKVHIKVLQTVISFFLLRAIYFVSVIISVWSFKNLENKPVFMFCQAIGFSCSSAHPFILIWGNKKLKQTYLSVLWQMRY

SEQ ID NO: 13 - protein, 309 aa, Homo sapiens
MITFLPIIFSILIVVTFVIGNFANGFIALVNSIEWFKRQKISFADQILTALAVSRVGLLWVLVLNWYATELNPAFNSIEVRITAYNVWAVINHFSNWLATSLSIFYLLKIANFSNLIFLHLKRRVKSVVLVILLGPLLFLVCHLFVINMNQIIWTKEYEGNMTWKIKLRSAMYLSNTTVTILANLVPFTLTLISFLLLICSLCKHLKKMQLHGKGSQDPSMKVHIKALQTVTSFLLLCAIYFLSIIMSVWSFESLENKPVFMFCEAIAFSYPSTHPFILIWGNKKLKQTFLSVLWHVRYWVKGEKPSSS

SEQ ID NO: 14 - protein, 309 aa, Homo sapiens
MTTFIPIIFSSVVVVLFVIGNFANGFIALVNSIERVKRQKISFADQILTALAVSRVGLLWVLLLNWYSTVFNPAFYSVEVRTTAYNVWAVTGHFSNWLATSLSIFYLLKIANFSNLIFLHLKRRVKSVILVMLLGPLLFLACQLFVINMKEIVRTKEYEGNLTWKIKLRSAVYLSDATVTTLGNLVPFTLTLLCFLLLICSLCKHLKKMQLHGKGSQDPSTKVHIKALQTVIFFLLLCAVYFLSIMISVWSFGSLENKPVFMFCKAIRFSYPSIHPFILIWGNKKLKQTFLSVLRQVRYWVKGEKPSSP

SEQ ID NO: 15 - protein, 259 aa, Homo sapiens
MAPLDLLLSCLAVSRIFLQLFIFYVNVIVIFFIEFIMCSANCAILLFINELELWLATWLGVFYCAKVASVRHPLFIWLKMRISKLVPWMILGSLLYVSMICVFHSKYAGFMVPYFLRKFFSQNATIQKEDTLAIQIFSFVAEFSVPLLIFLFAVLLLIFSLGRHTRQMRNTVAGSRVPGRGAPISALLSILSFLILYFSHCMIKVFLSSLKFHIRRFIFLFFILVIGIYPSGHSLILILGNPKLKQNAKKFLLHSKCCQ

SEQ ID NO: 16 - protein, 316 aa, Homo sapiens
MMGLTEGVFLILSGTQFTLGILVNCFIELVNGSSWFKTKRMSLSDFIITTLALLRIILLCIILTDSFLIEFSPNTHDSGIIMQIIDVSWTFTNHLSIWLATCLGVLYCLKIASFSHPTFLWLKWRVSRVMVWMLLGALLLSCGSTASLINEFKLYSVFRGIEATRNVTEHFRKKRSEYYLIHVLGTLWYLPPLIVSLASYSLLIFSLGRHTRQMLQNGTSSRDPTTEAHKRAIRIILSFFFLFLLYFLAFLIASFGNFLPKTKMAKMIGEVMTMFYPAGHSFILILGNSKLKQTFVVMLRCESGHLKPGSKGPIFS

SEQ ID NO: 17 - protein, 299 aa, Homo sapiens
MLRLFYFSAIIASVILNFVGIIMNLFITVVNCKTWVKSHRISSSDRILFSLGITRFLMLGLFLVNTIYFVSSNTERSVYLSAFFVLCFMFLDSSSVWFVTLLNILYCVKITNFQHSVFLLLKRNISPKIPRLLLACVLISAFTTCLYITLSQASPFPELVTTRNNTSFNISEGILSLVVSLVLSSSLQFIINVTSASLLIHSLRRHIQKMQKNATGFWNPQTEAHVGAMKLMVYFLILYIPYSVATLVQYLPFYAGMDMGTKSICLIFATLYSPGHSVLIIITHPKLKTTAKKILCFKK

SEQ ID NO: 18 - protein, 299 aa, Homo sapiens
MLSAGLGLLMLVAVVEFLIGLIGNGSLVVWSFREWIRKFNWSSYNLIILGLAGCRFLLQWLIILDLSLFPLFQSSRWLRYLSIFWVLVSQASLWFATFLSVFYCKKITTFDRPAYLWLKQRAYNLSLWCLLGYFIINLLLTVQIGLTFYHPPQGNSSIRYPFESWQYLYAFQLNSGSYLPLVVFLVSSGMLIVSLYTHHKKMKVHSAGRRDVRAKAHITALKSLGCFLLLHLVYIMASPFSITSKTYPPDLTSVFIWETLMAAYPSLHSLILIMGIPRVKQTCQKILWKTVCARRCWGP

SEQ ID NO: 19 - protein, 318 aa, Homo sapiens
MADKVQTTLLFLAVGEFSVGILGNAFIGLVNCMDWVKKRKIASIDLILTSLAISRICLLCVILLDCFILVLYPDVYATGKEMRIIDFFWTLTNHLSIWFATCLSIYYFFKIGNFFHPLFLWMKWRIDRVISWILLGCVVLSVFISLPATENLNADFRFCVKAKRKTNLTWSCRVNKTQHASTKLFLNLATLLPFCVCLMSFFLLILSLRRHIRRMQLSATGCRDPSTEAHVRALKAVISFLLLFIAYYLSFLIATSSYFMPETELAVIFGESIALIYPSSHSFILILGNNKLRHASLKVIWKVMSILKGRKFQQHKQI

SEQ ID NO: 20 - protein, 312 aa, Homo sapiens
MPSAIEAIYIILIAGELTIGIWGNGFIVLVNCIDWLKRRDISLIDIILISLAISRICLLCVISLDGFFMLLFPGTYGNSVLVSIVNVVWTFANNSSLWFTSCLSIFYLLKIANISHPFFFWLKLKINKVMLAILLGSFLISLIISVPKNDDMWYHLFKVSHEENITWKFKVSKIPGTFKQLTLNLGVMVPFILCLISFFLLLFSLVRHTKQIRLHATGFRDPSTEAHMRAIKAVIIFLLLLIVYYPVFLVMTSSALIPQGKLVLMIGDIVTVIFPSSHSFILIMGNSKLREAFLKMLRFVKCFLRRRKPFVP

SEQ ID NO: 21 - protein, 307 aa, Homo sapiens
MLRVVEGIFIFVVVSESVFGVLGNGFIGLVNCIDCAKNKLSTIGFILTGLAISRIFLIWIIITDGFIQIFSPNIYASGNLIEYISYFWVIGNQSSMWFATSLSIFYFLKIANFSNYIFLWLKSRTNMVLPFMIVFLLISSLLNFAYIAKILNDYKTKNDTVWDLNMYKSEYFIKQILLNLGVIFFFTLSLITCIFLIISLWRHNRQMQSNVTGLRDSNTEAHVKAMKVLISFIILFILYFIGMAIEISCFTVRENKLLLMFGMTTTAIYPWGHSFILILGNSKLKQASLRVLQQLKCCEKRKNLRVT

SEQ ID NO: 22 - protein, 303 aa, Homo sapiens
MESALPSIFTLVIIAEFIIGNLSNGFIVLINCIDWVSKRELSSVDKLLIILAISRIGLIWEILVSWFLALHYLAIFVSGTGLRIMIFSWIVSNHFNLWLATIFSIFYLLKIASFSSPAFLYLKWRVNKVILMILLGTLVFLFLNLIQINMHIKDWLDRYERNTTWNFSMSDFETFSVSVKFTMTMFSLTPFTVAFISFLLLIFSLQKHLQKMQLNYKGHRDPRTKVHTNALKIVISFLLFYASFFLCVLISWISELYQNTVIYMLCETIGVFSPSSHSFLLILGNAKLRQAFLLVAAKVWAKR

SEQ ID NO: 23 - protein, 317 aa, Homo sapiens
MGGVIKSIFTFVLIVEFIIGNLGNSFIALVNCIDWVKGRKISSVDRILTALAISRISLVWLIFGSWCVSVFFPALFATEKMFRMLTNIWTVINHFSVWLATGLGTFYFLKIANFSNSIFLYLKWRVKKVVLVLLLVTSVFLFLNIALINIHINASINGYRRNKTCSSDSSNFTRFSSLIVLTSTVFIFIPFTLSLAMFLLLIFSMWKHRKKMQHTVKISGDASTKAHRGVKSVITFFLLYAIFSLSFFISVWTSERLEENLIILSQVMGMAYPSCHSCVLILGNKKLRQASLSVLLWLRYMFKDGEPSGHKEFRESS

SEQ ID NO: 24 - protein, 309 aa, Homo sapiens
MMSFLHIVFSILVVVAFILGNFANGFIALINFIAWVKRQKISSADQIIAALAVSRVGLLWVILLHWYSTVLNPTSSNLKVIIFISNAWAVTNHFSIWLATSLSIFYLLKIVNFSRLIFHHLKRKAKSVVLVIVLGSLFFLVCHLVMKHTYINVWTEECEGNVTWKIKLRNAMHLSNLTVAMLANLIPFTLTLISFLLLIYSLCKHLKKMQLHGKGSQDPSTKIHIKALQTVTSFLILLAIYFLCLIISFWNFKMRPKEIVLMLCQAFGIIYPSFHSFILIWGNKTLKQTFLSVLWQVTCWAKGQNQSTP

SEQ ID NO: 25 - protein, 319 aa, Homo sapiens
MITFLPIIFSILIVVIFVIGNFANGFIALVNSIEWVKRQKISFVDQILTALAVSRVGLLWVLLLHWYATQLNPAFYSVEVRITAYNVWAVTNHFSSWLATSLSMFYLLRIANFSNLIFLRIKRRVKSVVLVILLGPLLFLVCHLFVINMDETVWTKEYEGNVTWKIKLRSAMYHSNMTLTMLANFVPLTLTLISFLLLICSLCKHLKKMQLHGKGSQDPSTKVHIKALQTVTSFLLLCAIYFLSMIISVCNFGRLEKQPVFMFCQAIIFSYPSTHPFILILGNKKLKQIFLSVLRHVRYWVKDRSLRLHRFTRGALCVF

SEQ ID NO: 26 - protein, 338 aa, Homo sapiens
MLGRCFPPDTKEKQQLRMTKLCDPAESELSPFLITLILAVLLAEYLIGIIANGFIMAIHAAEWVQNKAVSTSGRILVFLSVSRIALQSLMMLEITISSTSLSFYSEDAVYYAFKISFIFLNFCSLWFAAWLSFFYFVKIANFSYPLFLKLRWRITGLIPWLLWLSVFISFSHSMFCINICTVYCNNSFPIHSSNSTKKTYLSEINVVGLAFFFNLGIVTPLIMFILTATLLILSLKRHTLHMGSNATGSNDPSMEAHMGAIKAISYFLILYIFNAVALFIYLSNMFDINSLWNNLCQIIMAAYPASHSILLIQDNPGLRRAWKRLQLRLHLYPKEWTL

SEQ ID NO: 27 - protein, 323 aa, Homo sapiens
MATVNTDATDKDISKFKVTFTLVVSGIECITGILGSGFITAIYGAEWARGKTLPTGDRIMLMLSFSRLLLQIWMMLENIFSLLFRIVYNQNSVYILFKVITVFLNHSNLWFAAWLKVFYCLRIANFNHPLFFLMKRKIIVLMPWLLRLSVLVSLSFSFPLSRDVFNVYVNSSIPIPSSNSTEKKYFSETNMVNLVFFYNMGIFVPLIMFILAATLLILSLKRHTLHMGSNATGSRDPSMKAHIGAIKATSYFLILYIFNAIALFLSTSNIFDTYSSWNILCKIIMAAYPAGHSVQLILGNPGLRRAWKRFQHQVPLYLKGQTL

SEQ ID NO: 28 - protein, 309 aa, Homo sapiens
MITFLPIIFSSLVVVTFVIGNFANGFIALVNSIEWFKRQKISFADQILTALAVSRVGLLWVLLLNWYSTVLNPAFNSVEVRTTAYNIWAVINHFSNWLATTLSIFYLLKIANFSNFIFLHLKRRVKSVILVMLLGPLLFLACHLFVINMNEIVRTKEFEGNMTWKIKLKSAMYFSNMTVTMVANLVPFTLTLLSFMLLICSLCKHLKKMQLHGKGSQDPSTKVHIKALQTVISFLLLCAIYFLSIMISVWSFGSLENKPVFMFCKAIRFSYPSIHPFILIWGNKKLKQTFLSVFWQMRYWVKGEKTSSP

SEQ ID NO: 29 - protein, 299 aa, Homo sapiens
MITFLYIFFSILIMVLFVLGNFANGFIALVNFIDWVKRKKISSADQILTALAVSRIGLLWALLLNWYLTVLNPAFYSVELRITSYNAWVVTNHFSMWLAANLSIFYLLKIANFSNLLFLHLKRRVRSVILVILLGTLIFLVCHLLVANMDESMWAEEYEGNMTGKMKLRNTVHLSYLTVTTLWSFIPFTLSLISFLMLICSLCKHLKKMQLHGEGSQDLSTKVHIKALQTLISFLLLCAIFFLFLIVSVWSPRRLRNDPVVMVSKAVGNIYLAFDSFILIWRTKKLKHTFLLILCQIRC

SEQ ID NO: 30 - protein, 318 aa, Homo sapiens
MNGDHMVLGSSVTDKKAIILVTILLLLRLVAIAGNGFITAALGVEWVLRRMLLPCDKLLVSLGASRFCLQSVVMGKTIYVFLHPMAFPYNPVLQFLAFQWDFLNAATLWSSTWLSVFYCVKIATFTHPVFFWLKHKLSGWLPWMLFSSVGLSSFTTILFFIGNHRMYQNYLRNHLQPWNVTGDSIRSYCEKFYLFPLKMITWTMPTAVFFICMILLITSLGRHRKKALLTTSGFREPSVQAHIKALLALLSFAMLFISYFLSLVFSAAGIFPPLDFKFWVWESVIYLCAAVHPIILLFSNCRLRAVLKSRRSSRCGTP

SEQ ID NO: 31 - protein, 339 aa, Homo sapiens
MMPFCHNIINISCVKNNWSNDVRASLYSLMVLIILTTLVGNLIVIVSISHFKQLHTPTNWLIHSMATVDFLLGCLVMPYSMVRSAEHCWYFGEVFCKIHTSTDIMLSSASIFHLSFISIDRYYAVCDPLRYKAKMNILVICVMIFISWSVPAVFAFGMIFLELNFKGAEEIYYKHVHCRGGCSVFFSKISGVLTFMTSFYIPGSIMLCVYYRIYLIAKEQARLISDANQKLQIGLEMKNGISQSKERKAVKTLGIVMGVFLICWCPFFICTVMDPFLHYIIPPTLNDVLIWFGYLNSTFNPMVYAFFYPWFRKALKMMLFGKIFQKDSSRCKLFLELSS

SEQ ID NO: 32 - protein, 351 aa, Homo sapiens
MAVSSEQHELSHFKRTQTKKEKFNCSEYGNRSCPENERSLGVRVAMYSFMAGSIFITIFGNLAMIISISYFKQLHTPTNFLILSMAITDFLLGFTIMPYSMIRSVENCWYFGLTFCKIYYSFDLMLSITSIFHLCSVAIDRFYAICYPLLYSTKITIPVIKRLLLLCWSVPGAFAFGVVFSEAYADGIEGYDILVACSSSCPVMFNKLWGTTLFMAGFFTPGSMMVGIYGKIFAVSRKHAHAINNLRENQNNQVKKDKKAAKTLGIVIGVFLLCWFPCFFTILLDPFLNFSTPVVLFDALTWFGYFNSTCNPLIYGFFYPWFRRALKYILLGKIFSSCFHNTILCMQKESE

SEQ ID NO: 33 - protein, 337 aa, Homo sapiens
MRAVFIQGAEEHPAAFCYQVNGSCPRTVHTLGIQLVIYLACAAGMLIIVLGNVFVAFAVSYFKALHTPTNFLLLSLALADMFLGLLVLPLSTIRSVESCWFFGDFLCRLHTYLDTLFCLTSIFHLCFISIDRHCAICDPLLYPSKFTVRVALRYILAGWGVPAAYTSLFLYTDVVETRLSQWLEEMPCVGSCQLLLNKFWGWLNFPLFFVPCLIMISLYVKIFVVATRQAQQITTLSKSLAGAAKHERKAAKTLGIAVGIYLLCWLPFTIDTMVDSLLHFITPPLVFDIFIWFAYFNSACNPIIYVFSYQWFRKALKLTLSQKVFSPQTRTVDLYQE

SEQ ID NO: 34 - protein, 342 aa, Homo sapiens
MTSNFSQPVVQLCYEDVNGSCIETPYSPGSRVILYTAFSFGSLLAVFGNLLVMTSVLHFKQLHSPTNFLIASLACADFLVGVTVMLFSMVRTVESCWYFGAKFCTLHSCCDVAFCYSSVLHLCFICIDRYIVVTDPLVYATKFTVSVSGICISVSWILPLTYSGAVFYTGVNDDGLEELVSALNCVGGCQIIVSQGWVLIDFLLFFIPTLVMIILYSKIFLIAKQQAIKIETTSSKVESSSESYKIRVAKRERKAAKTLGVTVLAFVISWLPYTVDILIDAFMGFLTPAYIYEICCWSAYYNSAMNPLIYALFYPWFRKAIKLILSGDVLKASSSTISLFLE

SEQ ID NO: 35 - protein, 348 aa, Homo sapiens
MVNNFSQAEAVELCYKNVNESCIKTPYSPGPRSILYAVLGFGAVLAAFGNLLVMIAILHFKQLHTPTNFLIASLACADFLVGVTVMPFSTVRSVESCWYFGDSYCKFHTCFDTSFCFASLFHLCCISVDRYIAVTDPLTYPTKFTVSVSGICIVLSWFFSVTYSFSIFYTGANEEGIEELVVALTCVGGCQAPLNQNWVLLCFLLFFIPNVAMVFIYSKIFLVAKHQARKIESTASQAQSSSESYKERVAKRERKAAKTLGIAMAAFLVSWLPYLVDAVIDAYMNFITPPYVYEILVWCVYYNSAMNPLIYAFFYQWFGKAIKLIVSGKVLRTDSSTTNLFSEEVETD

SEQ ID NO: 36 - protein, 345 aa, Homo sapiens
MSSNSSLLVAVQLCYANVNGSCVKIPFSPGSRVILYIVFGFGAVLAVFGNLLVMISILHFKQLHSPTNFLVASLACADFLVGVTVMPFSMVRTVESCWYFGRSFCTFHTCCDVAFCYSSLFHLCFISIDRYIAVTDPLVYPTKFTVSVSGICISVSWILPLMYSGAVFYTGVYDDGLEELSDALNCIGGCQTVVNQNWVLTDFLSFFIPTFIMIILYGNIFLVARRQAKKIENTGSKTESSSESYKARVARRERKAAKTLGVTVVAFMISWLPYSIDSLIDAFMGFITPACIYEICCWCAYYNSAMNPLIYALFYPWFRKAIKVIVTGQVLKNSSATMNLFSEHI

SEQ ID NO: 37 - protein, 312 aa, Homo sapiens
MMEPREAGQHVGAANGAQEDVAFNLIILSLTEGLGLGGLLGNGAVLWLLSSNVYRNPFAIYLLDVACADLIFLGCHMVAIVPDLLQGRLDFPGFVQTSLATLRFFCYIVGLSLLAAVSVEQCLAALFPAWYSCRRPRHLTTCVCALTWALCLLLHLLLSGACTQFFGEPSRHLCRTLWLVAAVLLALLCCTMCGASLMLLLRVERGPQRPPPRGFPGLILLTVLLFLFCGLPFGIYWLSRNLLWYIPHYFYHFSFLMAAVHCAAKPVVYFCLGSAQGRRLPLRLVLQRALGDEAELGAVRETSRRGLVDIAA

SEQ ID NO: 38 - protein, 343 aa, Homo sapiens
MAGNCSWEAHPGNRNKMCPGLSEAPELYSRGFLTIEQIAMLPPPAVMNYIFLLLCLCGLVGNGLVLWFFGFSIKRNPFSIYFLHLASADVGYLFSKAVFSILNTGGFLGTFADYIRSVCRVLGLCMFLTGVSLLPAVSAERCASVIFPAWYWRRRPKRLSAVVCALLWVLSLLVTCLHNYFCVFLGRGAPGAACRHMDIFLGILLFLLCCPLMVLPCLALILHVECRARRRQRSAKLNHVILAMVSVFLVSSIYLGIDWFLFWVFQIPAPFPEYVTDLCICINSSAKPIVYFLAGRDKSQRLWEPLRVVFQRALRDGAELGEAGGSTPNTVTMEMQCPPGNAS

SEQ ID NO: 39 - protein, 325 aa, Homo sapiens
MDGSNVTSFVVEEPTNISTGRNASVGNAHRQIPIVHWVIMSISPVGFVENGILLWFLCFRMRRNPFTVYITHLSIADISLLFCIFILSIDYALDYELSSGHYYTIVTLSVTFLFGYNTGLYLLTAISVERCLSVLYPIWYRCHRPKYQSALVCALLWALSCLVTTMEYVMCIDREEESHSRNDCRAVIIFIAILSFLVFTPLMLVSSTILVVKIRKNTWASHSSKLYIVIMVTIIIFLIFAMPMRLLYLLYYEYWSTFGNLHHISLLFSTINSSANPFIYFFVGSSKKKRFKESLKVVLTRAFKDEMQPRRQKDNCNTVTVETVV

SEQ ID NO: 40 - protein, 378 aa, Homo sapiens
MVWGKICWFSQRAGWTVFAESQISLSCSLCLHSGDQEAQNPNLVSQLCGVFLQNETNETIHMQMSMAVGQQALPLNIIAPKAVLVSLCGVLLNGTVFWLLCCGATNPYMVYILHLVAADVIYLCCSAVGFLQVTLLTYHGVVFFIPDFLAILSPFSFEVCLCLLVAISTERCVCVLFPIWYRCHRPKYTSNVVCTLIWGLPFCINIVKSLFLTYWKHVKACVIFLKLSGLFHAILSLVMCVSSLTLLIRFLCCSQQQKATRVYAVVQISAPMFLLWALPLSVAPLITDFKMFVTTSYLISLFLIINSSANPIIYFFVGSLRKKRLKESLRVILQRALADKPEVGRNKKAAGIDPMEQPHSTQHVENLLPREHRVDVET

SEQ ID NO: 41 - protein, 321 aa, Homo sapiens
MNQTLNSSGTVESALNYSRGSTVHTAYLVLSSLAMFTCLCGMAGNSMVIWLLGFRMHRNPFCIYILNLAAADLLFLFSMASTLSLETQPLVNTTDKVHELMKRLMYFAYTVGLSLLTAISTQRCLSVLFPIWFKCHRPRHLSAWVCGLLWTLCLLMNGLTSSFCSKFLKFNEDRCFRVDMVQAALIMGVLTPVMTLSSLTLFVWVRRSSQQWRRQPTRLFVVVLASVLVFLICSLPLSIYWFVLYWLSLPPEMQVLCFSLSRLSSSVSSSANPVIYFLVGSRRSHRLPTRSLGTVLQQALREEPELEGGETPTVGTNEMGA

SEQ ID NO: 42 - protein, 289 aa, Homo sapiens
MFGLFGLWRTFDSVVFYLTLIVGLGGPVGNGLVLWNLGFRIKKGPFSIYLLHLAAADFLFLSCRVGFSVAQAALGAQDTLYFVLTFLWFAVGLWLLAAFSVERCLSDLFPACYQGCRPRHASAVLCALVWTPTLPAVPLPANACGLLRNSACPLVCPRYHVASVTWFLVLARVAWTAGVVLFVWVTCCSTRPRPRLYGIVLGALLLLFFCGLPSVFYWSLQPLLNFLLPVFSPLATLLACVNSSSKPLIYSGLGRQPGKREPLRSVLRRALGEGAELGARGQSLPMGLL

SEQ ID NO: 43 - protein, 322 aa, Homo sapiens
MDPTISTLDTELTPINGTEETLCYKQTLSLTVLTCIVSLVGLTGNAVVLWLLGCRMRRNAFSIYILNLAAADFLFLSGRLIYSLLSFISIPHTISKILYPVMMFSYFAGLSFLSAVSTERCLSVLWPIWYRCHRPTHLSAVVCVLLWALSLLRSILEWMLCGFLFSGADSAWCQTSDFITVAWLIFLCVVLCGSSLVLLIRILCGSRKIPLTRLYVTILLTVLVFLLCGLPFGIQFFLFLWIHVDREVLFCHVHLVSIFLSALNSSANPIIYFFVGSFRQRQNRQNLKLVLQRALQDASEVDEGGGQLPEEILELSGSRLEQ

SEQ ID NO: 44 - protein, 330 aa, Homo sapiens
MDPTTPAWGTESTTVNGNDQALLLLCGKETLIPVFLILFIALVGLVGNGFVLWLLGFRMRRNAFSVYVLSLAGADFLFLCFQIINCLVYLSNFFCSISINFPSFFTTVMTCAYLAGLSMLSTVSTERCLSVLWPIWYRCRRPRHLSAVVCVLLWALSLLLSILEGKFCGFLFSDGDSGWCQTFDFITAAWLIFLFMVLCGSSLALLVRILCGSRGLPLTRLYLTILLTVLVFLLCGLPFGIQWFLILWIWKDSDVLFCHIHPVSVVLSSLNSSANPIIYFFVGSFRKQWRLQQPILKLALQRALQDIAEVDHSEGCFRQGTPEMSRSSLV

SEQ ID NO: 45 - protein, 322 aa, Homo sapiens
MDSTIPVLGTELTPINGREETPCYKQTLSFTGLTCIVSLVALTGNAVVLWLLGCRMRRNAVSIYILNLVAADFLFLSGHIICSPLRLINIRHPISKILSPVMTFPYFIGLSMLSAISTERCLSILWPIWYHCRRPRYLSSVMCVLLWALSLLRSILEWMFCDFLFSGANSVWCETSDFITIAWLVFLCVVLCGSSLVLLVRILCGSRKMPLTRLYVTILLTVLVFLLCGLPFGIQWALFSRIHLDWKVLFCHVHLVSIFLSALNSSANPIIYFFVGSFRQRQNRQNLKLVLQRALQDTPEVDEGGGWLPQETLELSGSRLEQ

SEQ ID NO: 46 - protein, 322 aa, Homo sapiens
MDPTVPVFGTKLTPINGREETPCYNQTLSFTVLTCIISLVGLTGNAVVLWLLGYRMRRNAVSIYILNLAAADFLFLSFQIIRLPLRLINISHLIRKILVSVMTFPYFTGLSMLSAISTERCLSVLWPIWYRCRRPTHLSAVVCVLLWGLSLLFSMLEWRFCDFLFSGADSSWCETSDFIPVAWLIFLCVVLCVSSLVLLVRILCGSRKMPLTRLYVTILLTVLVFLLCGLPFGILGALIYRMHLNLEVLYCHVYLVCMSLSSLNSSANPIIYFFVGSFRQRQNRQNLKLVLQRALQDKPEVDKGEGQLPEESLELSGSRLGP

SEQ ID NO: 47 - protein, 330 aa, Homo sapiens
MMWGAGSPLAWLSAGSGNVNVSSVGPAEGPTGPAAPLPSPKAWDVVLCISGTLVSCENALVVAIIVGTPAFRAPMFLLVGSLAVADLLAGLGLVLHFAAVFCIGSAEMSLVLVGVLAMAFTASIGSLLAITVDRYLSLYNALTYYSETTVTRTYVMLALVWGGALGLGLLPVLAWNCLDGLTTCGVVYPLSKNHLVVLAIAFFMVFGIMLQLYAQICRIVCRHAQQIALQRHLLPASHYVATRKGIATLAVVLGAFAACWLPFTVYCLLGDAHSPPLYTYLTLLPATYNSMINPIIYAFRNQDVQKVLWAVCCCCSSSKIPFRSRSPSDV

SEQ ID NO: 48 - protein, 362 aa, Homo sapiens
MGNHTWEGCHVDSRVDHLFPPSLYIFVIGVGLPTNCLALWAAYRQVQQRNELGVYLMNLSIADLLYICTLPLWVDYFLHHDNWIHGPGSCKLFGFIFYTNIYISIAFLCCISVDRYLAVAHPLRFARLRRVKTAVAVSSVVWATELGANSAPLFHDELFRDRYNHTFCFEKFPMEGWVAWMNLYRVFVGFLFPWALMLLSYRGILRAVRGSVSTERQEKAKIKRLALSLIAIVLVCFAPYHVLLLSRSAIYLGRPWDCGFEERVFSAYHSSLAFTSLNCVADPILYCLVNEGARSDVAKALHNLLRFLASDKPQEMANASLTLETPLTSKRNSTAKAMTGSWAATPPSQGDQVQLKMLPPAQ

SEQ ID NO: 49 - protein, 377 aa, Homo sapiens
MTLLAWCTRGANPAAMNASAASLNDSQVVVVAAEGAAAAATAAGGPDTGEWGPPAAAALGAGGGANGSLELSSQLSAGPPGLLLPAVNPWDVLLCVSGTVIAGENALVVALIASTPALRTPMFVLVGSLATADLLAGCGLILHFVFQYLVPSETVSLLTVGFLVASFAASVSSLLAITVDRYLSLYNALTYYSRRTLLGVHLLLAATWTVSLGLGLLPVLGWNCLAERAACSVVRPLARSHVALLSAAFFMVFGIMLHLYVRICQVVWRHAHQIALQQHCLAPPHLAATRKGVGTLAVVLGTFGASWLPFAIYCVVGSHEDPAVYTYATLLPATYNSMINPIIYAFRNQEIQRALWLLLCGCFQSKVPFRSRSPSEV

SEQ ID NO: 50 - protein, 334 aa, Homo sapiens
MNEDLKVNLSGLPRDYLDAAAAENISAAVSSRVPAVEPEPELVVNPWDIVLCTSGTLISCENAIVVLIIFHNPSLRAPMFLLIGSLALADLLAGIGLITNFVFAYLLQSEATKLVTIGLIVASFSASVCSLLAITVDRYLSLYYALTYHSERTVTFTYVMLVMLWGTSICLGLLPVMGWNCLRDESTCSVVRPLTKNNAAILSVSFLFMFALMLQLYIQICKIVMRHAHQIALQHHFLATSHYVTTRKGVSTLAIILGTFAACWMPFTLYSLIADYTYPSIYTYATLLPATYNSIINPVIYAFRNQEIQKALCLICCGCIPSSLAQRARSPSDV

SEQ ID NO: 51 - protein, 360 aa, Homo sapiens
MDPEETSVYLDYYYATSPNSDIRETHSHVPYTSVFLPVFYTAVFLTGVLGNLVLMGALHFKPGSRRLIDIFIINLAASDFIFLVTLPLWVDKEASLGLWRTGSFLCKGSSYMISVNMHCSVLLLTCMSVDRYLAIVWPVVSRKFRRTDCAYVVCASIWFISCLLGLPTLLSRELTLIDDKPYCAEKKATPIKLIWSLVALIFTFFVPLLSIVTCYCCIARKLCAHYQQSGKHNKKLKKSIKIIFIVVAAFLVSWLPFNTFKFLAIVSGLRQEHYLPSAILQLGMEVSGPLAFANSCVNPFIYYIFDSYIRRAIVHCLCPCLKNYDFGSSTETSDSHLTKALSTFIHAEDFARRRKRSVSL

SEQ ID NO: 52 - protein, 367 aa, Homo sapiens
MSKRSWWAGSRKPPREMLKLSGSDSSQSMNGLEVAPPGLITNFSLATAEQCGQETPLENMLFASFYLLDFILALVGNTLALWLFIRDHKSGTPANVFLMHLAVADLSCVLVLPTRLVYHFSGNHWPFGEIACRLTGFLFYLNMYASIYFLTCISADRFLAIVHPVKSLKLRRPLYAHLACAFLWVVVAVAMAPLLVSPQTVQTNHTVVCLQLYREKASHHALVSLAVAFTFPFITTVTCYLLIIRSLRQGLRVEKRLKTKAVRMIAIVLAIFLVCFVPYHVNRSVYVLHYRSHGASCATQRILALANRITSCLTSLNGALDPIMYFFVAEKFRHALCNLLCGKRLKGPPPSFEGKTNESSLSAKSEL

SEQ ID NO: 53 - protein, 415 aa, Homo sapiens
MVFAHRMDNSKPHLIIPTLLVPLQNRSCTETATPLPSQYLMELSEEHSWMSNQTDLHYVLKPGEVATASIFFGILWLFSIFGNSLVCLVIHRSRRTQSTTNYFVVSMACADLLISVASTPFVLLQFTTGRWTLGSATCKVVRYFQYLTPGVQIYVLLSICIDRFYTIVYPLSFKVSREKAKKMIAASWVFDAGFVTPVLFFYGSNWDSHCNYFLPSSWEGTAYTVIHFLVGFVIPSVLIILFYQKVIKYIWRIGTDGRTVRRTMNIVPRTKVKTIKMFLILNLLFLLSWLPFHVAQLWHPHEQDYKKSSLVFTAITWISFSSSASKPTLYSIYNANFRRGMKETFCMSSMKCYRSNAYTITTSSRMAKKNYVGISEIPSMAKTITKDSIYDSFDREAKEKKLAWPINSNPPNTFV

SEQ ID NO: 54 - protein, 358 aa, Homo sapiens
MPSVSPAGPSAGAVPNATAVTTVRTNASGLEVPLFHLFARLDEELHGTFPGLWLALMAVHGAIFLAGLVLNGLALYVFCCRTRAKTPSVIYTINLVVTDLLVGLSLPTRFAVYYGARGCLRCAFPHVLGYFLNMHCSILFLTCICVDRYLAIVRPEGSRRCRQPACARAVCAFVWLAAGAVTLSVLGVTGSRPCCRVFALTVLEFLLPLLVISVFTGRIMCALSRPGLLHQGRQRRVRAMQLLLTVLIIFLVCFTPFHARQVAVALWPDMPHHTSLVVYHVAVTLSSLNSCMDPIVYCFVTSGFQATVRGLFGQHGEREPSSGDVVSMHRSSKGSGRHHILSAGPHALTQALANGPEA

SEQ ID NO: 55 - protein, 349 aa, Homo sapiens
MNSTLDGNQSSHPFCLLAFGYLETVNFCLLEVLIIVFLTVLIISGNIIVIFVFHCAPLLNHHTTSYFIQTMAYADLFVGVSCVVPSLSLLHHPLPVEESLTCQIFGFVVSVLKSVSMASLACISIDRYIAITKPLTYNTLVTPWRLRLCIFLIWLYSTLVFLPSFFHWGKPGYHGDVFQWCAESWHTDSYFTLFIVMMLYAPAALIVCFTYFNIFRICQQHTKDISERQARFSSQSGETGEVQACPDKRYAMVLFRITSVFYILWLPYIIYFLLESSTGHSNRFASFLTTWLAISNSFCNCVIYSLSNSVFQRGLKRLSGAMCTSCASQTTANDPYTVRSKGPLNGCHI

SEQ ID NO: 56 - protein, 433 aa, Homo sapiens
MCFSPILEINMQSESNITVRDDIDDINTNMYQPLSYPLSFQVSLTGFLMLEIVLGLGSNLTVLVLYCMKSNLINSVSNIITMNLHVLDVIICVGCIPLTIVILLLSLESNTALICCFHEACVSFASVSTAINVFAITLDRYDISVKPANRILTMGRAVMLMISIWIFSFFSFLIPFIEVNFFSLQSGNTWENKTLLCVSTNEYYTELGMYYHLLVQIPIFFFTVVVMLITYTKILQALNIRIGTRFSTGQKKKARKKKTISLTTQHEATDMSQSSGGRNVVFGVRTSVSVIIALRRAVKRHRERRERQKRVFRMSLLIISTFLLCWTPISVLNTTILCLGPSDLLVKLRLCFLVMAYGTTIFHPLLYAFTRQKFQKVLKSKMKKRVVSIVEADPLPNNAVIHNSWIDPKRNKKITFEDSEIREKCLVPQVVTD

SEQ ID NO: 57 - protein, 361 aa, Homo sapiens
MAPTEPWSPSPGSAPWDYSGLDGLEELELCPAGDLPYGYVYIPALYLAAFAVGLLGNAFVVWLLAGRRGPRRLVDTFVLHLAAADLGFVLTLPLWAAAAALGGRWPFGDGLCKLSSFALAGTRCAGALLLAGMSVDRYLAVVKLLEARPLRTPRCALASCCGVWAVALLAGLPSLVYRGLQPLPGGQDSQCGEEPSHAFQGLSLLLLLLTFVLPLVVTLFCYCRISRRLRRPPHVGRARRNSLRIIFAIESTFVGSWLPFSALRAVFHLARLGALPLPCPLLLALRWGLTIATCLAFVNSCANPLIYLLLDRSFRARALDGACGRTGRLARRISSASSLSRDDSSVFRCRAQAANTASASW

SEQ ID NO: 58 - protein, 337 aa, Homo sapiens
MNSWDAGLAGLLVGTMGVSLLSNALVLLCLLHSADIRRQAPALFTLNLTCGNLLCTVVNMPLTLAGVVAQRQPAGDRLCRLAAFLDTFLAANSMLSMAALSIDRWVAVVFPLSYRAKMRLRDAALMVAYTWLHALTFPAAALALSWLGFHQLYASCTLCSRRPDERLRFAVFTGAFHALSFLLSFVVLCCTYLKVLKVARFHCKRIDVITMQTLVLLVDLHPSVRERCLEEQKRRRQRATKKISTFIGTFLVCFAPYVITRLVELFSTVPIGSHWGVLSKCLAYSKAASDPFVYSLLRHQYRKSCKEILNRLLHRRSIHSSGLTGDSHSQNILPVSE

SEQ ID NO: 59 - protein, 373 aa, Homo sapiens
MANASEPGGGGEAAALGLKLATLSLLLCVSLAGNVLFALLIVRERSLHRAPYYLLLDLCLADGLRALACLPVMLAARRAAAAAGAPPGALGCKLLAFLAALFCFHAAFLLLGVGVTRYLAIAHHRFYAERLAGWPCAALVCAAWALALAAAFPPVLDGGGYGDDEDAPCALEQRPDGAPGALGFLLLLAVVVGATHLVYLRLLFFIHDRRKMRPARLVPAVSHDWTFHGPGATGQAAANWTAGFGRGPTPPALVGIRPAGPGRGARRLLVLEEFKTEKRLCKMFYAITLLFLLLWGPYVVASYLRVLVRPGAVPQAYLTASVWLTFAQAGINPVVCFLFNRELRDCFRAQFPCCQSPQTTQATLPCDLKGIGL

SEQ ID NO: 60 - protein, 319 aa, Homo sapiens
MPFPNCSAPSTVVATAVGVLLGLECGLGLLGNAVALWTFLFRVRVWKPYAVYLLNLALADLLLAACLPFLAAFYLSLQAWHLGRVGCWALHFLLDLSRSVGMAFLAAVALDRYLRVVHPRLKVNLLSPQAALGVSGLVWLLMVALTCPGLLISEAAQNSTRCHSFYSRADGSFSIIWQEALSCLQFVLPFGLIVFCNAGIIRALQKRLREPEKQPKLQRAQALVTLVVVLFALCFLPCFLARVLMHIFQNLGSCRALCAVAHTSDVTGSLTYLHSVLNPVVYCFSSPTFRSSYRRVFHTLRGKGQAAEPPDFNPRDSYS

SEQ ID NO: 61 - protein, 356 aa, Homo sapiens
MNGVSEGTRGCSDRQPGVLTRDRSCSRKMNSSGCLSEEVGSLRPLTVVILSASIVVGVLGNGLVLWMTVFRMARTVSTVCFFHLALADFMLSLSLPIAMYYIVSRQWLLGEWACKLYITFVFLSYFASNCLLVFISVDRCISVLYPVWALNHRTVQRASWLAFGVWLLAAALCSAHLKFRTTRKWNGCTHCYLAFNSDNETAQIWIEGVVEGHIIGTIGHFLLGFLGPLAIIGTCAHLIRAKLLREGWVHANRPKRLLLVLVSAFFIFWSPFNVVLLVHLWRRVMLKEIYHPRMLLILQASFALGCVNSSLNPFLYVFVGRDFQEKFFQSLTSALARAFGEEEFLSSCPRGNAPRE

SEQ ID NO: 62 - protein, 333 aa, Homo sapiens
MDLINSTDYLINASTLVRNSTQFLAPASKMIIALSLYISSIIGTITNGLYLWVLRFKMKQTVNTLLFFHLILSYFISTMILPFMATSQLQDNHWNFGTALCKVFNGTLSLGMFTSVFFLSAIGLDRYLLTLHPVWSQQHRTPRWASSIVLGVWISAAALSIPYLIFRETHHDRKGKVTCQNNYAVSTNWESKEMQASRQWIHVACFISRFLLGFLLPFFIIIFCYERVASKVKERSLFKSSKPFKVMMTAIISFFVCWMPYHIHQGLLLTTNQSLLLELTLILTVLTTSFNTIFSPTLYLFVGENFKKVFKKSILALFESTFSEDSSVERTQT

SEQ ID NO: 63 - protein, 381 aa, Homo sapiens
MRSHTITMTTTSVSSWPYSSHRMRFITNHSDQPPQNFSATPNVTTCPMDEKLLSTVLTTSYSVIFIVGLVGNIIALYVFLGIHRKRNSIQIYLLNVAIADLLLIFCLPFRIMYHINQNKWTLGVILCKVVGTLFYMNMYISIILLGFISLDRYIKINRSIQQRKAITTKQSIYVCCIVWMLALGGFLTMIILTLKKGGHNSTMCFHYRDKHNAKGEAIFNFILVVMFWLIFLLIILSYIKIGKNLLRISKRRSKFPNSGKYATTARNSFIVLIIFTICFVPYHAFRFIYISSQLNVSSCYWKEIVHKTNEIMLVLSSFNSCLDPVMYFLMSSNIRKIMCQLLFRRFQGEPSRSESTSEFKPGYSLHDTSVAVKIQSSSKST

SEQ ID NO: 64 - protein, 340 aa, Homo sapiens
MLSGSRAVPTPHRGSEELLKYMLHSPCVSLTMNGTYNTCGSSDLTWPPAIKLGFYAYLGVLLVLGLLLNSLALWVFCCRMQQWTETRIYMTNLAVADLCLLCTLPFVLHSLRDTSDTPLCQLSQGIYLTNRYMSISLVTAIAVDRYVAVRHPLRARGLRSPRQAAAVCAVLWVLVIGSLVARWLLGIQEGGFCFRSTRHNFNSMAFPLLGFYLPLAVVVFCSLKVVTALAQRPPTDVGQAEATRKAARMVWANLLVFVVCFLPLHVGLTVRLAVGWNACALLETIRRALYITSKLSDANCCLDAICYYYMAKEFQEASALAVAPSAKAHKSQDSLCVTLA

SEQ ID NO: 65 - protein, 613 aa, Homo sapiens
MRAPGALLARMSRLLLLLLLKVSASSALGVAPASRNETCLGESCAPTVIQRRGRDAWGPGNSARDVLRARAPREEQGAAFLAGPSWDLPAAPGRDPAAGRGAEASAAGPPGPPTRPPGPWRWKGARGQEPSETLGRGNPTALQLFLQISEEEEKGPRGAGISGRSQEQSVKTVPGASDLFYWPRRAGKLQGSHHKPLSKTANGLAGHEGWTIALPGRALAQNGSLGEGIHEPGGPRRGNSTNRRVRLKNPFYPLTQESYGAYAVMCLSVVIFGTGIIGNLAVMCIVCHNYYMRSISNSLLANLAFWDFLIIFFCLPLVIFHELTKKWLLEDFSCKIVPYIEVASLGVTTFTLCALCIDRFRAATNVQMYYEMIENCSSTTAKLAVIWVGALLLALPEVVLRQLSKEDLGFSGRAPAERCIIKISPDLPDTIYVLALTYDSARLWWYFGCYFCLPTLFTITCSLVTARKIRKAEKACTRGNKRQIQLESQMNCTVVALTILYGFCIIPENICNIVTAYMATGVSQQTMDLLNIISQFLLFFKSCVTPVLLFCLCKPFSRAFMECCCCCCEECIQKSSTVTSDDNDNEYTTELELSPFSTIRREMSTFASVGTHC

SEQ ID NO: 66 - protein, 481 aa, Homo sapiens
MRWLWPLAVSLAVILAVGLSRVSGGAPLHLGRHRAETQEQQSRSKRGTEDEEAKGVQQYVPEEWAEYPRPIHPAGLQPTKPLVATSPNPGKDGGTPDSGQELRGNLTGAPGQRLQIQNPLYPVTESSYSAYAIMLLALVVFAVGIVGNLSVMCIVWHSYYLKSAWNSILASLALWDFLVLFFCLPIVIFNEITKQRLLGDVSCRAVPFMEVSSLGVTTFSLCALGIDRFHVATSTLPKVRPIERCQSILAKLAVIWVGSMTLAVPELLLWQLAQEPAPTMGTLDSCIMKPSASLPESLYSLVMTYQNARMWWYFGCYFCLPILFTVTCQLVTWRVRGPPGRKSECRASKHEQCESQLNSTVVGLTVVYAFCTLPENVCNIVVAYLSTELTRQTLDLLGLINQFSTFFKGAITPVLLLCICRPLGQAFLDCCCCCCCEECGGASEASAANGSDNKLKTEVSSSIYFHKPRESPPLLPLGTPC

SEQ ID NO: 67 - protein, 453 aa, Homo sapiens
MASPSLPGSDCSQIIDHSHVPEFEVATWIKITLILVYLIIFVMGLLGNSATIRVTQVLQKKGYLQKEVTDHMVSLACSDILVFLIGMPMEFYSIIWNPLTTSSYTLSCKLHTFLFEACSYATLLHVLTLSFERYIAICHPFRYKAVSGPCQVKLLIGFVWVTSALVALPLLFAMGTEYPLVNVPSHRGLTCNRSSTRHHEQPETSNMSICTNLSSRWTVFQSSIFGAFVVYLVVLLSVAFMCWNMMQVLMKSQKGSLAGGTRPPQLRKSESEESRTARRQTIIFLRLIVVTLAVCWMPNQIRRIMAAAKPKHDWTRSYFRAYMILLPFSETFFYLSSVINPLLYTVSSQQFRRVFVQVLCCRLSLQHANHEKRLRVHAHSTTDSARFVQRPLLFASRRQSSARRTEKIFLSTFQSEAEPQSKSQSLSLESLEPNSGAKPANSAAENGFQEHEV

SEQ ID NO: 68 - protein, 372 aa, Homo sapiens
MACNSTSLEAYTYLLLNTSNASDSGSTQLPAPLRISLAIVMLLMTVVGFLGNTVVCIIVYQRPAMRSAINLLLATLAFSDIMLSLCCMPFTAVTLITVRWHFGDHFCRLSATLYWFFVLEGVAILLIISVDRFLIIVQRQDKLNPRRAKVIIAVSWVLSFCIAGPSLTGWTLVEVPARAPQCVLGYTELPADRAYVVTLVVAVFFAPFGVMLCAYMCILNTVRKNAVRVHNQSDSLDLRQLTRAGLRRLQRQQQVSVDLSFKTKAFTTILILFVGFSLCWLPHSVYSLLSVFSQRFYCGSSFYATSTCVLWLSYLKSVFNPIVYCWRIKKFREACIELLPQTFQILPKVPERIRRRIQPSTVYVCNENQSAV

SEQ ID NO: 69 - protein, 927 aa, Homo sapiens
MPGPLGLLCFLALGLLGSAGPSGAAPPLCAAPCSCDGDRRVDCSGKGLTAVPEGLSAFTQALQLAGNDLSFIHPKALSGLKELKVLTLQNNQLKTVPSEAIRGLSALQSLRLDANHITSVPEDSFEGLVQLRHLWLDDNSLTEVPVHPLSNLPTLQALTLALNKISSIPDFAFTNLSSLVVLHLHNNKIRSLSQHCFDGLDNLETLDLNYNNLGEFPQAIKALPSLKELGFHSNSISVIPDGAFDGNPLLRTIHLYDNPLSFVGNSAFHNLSDLHSLVIRGASMVQQFPNLTGTVHLESLTLTGTKISSIPNNLCQEQKMLRTLDLSYNNIRDLPSFNGCHALEEISLQRNQIYQIKEGTFQGLISLRILDLSRNLIHEIHSRAFATLGPITNLDVSFNELTSFPTEGLNGLNQLKLVGNFKLKEALAAKDFVNLRSLSVPYAYQCCAFWGCDSYANLNTEDNSLQDHSVAQEKGTADAANVTSTLENEEHSQIIIHCTPSTGAFKPCEYLLGSWMIRLTVWFIFLVALFFNLLVILTTFASCTSLPSSKLFIGLISVSNLFMGIYTGILTFLDAVSWGRFAEFGIWWETGSGCKVAGFLAVFSSESAIFLLMLATVERSLSAKDIMKNGKSNHLKQFRVAALLAFLGATVAGCFPLFHRGEYSASPLCLPFPTGETPSLGFTVTLVLLNSLAFLLMAVIYTKLYCNLEKEDLSENSQSSMIKHVAWLIFTNCIFFCPVAFFSFAPLITAISISPEIMKSVTLIFFPLPACLNPVLYVFFNPKFKEDWKLLKRRVTKKSGSVSVSISSQGGCLEQDFYYDCGMYSHLQGNLTVCDCCESFLLTKPVSCKHLIKSHSCPALAVASCQRPEGYWSDCGTQSAHSDYADEEDSFVSDSSDQVQACGRACFYQSRGFPLVRYAYNLPRVKD

SEQ ID NO: 70 - protein, 883 aa, Homo sapiens
MDTSRLGVLLSLPVLLQLATGGSSPRSGVLLRGCPTHCHCEPDGRMLLRVDCSDLGLSELPSNLSVFTSYLDLSMNNISQLLPNPLPSLRFLEELRLAGNALTYIPKGAFTGLYSLKVLMLQNNQLRHVPTEALQNLRSLQSLRLDANHISYVPPSCFSGLHSLRHLWLDDNALTEIPVQAFRSLSALQAMTLALNKIHHIPDYAFGNLSSLVVLHLHNNRIHSLGKKCFDGLHSLETLDLNYNNLDEFPTAIRTLSNLKELHFYDNPIQFVGRSAFQHLPELRTLTLNGASQITEFPDLTGTANLESLTLTGAQISSLPQTVCNQLPNLQVLDLSYNLLEDLPSFSVCQKLQKIDLRHNEIYEIKVDTFQQLLSLRSLNLAWNKIAIIHPNAFSTLPSLIKLDLSSNLLSSFPITGLHGLTHLKLTGNHALQSLISSENFPELKVIEMPYAYQCCAFGVCENAYKISNQWNKGDNSSMDDLHKKDAGMFQAQDERDLEDFLLDFEEDLKALHSVQCSPSPGPFKPCEHLLDGWLIRIGVWTIAVLALTCNALVTSTVFRSPLYISPIKLLIGVIAAVNMLTGVSSAVLAGVDAFTFGSFARHGAWWENGVGCHVIGFLSIFASESSVFLLTLAALERGFSVKYSAKFETKAPFSSLKVIILLCALLALTMAAVPLLGGSKYGASPLCLPLPFGEPSTMGYMVALILLNSLCFLMMTIAYTKLYCNLDKGDLENIWDCSMVKHIALLLFTNCILNCPVAFLSFSSLINLTFISPEVIKFILLVVVPLPACLNPLLYILFNPHFKEDLVSLRKQTYVWTRSKHPSLMSINSDDVEKQSCDSTQALVTFTSSSITYDLPPSSVPSPAYPVTESCHLSSVAFVPCL

SEQ ID NO: 71 - protein, 617 aa, Homo sapiens
MGPTLAVPTPYGCIGCKLPQPEYPPALIIFMFCAMVITIVVDLIGNSMVILAVTKNKKLRNSGNIFVVSLSVADMLVAIYPYPLMLHAMSIGGWDLSQLQCQMVGFITGLSVVGSIFNIVAIAINRYCYICHSLQYERIFSVRNTCIYLVITWIMTVLAVLPNMYIGTIEYDPRTYTCIFNYLNNPVFTVTIVCIHFVLPLLIVGFCYVRIWTKVLAARDPAGQNPDNQLAEVRNFLTMFVIFLLFAVCWCPINVLTVLVAVSPKEMAGKIPNWLYLAAYFIAYFNSCLNAVIYGLLNENFRREYWTIFHAMRHPIIFFSGLISDIREMQEARTLARARAHARDQAREQDRAHACPAVEETPMNVRNVPLPGDAAAGHPDRASGHPKPHSRSSSAYRKSASTHHKSVFSHSKAASGHLKPVSGHSKPASGHPKSATVYPKPASVHFKADSVHFKGDSVHFKPDSVHFKPASSNPKPITGHHVSAGSHSKSAFSAATSHPKPTTGHIKPATSHAEPTTADYPKPATTSHPKPTAADNPELSASHCPEIPAIAHPVSDDSDLPESASSPAAGPTKPAASQLESDTIADLPDPTVVTTSTNDYHDVVVIDVEDDPDEMAV

SEQ ID NO: 72 - protein, 361 aa, Homo sapiens
MNESRWTEWRILNMSSGIVNVSERHSCPLGFGHYSVVDVCIFETVVIVLLTFLIIAGNLTVIFVFHCAPLLHHYTTSYFIQTMAYADLFVGVSCLVPTLSLLHYSTGVHESLTCQVFGYIISVLKSVSMACLACISVDRYLAITKPLSYNQLVTPCRLRICIILIWIYSCLIFLPSFFGWGKPGYHGDIFEWCATSWLTSAYFTGFIVCLLYAPAAFVVCFTYFHIFKICRQHTKEINDRRARFPSHEVDSSRETGHSPDRRYAMVLFRITSVFYMLWLPYIIYFLLESSRVLDNPTLSFLTTWLAISNSFCNCVIYSLSNSVFRLGLRRLSETMCTSCMCVKDQEAQEPKPRKRANSCSI

SEQ ID NO: 73 - protein, 451 aa, Homo sapiens
MESSPIPQSSGNSSTLGRVPQTPGPSTASGVPEVGLRDVASESVALFFMLLLDLTAVAGNAAVMAVIAKTPALRKFVFVFHLCLVDLLAALTLMPLAMLSSSALFDHALFGEVACRLYLFLSVCFVSLAILSVSAINVERYYYVVHPMRYEVRMTLGLVASVLVGVWVKALAMASVPVLGRVSWEEGAPSVPPGCSLQWSHSAYCQLFVVVFAVLYFLLPLLLILVVYCSMFRVARVAAMQHGPLPTWMETPRQRSESLSSRSTMVTSSGAPQTTPHRTFGGGKAAVVLLAVGGQFLLCWLPYFSFHLYVALSAQPISTGQVESVVTWIGYFCFTSNPFFYGCLNRQIRGELSKQFVCFFKPAPEEELRLPSREGSIEENFLQFLQGTGCPSESWVSRPLPSPKQEPPAVDFRIPGQIAEETSEFLEQQLTSDIIMSDSYLRPAASPRLES

SEQ ID NO: 74 - protein, 368 aa, Homo sapiens
MANSTGLNASEVAGSLGLILAAVVEVGALLGNGALLVVVLRTPGLRDALYLAHLCVVDLLAAASIMPLGLLAAPPPGLGRVRLGPAPCRAARFLSAALLPACTLGVAALGLARYRLIVHPLRPGSRPPPVLVLTAVWAAAGLLGALSLLGTPPAPPPAPARCSVLAGGLGPFRPLWALLAFALPALLLLGAYGGIFVVARRAALRPPRPARGSRLHSDSLDSRLSILPPLRPRLPGGKAALAPALAVGQFAACWLPYGCACLAPAARAAEAEAAVTWVAYSAFAAHPFLYGLLQRPVRLALGRLSRRALPGPVRACTPQAWHPRALLQCLQRPPEGPAVGPSEAPEQTPELAGGRSPAYQGPPESSLS

SEQ ID NO: 75 - protein, 419 aa, Homo sapiens
MVFSAVLTAFHTGTSNTTFVVYENTYMNITLPPPFQHPDLSPLLRYSFETMAPTGLSSLTVNSTAVPTTPAAFKSLNLPLQITLSAIMIFILFVSFLGNLVVCLMVYQKAAMRSAINILLASLAFADMLLAVLNMPFALVTILTTRWIFGKFFCRVSAMFFWLFVIEGVAILLIISIDRFLIIVQRQDKLNPYRAKVLIAVSWATSFCVAFPLAVGNPDLQIPSRAPQCVFGYTTNPGYQAYVILISLISFFIPFLVILYSFMGILNTLRHNALRIHSYPEGICLSQASKLGLMSLQRPFQMSIDMGFKTRAFTTILILFAVFIVCWAPFTTYSLVATFSKHFYYQHNFFEISTWLLWLCYLKSALNPLIYYWRIKKFHDACLDMMPKSFKFLPQLPGHTKRRIRPSAVYVCGEHRTVV

SEQ ID NO: 76 - protein, 337 aa, Homo sapiens
MNSTCIEEQHDLDHYLFPIVYIFVIIVSIPANIGSLCVSFLQAKKESELGIYLFSLSLSDLLYALTLPLWIDYTWNKDNWTFSPALCKGSAFLMYMNFYSSTAFLTCIAVDRYLAVVYPLKFFFLRTRRFALMVSLSIWILETIFNAVMLWEDETVVEYCDAEKSNFTLCYDKYPLEKWQINLNLFRTCTGYAIPLVTILICNRKVYQAVRHNKATENKEKKRIIKLLVSITVTFVLCFTPFHVMLLIRCILEHAVNFEDHSNSGKRTYTMYRITVALTSLNCVADPILYCFVTETGRYDMWNILKFCTGRCNTSQRQRKRILSVSTKDTMELEVLE

SEQ ID NO: 77 - protein, 365 aa, Homo sapiens
MGNITADNSSMSCTIDHTIHQTLAPVVYVTVLVVGFPANCLSLYFGYLQIKARNELGVYLCNLTVADLFYICSLPFWLQYVLQHDNWSHGDLSCQVCGILLYENIYISVGFLCCISVDRYLAVAHPFRFHQFRTLKAAVGVSVVIWAKELLTSIYFLMHEEVIEDENQHRVCFEHYPIQAWQRAINYYRFLVGFLFPICLLLASYQGILRAVRRSHGTQKSRKDQIQRLVLSTVVIFLACFLPYHVLLLVRSVWEASCDFAKGVFNAYHFSLLLTSFNCVADPVLYCFVSETTHRDLARLRGACLAFLTCSRTGRAREAYPLGAPEASGKSGAQGEEPELLTKLHPAFQTPNSPGSGGFPTGRLA

SEQ ID NO: 78 - protein, 540 aa, Homo sapiens
MNSTGHLQDAPNATSLHVPHSQEGNSTSLQEGLQDLIHTATLVTCTFLLAVIFCLGSYGNFIVFLSFFDPAFRKFRTNFDFMILNLSFCDLFICGVTAPMFTFVLFFSSASSIPDAFCFTFHLTSSGFIIMSLKTVAVIALHRLRMVLGKQPNRTASFPCTVLLTLLLWATSFTLATLATLKTSKSHLCLPMSSLIAGKGKAILSLYVVDFTFCVAVVSVSYIMIAQTLRKNAQVRKCPPVITVDASRPQPFMGVPVQGGGDPIQCAMPALYRNQNYNKLQHVQTRGYTKSPNQLVTPAASRLQLVSAINLSTAKDSKAVVTCVIIVLSVLVCCLPLGISLVQVVLSSNGSFILYQFELFGFTLIFFKSGLNPFIYSRNSAGLRRKVLWCLQYIGLGFFCCKQKTRLRAMGKGNLEVNRNKSSHHETNSAYMLSPKPQKKFVDQACGPSHSKESMVSPKISAGHQHCGQSSSTPINTRIEPYYSIYNSSPSQEESSPCNLQPVNSFGFANSYIAMHYHTTNDLVQEYDSTSAKQIPVPSV

SEQ ID NO: 79 - protein, 363 aa, Homo sapiens
MGPGEALLAGLLVMVLAVALLSNALVLLCCAYSAELRTRASGVLLVNLSLGHLLLAALDMPFTLLGVMRGRTPSAPGACQVIGFLDTFLASNAALSVAALSADQWLAVGFPLRYAGRLRPRYAGLLLGCAWGQSLAFSGAALGCSWLGYSSAFASCSLRLPPEPERPRFAAFTATLHAVGFVLPLAVLCLTSLQVHRVARRHCQRMDTVTMKALALLADLHPSVRQRCLIQQKRRRHRATRKIGIAIATFLICFAPYVMTRLAELVPFVTVNAQWGILSKCLTYSKAVADPFTYSLLRRPFRQVLAGMVHRLLKRTPRPASTHDSSLDVAGMVHQLLKRTPRPASTHNGSVDTENDSCLQQTH

SEQ ID NO: 80 - protein, 336 aa, Homo sapiens
MNNNTTCIQPSMISSMALPIIYILLCIVGVFGNTLSQWIFLTKIGKKTSTHIYLSHLVTANLLVCSAMPFMSIYFLKGFQWEYQSAQCRVVNFLGTLSMHASMFVSLLILSWIAISRYATLMQKDSSQETTSCYEKIFYGHLLKKFRQPNFARKLCIYIWGVVLGIIIPVTVYYSVIEATEGEESLCYNRQMELGAMISQIAGLIGTTFIGFSFLVVLTSYYSFVSHLRKIRTCTSIMEKDLTYSSVKRHLLVIQILLIVCFLPYSIFKPIFYVLHQRDNCQQLNYLIETKNILTCLASARSSTDPIIFLLLDKTFKKTLYNLFTKSNSAHMQSYG

SEQ ID NO: 81 - protein, 381 aa, Homo sapiens
MVPHLLLLCLLPLVRATEPHEGRADEQSAEAALAVPNASHFFSWNNYTFSDWQNFVGRRRYGAESQNPTVKALLIVAYSFIIVFSLFGNVLVCHVIFKNQRMHSATSLFIVNLAVADIMITLLNTPFTLVIMHPLKPRISITKGVIYIAVIWTMATFFSLPHAICQKLFTFKYSEDIVRSLCLPDFPEPADLFWKYLDLATFILLYILPLLIISVAYARVAKKLWLCNMIGDVTTEQYFALRRKKKKTIKMLMLVVVLFALCWFPLNCYVLLLSSKVIRTNNALYFAFHWFAMSSTCYNPFIYCWLNENFRIELKALLSMCQRPPKPQEDRPPSPVPSFRVAWTEKNDGQRAPLANNLLPTSQLQSGKTDLSSVEPIVTMS

SEQ ID NO: 82 - protein, 396 aa, Homo sapiens
MWNSSDANFSCYHESVLGYRYVAVSWGVVVAVTGTVGNVLTLLALAIQPKLRTRFNLLIANLTLADLLYCTLLQPFSVDTYLHLHWRTGATFCRVFGLLLFASNSVSILTLCLIALGRYLLIAHPKLFPQVFSAKGIVLALVSTWVVGVASFAPLWPIYILVPVVCTCSFDRIRGRPYTTILMGIYFVLGLSSVGIFYCLIHRQVKRAAQALDQYKLRQASIHSNHVARTDEAMPGRFQELDSRLASGGPSEGISSEPVSAATTQTLEGDSSEVGDQINSKRAKQMAEKSPPEASAKAQPIKGARRAPDSSSEFGKVTRMCFAVFLCFALSYIPFLLLNILDARVQAPRVVHMLAANLTWLNGCINPVLYAAMNRQFRQAYGSILKRGPRSFHRLH

SEQ ID NO: 83 - protein, 370 aa, Homo sapiens
MANYSHAADNILQNLSPLTAFLKLTSLGFIIGVSVVGNLLISILLVKDKTLHRAPYYFLLDLCCSDILRSAICFPFVFNSVKNGSTWTYGTLTCKVIAFLGVLSCFHTAFMLFCISVTRYLAIAHHRFYTKRLTFWTCLAVICMVWTLSVAMAFPPVLDVGTYSFIREEDQCTFQHRSFRANDSLGFMLLLALILLATQLVYLKLIFFVHDRRKMKPVQFVAAVSQNWTFHGPGASGQAAANWLAGFGRGPTPPTLLGIRQNANTTGRRRLLVLDEFKMEKRISRMFYIMTFLFLTLWGPYLVACYWRVFARGPVVPGGFLTAAVWMSFAQAGINPFVCIFSNRELRRCFSTTLLYCRKSRLPREPYCVI

SEQ ID NO: 84 - protein, 358 aa, Homo sapiens
MGFNLTLAKLPNNELHGQESHNSGNRSDGPGKNTTLHNEFDTIVLPVLYLIIFVASILLNGLAVWIFFHIRNKTSFIFYLKNIVVADLIMTLTFPFRIVHDAGFGPWYFKFILCRYTSVLFYANMYTSIVFLGLISIDRYLKVVKPFGDSRMYSITFTKVLSVCVWVIMAVLSLPNIILTNGQPTEDNIHDCSKLKSPLGVKWHTAVTYVNSCLFVAVLVILIGCYIAISRYIHKSSRQFISQSSRKRKHNQSIRVVVAVFFTCFLPYHLCRIPFTFSHLDRLLDESAQKILYYCKEITLFLSACNVCLDPIIYFFMCRSFSRRLFKKSNIRTRSESIRSLQSVRRSEVRIYYDYTDV

SEQ ID NO: 85 - protein, 384 aa, Homo sapiens
MTNSSSTSTSSTTGGSLLLLCEEEESWAGRRIPVSLLYSGLAIGGTLANGMVIYLVSSFRKLQTTSNAFIVNGCAADLSVCALWMPQEAVLGLLPTGSAEPPADWDGAGGSYRLLRGGLLGLGLTVSLLSHCLVALNRYLLITRAPATYQALYQRRHTAGMLALSWALALGLVLLLPPWAPRPGAAPPRVHYPALLAAAALLAQTALLLHCYLGIVRRVRVSVKRVSVLNFHLLHQLPGCAAAAAAFPGAQHAPGPGGAAHPAQAQPLPPALHPRRAQRRLSGLSVLLLCCVFLLATQPLVWVSLASGFSLPVPWGVQAASWLLCCALSALNPLLYTWRNEEFRRSVRSVLPGVGDAAAAAVAATAVPAVSQAQLGTRAAGQHW

SEQ ID NO: 86 - protein, 508 aa, Homo sapiens
MTSTCTNSTRESNSSHTCMPLSKMPISLAHGIIRSTVLVIFLAASFVGNIVLALVLQRKPQLLQVTNRFIFNLLVTDLLQISLVAPWVVATSVPLFWPLNSHFCTALVSLTHLFAFASVNTIVVVSVDRYLSIIHPLSYPSKMTQRRGYLLLYGTWIVAILQSTPPLYGWGQAAFDERNALCSMIWGASPSYTILSVVSFIVIPLIVMIACYSVVFCAARRQHALLYNVKRHSLEVRVKDCVENEDEEGAEKKEEFQDESEFRRQHEGEVKAKEGRMEAKDGSLKAKEGSTGTSESSVEARGSEEVRESSTVASDGSMEGKEGSTKVEENSMKADKGRTEVNQCSIDLGEDDMEFGEDDINFSEDDVEAVNIPESLPPSRRNSNSNPPLPRCYQCKAAKVIFIIIFSYVLSLGPYCFLAVLAVWVDVETQVPQWVITIIIWLFFLQCCIHPYVYGYMHKTIKKEIQDMLKKFFCKEKPPKEDSHPDLPGTEGGTEGKIVPSYDSATFP

SEQ ID NO: 87 - protein, 380 aa, Homo sapiens
MCPMLLKNGYNGNATPVTTTAPWASLGLSAKTCNNVSFEESRIVLVVVYSAVCTLGVPANCLTAWLALLQVLQGNVLAVYLLCLALCELLYTGTLPLWVIYIRNQHRWTLGLLACKVTAYIFFCNIYVSILFLCCISCDRFVAVVYALESRGRRRRRTAILISACIFILVGIVHYPVFQTEDKETCFDMLQMDSRIAGYYYARFTVGFAIPLSIIAFTNHRIFRSIKQSMGLSAAQKAKVKHSAIAVVVIFLVCFAPYHLVLLVKAAAFSYYRGDRNAMCGLEERLYTASVVFLCLSTVNGVADPIIYVLATDHSRQEVSRIHKGWKEWSMKTDVTRLTHSRDTEELQSPVALADHYTFSRPVHPPGSPCPAKRLIEESC

SEQ ID NO: 88 - protein, 494 aa, Homo sapiens
MEEPQPPRPPASMALLGSQHSGAPSAAGPPGGTSSAATAAVLSFSTVATAALGNLSDASGGGTAAAPGGGGLGGSGAAREAGAAVRRPLGPEAAPLLSHGAAVAAQALVLLLIFLLSSLGNCAVMGVIVKHRQLRTVTNAFILSLSLSDLLTALLCLPAAFLDLFTPPGGSAPAAAAGPWRGFCAASRFFSSCFGIVSTLSVALISLDRYCAIVRPPREKIGRRRALQLLAGAWLTALGFSLPWELLGAPRELAAAQSFHGCLYRTSPDPAQLGAAFSVGLVVACYLLPFLLMCFCHYHICKTVRLSDVRVRPVNTYARVLRFFSEVRTATTVLIMIVFVICCWGPYCFLVLLAAARQAQTMQAPSLLSVVAVWLTWANGAINPVIYAIRNPNISMLLGRNREEGYRTRNVDAFLPSQGPGLQARSRSRLRNRYANRLGACNRMSSSNPASGVAGDVAMWARKNPVVLFCREGPPEPVTAVTKQPKSEAGDTSL

SEQ ID NO: 89 - protein, 353 aa, Homo sapiens
MEHTHAHLAANSSLSWWSPGSACGLGFVPVVYYSLLLCLGLPANILTVIILSQLVARRQKSSYNYLLALAAADILVLFFIVFVDFLLEDFILNMQMPQVPDKIIEVLEFSSIHTSIWITVPLTIDRYIAVCHPLKYHTVSYPARTRKVIVSVYITCFLTSIPYYWWPNIWTEDYISTSVHHVLIWIHCFTVYLVPCSIFFILNSIIVYKLRRKSNFRLRGYSTGKTTAILFTITSIFATLWAPRIIMILYHLYGAPIQNRWLVHIMSDIANMLALLNTAINFFLYCFISKRFRTMAAATLKAFFKCQKQPVQFYTNHNFSITSSPWISPANSHCIKMLVYQYDKNGKPIKVSP

SEQ ID NO: 90 - protein, 305 aa, Homo sapiens
MPGHNTSRNSSCDPIVTPHLISLYFIVLIGGLVGVISILFLLVKMNTRSVTTMAVINLVVVHSVFLLTVPFRLTYLIKKTWMFGLPFCKFVSAMLHIHMYLTFLFYVVILVTRYLIFFKCKDKVEFYRKLHAVAASAGMWTLVIVIVVPLVVSRYGIHEEYNEEHCFKFHKELAYTYVKIINYMIVIFVIAVAVILLVFQVFIIMLMVQKLRHSLLSHQEFWAQLKNLFFIGVILVCFLPYQFFRIYYLNVVTHSNACNSKVAFYNEIFLSVTAISCYDLLLFVFGGSHWFKQKIIGLWNCVLCR

SEQ ID NO: 91 - protein, 374 aa, Homo sapiens
MLTGSCGDPQKKPQVTQDSGPQSMGLEGRETAGQPRVTLLPTPHVSGLSQEFESHWPEIAERSPCVAGVIPVIYYSVLLGLGLPVSLLTAVALARLATRTRRPSYYYLLALTASDIIIQVVIVFAGFLLQGAVLARQVPQAVVRTANILEFAANHASVWIAILLTVDRYTALCHPLHHRAASSPGRTRRAIAAVLSAALLTGIPFYWWLDMWRDTDSPRTLDEVLKWAHCLTVYFIPCGVFLVTNSAIIHRLRRRGRSGLQPRVGKSTAILLGITTLFTLLWAPRVFVMLYHMYVAPVHRDWRVHLALDVANMVAMLHTAANFGLYCFVSKTFRATVRQVIHDAYLPCTLASQPEGMAAKPVMEPPGLPTGAEV

SEQ ID NO: 92 - protein, 333 aa, Homo sapiens
MWSCSWFNGTGLVEELPACQDLQLGLSLLSLLGLVVGVPVGLCYNALLVLANLHSKASMTMPDVYFVNMAVAGLVLSALAPVHLLGPPSSRWALWSVGGEVHVALQIPFNVSSLVAMYSTALLSLDHYIERALPRTYMASVYNTRHVCGFVWGGALLTSFSSLLFYICSHVSTRALECAKMQNAEAADATLVFIGYVVPALATLYALVLLSRVRREDTPLDRDTGRLEPSAHRLLVATVCTQFGLWTPHYLILLGHTVIISRGKPVDAHYLGLLHFVKDFSKLLAFSSSFVTPLLYRYMNQSFPSKLQRLMKKLPCGDRHCSPDHMGVQQVLA

SEQ ID NO: 93 - protein, 347 aa, Homo sapiens
MGDELAPCPVGTTAWPALIQLISKTPCMPQAASNTSLGLGDLRVPSSMLYWLFLPSSLLAAATLAVSPLLLVTILRNQRLRQEPHYLLPANILLSDLAYILLHMLISSSSLGGWELGRMACGILTDAVFAACTSTILSFTAIVLHTYLAVIHPLRYLSFMSHGAAWKAVALIWLVACCFPTFLIWLSKWQDAQLEEQGASYILPPSMGTQPGCGLLVIVTYTSILCVLFLCTALIANCFWRIYAEAKTSGIWGQGYSRARGTLLIHSVLITLYVSTGVVFSLDMVLTRYHHIDSGTHTWLLAANSEVLMMLPRAMLTYLYLLRYRQLLGMVRGHLPSRRHQAIFTIS

SEQ ID NO: 94 - protein, 731 aa, Homo sapiens
MSLFLSNLSTNDSSLWKENHNSTDLLNPPGTLNIYLFCLTCLMTFAALVGSIYSLISLLKMQNRTVVSMLVASWSVDDLMSVLSVTIFMFLQWPNEVPGYFQFLCTTSALMYLCQGLSSNLKATLLVSYNFYTMHRGVGSQTASRRSGQVLGVVLTVWAASLLLSALPLCGWGAFVRTPWGCLVDCSSSYVLFLSIVYALAFGLLVGLSVPLTHRLLCSEEPPRLHSNYQEISRGASIPGTPPTAGRVVSLSPEDAPGPSLRRSGGCSPSSDTVFGPGAPAAAGAEACRRENRGTLYGTRSFTVSVAQKRFALILALTKVVLWLPMMMHMVVQNVVGFQSLPLETFSFLLTLLATTVTPVFVLSKRWTHLPCGCIINCRQNAYAVASDGKKIKRKGFEFNLSFQKSYGIYKIAHEDYYDDDENSIFYHNLMNSECETTKDPQRDNRNIFNAIKVEISTTPSLDSSTQRGINKCTNTDITEAKQDSNNKKDAFSDKTGGDINYEETTFSEGPERRLSHEESQKPDLSDWEWCRSKSERTPRQRSGYALAIPLCAFQGTVSLHAPTGKTLSLSTYEVSAEGQKITPASKKIEVYRSKSVGHEPNSEDSSSTFVDTSVKIHLEVLEICDNEEALDTVSIISNISQSSTQVRSPSLRYSRKENRFVSCDLGETASYSLFLPTSNPDGDINISIPDTVEAHRQNSKRQHQERDGYQEEIQLLNKAYRKREEESKGS

SEQ ID NO: 95 - protein, 434 aa, Homo sapiens
MEDLFSPSILPPAPNISVPILLGWGLNLTLGQGAPASGPPSRRVRLVFLGVILVVAVAGNTTVLCRLCGGGGPWAGPKRRKMDFLLVQLALADLYACGGTALSQLAWELLGEPRAATGDLACRFLQLLQASGRGASAHLVVLIALERRRAVRLPHGRPLPARALAALGWLLALLLALPPAFVVRGDSPSPLPPPPPPTSLQPGAPPAARAWPGERRCHGIFAPLPRWHLQVYAFYEAVAGFVAPVTVLGVACGHLLSVWWRHRPQAPAAAAPWSASPGRAPAPSALPRAKVQSLKMSLLLALLFVGCELPYFAARLAAAWSSGPAGDWEGEGLSAALRVVAMANSALNPFVYLFFQAGDCRLRRQLRKRLGSLCCAPQGGAEDEEGPRGHQALYRQRWPHPHYHHARREPLDEGGLRPPPPRPRPLPCSCESAF

SEQ ID NO: 96 - protein, 419 aa, Homo sapiens
MLAAAFADSNSSSMNVSFAHLHFAGGYLPSDSQDWRTIIPALLVAVCLVGFVGNLCVIGILLHNAWKGKPSMIHSLILNLSLADLSLLLFSAPIRATAYSKSVWDLGWFVCKSSDWFIHTCMAAKSLTIVVVAKVCFMYASDPAKQVSIHNYTIWSVLVAIWTVASLLPLPEWFFSTIRHHEGVEMCLVDVPAVAEEFMSMFGKLYPLLAFGLPLFFASFYFWRAYDQCKKRGTKTQNLRNQIRSKQVTVMLLSIAIISALLWLPEWVAWLWVWHLKAAGPAPPQGFIALSQVLMFSISSANPLIFLVMSEEFREGLKGVWKWMITKKPPTVSESQETPAGNSEGLPDKVPSPESPASIPEKEKPSSPSSGKGKTEKAEIPILPDVEQFWHERDTVPSVQDNDPIPWEHEDQETGEGVK

SEQ ID NO: 97 - protein, 470 aa, Homo sapiens
MDTTMEADLGATGHRPRTELDDEDSYPQGGWDTVFLVALLLLGLPANGLMAWLAGSQARHGAGTRLALLLLSLALSDFLFLAAAAFQILEIRHGGHWPLGTAACRFYYFLWGVSYSSGLFLLAALSLDRCLLALCPHWYPGHRPVRLPLWVCAGVWVLATLFSVPWLVFPEAAVWWYDLVICLDFWDSEELSLRMLEVLGGFLPFLLLLVCHVLTQATACRTCHRQQQPAACRGFARVARTILSAYVVLRLPYQLAQLLYLAFLWDVYSGYLLWEALVYSDYLILLNSCLSPFLCLMASADLRTLLRSVLSSFAAALCEERPGSFTPTEPQTQLDSEGPTLPEPMAEAQSQMDPVAQPQVNPTLQPRSDPTAQPQLNPTAQPQSDPTAQPQLNLMAQPQSDSVAQPQADTNVQTPAPAASSVPSPCDEASPTPSSHPTPGALEDPATPPASEGESPSSTPPEAAPGAGPT

SEQ ID NO: 98 - protein, 609 aa, Homo sapiens
MSDERRLPGSAVGWLVCGGLSLLANAWGILSVGAKQKKWKPLEFLLCTLAATHMLNVAVPIATYSVVQLRRQRPDFEWNEGLCKVFVSTFYTLTLATCFSVTSLSYHRMWMVCWPVNYRLSNAKKQAVHTVMGIWMVSFILSALPAVGWHDTSERFYTHGCRFIVAEIGLGFGVCFLLLVGGSVAMGVICTAIALFQTLAVQVGRQADRRAFTVPTIVVEDAQGKRRSSIDGSEPAKTSLQTTGLVTTIVFIYDCLMGFPVLVVSFSSLRADASAPWMALCVLWCSVAQALLLPVFLWACDRYRADLKAVREKCMALMANDEESDDETSLEGGISPDLVLERSLDYGYGGDFVALDRMAKYEISALEGGLPQLYPLRPLQEDKMQYLQVPPTRRFSHDDADVWAAVPLPAFLPRWGSGEDLAALAHLVLPAGPERRRASLLAFAEDAPPSRARRRSAESLLSLRPSALDSGPRGARDSPPGSPRRRPGPGPRSASASLLPDAFALTAFECEPQALRRPPGPFPAAPAAPDGADPGEAPTPPSSAQRSPGPRPSAHSHAGSLRPGLSASWGEPGGLRAAGGGGSTSSFLSSPSESSGYATLHSDSLGSAS

SEQ ID NO: 99 - protein, 338 aa, Homo sapiens
MTALSSENCSFQYQLRQTNQPLDVNYLLFLIILGKILLNILTLGMRRKNTCQNFMEYFCISLAFVDLLLLVNISIILYFRDFVLLSIRFTKYHICLFTQIISFTYGFLHYPVFLTACIDYCLNFSKTTKLSFKCQKLFYFFTVILIWISVLAYVLGDPAIYQSLKAQNAYSRHCPFYVSIQSYWLSFFMVMILFVAFITCWEEVTTLVQAIRITSYMNETILYFPFSSHSSYTVRSKKIFLSKLIVCFLSTWLPFVLLQVIIVLLKVQIPAYIEMNIPWLYFVNSFLIATVYWFNCHKLNLKDIGLPLDPFVNWKCCFIPLTIPNLEQIEKPISIMIC

SEQ ID NO: 100 - protein, 549 aa, Homo sapiens
MSARGVVQHALPTPRRGALTMSLNSSLSCRKELSNLTEEEGGEGGVIITQFIAIIVITIFVCLGNLVIVVTLYKKSYLLTLSNKFVFSLTLSNFLLSVLVLPFVVTSSIRREWIFGVVWCNFSALLYLLISSASMLTLGVIAIDRYYAVLYPMVYPMKITGNRAVMALVYIWLHSLIGCLPPLFGWSSVEFDEFKWMCVAAWHREPGYTAFWQIWCALFPFLVMLVCYGFIFRVARVKARKVHCGTVVIVEEDAQRTGRKNSSTSTSSSGSRRNAFQGVVYSANQCKALITILVVLGAFMVTWGPYMVVIASEALWGKSSVSPSLETWATWLSFASAVCHPLIYGLWNKTVRKELLGMCFGDRYYREPFVQRQRTSRLFSISNRITDLGLSPHLTALMAGGQPLGHSSSTGDTGFSCSQDSGTDMMLLEDYTSDDNPPSHCTCPPKRRSSVTFEDEVEQIKEAAKNSILHVKAEVHKSLDSYAASLAKAIEAEAKINLFGEEALPGVLVTARTVPGGGFGGRRGSRTLVSQRLQLQSIEEGDVLAAEQR

SEQ ID NO: 101 - protein, 304 aa, Homo sapiens
MLSTGVVSFFSLKSDSAPPWMVLAVLWCSMAQTLLLPSFIWSCERYRADVRTVWEQCVAIMSEEDGDDDGGCDDYAEGRVCKVRFDANGATGPGSRDPAQVKLLPGRHMLFPPLERVHYLQVPLSRRLSHDETNIFSTPREPGSFLHKWSSSDDIRVLPAQSRALGGPPEYLGQRHRLEDEEDEEEAEGGGLASLRQFLESGVLGSGGGPPRGPGFFREEITTFIDETPLPSPTASPGHSPRRPRPLGLSPRRLSLGSPESRAVGLPLGLSAGRRCSLTGGEESARAWGGSWGPGNPIFPQLTL

SEQ ID NO: 102 - protein, 319 aa, Homo sapiens
MTNSSFFCPVYKDLEPFTYFFYLVFLVGIIGSCFATWAFIQKNTNHRCVSIYLINLLTADFLLTLALPVKIVVDLGVAPWKLKIFHCQVTACLIYINMYLSIIFLAFVSIDRCLQLTHSCKIYRIQEPGFAKMISTVVWLMVLLIMVPNMMIPIKDIKEKSNVGCMEFKKEFGRNWHLLTNFICVAIFLNFSAIILISNCLVIRQLYRNKDNENYPNVKKALINILLVTTGYIICFVPYHIVRIPYTLSQTEVITDCSTRISLFKAKEATLLLAVSNLCFDPILYYHLSKAFRSKVTETFASPKETKAQKEKLRCENNA

SEQ ID NO: 103 - protein, 373 aa, Homo sapiens
MANTTGEPEEVSGALSPPSASAYVKLVLLGLIMCVSLAGNAILSLLVLKERALHKAPYYFLLDLCLADGIRSAVCFPFVLASVRHGSSWTFSALSCKIVAFMAVLFCFHAAFMLFCISVTRYMAIAHHRFYAKRMTLWTCAAVICMAWTLSVAMAFPPVFDVGTYKFIREEDQCIFEHRYFKANDTLGFMLMLAVLMAATHAVYGKLLLFEYRHRKMKPVQMVPAISQNWTFHGPGATGQAAANWIAGFGRGPMPPTLLGIRQNGHAASRRLLGMDEVKGEKQLGRMFYAITLLFLLLWSPYIVACYWRVFVKACAVPHRYLATAVWMSFAQAAVNPIVCFLLNKDLKKCLRTHAPCWGTGGAPAPREPYCVM

SEQ ID NO: 104 - protein, 333 aa, Homo sapiens
MPANYTCTRPDGDNTDFRYFIYAVTYTVILVPGLIGNILALWVFYGYMKETKRAVIFMINLAIADLLQVLSLPLRIFYYLNHDWPFGPGLCMFCFYLKYVNMYASIYFLVCISVRRFWFLMYPFRFHDCKQKYDLYISIAGWLIICLACVLFPLLRTSDDTSGNRTKCFVDLPTRNVNLAQSVVMMTIGELIGFVTPLLIVLYCTWKTVLSLQDKYPMAQDLGEKQKALKMILTCAGVFLICFAPYHFSFPLDFLVKSNEIKSCLARRVILIFHSVALCLASLNSCLDPVIYYFSTNEFRRRLSRQDLHDSIQLHAKSFVSNHTASTMTPELC

SEQ ID NO: 105 - protein, 514 aa, Homo sapiens
MGHNGSWISPNASEPHNASGAEAAGVNRSALGEFGEAQLYRQFTTTVQVVIFIGSLLEFGNMEVTRKLDKSRLPGIKFIKNLACSGICASLVCVPFDIILSTSPHCCWWIYTMLFCKVVKFLHKVFCSVTILSFPAIALDRYYSVLYPLERKISDAKSRELVMYIWAHAVVASVPVFAVTNVADIYATSTCTEVWSNSLGHLVYVLVYNITTVIVPVVVVFLFLILIRRALSASQKKKVIIAALRTPQNTISIPYASQREAELHATLLSMVMVFILCSVPYATLVVYQTVLNVPDTSVFLLLTAVWLPKVSLLANPVLFLTVNKSVRKCLIGTLVQLHHRYSRRNVVSTGSGMAEASLEPSIRSGSQLLEMFHIGQQQIFKPTEDEEESEAKYIGSADFQAKEIFSTCLEGEQGPQFAPSAPPLSTVDSVSQVAPAAPVEPETFPDKYSLQFGFGPFELPPQWLSETRNSKKRLLPPLGNTPEELIQTKVPKVGRVERKMSRNNKVSIFPKVDS

SEQ ID NO: 106 - protein, 404 aa, Homo sapiens
MSVKPSWGPGPSEGVTAVPTSDLGEIHNWTELLDLFNHTLSECHVELSQSTKRVVLFALYLAMFVVGLVENLLVICVNWRGSGRAGLMNLYILNMAIADLGIVLSLPVWMLEVTLDYTWLWGSFSCRFTHYFYFVNMYSSIFFLVCLSVDRYVTLTSASPSWQRYQHRVRRAMCAGIWVLSAIIPLPEVVHIQLVEGPEPMCLFMAPFETYSTWALAVALSTTILGFLLPFPLITVFNVLTACRLRQPGQPKSRRHCLLLCAYVAVFVMCWLPYHVTLLLLTLHGTHISLHCHLVHLLYFFYDVIDCFSMLHCVINPILYNFLSPHFRGRLLNAVVHYLPKDQTKAGTCASSSSCSTQHSIIITKGDSQPAAAAPHPEPSLSFQAHHLLPNTSPISPTQPLTPS

SEQ ID NO: 107 - protein, 361 aa, Homo sapiens [sequence omitted]

SEQ ID NO: 108 - protein, 353 aa, synthetic construct
MVGDTLKLLSPLMTRYFFLLFYSTDSSDFNENQHPLDFDGMASGKLESGISFLIQTGVGILGNSFLLCFYNFILLTGNKLRPMDLILSQLALANSLVLFSKGIPQTMAAFGLKYFLDDTGCKLVFYYHRVGTGVSFSTICLLNGFQAIKLNPSICRWLELKIRSPKFIGFCCFLCWAPHLLINTSVLFLVNGPLNSKNLSVKNNYGYCSWKMPERFGTLYTVLYFSPDFMSLGFMVWASGSMVFVLYRHKQRVQHIHSNRLSSRPSHEARATHTIMVLVSSFFAFYSVHSILTIWMTVVANPGQWIVNNSVFVASCFPAFSPFVLIFSDTHVSQFCFACRTKKTLFPDLVAMP

SEQ ID NO: 109 - protein, 305 aa, synthetic construct
MASVDLFIGMIVLFQVVVGILGNFSLLYHYMFLYFRGCKPRSTDLILRHLTVANSLVILSRGIPETMAAFGLKHFDNYFGCKFLLYVHRVARGVSIGSTCLLSVFQVITINPRNSRWAEMKVKAPKYIGLSSILCWVLHMLVNAIFPIYTTGKWSNKNITKKGDLGYCSAPLHDEVIKSVYAALTSFHDVLCLGLMTWASSSMVFVLYRHKQQVQHIHRNNLSPRSSPENRATQSILVLVSTFVSFYALSSIIYVYLALFDNSSWWLVNTAALITACFPTISPFVLMCHDPSISRLCCICCGRNR

SEQ ID NO: 110 - protein, 302 aa, synthetic construct
MASRYVAVGMIFLSQTVVGVLGNFSLLLHYLSLYCTGCRLRSTDLIVKHLIVANFLALLCKGVPQTMAAFGVRYFLNAIGCKLVFYLHRVGRGVSIGTTCLLSVFQVITISSRKSRWAKLKEKAPKHVGFSVLLCWILCMLVNIIFPMYVTGKWNYTNITVNKDLGYCSGGGNNKIAQTLRAMLLSFPDVLCLGLMLWASSSMVCILHRHKQRVQHIDRSNLSPRASPENRATQSILILVSTFVSSYTLSCLFQVCIALLDNPNSLLVNTSALMSVCFPTLSPFVLMSCDPSVYRLCFAWKR

SEQ ID NO: 111 - protein, 357 aa, synthetic construct
MLKLVIIENMAEIMLFSLDLLLFSTDILCFNFPSKMIKLPGFITIQIFFYPQASFGISANTILLLFHIFTFVFSHRSKSIDMIISHLSLIHILLLFTQAILVSLDFFGSQNTQDDLRCKVIVFLNKVMRGLSICTPCLLSVLQAIISPSIFSLAKLKHPSASHILGFFLFSWVLNMFIGVIFCCTLRLPPVKRGQSSVCHTALFLFAHELHPQETVFHTNDFEGCHLYRVHGPLKRLHGDYFIQTIRGYLSAFTQPACPRVSPVKRASQTILLLVSFVFIYWVDFTFSFSRGVTWINDSLLVWFQVIVANSYATISPLMLIYADNQIFKTLQMLWFKYLSPPKLMLKFNRQCGSTKK

SEQ ID NO: 112 - protein, 841 aa, synthetic construct
MLLCTARLVGLQLLLSCCWAFACHSTESSPDFSLPGDYLLAGLFPLHSGCLQVRHRPEVTLCDRSCSFNEHGYHLFQAMRFGIEEINNSTALLPNVTLGYELYDVCSESANVYATLRVLSLPGQHHIELQGDLLHYSPTVVAVIGPDSTNRAATTAALLSPFLVPLISYEASSETLSVKRQYPSFLRTIPSDKYQVETMVLLLQKFGWTWISLVGSSGDYGQLGVQALENQATGQGICIAFKDIMPFSAQVGDERMQCMMRHLAQARATVVVVFSSRQLARVFFESVVLANLTGKVWIASEDWAISRHITGVPGIQRIGTVLGVAIQQRAVPGLKEFEEAYARADKGAPRPCHKGSWCSSNQLCRECQAFTAHTMPKLKAFSMSSAYNVYRAVYAVAHGLHQLLGCASGACSRGRVYPWQLLEQIHKVNFLLHKDTVAFNDNGDPLSGYDIIAWDWSGPKWTFTVIGSSTWSPVQLDINETKIQWHGKDNQVPKSVCSSDCLEGHQRVVVGFHHCCFECVPCEAGTFLNKSDLYRCQPCGKEEWAPEGSQTCFPRTVVFLAWHEPTSWVLLAANTLLLLLLLGTAGLFAWHLDTPVVRSAGGRLCFLMLGSLAAGSCSLYGFFGEPTRPTCLLRQALFALGFAIFLSCLTVRSFQLVIIFKFSTKVPTFYHAWVQNHGAGLFVMISSAAQLLICLTWLVVWTPLPTREYQRFPHLVVLECTEANSLGFILAFLYNGLLSISAFACSYLGKDLPENYNEAKCVTFSLLLNFVSWIAFFTTASVYQGKYLPAVNVLAGLSSLSGGFSGYFLPKCYVILCRPDLNSTEHFQASIQDYTRRCGST

SEQ ID NO: 113 - protein, 837 aa, synthetic construct
MGPRAKTICSLFFLLWVLAEPAEDFYLPGDYLLGGLFTLHANMKGIVHLNFLQVPMCKEYEVKVLGYNLMQAMRFAVEEINNDSSLLPGVLLGYEMVDVCYISNNVQPVLYFLAQEDNLLPIQEDYSNYIPRVVAVIGPDNSESVMTVANFLSLFLLPQITYSAISDELRDKVRFPALLRTVPSADHHIEAMVQLMLHFRWNWIIVLVSSDDYGRDNSQLLGERLARRDICIAFQETLPTPQPNQNMTSEERQRLVTIVDKLQQSTARVVVVFSPDLTLHNFFNEVLRQNFTGAVWIASESWAIDPVLHNLTELRHTGTFLGITIQSVPIPGFSEFRVRGPQAGPPPLNRTSQSYTCNQECDNCLNATLSFNTILRLSGERVVYSVYSAVYAVAHALHSLLGCDKSTCTKRVVYPWQLLEEIWKVNFTLLGHQIFFDPQGDVPLHLEIIQWQWDLSQNPFQSIASYYPLQRQLKNIQDISWHTPNNTIPVSMCSKRCQPGQKKKPVGIHPCCFECIDCLPGTFLNHTADEFECQPCPSNEWSHQSDTSCFKRRLAFLEWHEAPTIAVALLAALGFLSTLAILVIFWRHFQTPMVRSAGGPMCFLMLTPLLVAYMVVPVYVGPPTVSTCLCRQALFTLCFTICISCITVRSFQIVCAFKMASRLPRAYSYWVRYHGPYVFVAFITVLKVVIVVINMLATGLSPTTRTDPDDPKIMILSCNPNYRNSLLFNTSLDLLLSVVGFSFAYMGKELPTNYNEAKFITLSMTFYFTSSVSLCTFMSVYSGVLVTIVDLLVTVLNLLGISLGYFGPKCYMILFYPERNTPAYFNSMIQGYTMRRD

SEQ ID NO: 114 - protein, 848 aa, synthetic construct
MLGPAVLGLSLWLHPGTGAPLCLSQQLRMKGDYVLGGLFPLGAEEAGLRSRTRPSSPVCTRFSSNGLLWALAMKMAVEEINNKSDLLPGLRLGYDLFDTCSEPVVAMKPSLMFLAKAGSRDIAAYCNYTQYQPRVLAVIGPHSSELALVTGKFFSFFLMPQVSYGASMDRLSNRETFPSFFRTVPSDRVQLTAAVELLQEFGWNWVAALGSDDEYGRQGLSLFSSLAAARGICIAHEGLVPLPRADDSRLGKVQDLLHQVNQSSVQVVVLFASARAAHALFSYSISSRLSPKVWVASEAWLTSDLVMTLPGMAQVGTVLGFLQRGAQLPEFPQYVKTHLALAADPAFCASLGAREQGLEEHVVGPRCPQCDHITLQNVSAGLLHHQTFAAYAAVYSVAQALHNTLQCNASGCPAQEPVRPQLLENMYNLSFHARGLPLRFDSSGNVDMEYDLKLWVWQGSVPRLHTVGRFNGSLQLERSKMRWHTPGNQKPVSQCSRQCQEGQVRRVKGFHSCCYDCVDCKAGSYRQNPDDLACTFCGQDQWSPERSTRCFPRRPRFLAWGEPAVLLLLLLLSLALGLVLAALGLFVHHRDSPLVQASGGPLACFGLVCLGLVCLSVLLFPGQPSPASCLAQQPLSHLPLTGCLSTLFLQAAEIFVESELPLSWADRLSGCLRGPWAWLVVLLAMLVEAALCAWYLVAFPPEVVTDWHVLPTEALVHCRTRSWVSFGLVHATNATLAFLCFLGTFLVQSQPGRYNRARGLTFAMLAYFITWVSFVPLFANVQVVYQPAVQMGAILLCALGILATFHLPKCYLLLWQPGLNTPEFFLGGGPGDAQGQNDGNTGNQGKHE

SEQ ID NO: 115 - protein, 309 aa, synthetic construct
MFSPEDNIFIIIITGEFIIGILGNGYIGLVNWIDWIKKKKISSIDYILTSLAISRICLICVMVLNGIIIVLYPDVYTNNKLQIVIFTFWTFANYLSMWFATCLNVFYFLKIANFSHPLFLWLKWRIDRVVHWILLGCLAISLLVSLIAAIVLSCDYRFHKIAKHKRNITEMFHVSKIQYFEPLTLFNLLAIVPFTVSLISFFLLIRSLWRHTKQMKLYVTGCRDPSTEAHVRAMKTMTSFLFLLFVYYISSLLMTFSYLMKEYKLAVMFGEIIAILYPSGHSLILIILNNKLRQASVRMLTCRKIACMM

SEQ ID NO: 116 - protein, 295 aa, synthetic construct
MIPIQLTVFFMIIYVLESLTIIVQSSLIVAVLGREWVQVRRLSPVDMILISLGICRFCLQWASMLYNFCSYFNPNYVFWYLTITWEFTNILTFWLTSLLAVFYCVKVSSFTHPIFLWLRWRILRLVPWLLLGSLMISCVTIIPSAIGNYIQIQLITMEHLPRNSTVTERLENFHQYFFQAHKTVALVIPFLLFLASTILLMASLTQHLEQMQHHSTGHCNSSMKAHFTALRSLAVFLIFFTSYFLTILISIIGTLFDKRSWFWVWEAFIYAFVSIHSTSLMLSSPTLKRVLKGKC

SEQ ID NO: 117 - protein, 335 aa, synthetic construct
MLTLTPIRTVSYEVKSTFLFLSVLEFAVGILTNAFIFLVNFWDVVRRQPLSNCDLVLLCLSITRLFLHGLLFLDAIQLTHFQKMKDPLSHSYQTIIMLWMIANQANLWLATCLSLLYCSKIVRFSHTFLLCLASWVSRKIPQMLLGAILFSCICTVLCLWDFFSRSHFTVTTVLFMNNNTELNLQIKKLNFFYSFLFCYLGSIPPFLLFLVSSGVLIVSLGRHMRTMKAYTRDSRDPSLEAHIKALKSLVSFLCFYVVSFCAALISVPLLILWHNKIGVMVCVGIMAACPSGHAAILISGNAKLRRAVMTILLWAQSSLKVRADHKADPRTPDLC

SEQ ID NO: 118 - protein, 312 aa, synthetic construct
MATGLDKIFLILAIAEFIIGMLGNVFIGLVNCSEWVKNQKVSSADFILTCLAISRIGQLLVILFDSFLVGLAPHLYTTYRLGKTVIMLWHMTNHLTTWLATCLSIFYFLKIAHFSHSLFLWLRWRMNRVILMLLILSLFLLIFDSLLLEIFIDISLNYIIDKSNLTLYLDESKTLYDKLLILLSLTYFIPFSLSLTSLLLLFLSLVRHTRNLQLNSLGSRDSSTEAHKRAMKMVMSFLFLFIVHFFSLQLANWIFFMLWNNKCIKFVMLALNAFPSGHSFILILGNSKLRQTALRLLWHLRNYLKTPNPLPL

SEQ ID NO: 119 - protein, 309 aa, synthetic construct
MITFLPIIFSILVVVTFVIGNFANGFIALVNSTEWVKRQKISFADQILTALAVSRIGLLWVLLLHWYSIVLNPAFYSVEVRITTYNVWAVTSHFSNWLATSLSIFYLLKIANFSNLIFLHLKRRVKSVILVMLLGPLLFLPCHLFVINMNQIVQTKEYEGNMTWKIKLRRTMFLSDTTVTMLANLVPFTLTLISFLLLICSLCKHLKKMQLHGKGSQDPNTKVHIKALQTVISFLLLCAIYFVFVTISVWSFQTLDNNPVFMFCQAITFSYPSAHPFILIWGNKKLKQTFLSVLWQVRYWVKGQKPSSP

SEQ ID NO: 120 - protein, 309 aa, synthetic construct
MITFLPIIFSILIVVTFVIGNFANGFIALVNSIEWVKRQKISFADQILTALAVSRVGLLWVLLLHWYATEFNLAFYSIEVRITAYNVWAVTNHFSNWLATSLSIFYLLKIANFSNLIFLHLKRRVKSVILVILLGPLLFLVCHLFVINMNQIVQTKEYEGNMTWKIKLRSAMYLSNMTVTMLANFVPFTLTLISFLLLICSLCKHLKKMQLHGKGSQDPSTKVHIKALQTVTSFLLLCAIYFLSIIMSVWSFESLENKPVFMFCQAIAFSYPSTHPFILIWGNKKLKQTFLSVLWHVRYWVKGQKPSSS

SEQ ID NO: 121 - protein, 309 aa, synthetic construct
MITFLPIIFSILVVVTFVIGNFANGFIALVNSIEWVKRQKISFADQILTALAVSRVGLLWVLLLNWYATVLNPAFYSVEVRTTTYNVWAVTSHFSNWLATSLSIFYLLKIANFSNLIFLHLKRRVKSVILVMLLGPLLFLACHLFVVNMNEIVRTKEYEGNMTWKIKLRSAVYLSDMTVTTLGNLVPFTLTLISFLLLICSLCKHLKKMQLHGKGSQDPSTKVHIKALQTVISFLLLCAIYFVSIIISVWSFESLENKPVFMFCQAIRFSYPSAHPFILIWGNKKLKQTFLSVLRQVRYWVKGQKPSSP

SEQ ID NO: 122 - protein, 298 aa, synthetic construct
MLESHLIIHFLLVIQFLTGVLANGIIVVVNGIDLIKQRKMAPLDLLLSCLAVSRIFLQLFIFYVNLIVLSLIEFIMCSANFAILLFVNELGLWLATWLGVFYCAKIASIRHPLFFWLKMRISKLVPWLILGSLLYVSMICVFHSKYAWFMVPYFLRKFFSQNATIQKEDTLAIQIFSLVAELSLPLLIFLFAVLLLIFSLGRHTRQMRNTVAGSRVPGRGAHISALLSILSFLILYFSHYMIKVLLSSQKFHIRSFIFLFCILVIGIYPSGHSLILILGNPKLKQNAKKFLLHSKCCQ

SEQ ID NO: 123 - protein, 316 aa, synthetic construct
MMGLTEGVFLVLSGTQFILGMLGNGFIGLVNGSSWFKSKRISLSDFIITTLALSRIVLLWILLTDGVLIVFSPKTHDSGIIMQIIDIFWTFTNHLSIWLATCLGVLYCLKIASFSHPTFLWLKWRVSRVVVWMLLGALLLSCGSTASLINEFKIYSVLRGIEATGNVTEHFRKKRSEYYLIHVLGTLWYLPPLIVSLASYFLLILSLGRHTRQMQQNGTSSRDPSTEAHKRAIRIILSFLFLFLLYFLAFLIASSSNFLPKTKMAKMIGEVITMFYPAGHSFILILGNNKLKQTFVEMLRCESGHLKPGSKGPIFP

SEQ ID NO: 124 - protein, 299 aa, synthetic construct
MLRLFYFSAIIASVILNFVGIIMNLFITVVNYKTWVKSHRISSSDRILFSLGITRFLMLGLFLLNTIYFVSSNTERSVYLSAFFLLCWMFLDSSSLWFVTLLNILYCVKITNFQHSVFLLLKRNLSPKIPRLLLACVLISAFTTLLYIVLSQASPFPELVTGRNNTSFDISEGILSLVVSLVLSSFLQFIINVTSASLLIHSLRRHIQKMQRNATGFWNPQTEAHVGAMKLMIYFLILYIPYSVATLLQYLPFYAGMDLGTKSICLIISTLYPPGHSVLIILTHPKLKTKAKKILCFNK

SEQ ID NO: 125 - protein, 295 aa, synthetic construct
MLSAGLGLLMLVAVAEFLIGLVGNGVLVVWSFGEWIRKFNWSSYNLIVLGLAGCRFLLQWLIMLDLSLFPLFQSSRWLRYLSVFWVLVSQASLWFATFLSVFYCKKITTFEHPVYLWLKQRAYNLSLWCLLGYFIINLLLTVQIGLTFYHPSQGNSSILYPFSSWHYLYILQLNSGSYLPFMVFLVSSGMLIVSLYRHHRKMKVHTAGRRDARAKAHITVLKSLGCFLILHLVYILASPFSITSKTYPADLTSVFISETLMAAYPSLHSVILIMGNPRVKQTCQRILWKTVCAWR

SEQ ID NO: 126 - protein, 312 aa, synthetic construct
MADKVQTTLMLIAVGEFSVGILGNAFIGLVNCMDWIKNRKIASIDLILTSLAISRICLLCIILLDCFILVLYPDVYATGKQMRIIDFFWTLTNHLSVWFATCLSIFYFLKIANFFHPLFLWMKWRIDRVISRILLGCLVLSVFISLPVTENLNDDFRFCVKAKRKTNLTWRCRVNKAQYASTKLFLNLLTLFPFSVSLISFLLLILSLWRHTRQMQLSATGCRDPSTEAHVGAMKAVISFLLLFIAYYLAFLIATSSYFMPETELAVIFGELIALIYPSSHSFILILGNNKLRQASLRVLWKVKSILKRRKF

SEQ ID NO: 127 - protein, 311 aa, synthetic construct
MPSTIEAIYIILIAGELTIGIWGNGFIVLVNCIGWLKRRDISLIDIILVSLAISRICLLCVISLDGFFMLLSPDTYGNSVLMSIVDVFWTLSNHSSVWFTSCLSIFYLLKIANISHPFFLWLKLKINRVILGILLGSFLISLIISVSLNEMWWHLFKVNHEENITWEFKVSKIPGAFKQIILNLGAMVPFILCLISFFLLLFSLFRHTKQMKLHATGSRDPSTEAHMRAIKAVIIFLLLFIMYYAVFLVVTSSALIPQGKLVLMFGGIVTVIFPSSHSFILIMGNSKLREAFLKVLRFVKGFHKRRKPFVP

SEQ ID NO: 128 - protein, 308 aa, synthetic construct
MLSVVEGILIFVAVSESVLGVLGNGFIGLVNCIDCVKNKKLSTIGFILTGLAISRICLIWIIITDGFIKIFSPDMYASGNLIEYISYFWVIGNQSSMWFATSLSIFYFLKIANFSHYIFLWLKSRINMVLPLLMGFLLISWLLNFPQIVKILNDYKMKNRNTTWDLNMYKSEYFIKQILLNLGVIFFFTLSLITCFLLIISLWRHNRQMQLNVTGFRDSSTEAHVKAMKVLISFIILFILYFIGIAIEISCTVRENNKLLFIFGMTTTAIYPWGHSFILILGNSKLKQASLRVLQQLKCEKRKNLRVT

SEQ ID NO: 129 - protein, 303 aa, synthetic construct
MESALPSIFTLVIIAEFIIGNLSNGFIVLINCIDWVSKRELSSVDKILIILAISRIGLIWEILVSWFLALHYLAIFVSGTGLRIMIFSWIVSNHFSLWLATILSIFYLLKIASFSSPAFLYLKWRVKKVILMILLGTLVFLFLNLIQINMHIKDWLDRYERNTTWNFSMSDFETFSVLVKFTMTMFSLTPFTVALISFLLLIFSLWKHLQKMQLNYKGHRDPRTKAHINALKIVISFLLLYASFFLSVLISWISELYQNTLIHMLCETIGVFYPSSHSFILILGNAKLRQAFLLVAAKVWAKR

SEQ ID NO: 130 - protein, 312 aa, synthetic construct
MGGVIKSIFTFILIVEFIIGNLGNGFIALVNCIDWVKRRKISSVDQILTALAISRISLLWLIFGSWCVSVFFPALFATEKMFRMLTNIWTVTNHFSVWLATGLSIFYFLKIANFSNSIFLYLKWRVKKVVSVTLLVSLVLLFLNIALINIHINASINGYRRNKTCSSDSSNFTRFSSLILLTNTVFIFIPFTVSLATFLLLIFSLWKHLKKMQHTAKGSRDASTKAHRKALQTVITFLLLYAIFFLSFFISVWTSERLEENLIIIFSQVMGMAFPSGHSCVLILGNKKLRQASLSVLLWLRCRFSGHKEFRE

SEQ ID NO: 131 - protein, 309 aa, synthetic construct
MMSFLPIVFSILVVVAFILGNFANGFIALINFIAWVKRQKISSADQIIAALAVSRVGLLWVILLHWYATVLNPTSSSLKVRIFISNAWAVTNHFSIWLATSLSIFYLLKIVNFSRLIFHHLKRKVKSVVLVIVLGSLFFLVCHLVMKNTYINVWTKEYEGNVTWKIKLRNAMHLSNLTVATLANLIPFTLTLISFLLLIYSLCKHLKKMQLHGKGSQDPSTKIHIKALQTVTSFLILFAIYFLCLIISFWNSKMQQKELVLMLCQAFGIIYPSFHSFILIWGNKKLKQTFLSVLWQVTCWAKGQNQSTP

SEQ ID NO: 132 - protein, 309 aa, synthetic construct
MITFLPIIFSILIVVIFVIGNFANGFIALVNSIEWVKRQKISFVDQILTALAVSRVGLLWVLLLHWYATQLNPAFYSVEVRITAYNVWAVTNHFSSWLATSLSMFYLLKIANFSNLIFLRIKRRVKSVVLVILLGPLLFLVCHLFVINMDETVWTKEYEGNVTWKIKLRSAMYHSNMTLTMLANFVPLTLTLISFLLLICSLCKHLKKMQLHGKGSQDPSTKVHIKALQTVTSFLLLCAIYFLSMIISVCNFGRLEKQPVFMFCQAIIFSYPSTHPFILILGNKKLKQIFLSVLWHVRYWVKXQKPSSP

SEQ ID NO: 133 - protein, 321 aa, synthetic construct
MTKTCDPAENELSPFLITLILTIIGTECIIGIIANGFIMAINAAEWIQNKAVSTSGRILVFLSVSRIALQSFMMLEITISSTSPSFYNEDAVYYAFKVSFMFLNFCSLWFAAWLSFFYFVKIADFSYPLFLKLKWRISGLMPWLLWLSVFISLGHSVLFCINIYTVYCNNSFPIPSSNSTKKKYFTETNVVNLALLYNLGIFIPLIMFILAATLLIISLKRHTLHMGSNATGSRDPSMEAHMGAIKATSYFLILYIFNAVALFLYMSNIFDINSLWNILCKIIMAAYPAGHSILLIQDNPGLRRAWKRLQLQVHLYLKWTL

SEQ ID NO: 134 - protein, 318 aa, synthetic construct
MATVNTDATDKDISRFKITFTLVVSGIECITGILGNGFITAIYGAEWARGKRLPTGDCILLMLSFSRLLLQIWMMLENTYSLLFRIVYNQNTVYILFKVITVFLNYSNLWLAAWLNVFYCLRIANFNHPLFFLMKRKIIVLMPWLLRLSVLVSLCFSFPFSKDIFNVYVNSSIPIPSSNSTEKKYFSETNVVNLVFLYNLGIFIPLIMFILAATLLILSLKRHTLHMGSNATGSRDPSMEAHIGAIKATSYFLILYIFNAVALFLSMSNIFDTYSSWNILCKIIMAAYPAGHSVLLILGNPGLRRAWKRFQHQVHLYL

SEQ ID NO: 135 - protein, 308 aa, synthetic construct
MITFLPIIFSILVVVTFVIGNFANGFIALVNSIEWVKRQKISFADQILTALAVSRVGLLWVLLLNWYSTVLNPAFYSVEVRTTAYNLWAVTSHFSNWLATSLSIFYLLKIANFSNLIFLHLKRRVKSVILVILLGPLLFLVCHLFVINMNEIVRTKEYEGNMTWKIKLRSAMYLSNTTVTMLANLVPFTLTLISFLLLICSLCKHLKKMQLHGKGSQDPSTKVHIKALQTVISLLLCAIYFLSIMISVWSLGRLENKAVFMFCKAIRFSYPSAHAFILIWGNKKLKQTFLSVLWQVRYWVKGQKTSSP

SEQ ID NO: 136 - protein, 299 aa, synthetic construct
MITFLHIFFSVLILVLFVLGNFANGFIALVNFIDWVKRKKISSADQILTALAVSRVGLLWALLLNWYLTVLNPAFYSVELRITSYNAWVVTNHFSMWLAASLSIFYLLKIANFSNLIFLHLKRRVRSIILVILLGTLLFLVCHLLVVNMDENMWTEEYEGNMTGKMKLRNTAHLSYMTVTTLWSFIPFTLSLISFLMLIFSLCKHLKKMQLHGEGSQDPSTKVHIKALQTLISFLLLCAIFFLFLIISVWSPRRLQNEPVFMVCKAVGNIYLSFDSFILIWRTKKLKHTFLLILCQIRC

SEQ ID NO: 137 - protein, 318 aa, synthetic construct
MNGDHMVLGSSVTDKKAIILVIILLLLCLVAIVGNGFITAALGMEWLLRRTLSPCDKLLVSLGASRFCLQWVVMGKTIYVFLHPMAFPYNPVLQFLAFQWDFLNAATLWFSTWLSVFYCVKIATFTHPVFLWLKHKVSGWVPWMLLSSVGLSSLSTILFFIGNQRIYQNYLRNHLQPWNVTGNSIRSYCEKFYFFPLKMVTWTVPTVVFFICMILLITSLGRHRKKALLTTSGFRDPSAQAHIKALLALLSFAILFISYFLSLVLSAAGIFPPLEFRFWVWQSVIYLCTAVHPIILLFSNCRLRAVLKRGCSSRCGTP

SEQ ID NO: 138 - protein, 335 aa, synthetic construct
MPFCHNIINISCVKSSWSNDVRASLYSLMVLIILTTLVGNLIVIISISHFKQLHTPTNWLIHSMATVDFLLGCLVMPYSMVRSVEHCWYFGEVFCKIHTSTDIMLSSASIFHLSFISIDRYYAVCDPLRYKAKINILVICVMIFISWSVPAVFAFGMIFLELNFKGAEEIYYKHVHCRGGCSVFFSKTSGVLAFMTSFYIPGSIMLCVYYRIYLIAKEQARSISDANQKLQIGLEMKNGISQSKERKAAKTLGIVMGVFLICWCPFFICTVMDPFLHYIIPPTLNDALIWFGYLNSTFNPMVYAFFYPWFRRALKMILFGKIFQKDSSRCKLFLE

SEQ ID NO: 139 - protein, 306 aa, synthetic construct
MYSFMAGAIFITVFGNLAMIISISYFKQLHTPTNFLILSMAVTDFLLGFTIMPYSMIRSVENCWYFGLTFCKIHYSFDLMLSITSIFHLCSVAIDRFYAICYPLLYSTKMTIPVIKRLLLLCWSVPGAFAFGVVFSEAYADGIEGYDILVACSSSCPVMFNKLWGTTLFMAGFFTPGSVMVGIYGKIFAVSRKHARAINNLPENQNNQMRKDKKAAKTLGIVMGVFLLCWFPCFFTILLDPFLNFSTPVVLFDALTWFGYFNSTCNPLIYGFFYPWFRRALKYILLGKIFSSHFHNTNLFTQKETE

SEQ ID NO: 140 - protein, 337 aa, synthetic construct
MRAVFIQGAEEHPAAFCYQVNGSCPRTVHPLGIQLAIYLACAAGMLITVLGNLFVVFAVSYFKALHTPTNFLLLSLALADMLLGLLVLPLSTIRSVESCWFFGDFLCRLHTYLDTLFCLTSIFHLCFISIDRHCAICDPLLYPSKFTVRVALRYILAGWGVPAAYTAFFLYTDVVETGLSQWLEEMPCVGSCQLLFNKFWGWLNFPVFFFPCLIMISLYVKIFVVATRQAQQITTLSKSLAGAAKRERKAAKTLGIAVGIYLLCWLPFTIDTMVDSLLNFITPPLVFDIFIWFAYFNSACNPIIYVFSYRWFRKALKLTLSQKIFSPRTRTVDLYQE

SEQ ID NO: 141 - protein, 342 aa, synthetic construct
MTSNFSQPVVQLCYENVNGSCIKTPYSPGSRVILYTVFGFGSLLAVFGNLLVMTSVLHFKQLHSPANFLIASLACADFLVGVTVMPFSMVRSVESCWYFGAKFCTLHSCCDVAFCYSSLFHLCFISIDRYIAVTDPLVYPTKFTVSVSGICISISWILPLVYSGAVFYTGVSDDGMEELVSALNCVGGCQIVVNQDWVLIDFLLFFIPTLVMIILYSKIFLVAKQQAIKIETTGSKAESSSESYKARVAKRERKAAKTLGVTVVAFMISWLPYTIDTLIDAFMGFITPAYIYEICCWGAYYNSAMNPLIYALFYPWFRKAIKLILSGEVLKASSSTISLFSE

SEQ ID NO: 142 - protein, 348 aa, synthetic construct
MVNNFSQAEAVELCYENVNGSCIKTPYSPGPRAILYAVLGFGAVLAVFGNLLVIIAILHFKQLHTPTNFLIASLACADFLVGVTVMPFSTVRSVESCWYFGESYCKFHTCFDTSFCFASLFHLCCISIDRYIAVTDPLTYPTKFTVSVSGICIVLSWFFSVTYSFSIFYTGANEEGIEELVVALTCVGGCQAPLNQNWVLLCFLLFFIPTVAMVFIYGKIFLVAKHQARKIESTASQAQSSSESYKERVAKRERKAAKTLGIAMAAFLVSWLPYIIDAVIDAYMNFITPPYVYEILVWCVYYNSAMNPLIYAFFYPWFRKAIKLIVSGKVLRTDSSTTNLFSEEADTD

SEQ ID NO: 143 - protein, 345 aa, synthetic construct
MSSNSSPLAAVQLCYENVNGSCVKTPYSPGSRVILYIVFGFGAVLAVFGNLLVMISILHFKQLHSPTNFLIASLACADFLVGVTVMPFSMVRSVESCWYFGRSFCTFHTCCDVAFCYSSLFHLCFISIDRYIAVTDPLVYPTKFTVSVSGICISISWILPLVYSGAVFYTGAYDDGLEELSSALNCVGGCQTVVNQNWVLIDFLSFFIPTLVMIILYSNIFLVARQQAKKIENTGSKTESSSESYKARVAKRERKAAKTLGITVVAFMISWLPYSIDSLIDAFMGFITPAYIYEICCWCAYYNSAMNPLIYALFYPWFRKAIKVIVSGQVFKNSSATMNLFSEQI

SEQ ID NO: 144 - protein, 311 aa, synthetic construct
MEPREAGQHVGAANGAQEDVAFNLIILSLTEGLGLGGLLGNGAVLWLLSSNVYRNPFSIYLLDVACADLIFLGCHMVAIIPDLLQGRLDFPGFVQTSLATLRFFCYIVGLSLLAAVSVEQCLATLFPAWYSCRRPRHLTTCVCALTWALCLLLHLLLSGACTQFFGEPSRHLCRTLWLVAAVLLALLCCTMCGASLLLLLRVERGPQRPQPRGFPGLVLLAVLLFLFCGLPFGIYWLSRNLLWHIPHYFYHFSFLMAAVHCAAKPVIYFCLGSAQGRRLPLRLVLQRALGDEAELGAVRETSRRGLVDIAA

SEQ ID NO: 145 - protein, 343 aa, synthetic construct
MAGNCSWEAHPGNRNKMCPGLSEAPELYSRGFLTIEQIAMLPPPAVMNYIFLLLCLCGLVGNGLVLWFFGFSIKRNPFSIYFLHLASADVGYLFSKAVFSILNTGGFLGTFADYVRAVCRILGLCMFLTGVSLLPAISAERCLSVIFPAWYWRRRPKRLSAVVCALLWVLSLLVTCIHNYFCVFLGRGASGAACRHMDIFLGILLFLVFCPLMVLPCLALILHVECRARRRQRSAKLNHVILAMVSVFLVSSIYLGIDWFLFWVFQIPAPFPEYVTDLCICINSSAKPVVYFLAGRDKSQRLWEPLRVVFQRALRDGAELGEAGGGTPNTVTMEMQCPSGNAS

SEQ ID NO: 146 - protein, 325 aa, synthetic construct
MDGSNVTSFVVEEPTNISTGRNASVGNAHRQIPIVHWVIMSISPVGFVENGILLWFLCFRMRRNPFTVYITHLSIADISLLFCIFILSIDYALDYELSSGHYYTIVTLSVTFLFGYNTGLYLLTAISVERCLSVLYPIWYRCHRPKYQSALVCALLWALSCLVTTMEYVMCIDREEESHSRSDCRAVIIFIAILSFLVFTPLMLVSSTILVVKIRKNTWASHSSKLYIVIMVTIIIFLIFAMPMRLLYLLYYEYWSTFGNLHHISLLFSTINSSANPFIYFFVGSSKKKRFKESLKVVLTRAFKDEMQPRRQEDNCNTVTVETVV

SEQ ID NO: 147 - protein, 317 aa, synthetic construct [sequence omitted]

SEQ ID NO: 148 - protein, 312 aa, synthetic construct
MNQTLNSSGTSALNSYSRGSTVHTAYLVLSSLAMFTCVCGMAGNGMVIWLLGFRMQRTPFCIYVLNLAVADLLFLLCMASTLSLETQPLDKVHEVMKRLKYFAYTAGLSLLTAISTQRCLSVLFPIWYKCHRPRHLSAVVCALLWALCLLMNGLASSFCSKFWKFNEDQCFRVDMVQAALIMGVFTPVMTLSSLTLFVRVRRSSQQWRRPTRLYVVILASVLVFLICSLPLGIYWFVLYWLSLPPEMQVLCFSLSRLSSSVSSSANPVIYFLVGSRRSLPEPLGAVLQRALREEPELEGRETPSTGTNEMGA

SEQ ID NO: 149 - protein, 289 aa, synthetic construct
MFGLFGLWRTFDSVVFYLTLAVGLGGLVGNGLVLWHLGFHIKKGPFSVYLLHLAAADFLFLSCQVGFSVAQAALGAQDTLYFVVTFLWFAVGLWLLAAFSVERCLSDLFPACYQGCRPRHTSAVLCALVWALTLPAVLLPANACGLLRNSARPLVCLRYHVASVTWLLVLACVACTAGLVLFVWVTCCSTRPRPRFYGIVLGSLLLLFFCGLPSVLYWSLRPLLNFLLPVFSPLATLLACVNSSSKPLIYFGLGRQPGKREPLRSVLQRALGEGAELGAGGQSLPMGLL

SEQ ID NO: 150 - protein, 321 aa, synthetic construct
MDPTISALDTELTPINGTEETLCYKQTLSLTVLTCIISLVGLTGNAVVLWLLGFRMRRNAFSIYILNLAAADFLFLSGRLIYSLLSFISIPHTISKILYPVMMFSYFAGLSFLSAISTERCLSVLWPIWYRCRRPTHLSAVVCVLLWALSLLRSILEWMLCGFLFSGADSVWCQTSDFITVAWLIFLFVVLCGSSLVLLIRILCGSRKIPLTRLYVTILLTVLVFLLCGLPFGIQFFLFLWIHVDREVLFCHVLVSIFLSALNSSANPIIYFFVGSFRQRQNRQNLKLVLQRALQDTPEVDEGGGQLPEETLELSGSRLEQ

SEQ ID NO: 151 - protein, 329 aa, synthetic construct
MDPTTPAWGTESTTVNGSDQALLLLCGKETLIPVLLILIIALVGLAGNAFVLWLLGFRMRRNAFSVYILNLAGADFLFLCFQIINCLVYLINFFHSISINIPSFFTTVMTFAYIAGLSMLSAISTERCLSVLWPIWYRCRRPRHLSAVMCALLWALSLLLSILEGKYCGFLFSDFGDSWCQTFDFITAAWLIFLFVLLSGSSLALLVRILCGSRRLPLTRLYVTILLTVLVFLLCGLPFGIQWFLLLWIWKDSDVLFCHLHLVSVVLSCVNSCANPIIYFFVGSFRQRWRLQPTLKLVLQRALQDTAEVDESEGSLPQETLEMSGSSLV

SEQ ID NO: 152 - protein, 322 aa, synthetic construct
MDPTIPALGTELTPINGREETPCYKQTLSLTVLTCIISLVGLTGNAVVLWLLGFRMRRNAVSTYILNLAAADFLFLSGHVIRSPLRLINIRHPISKILNPVMTFPYFIGLSMLSAISTERCLSVLWPIWYRCRRPRHLSSVVCVLLWVLSLLRSILEWMFCDFLFSGADSVWCETSDFITIAWLIFLCVVLCGSSLVLLVRILCGSRKMPLTRLYVTILLTVLVFLLCGLPFGIQWALFSRIHLDWKVLFCHVHLVSIFLSSLNSSANPIIYFFVGSFRQRQNRQNLKLVLQRALQDTPEVDEGGGRLPEETLELSGSRLEQ

SEQ ID NO: 153 - protein, 322 aa, synthetic construct
MDPTIPALGTSLTPINGREETPCYKLTLSLTVLTCIISLVGLTGNAVVLWLLGFRMRRNAVSIYILNLAAADFLFLSGHVIRFLLRLINIPHTIRRILVCVMTVPYLTGLSMLSAISTERCLSVLWPIWYRCRRPTHLSAVVCVLLWALSLLRSILEWRFCDFLFSGADSCWCETSNFIPIAWLTFLCVVLCVSSLVLLVRILCGSRKMPLTRLYVTILLTVLVFLLCGLPFGILGSLNYMIHRDLEVLYCHVYRVCMFLSSLNSSANPIIYFFVGSFRQRQNRQNLKLVLQRALQDTPEVDEGGGRLPEETLELSGSRLRQ

SEQ ID NO: 154 - protein, 330 aa, synthetic construct
MMWGAGSPLAWLSAGSGNVNVSSVGSAEGPTGPAAPLPSPKAWDVVLCISGTLVSCENALVVAIIVGTPAFRAPMFLLVGSLAVADLLAGLGLVLHFAAVFCIGSAEMSLVLVGVLAMAFTASIGSLLAITVDRYLSLYNALTYYSETTVTRTYVMLALVWGGALGLGLLPVLAWNCLDGLTTCGVVYPLSKNHLVVLAVAFFMVFGIMLQLYAQICRIVCRHAQQIALQRHLLPASHYVATRKGIATLAVVLGAFAACWLPFTVYCLLGDAHSPPLYTYLTLLPATYNSMINPIIYAFRNQDVQKVLWAVCCCCSSSKIPFRSRSPSDV

SEQ ID NO: 155 - protein, 359 aa, synthetic construct
MGNHTWEGCHVDSRVDHLFPPSLYIFVIGVGLPTNCLALWAAYRQVRQRNELGVYLMNLSIADLLYICTLPLWVDYFLHHDNWIHGPGSCKLFGFIFYTNIYISIAFLCCISVDRYLAVAHPLRFARLRRVKTAVAVSSVVWATELGANSAPLFHDELFRDRYNHTFCFEKFPMEGWVAWMNLYRVFVGFLFPWALMLLSYRGILRAVRGSVSTERQEKAKIKRLALSLIAIVLVCFAPYHVLLLSRSAVYLGRPWDCGFEERVFSAYHSSLAFTSLNCVADPILYCLVNEGARSDVAKALHNLLRFLASDKPQEMANASLTLETPLTSKRNSAKAMTGSWAATPPSQGDQVQLKMLPP

SEQ ID NO: 156 - protein, 356 aa, synthetic construct
MNASAASLNESQVVAVAAEGAAAAAPDTGEWGPPAAALGAGGAANGSLELSSQLPAGPPGLLLSAVNPWDVLLCVSGTVIAGENALVVALIASTPALRTPMFVLVGSLATADLLAGCGLILHFVFQYVVPSETVSLLTVGFLVASFAASVSSLLAITVDRYLSLYNALTYYSRRTLLGVHLLLAATWTVSLGLGLLPVLGWNCLAERAACSVVRPLTRSHVALLSAAFFMVFGIMLHLYVRICQVVWRHAHQIALQQHCLAPPHLAATRKGVGTLAVVLGTFGASWLPFAIYCVVGSHEDPAVYTYATLLPATYNSMINPIIYAFRNQEIQRALWLLFCGCFQSKVPFRSRSPSEV

SEQ ID NO: 157 - protein, 333 aa, synthetic construct
MNEDLKVNLSGLPRDYLDAAAAENSAAVSSQVPVVEPEPELVVNPWDIVLCTSGTLISCENAIVVLIIFHNPSLRAPMFLLIGSLALADLLAGIGLIINFVFAYLLQSEATKLVTIGLIVASFSASVCSLLAITVDRYLSLYYALTYHSERTVTFTYVMLIMLWGTSICLGLLPVMGWNCLRDESTCSVVRPLTKNNAAILSVSFLFMFALMLQLYIQICKIVMRHAHQIALQHHFLATSHYVTTRKGVSTLAIILGTFAACWMPFTLYSLIADYTYPSIYTYATLLPATYNSIINPVIYAFRNQEIQKALCLICCGCIPSSLSQRARSPSDV

SEQ ID NO: 158 - protein, 360 aa, synthetic construct
MDPEATSVYLDYYYATSPNPDIRETHSHVPYTSVFLPIFYTAVFLTGVLGNLILMGALHFKRGSRRLIDIFIINLAASDFIFLVTLPLWVDKEASLGLWRTGSFLCKGSSYMISVNMHCSVFLLTCMSVDRYLAIMCPAVSRKFRRRDCAYGVCASVWFISCLLGLPTLLSRELTLIDDKPYCAEKKATPIKLIWALVALIFTFFVPLLSIVTCYCCITRKLCAHYQQSGKHNKKLRKSIKIIFIVVAAFVFSWLPFNTFKLLAIVSGLQQEHYFSSAILQLGMEVSGPLAFANSCVNPFIYYIFDSYIRRAIVHCLCPCLKNYDFGSSTETSDSHLTKALSNFIHAEDFARRRKRSVSL

SEQ ID NO: 159 - protein, 339 aa, synthetic construct
MNGLEVAPPSLITNFSLATAEQCGQETPLENMLFASFYLLDFILAFVGNALALWLFIRDHKSGTPANVFLMHLAVADLSCVLVLPTRLVYHFSGNHWPFGEIPCRLTGFLFYLNMYASIYFLTCISADRFLAIVHPVKSLKLRRPLYAHLACAFLWVVVAVAMAPLLVSPQTVQTNHTVVCLQLYREKASHHALVSLAVAFTFPFVTTVTCYLLIIRSLRQGPRVEKRLKTKAVRMIAMVLAIFLVCFVPYHVHRSVYVLHYRGSHTSCAAQRILALGNRITSCLTSLNGALDPVMYFFVAEKFRHALCNLLCGKRLKGPPPSFEGKTNESSLSARSEL

SEQ ID NO: 160 - protein, 415 aa, synthetic construct
MVFAHRMDNSKPPLVIPTLLVPLQNHSCTETATPLPSHDLMELSEEHSWMSNRTDLQYGLKPGEVATASIFFGALWLFSIFGNSLVCLVIHRSRRTQSTTNYFVVSMACADLLISVASTPFVLLQFTTGRWTLGSAMCKVVRYFQYLTPGVQIYVLLSICIDRFYTIVYPLSFKVSREKAKKMIAASWIFDAAFVTPVFFFYGSNWDSHCNYFLPSSWEGTAYTVIHFLVGFVIPSVLIILFYQKVIKYIWRIGTDGRTVRRTMNIVPRTKVKTIKMFLILNLLFLLSWLPFHVAQLWHPHEQDYKKSSLVFTAITWISFSSSASKPTLYSIYNANFRRGMKETFCMSSMKCYRSNAYTITTSSRMAKKNYVGISEIPPMAKTITKDSIYDSFDREAKEKKLAWPINSNPPNTFV

SEQ ID NO: 161 - protein, 358 aa, synthetic construct
MPSVSPAGPSAGAAPNATAVTNASGPEVPLFHLFARLDEELHGTFPGLWLALMAVHGAIFLAGLVLNGLALYVFCCRTRAKTPSVIYTINLVVTDLLVGLSLPTRFAVFYGARGCLRCAFPHVFGYFLNMHCSILFLTCICVDRYLAIVQPEGSRRWRQPACARAVCAFVWLAAGAVTLSVLGVTGSGRPCCRVFALTVLEFLLPLLVISVFTGRIMCALSRPGLLRQGRQRRVRAMQLLLTVLVIFLVCFTPFHARQVAVALWPDMPHHTSLVVYHVAVTLSSLNSCMDPIVYCFVTSGFQATVRGLFRQHGAEREPSSGDVVSMHKSSKGSGGRHHILSAGPHALTQQALANGPEA

SEQ ID NO: 162 - protein, 348 aa, synthetic construct
MNSTLDGNQSSHPFCLLAFGYLETVNFCLLEVLIIVFLTVLIISGNIIVIFVFHCAPLLNHHTTSYFIQTMAYADLLVGVSCLVPSLSLLHYPLPVEESLTCQIFGFVVSVLKSVSMASLACISIDRYIAITKPLTYNTLVTPWRLRLCIFLIWLYSTLVFLPSFFHWGKPGYHGDVFQWCAESWHTDPYFTLFIVMMLYAPAALIVCFTYFNIFRICQQHTKEISERQARFSSQSGETGEVQACPDKRYAMVLFRITSVFYILWLPYIIYFLLESSTGHSNRFASFLTTWLAISNSFCNCVIYSLSNSVFQRGLKRLSGAMCTSCASQTTAKDPYTVRSKPLNGCHV

SEQ ID NO: 163 - protein, 433 aa, synthetic construct
MCFSPILEINMQSESNITVRDDIDDINTNMYQPLSYPLSFQVSLTGFLMLEIVLGLGSNLTVLVLYCMKSNLINSVSNIITMNLHVLDVIICVGCIPLTIVILLLSLESNTALICCFHEACVSFASVSTAINVFAITLDRYDISVKPANRILTMGRAVMLMTSIWIFSFFSFLIPFIEVNFFSLQSGNTWENKTLLCVSTNEYYTELGMYYHLLVQIPIFFFTVIVMLITYTKILQALNIRIGTRFSTGQKKKARKKKTISLTTQHETTDMSQSSGGRNVVFGVRTSVSVIIALRRAVKRHRERRERQKRVFRMSLLIISTFLLCWTPISVLNTTILCLGPSDLLVKLRLCFLVMAYGTTIFHPLLYAFTRQKFQKVLKSKMKKRVVSIVEADPMPNNAVIHNSWIDPKRNKKITFEDSEIREKCLVPQVVTD

SEQ ID NO: 164 - protein, 362 aa, synthetic construct
MAPTEPWSPSPGSAPWDYSGSGGLEELELCPAGDLPYGYVYIPALYLAAFAVGLLGNAFVVWLLAGRRGPRRLVDTFVLHLAAADLGFVLTLPLWAAAAALGGRWPFGEGLCKLSSFALAGTRCAGALLLAGMSVDRYLAVVKLLDARPLRTPRCALASCCGVWAVALLAGLPSLVYRGLQPLPGGQDSSQCGEEPSDAFQGLSLLLLLLTFVLPLVVTLFCYCRISRRLRRPPHVGRARRNSLRIIFAIESAFVGSWLPFSALRAVFHLARLGALPLPCPLLLALRWGLTIATCLAFVNSCANPLIYLLLDRSFRARALWDGACGRTGRLARRISSASSLSRDDSSVFRCRAQAANTASAS

SEQ ID NO: 165 - protein, 335 aa, synthetic construct
MNSWDAGLAGLLVGTMGVSLLSNALVLLCLLHSADIRRQAPALFTLNLTCGNLLCTVVNMPLTLAGVVAQRQPAGDRLCRLAAFLDTFLATNSMLSMAALSIDRWVAVVFPLSYRAKMRLRDAALMVAYTWLHALTFPAAALALSWLGFHQLYASCTLCSRRPRLRFAVFTGAFHALSFLLSFVVLCFTYLKVLKVARFHCKRIDVITMQTLVLLVDIHPSVRERCLEEQKRRRQRATKKISTFIGTFLVCFAPYVITRLVELSSTVPIGSHWGVLSKCLAYSKAASDPFVYSLLRHQYRKSCKDILNRILHRRSIHSSGLTGDSHSQNILPVSE

SEQ ID NO: 166 - protein, 373 aa, synthetic construct; identical to SEQ ID NO: 59

SEQ ID NO: 167 - protein, 312 aa, synthetic construct
MPFPNCSAPSTVVETAVAVLLGLECGLGLLGNAVALWTFFFRLKVWKPYAVYLLNLVLADLLLAACLPFLAAFYLRLKTWHLGRVGCQALLFLLDLSRGVGVAFLTAVALDRYLRVVHPRLKVNLLSPRAAWGISGLVWLLMVALTHLSLISESTECPSFYPRDGSFSIIWQEALFFLQFVLPFGLILFCNAGIIRTLQKRLRDPDKQPKLQRAQALVTLVVVLFALCFLPSFLARVLMAIFRNLGSCRALCAVVHTSDVTGSLTYLQSVLNPVVYCFSNPAFRSSYRKVFHLRGRGQAAEPPGFDPRDSYS

SEQ ID NO: 168 - protein, 327 aa, synthetic construct
MNSSGCLPEEVGSLRPLTVAVLSVSFVVGVVGNGLVLWMTVFRMARTVTTVWFFNLALADFMLLLSLPIAIYYIASGQWLLGEWACKLYITFLFLSFFASICLLVLISVDRCISVLYPVWALNHRTVQRASWLAFGVWLLAAVLCSPHLKFRTTRKWNGCTYCYFAFNSENETAQIWIEGVVEGHIIVTIGHFLLGFLVPLAIIGTCAHLIRAKLLREGWVHANRPKRLLLVLVSAFFIFWFPFNVVLLVHLWRRMLKEIYHPRMLLILWATFSLGCVNSCLNPFLYVFIGRDFQEKFFQSLPSALARAFGEEGFLSSCPRGNAPRE

SEQ ID NO: 169 - protein, 340 aa, synthetic construct
MDLINSTDYLINASTLVRNSTQFLAPASKMIIALLLFISFIIGTITNGLYLWVLKFKMKKTVNTLLFFHLILSYFISTLILPFMATSQLQDNHWNFGTAMCKVFNGTLSLGMFASVFFLSAISLDRYLLTLHPVWSQQHRTPRWASSIVLGVWISAAALSIPYLVFRETHHDHKGRVTCQNNYAVSTNWESKEMQTLRQWIHVACFISRFLLGFLLPFFIIIFCYERVASKMKERGLFKSSKPFKVMMTAIISFFVCWMPYHVYQGLLLTKNQSLLLELTLILTVLTTSFNTIFSPTLYLFVGENFKKVFKKSILALFESTFSEDSSVERTQNLNSEAYI

SEQ ID NO: 170 - protein, 374 aa, synthetic construct
MTTTSVSSWPYSSHRMRFITNHSDQPPQNFSATPNTTSCPMDEKLLSTVLTTFYSVIFIVGLVGNIIALYVFLGIHRKRNSIQIYLLNVAIADLLLIFCLPFRIMYHINQNKWTLGVILCKVVGTLFYMNMYISIILLGFISLDRYIKINRSIQQRKAITTKQSIYVCCIVWMLALGGFLTMIILTLKKGGHNSTMCFHYRDKHNAKGEAIFNYILVVMFWLIFLLIILSYIKIGKNLLRISKRRSKFPNSGKYATTARNSFIVLIIFTICFVPYHAFRFVYISSQLNVSSCYWKEIVHKTNEIMLVFSSFNSCLDPVMYFLMSSNIRKIMCQLLFRRFQGEPSRSESTSEFKPGYSLHDTSVAAKIQQSSSKS

SEQ ID NO: 171 - protein, 305 aa, synthetic construct
MNGTNNTCGSSDLWPPAIKLGFYAYLGVLLVLGLLLNGLALWVFCCRMQQWTETRIYMTNLAVADLCLLCALPFVLHSLRDTSDTPLCQLSQGIYLTNRYMSISLVTAIAVDRYVAVRHPLRARGLRSPRQAAAVCAALWVLVIGSLVLRWLLGIQEGGFCFRSTSRHNFNTMAFSLLGFYLPLAVLVFCSLQVVTALAQRPAADGGQAEATRKAARMVWANLLVFVVCFLPLHVVLTVRLAVGWNTETIRRALYITSKLSDANCCLDAICYYYMAKEFQEASALAVAPSAKAHKSQDSLCVTLA

SEQ ID NO: 172 - protein, 606 aa, synthetic construct
MRAPGAPLARTSLLLLLLLKVSASSALGVAPASRNETCLGESCSTVIQRRSRDAWGPGNSARRARAPREEQGAAAVRAAPSWDLPAAPGRDPGGAEASAAGPPGPPTRPPGAWRWKGARGQEPPGTLGRGNPTALQLFLQTSEEEEKGPRGAGISGRSQEQSVKTEPGASDLFYWPRRAGKLQGSHHKPLPKTANGPAGHEGRTIAPPGRALAQNGSSGEGIHEPGGPRRGNSTNRRVRLKNPFYPLTQESYGAYAVMCLSVVIFGTGIIGNLAVMCIVCHNYYMRSISNSLLANLAFWDFLIIFFCLPLVIFHELTKKWLLEDFSCKIVPYIEVASLGVTTFTLCALCIDRFRAATNVQMYYEMIENCSSTTAKLAVIWVGALLLALPEVVLRQLSKEDLGFSGRAPAERCVIKISPDLPDTIYVLALTYDSARLWWYFGCYFCLPTLFTITCSLVTARKIRKAEKACTRGNKRQIQLESQMNCTVVALTILYGFCIIPENICNIVTAYMATGVSQQTMDLLNIISQFLLFFKSCVTPVLLFCLCKPFSRAFMECCCCCCDECIQKSSTVTSDDNDNEYTTELELSPFSTIRREMSTFASVGTHC

SEQ ID NO: 173 - protein, 479 aa, synthetic construct
MRWLWPLAVSLAVILVGLSRVSGGGPLHLGRHRAETQEQQSRSRRGTEDEEAKGVQQYVPEEWAEYPRPIHPAGLQPTKPLVATSPNPDKDGGTPGSGQEPRGNLTGAPGQRLQIQNPLYPVTESSYSAYAVMLLALVVFAVGIVGNLSVMCIVWHSYYLKSAWNSILASLALWDFLVLFFCLPVVIFNEITKQRLLGDVSCRAVPFMEVSSLGVTTFSLCALGIDRFHVATSTLPKVRPIERCQSILAKLAVIWVGSMTLAVPELLLWQLAQEPAPTMGTVDSCIMKPSASLPESLYSLVMTYQNARMWWYFGCYFCLPILFTVTCQLVTWRVRGPPGRKPECRAGKHEQCESQLNSTVVGLTVVYALCTLPENVCNIVVAYLSTELTRQTLDLLGLINQFSTFFKGAITPVLLLCICRPLGQAFLDCCCCCCEECGGASEASAANGSDSKLKTEVSSSIYFHKPRESPPLLPLGTPC

SEQ ID NO: 174 - protein, 455 aa, synthetic construct
MASPSLPSSDCSQVIDHSHVPEFEVATWIKITLILVYLIIFVMGILGNSVTIRVTQVLQKKGYLQKEVTDHMVSLACSDILVFLIGMPMEFYSIIWNPLTTPSYTLSCKLHTFLFEACSYATLLHVLTLSFERYVAICHPFRYKAVSGPCQVKLLIGFVWVTSALVALPLLFAMGTEYPLVNVPSHRGLTCNRSRTRHHEQPETSNMSICTNLSSRWTVFQSSIFGAFVVYLVVLVSVAFMCWNMMQVLMKSKQGTLAGGGQPPQLRKSESEESRTARRQTIIFLRLIVVTLAVCWMPNQVRRIMAAAKPKHDWTRSYFRAYMILLPFSDTFFYLSSVVNPLLYNVSSQQFRRVFVQVLRCRLTLQHANHEKRLRAHAHSTTDSARSVRRPLIFAASRRQSSSARRTNKVFLSTFQSEAKPQSKPQSLSLESLEPNSEAKPANSAAENGFQEHEV

SEQ ID NO: 175 - protein, 372 aa, synthetic construct
MACNSTSLETYTYLLLNTSNASDSGSTQLPAPLRISLAIVMLLMIVVGFLGNAVVCIIVYQRPAMRSAINLLLATLAFSDIMLSLCCMPFTAVTLITVRWHFGDHFCRLSATLYWFFVLEGVAILLIISVDRFLIIVQRQDKLNPRRAKVIIAVSWALSFCISAPSLTGWTLVEVPARAPQCVLGYTEFPADRAYVVTLVVAVFFVPFGVMLCSYLCILNTVRKNAVRVHNQSDSLDLRQLTRAGLRRLQRQQQVSLDLSFKTKAFTTILILFVGFSLCWLPHSVYSLLSVFSRRFYCSSSFYATSTCVLWLSYLKSVFNPIVYCWRIKKFREACIELLPQTFQILPKVPERIRRRIQPSTVYVCNENQSAV

SEQ ID NO: 176 - protein, 946 aa, synthetic construct
MPGPLGLLCFLALGLLGSAGPSGLCAAPCSCDGDRRVDCSGKGLTAVPEGLSAFTQLDISMNNITQLPEDAFKNFPFLEELRLAGNDLSFIHPKALSGLKELKVLTLQNNQLKTVPSEAIRGLSALQSLRLDANHITSVPEDSFEGLVQLRHLWLDDNSLTEVPVHPLSNLPTLQALTLALNKISSIPDFAFTNLSSLVVLHLHNNKIKSLGQHCFDGLDNLETLDLNYNNLGEFPQAIKALPSLKELLFHSNSISVIPDGAFDGNPLLRTIHLYDNPLSFVGNSAFHNLSDLHSLVIRGASMVQQFPNLTGTVHLESLTLTGTKISSISSNLCQEQKMLRTLDLSYNNIKDLPSFNGCHALEEISLQRNQIHQIKEGTFQGLISLRILDLSRNLIHEIHSRAFAKLGSITNLDVSFNELTSFPTEGLNGLNQLKLVGNFKLKEALAAKDFVNLRSLSVPYAYQCCAFWGCDSYAHSNTEDNSLQDHSVAKDKGTADAANVTSSAENEEHSQIIIHCTPSTGAFKPCEYLLGSWMIRLTVWFIFLVALFFNLLVILTTFASCTSLPSSKLFIGLISVSNLFMGAYTGILTFLDAVSWGRFAEFGIWWEIGSGCKIAGFLAVFSSESAIFLLMLAAVERSLSAKDIMKNGKSNHLKQFRVAALLAFLGAAVAGCFPLFHRGEYSASPLCLPFPTGETPSLGFTVTLVLLNSLAFLLMAIIYTKLYCNLEKEDLSENSHSSMIKHVAWLIFTNCIFFCPVAFFSFAPLITAISISPEIMKSVTLIFFPLPACLNPVLYVFFNPKFKEDWKLLKRHVTKKSGSVSVSISSQAGCVEQDFYYDCGMYSHLQGNLTVCDCCESFLLTKPVSCKHLIKSHSCPALAVGSCQRPDGYWSDCGTQSAHSDYADEEDSFVSDSSDQVQACGRACFYQSRGFPLVRYAYNLPRVKD

SEQ ID NO: 177 - protein, 907 aa, synthetic construct
MDTSRVGVLLSLPVLLQLAAGGGSPRPGALLRGCPAHCQCEPDGRMLLRVDCSDLGLSELPSNLSVFTSYLDLSMNNISQLPPNPLHSLRFLEELRLAGNALTYIPKGAFAGLYSLKVLMLQNNHLRQVPTEALQNLRSLQSLRLDANHISYVPPSCFSGLHSLRHLWLDDNALTEIPVQAFRSLSALQAMTLALNKIHHIPDYAFGNLSSLVVLHLHNNRIHSLGKKCFDGLHSLETLDLNYNNLDEFPTAIRTLSNLKELGFHSNNIKSIPEKAFVGNPSLITIHFYDNPIQFVGRSAFQHLPELRTLTLNGASQITEFPDLTGTASLESLTLTGAQISSLPQTVCDQLPNLQVLDLSYNLLEDLPSFSVCQKLQKIDLRHNEIYEIKVDTFQQLLSLRSLNLAWNKIAIIHPNAFSTLPSLRKLDLSSNLLSSFPVTGLHGLTHLKLTGNHALQSLISSENFPELKVIEMPYAYQCCAFGVCENVYKISNQWNKGDNSSMDDLHKKDAGMFQVQDERDLEDFLLDFEEDLKALHSVQCSPSPGPFKLCEYLFGSWLIRIGVWTIAVLALTCNALVTSTVFRAPLYISSIKLLIGLIAAVNMLMGVSSAVLAGVDAFTFGSFAQHGAWWEQGVGCQVVGFLSIFASESSVFLLTLAALERGFSVKCSAKFETKTPFSSLKAIILLCALLALTIATVPLLGGSEYSASPLCLPLPFGEPSTTGYMVALVLLNSLCFLVMTIAYTKLYCNLEKGDLENIWDCSMVKHIALLLFTNCILYCPVAFLSFSSLLNLTFISPEVIKFILLVIVPLPACLNPLLYILFNPHFKEDLGSLGKQTHFWTRSKHPSLMSINSDDVEKQSCDSTQALVTFTSASIAYDLPSNSVSPPAYPVTESCHLSSVAFVPCL

SEQ ID NO: 178 - protein, 588 aa, synthetic construct
MGPTLAVPTPYGCIGCKLPQPDYPPALIIFMFCAMVITIVVDLIGNSMVILAVTKNKKLRNSGNIFVVSLSVADMLVAIYPYPLMLHAMSIGGWDLSQLQCQMVGFITGLSVVGSIFNIVAIAINRYCYICHSLQYERIFSVRNTCIYLVVTWIMTVLAVLPNMYIGTIEYDPRTYTCIFNYLNNPVFAVTIVCIHFVLPLLIVGFCYVRIWTKVLAARDPAGQNPDNQLAEVRNFLTMFVIFLLFAVCWCPINVLTVLVAVSPKEMAGKIPNWLYLAAYFIAYFNSCLNAVIYGLLNENFRREYWTIFHAMRHPILFFSGLITDIREMQEARALARARARDQARAEQDRAHACPAVEETPMNVRNVPLPGDAAAGHPDRASGHPKPHSSSAYRKSASTGHSKPASGHPKSATVYPKPASVHFKADSVHFKVHFKSVHFKPASSHPKPITGHHVSAGSHSKSAFSPATSHPKPTTGHIKPATSHAEPTTADYPEPATTSHPKPTAADHPELSASHCPEIPAIAHPESDDSDLPESASSPAAGPTKPAASQLESTAADLPDPTVVTTSTNDYHDVVVIDVEDDSDEMAV

SEQ ID NO: 179 - protein, 361 aa, synthetic construct
MNESRWTEWRILNMSSGIVNVSEHHSCPLGFGHYSAVDVCILETVVIVLLTFLIIAGNLTVIFVFHCAPLLHHYTTSYFIQTMAYADLFVGVSCLVPTLSLLHYSTGVHESLTCQVFGYIISVLKSVSMACLACISVDRYLAITKPLSYNQLVTPCRLRICIILIWIYSCLIFLPSFFGWGKPGYHGDIFEWCATSWLTSAYFTGFIVCLLYAPAAFVVCFTYFHIFKICRQHTKEINDRRARFPSHEVDASGETGHSPDRRYAMVLFRITSVFYMLWLPYIIYFLLESSRVLDNPTLSFLTTWLAISNSFCNCVIYSLSNSVFRLGLRRLSETMCTSCMCVKDQEARDPKPRKRANSCSI

SEQ ID NO: 180 - protein, 451 aa, synthetic construct
MESSPIPQSSGNSSTLGRVPQTPGPSTASGVPEVGLRDVASESVALFFMLLLDLTAVAGNAAVMAVIAKTPALRKFVFVFHLCLVDLLAALTLMPLAMLSSSALFDHALFGEVACRLYLFLSVCFVSLAILSVSAINVERYYYVVHPMRYEVRMTLGLVASVLVGVWVKALAMASVPVLGRVSWEEGAPSVPPGCSLQWSHSAYCQLFVVVFAVLYFLLPLLLILVVYCSMFRVARVAAMQHGPLPTWMETPRQRSESLSSRSTMVTSSGAPQTTPHRTFGGGKAAVVLLAVGGQFLLCWLPYFSFHLYVALSAQPISTGQVESVVTWIGYFCFTSNPFFYGCLNRQIRGELSKQFVCFFKQAPEEELRLPSREGSIEENFLQFLQGTGCPSESWVSRPLPSPKQEPPAVDFRIPGQIAEETSEFLEQQLTSDIIMSDSYLRPAPSPRLES

SEQ ID NO: 181 - protein, 362 aa, synthetic construct
MANSTGLNASEVAGSVGLILAAVVEAGALLGNGALLVVVLRTPGLRDALYLVHLCVVDLLAAASIMPLGLLAAPPPGLGRVRLGPAPCRAARFLSAALLPACTLGVAALGLARYRLIVHPLRPGARPPPVLVLTAVWAAAGLLGALSLLGPPPAPPPAPARCSVLAGGLGPFRPLWALLAFALPALLLLGAYGSIFLVARRAALRPPRPARGRLRSDSLDSRLSILPPLRPRLPGGKAALAPALAVGQFAACWLPYGCACLAPAAQAAEAEAAVTWVAYSAFAAHPFLYGLLQRPVRRALGRLARRALPRPPRACTPQAWHPRALLQCLQGPPEGPALGPSEAPEQTPELAGGRSLSMPGAT

SEQ ID NO: 182 - protein, 419 aa, synthetic construct
MVFSAVLTASHTGTSNTTFVVYENTYMNITLPPPFQHPGLSPLLRYSFETMAPTGLSSLTVNSTAVPPTPAVFKSLNLPLQIILSAIMIFILFVSFLGNLVVCLMVYQKAAMRSAINILLASLAFADMLLAVLNMPFALVTILTTRWIFGKFFCRVSAMFFWLFVIEGVAILLIISIDRFLIIVQRQDKLNPYRAKVLIAVSWATSFCVAFPLAVGNPDLQIPSRAPQCVFGYTTNPGYQAYVILISLISFFIPFLVILYSFMGILNTLRHNALRIHSYPEGICLSQASKLGLMSLQRPFQMSIDMGFKTRAFTTILILFAVFIVCWAPFTTYSLVATFSKHFYYKHNFFEISTWLLWLCYLKSALNPLIYYWRIKKFHDACLDMMPKSFKFLPQLPGHTRRRIRPSAVYVCGEHRTVV

SEQ ID NO: 183 - protein, 341 aa, synthetic construct
MNSTCIEEQHDLDHYLFPIVYIFVIIVSIPANIGSLCVSFLQAKKENELGIYLFSLSLSDLLYALTLPLWIDYTWNKDNWTFSPALCKGSAFLMYMNFYSSTAFLTCIAVDRYLAVVYPLKFSFLRTRRFAFMVSLSIWVLETIFNAVILWEDETFVEYCDAKKSNFTLCYDKYPLEKWQINLNLFRTCTGYAIPLVIIMICNQKVYQAVRHNQATENSEKKRIIKLLVSITLTFVLCFTPFHVMLLIRSILEHDVNFDDHYFDDPKSGKQTYKIYRITVALTSLNCVADPILYCFVTETGRSDMWNILKFCTGKLNKSQRQRKSILSMSTKDTVELEILE

SEQ ID NO: 184 - protein, 363 aa, synthetic construct
MGNITADNSSMSCTIDHTIHQTLAPVVYVTVLVVGFPANCLSLYFGYLQIKARNELGVYLCNLTVADLFYICSLPFWLQYVLQHDNWSHGDLSCQVCGILLYENIYISVGFLCCISIDRYLAVAHPFRFHQFRTLKAAVGVSVVIWAKELLTSIYFLMHEEVIEDEDQHRVCFEHYPIQAWQRAINYYRFLVGFLFPICLLLASYQGILRAVRRSHGTQKSRKDQIQRLVLSTVVIFLACFLPYHVLLLVRSLWEASCDFAKGIFNAYHFSLLLTSFNCVADPVLYCFVSETTHRDLARLRGACLAFLTCSRTGRAREAYPLGAPEASGKSGQGEEPELLTKLHPAFQTPNSPGSGFPTGRLA

SEQ ID NO: 185 - protein, 540 aa, synthetic construct
MNSTGHLQDAPNATSLHVPHSQGGNSTSLQEDLQDLIHTATLVTCTFLLAVIFCLGSYGNFIVFLSFFDPAFRKFRTNFDFMILNLSFCDLFICGVTAPMFTFVLFFSSASSIPDAFCFTFHLTSSGFIIMSLKTVAVIALHRLRMVLGKQPNRTASFPCTLLLTLLLWATSFTLATLATLKTSKSHLCLPMSSLIAGEGKAILSLYVVDFTFCVAVVSVSYIMIAQTLRKNAQVRKCPPVITVDASRPQPFMGAPVKGGGDPIQCTMPALYRNQNYNKLQHVQTHGYTKSPNQLPTPAASRLQLVSAVNLSTAKDSKAVVTCVIIVLSVLVCCLPLGISLVQVVLSSNGSFILYQFELFGFTLIFFKSGLNPFIYSRNSAGLRRKVLWCLQYIGLGFFCCKQKTRLRAMGKGNLEVNRNKSSHHETNSAYMLSPKPQKKFVDQACGPSHSKESVVSPKISAGHQHYGQSSSTPINTRIEPYYSIYNSSPSQEESSPCNLQPVNSFGFANSYIAMHYHTTNDLMQEYDSTSAKQIPVPSV

SEQ ID NO: 186 - protein, 339 aa, synthetic construct
MDLAEVLLAGLLVLVLVVSLLSNLLVLLCFAYSTEIRKQVSGVFLVNLSFCNLLLTVLNMPFTLLGILRGQQPSGPCACKAVGFLETFLTSNTMLSMAALSIDKWIAVVFPLSYTSKMRYKDAVILMGYSWLHSLTFPLVSLFCSWVDYSSVYASCTLHLPEEPERRRFTVFTIVFHATSFMLSLVILCFTYLKVLKVARFHCKRIDIITMQTLVLLVDIHPSVKQRCLNEQKRRRQRATKKISIFIGSFVICFAPYIITRLIELLPFVTINYYWGILSKCLTYSKAASDPFVYSLLRQQYKKVLINIVNRILKRDLYPSSGYNSSLDTENDYCLHRTN

SEQ ID NO: 187 - protein, 335 aa, synthetic construct
MNNNSTCIQPSMISSMALPIIYIFLCIVGLFGNSLSQWVFLTKIGKKTSTHIYLAHLVTANLLVCSAMPFMSIYFLKGFQWEYQSAQCRVVNFLGTLSMHVSMFVSLLILSWIAISRYATLMKKDSSQETTSCYEKIFYGHLLKKFRQPNFARKLCIYIWGVVLGIIIPVIIYYSVVEATEGEESLCYNRQMELGAMISQIAGLIGTTFIGFSFLVVLTSYYSFVSHLRKIRTCTSIMEKDLTYSSVKRHLLVIQILLIVCFLPYSIFKPIFYVLHQRDDCQQLNYLIEIKNILTCLASARSSTDPIIFLLLDKTFKKTLYNLFTKSNSHMQSYG

SEQ ID NO: 188 - protein, 421 aa, synthetic construct
MVPHLLLLCLLPLVRATEPPEGRADEQLEAALAVPNASHFFWNNYTFSDWQNFVGRRRYGAESQNPTVKALLIVAYSFIIVFSLFGNVLVCHVIFKNQRMHSATSLFIVNLAVADIMITLLNTPFTLVRFVNSTWVFGKGMCHVSRFAQYCSLHVSALTLTAIAVDRHQVIMHPLKPRISITKGVIYIAVIWTMATFFSLPHAICQKLFTFKYSEDIVRSLCLPDFPEPADLFWKYLDLATFILLYILPLLIISVAYARVAKKLWLCNTIGDVTTEQYLALRRKKKKTIKMLMLVVVLFALCWFPLNCYVLLLSSKVIHTNNALYFAFHWFAMSSTCYNPFIYCWLNENFRVELKALLSMCQRPPKPQEDRPPSPVPSFRVAWTEKSDGRRAPLANNLLPSSQLQSGKTDLSSVEPIVAMS

SEQ ID NO: 189 - protein, 395 aa, synthetic construct
MWNTSDANFSCYHESVLGYRYVAVSWGVVVAVTGTVGNVLTLLALAIQPKLRTRFNLLIANLTLADLLYCTLLQPFSVDTYLHLHWRTGATFCRVFGLLLFASNSVSILTLCLIALGRYLLIAHPKLFPQVFSAKGIVLALVGTWVVGVASFAPLWPVYILVPVVCTCSFDRIRGRPYTTILMGIYFVLGLSSVGIFYCLIHRQVKRAAQALDQYKLRQASIHSNHVAGTDEAMPGRFQELDSGLASGGPSEGISSEPVSAATTQTLEGDSSEVGDQINSKRAKQMAEKSPPEASAAQPTKGARRAQDSPSEFGKVTRMCFAVFLCFALSYIPFLLLNILDARVRAPRVVHMLAANLTWLNGCINPVLYAAMNRQFRQAYGSILKRGPQSFRRLH

SEQ ID NO: 190 - protein, 370 aa, synthetic construct
MANYSHAADNILQNLSPLTAFLKLTSLGFIIGVSVVGNLLISILLVKDKTLHRAPYYFLLDLCCSDILRSAICFPFVFTSVKNGSTWTYGTLTCKVIAFLGVLSCFHTAFMLFCISVTRYLAIAHHRFYTKRLTFWTCLAVICMVWTLSVAMAFPPVLDVGTYSFIREEDQCTFQHRSFRANDSLGFMLLLALILLATQLVYLKLIFFVHDRRKMKPVQFVAAVSQNWTFHGPGASGQAAANWLAGFGRGPTPPTLLGIRQNANTTGRRRLLVLDEFKMEKRISRMFYIMTFLFLTLWGPYLVACYWRVFARGPVVPGGFLTAAVWMSFAQAGINPFVCIFSNRELRRCFSTTLLYCRKSRLPREPYCVI

SEQ ID NO: 191 - protein, 358 aa, synthetic construct
MGLNLTLAKLPNNELHGQESHNSGNRSDGPGKNTTLHNEFDTIVLPVLYLIIFVASILLNGLAVWIFFHIRNKTSFIFYLKNIVVADLIMTLTFPFRIVHDAGFGPWYFKFILCRYTSVLFYANMYTSIVFLGLISIDRYLKVVKPFGDSRMYSITFTKVLSVCVWVIMAVLSLPNIILTNGQPTKENIHDCSKLKSPLGVKWHTAVIYVNSCLFVAVLVILIGCYIAISRYIHKSSRQFISQSSRKRKHNQSIRVVVAVFFTCFLPYHLCRIPFTFSHLDRLLDESAHKILYYCKEMTLFLSACNVCLDPIIYFFMCRSFSRRLFKKSNIRTRSESIRSLQSVRRSEVRIYYDYTDV

SEQ ID NO: 192 - protein, 334 aa, synthetic construct
MTNSTSGGSLLLLCSWAGRRIPVSLLYSGLAIGGTLANGMVIYLVSSFRKLQTTSNAFIVNGCAADLSVCALWMPQEAVLGLLPTGSAEPPGGSYRLLRGGLLGLGLTVSLLSHCLVALNRYLLITRAPAYQALYQRRHTAGMLALSWALALGLVLLLPPWAPRPGAAPPRVHYPALLAAAALLAQTALLLHCYLGIVRRVRVSVKRVSVLNFHLLHQLPGCAAAAHPRRAQRRLSGLSVLLLCCVFLLATQPLVWVSLASGFSLPVPWGVQAASWLLCCALSALNPLLYTWRNEEFRRSVRSVLPGVGDAAAAAVAAAVPAVQLGTRAAGQHW

SEQ ID NO: 193 - protein, 484 aa, synthetic construct
MTSTCTNSTRESNSSHTCMPLSKMPISLAHGIIRSTVLLIFLAASFVGNIVLALVLQRKPQLLQVTNRFIFNLLVTDLLQISLVAPWVVATSVPLFWPLNSHFCTALVSLTHLFAFASVNTIVVVSVDRYLSIIHPLSYPSKMTPRRGYLLLYGTWIVAILQSTPPLYGWGQAAFDERNALCSMIWGASPSYTILSVVSFIVIPLIVMIACYSVVFGAARRQHALLYNVKSHSLEVRVKDCVENEDEEAEDESEFRRQHGEVKAKEMEAKEGSTGTSEGSVEARGSEEVRESSMEGKEGSTKVNSMADKGRTEVNQCNIDLGEDDMEFGEDDINFSDDVEAVNIPESLPPSRRNSNSNPPLPRCYQCKAAKVIFLIIFSYVLSLGPYCFLAVLAVWVDVQTQVPQWVITIIIWLFFLQCCIHPYIYGYMHKTIKKEIQDMLKKFFCKEKPPKEDSHPDLPGTEAGTEGGTEGKIVPSHDSATSP

SEQ ID NO: 194 - protein, 367 aa, synthetic construct
MNGNATPVTTTAPWASLGLSAKTCNNFEESRVVLVVVYSAVCTLGLPANCLTAWLTLLQVLQGNVLAVYLFCLALCELLYTSTLPLWVIYIQNQHRWTLGLLACKVTAYIFFCNIYVSILFLCCISCDRFVAVVYALESRGRRRQRTAILISACVFILVGLVHYPVFQMEDKETCFEMLQMDSRIAGYYYARFTVGFAIPLSIIAFTNHRIFRSIKLSMGLSAAQKAKVKHSAIAVVVIFLVCFAPYHLVLLVKAAAFSYYRGDRNAVCAFEERLYTASVVFLCLSTVNSVADPIIYVLATDHSRQEVSRIHKGWKKWSMKTDVTRLTHSKDSEELQSPVALADHYTFPRPVHPPGSPPERLIEESC

SEQ ID NO: 195 - protein, 461 aa, synthetic construct
MALLGSQHPGAPSAAGGTSSAATAAAVLSFSTAAAAALGNLSDASGGGTAAAPGGGGLGGSGAPEAAPLLSHGAAVAAQALVLLLIFLLSSLGNCAVMGVIVKHRQLRTVTNAFILSLSLSDLLTALLCLPAAFLDLFTPPGGSAPWRGFCAASRFFSSCFGIVSTLSVALISLDRYCAIVRPPREKIGRRRALQLLAGAWLAALGFSLPWELLGAPRELAAAQSFHGCLYRTSPDPAQLGAAYSVGLVVACYLLPFLLMCFCHYHICKTVRLSDVRVRPVTTYARVLRFFSEVRTATTVLIMIVFVICCWGPYCFLVLLAAARQAQAMQAPSLLNVVAVWLTWANGAINPVIYAIRNPNISMLLGRNREEGYRTRNVDAFLPSQGPGLQARSRNRLRNRYANRLGACSRMSSSNPASGVGGDVAMWARKNPVVLFCREGPPEPVTAVTKQPKSEAGDTSL

SEQ ID NO: 196 - protein, 350 aa, synthetic construct
MEHTHAHLAANSSLSPGSACGLGFVPVVYYSLLLCLGLPANILTVIILSQLVARRQKSSYNYLLALAAADILVLFFIVFVDFLLEDFILNMQMPQVPDKIIEVLEFSSIHTSIWITVPLTIDRYIAVCHPLKYHTVSYPARTRKVIVSVYITCFLTSIPYYWWPNIWTEDYISTSMHHVLIWIHCFTVYLVPCSIFFILNSIIVYKLRRKSNFRLRGYSTGKTTAILFTITSIFATLWAPRIIMILYHLYGSPIQNRWLVHIMSDIANMLALLNTAINFFLYCFISKRFRTMAAATLKAFFKCQKQPVQFYTNHNFSITSSPWISPANSHCIKMLVYQYDKNGKPIKVSP

SEQ ID NO: 197 - protein, 305 aa, synthetic construct
MPGHNTSRNSSCDPIVTPHLTSLYFIVLIGGLVGVISILFLLVKMNTRSVTTTAVINLVVVHSVFLLTVPFRLTYLIKKTWMFGLPFCKFVSAMLHIHMYLTFLFYVVILVIRYLIFFKCKDKVEFYRKLHAVAASAGMWLLVIVIVVPLVVSQYGIHEEYNEEHCFKFHKELAYTYVKVINYMIVIFVIAIAVILLVFQVFIIMLMVRKLRHSLLSHQEFWAQLKNLFFIGVILICFLPYQFFRIYYLNVVTHSNACNSKVAFYNEIFLSVTAISCYDLLLFVLGGSHWFKQKIIDLWNCLLCR

SEQ ID NO: 198 - protein, 349 aa, synthetic construct
MGLEETAGQPRVTLLPTPNGSGLSQEFEGHWPEIPERSPCVAGVIPVIYYSVLLGLGLPVNLLTTVALARLATRTRKPSYYYLLALTASDIVTQVVIVFVGFLLQGAVLARQVPQAVVRTANILEFAANHASVWIAVLLTVDRYTALCHPLHHRAASSPGRTRRAIAAVLSAALLTGIPFYWWLDVWRDADPPSTLDEVLKWAHCLTVYFIPCGVFLVTNSAIIHRLRRRGRSGLRPRVGKSTAILLGVTTLFALLWAPRIFVMLYHLYVAPVHRDWRVHLALDVANMVAMLNTAVNFGLYCFVSKTFRATVREVIHDAHLPCTLGSQPEGMAAKPVLKPPGLPKGAEL

SEQ ID NO: 199 - protein, 333 aa, synthetic construct
MWSCGWLNGTGLVEDQPLCQDLHLVLSVFSLLYLVVGVPVGLGYNALLVLVNLHSKASMTMPDVYFVNMAVAGLVLSALAPVHLLGPPSSRWALWSVGSEAHVTLLILFNVSSLVTMYSTALLSLDYYIERALPRTYMSSVYNTRHVCGFVWGGALLTSFSSLLFYICSHVSTRILECSKMQNAEAADAIMVFIGYVVPALAVLYALVLISRIRKEDTPLDQDTGRLDPSVHRLLVATVCTQFGLWTPHYLTLLGHTVLISRGKPVDAHYLGILHFAKDLSKFLAFSSSFVTPLLYRYINQNFPSKLRRLMKKMHCGDQHCSPDHMGVQQVMA

SEQ ID NO: 200 - protein, 335 aa, synthetic construct
MGDELAPCPVGTTAWPALISKTPCMPQAASNTSLGLGDLRVPSSMLYWFFIPSSLLAAATLAVSPLLLVTILRSQRLRQETRYLLLANILLSDLAFLLLHMLISSSNLGGWELGRMACGILTDAVFAAYTSTILTFTAMVLDTYLAVIHPLRYLSFLSHGRAWKAVALIWLVACCFPTFLIWLSKWQDAQEQGASCILPPSLGTQPGVIVTYTSILCVLFLCTALIAYCYWRLYAETRTSGIWGQRYSRARGTLLIHSVLLTLYFSPGVVFSLEMVLTRYHHDSGTHVWLLAANSEVLMMLPRAMLPYLYGLRYRQLLGTVRGLSRRHQAIFTIS

SEQ ID NO: 201 - protein, 733 aa, synthetic construct
MSLFLSNLSTNDSSLWKENHNSTDLLNPPGTLNIYLFCLTCLMTLAALAGSIYSLVSLLKMQNRTVVSMLVASWSVDDLMSVLSVTIFMFLQWPNEVPGYFQSLCTTSALLYLCQGLSSNLKATLLVSYNFYTMHRAVGSQAASRRSGQVLGVALTVWAASLLLSALPLCGWGAFVRTPWGCLADCSSSYVLLLFAVYASAFGLLAGLSVPLTHQLLCSEEPPRLHANYQEISRGASTPGTPPTAGRVLSLSPEDAPGPALRCSGGCSPSSDTVFGPGPPAAAGAGACRRENRGTLYGTRSFTVSVAQKRFSLILALTKVILWLPMMIHMVVQHVVGFQSLPFETLSFLLTLLATTVTPVFVLSKRWTHLPCGCIINCKQNAYAVASDGKKIKRRGFEFNLSFQKSYGIYKIAHEDYYDDDENSISYHNLMNYECETTKDSQRDNRNIFNAIKVEISTTPSLDSSTLKGINKCTNTDITEAKQDSNNEKGADSLSDKTEGDINYEETTFLEGPERRLSHEESQKPDLSDWEWCRSKSERTPRQRSGGALAIPLCAFQGTVSLQAPTGKTLSLSTYEVSAEGQKITPASKKIEVYRSKSVGHEPNSEDSPSTFADTSVKIHLEVLEICDNEEALDTVSIISNISQSSTQVRSPSLRYSRKENRFVSCDLGETASYSLFLPTSNPDGDINISIPDTVEAHRQNSKRQHQERDGYQEEIQLLNKAYRKREEESKGN

SEQ ID NO: 202 - protein, 422 aa, synthetic construct
MEDPSPSIPPAPNLSVPILLGWGLNLTSGQGAPAPGPPPGPPSRRVRLVFLGVILVVAVAGNTTVLCRLCGGGGPWAGPKRRKMDFLLVQLALADLYACGGTALSQLAWELLGEPRAAAGDLACRFLQLLQASGRGASAHLVALIALERQRAVRRPQGPPLPARALAALGWLLALLLALPPAFVVRGDSPSPLGAPPAARAWPGERRCRGIFAPLPRWHLQVYALYEAVAGFVAPVAVLGVACGRLLCVWWQRRPQPAAAAPWSASPGRAPAPSALPRAKVQSLKMSLLLALLFVGCELPYFAARLAAAWSSGPAGDWEGEGLAAALRVVGVANSALNPFVYLFFQAGDCRLRRLRRRLGSLCCAPEGGAAEDEEPRGHQALHRHRWPHPHYHHARREQLDEGLRPPPPRPRPLPCSCESAF

SEQ ID NO: 203 - protein, 419 aa, synthetic construct
MLAAAFADSNSSSMNVSFAHLHFAGGYLPSDSKDWRTIIPALLVAVCLVGFVGNLCVIGILLHNAWKGKPSMIHSLILNLSLADLSLLLFSAPVRATAYSKGVWDLGWFVCKSSDWFIHTCMAAKSLTIVAVAKVCFMYASDPAKQVSIHNCTIWSVLVAIWAVASLLPLPEWFFSTTRHHAGVEMCLVDVPAVAEEFMSMFGKLYPLLVFCLPLLFASFYFWRAYGQCQKRGTKTQNLRNQMRSKQLTVMLLSIAITSALLWLPEWIAWLWVWHLKAGGPAPPQGFIALSQVLMFSISSANPLIFLVMSEEFKEGLKGLWKWMITKKPPTASESQETPAGNSEVLPDKVPSPESPASIPEKEKPGSPSSGKEKTEKAEIPILPDVEQFWHERDTVPSVQDNDPIPWEHEDQETGECVK

SEQ ID NO: 204 - protein, 451 aa, synthetic construct
MDTAMEANLGATGHGPRTELDDEDYYPQGGWDTVFLVALLLLGLPANGLMAWLAGSQARHGAGTRLALLLLSLALSDFLFLAAAAFQILEIQHGGHWPLGTAACRFYYFLWGVSYSSGLFLLAALSLDRCLLALCPRWYPGHRPARLPLWVCAGVWVLATLFSVPWLVFPEAAVWWYDLVICLDFWDSEELPLRMLEILGGFLPFLLLLVCHVLTQAACRTCHRRQPQPAACRGFARVAKTILSAYVVLRLPYQLAQLLYLAFLWDVYPGYLLWEALVYSDYLILLNSCLSPFLCLLASADLRALLRSVLSSFAAALCEERPGSFTPAEPQTQVDSEGPTLPGPMAEAQPVAQPQPTLQPRSDPTAQPTAQPQSDPTAQPQPQSDSVAQDTNAQTPAPAASSAPSPCDEASPTPSSDPTPGAPENPATPAASEGESPSSTPPEEAPGAGPT

SEQ ID NO: 205 - protein, 603 aa, synthetic construct
MSDERRLPGSAVGWLACGGLSLLANAWGILSVGAKQKKWKPLEFLLCTLAATHMLNVAVPIATYAVVQLRRQRPDYEWNEGLCKVFVSTFYTLTLATCFSVTSLSYHRMWMVRWPVNYRLSNAKKQAVHTVMGIWMVSFILSALPAVGWHDTSERFYTHGCRFIVAEIGLGFGVCFLLLVGGSVAMGVVCTAIALFQTLAVQVGRRADRRAFTVPTIVVEDAQGKRRSSIDGSEPAKTSLQITGLVATIVFIYDCLMGFPVLVVSFSSLRADASAPWMALCVLWCSVAQALLLPVFLWACDRYRADLKAVWEKCVALMANDEDSDDETSLEGGIPPDLVLERSLDYSYGGDFVALDRMAKYELSALEGGLPQLYPLRPLQEDKMQYLQVPPTRRFSHDDDVWAAVPPPAFLPRWGSGEDLAALALPAGPERRRSLLAFAEDAPPFRPRRRSAESLLSLRPSALDSGPRRARDSPPGSPRRRPGPGPRSASASLLPDAFALTAFEREPQALRRPPAPGPFPAADGADPGEAPTPPSGSAQRSPGPRPSAHSHAGSLRTGLSASWGEPGGLRAAGGGGSTSSFLSSPSESSGYVTLHSDSLGSAS

SEQ ID NO: 206 - protein, 338 aa, synthetic construct
MTALSSENCSFQYQLHQTNQPLDVNCLLFLIILGKILLNILTLGMRRKNTCQNFMEYFCISLAFVDLLLLVNISIILYFRDFVLLGIRFTKYHICLFTQIISFTYGFLHYPVFLIACIDYYLNFSKTTKLSFKCQKLFYFFTVILIWISVLAYVLGDPAIYQSLKAQNAYSYQCPFYVSIQSYWLSFSMVMILFVAFITSWSEVITLVQAVRITSYMNETILYFPFSSHSSYTVRSKKILLPKLIICFLGTWLPFVLLQVIILLLKVQIPAYIEMNIPWLYFVNSFLIATVYWFNCHKLNLRDIGLPLDPFVNWKCCFIPLTIHNLEQIEKPISIIIC

SEQ ID NO: 207 - protein, 529 aa, synthetic construct
MSLNSSLGHRKELSNLTEEEGGEGGVIVTEFIAIIVITIFVCLGNLVIVVTLYKKSYLLTLSNKFVFSLTLSNFLLSVLVLPFVVTSSIRREWIFGVVWCNFSALLYLLISSASMLTLGVIAIDRYYAVLYPMVYPMKITGNRAVMALVYIWLHSLIGCLPPLFGWSSVEFDEFKWMCVAAWHREPGYTAFWQIWCALFPFLVMLVCYGFIFRVARVKARKVHCGTVVIVEEDAQRTGRKNSSTSTSSSGSRRNAFQGVVYSANQCKALITILVVIGAFMVTWGPYMVVITSEALWGKNSVSPTLETWATWLSFTSAICHPLIYGLWNKTVRKELLGMCFGDRYYREPFVQRQRTSRLFSISNRITDLGLSPHLTALMAGGQPLGHSSSTGDTGFSCSQDSGTDVMLLEDYTSDDNPPSHCTCPPKRRSSVTFEDEVEQIKEAAKNPILHVKAEVHKSLDSYAASLAKAIEAEAKINLFGEEALPGVLVTARTVPGAGFGGRRGSRTLASQRLQLQSIEEGNVLAAEQR

SEQ ID NO: 208 - protein, 588 aa, synthetic construct
MARGGAGAEEASLRSNALSWLACGLLALLANAWIILSISAKQQKHKPLELLLCFLAGTHILMAAVPLTTFAVVQLRRQASSDYDWNESICKVFVSTYYTLALATCFTVASLSYHRMWMVRWPVNYRLSNAKKQALHAVMGIWMVSFILSTLPSIGWHNNGERYYARGCQFIVSKIGLGFGVCFSLLLLGGIVMGLVCVAITFYQTLWARPRRARQARRAGGGGGAKGGGPGGLGTRPAFEVPAIVVEDARGKRRSSLDGSESAKTSLQVTNLVSAIVFLYDSLTGVPILVVSFFSLKSDSAPPWMVLAVLWCSMAQTLLLPSFIWSCERYRADVRTVWEQCVAIMSEEDGDDDGGCDDYADGRVCKVRFDANGATGPGSRDPTQVKLLPGRHMLFPPLERVHYLQVPLSRRLSHDETNIFSTPRAPGSFLHKWSSSDDIRVLPAQSRALGGPPEYLGQRHRLEDEEDEEEAEGGGLASLRQFLEGGVLGSGGGPPRGPGFFREEITTFIDETPLPSPTASPGPSPRRPRPLGLSPRRLSLGSPDSRAVGLPLGLSAGRRCSLTGGEGSARAWGGSWGPGNPIFPQLTL

SEQ ID NO: 209 - protein, 319 aa, synthetic construct
MTNSSFFCPVYKDLEPFTYFFYLVFLVGIIGSCFATWAFIQKNTNHRCVSIYLINLLTADFLLTLALPVKIVVDLGVAPWKLRIFHCQVTACLIYINMYLSIIFLAFVSIDRCLQLTHSCKIYRIQEPGFAKMISTVVWLMVLLIMVPNMMIPIKDIKEKPNVGCMEFKKEFGRNWHLLTNFICVAIFLNFSAIILISNCLVIRQLYRNKDNENYPNVKKALINILLVTAGYIICFVPYHIVRIPYTLSQTEVISDCSTRISLFKAKEATLLLAVSNLCFDPILYYHLSKAFRLKVTETFASPKETKAQKEKLRCENNA

SEQ ID NO: 210 - protein, 381 aa, synthetic construct
MANTTGEPEGPGGPLAALSPPSSPSSAVSTYVKLVLLGLIICVSLVGNLIVSLLVLRDRALHKAPYYFLLDLCLADGIRSAVCFPFVLVSIRNGSAWTYSALSCKVVAFMAVLFCFHAAFMLFCISVTRYMAIAHHRFYAKRMTFWTCAAVICMVWTLSVAMAFPPVFDVGTYKFIREEDQCIFEHRYFKANDTLGFMLMLAVLILATHAVYGKLLLFEYRHRKMKPVQMVPAISQNWTFHGPGATGQAAANWIAGFGRGPMPPTLLGIRQNLHNQNRRLLGMEEFKGEKQLGRMFYAITLLFLVLWSPYIVACYWRVFVKACTIPHRYLSTTVWMSFAQAGVNPIVCFLLNKDLKKCLRTHLPCWGRTKPPLPREPYCVM

SEQ ID NO: 211 - protein, 330 aa, synthetic construct
MPANYTCTRPDGNTDFRYFIYAVTYTVILVPGLIGNILALWVFYGYMKETKRAVIFMINLAIADLLQVLSLPLRIFYYLNHDWPFGPGLCMFCFYLKYVNMYASIYFLVCISVRRFWFLMYPFRFHDCKQKYDLYISIAGWLIICLACLLFPLLRTSDDTSGNRCFVDLPTRNVNLAQSVAMMTIGELIGFVTPLLIVLYCTWKTVLSLQDKYPVAQDLGEKKKALKMILTCAGVFLICFAPYHFSFPLDFLVKSNEIKSCLARRVILIFHSVALCLASLNSCLDPVIYYFTTNEFRRRLSRQDLHDSIQLHAKSFVSNHTASTMTPELC

SEQ ID NO: 212 - protein, 507 aa, synthetic construct
MGHNNASEPRNASGAEAAGVNRSALGEFEAQLYRQFTTTVQVVIFIGSLLNFMVLWSTCRTTVFKSVTNRFIKNLACSGICASLVCVPFDIILSTSPHCCWWIYTMLFCKVVKFLHKVFCSVTILSFPAIALDRYYSVLYPLERKISDAKSRELVMYIWAHAVVASVPVFAVTNVADIYAMSTCTEVWSNSLGHLVYVLIYNITTVIVPVAVVFLFLILIRRALSASQKKKVIIAALRTPQNTISIPYASQREAELHATLLSMVMVFILCSVPYATLVVYQTVLNVPDTSVFLLLTAIWLPKVSLLANPVLFLTVNKSVRKCLVGTLVQLHHRYSRRNVVSTGSGVAEASLEPSMRSGSQLLEMFHIGQQQIFKPTEDEEESEAKYIGSADLQAKEILSTCLEGEQGPQFAPSAPPPGTVDSVSQVAPAAPVEPETFPDKYSLQFGFGPFELPPQWLSETRNSKKRLLPPLGNTPEELIQTKMPKVGRVERKMSRNNKVSIFPKVDS

SEQ ID NO: 213 - protein, 377 aa, synthetic construct
MSVKPSWGPGPSGVTAVPTSDLGEIHNWTELLDFFNHTLSECHVELSENTKRVVLFVLYLAIFVVGLVENLLVICVNWRGSGRAGLLNLYILNMAIADLGIVLSLPVWMLEVMLDYTWLWGSFSCRFTHYFYFANMYSSIFFLVCLSVDRYVTLTSASPSWQRHQHRVRRAVCAGVWVLSAIIPLPEVVHIQLVEGPEPMCLFMAPFETYSTWALAVALSTTILGFLLPFPLIAVFNVLTACRLRQPGQPESRRHCLLLCAYIAVFVICWLPYHVTLLLLTLHGTHISLHCHLAHLLYFFYDIIDCFSMLHCVINPILYNFLSPHFRGRLLSAVVHYLPKDQARATCASSSSSSTQHSIVITKEGSQPAAAAPPEPS

SEQ ID NO: 214 - protein, 361 aa, synthetic construct
MDIQMANNFTTPSATPQGSDCDLYAHHSTARILMPLHYSLVFIIGLVGNLLALVVIVQNRKKINSTTLYSTNLVISDILFTTALPTRIAYYALGFDWRIGEALCRITALVFYINTYAGVNFMTCLSIDRFFAVVHPLRYNKIKRIEHAKGICIFVWILVFAQTLPLLINPMSKQEAERTTCMEYPNFEETKSLPWILLGACLIGYVLPLIIILICYSQICCKLFRTAKQNPLTEKSGVNKKALNTIIFIIVVFVLCFTPYHVAIIQHMIKKLRFSNLLECSQRHSFQISLHFTVCLMNFNCCMDPFIYFFACKGYKRKVMKMLKRQVSVSISSAVRSAPEENSREMTETQMMIHSKSSNGK

SEQ ID NO: 215 - DNA, 1062 bp, synthetic construct
  source 1..1062: mol_type = other DNA
atggtgggcgacaccctgaagctgctgtccccactgatgacaaggtacttctttctgctgttctattctaccgacagctccgacttcaacgagaatcagcaccccctggacttcgatggaatggcaagcggcaagctggagtccggaatctctttcctgatccagaccggcgtgggcatcctgggcaactcctttctgctgtgcttctacaactttatcctgctgacaggcaataagctgaggcccatggatctgatcctgagccagctggccctggccaattccctggtgctgttctctaagggcatccctcagaccatggccgccttcggcctgaagtattttctggacgatacaggctgtaagctggtgttttactatcacagggtgggaaccggcgtgagcttctccacaatctgcctgctgaacggctttcaggccatcaagctgaatccttctatctgtcggtggctggagctgaagatcagaagcccaaagttcatcggcttttgctgtttcctgtgctgggccccccacctgctgatcaacacctctgtgctgttcctggtgaatggccctctgaactctaagaatctgagcgtgaagaacaattacggctattgttcctggaagatgcctgagcggtttggcaccctgtacacagtgctgtatttcagcccagactttatgtccctgggcttcatggtgtgggcctctggcagcatggtgtttgtgctgtaccggcacaagcagagagtgcagcacatccacagcaacaggctgtctagccgcccttcccacgaggccagagccacccacacaatcatggtgctggtgtcctctttctttgccttctatagcgtgcactccatcctgaccatctggatgacagtggtggccaatccaggccagtggatcgtgaacaatagcgtgttcgtggccagctgctttcccgccttctccccttttgtgctgatcttttccgacacacacgtgtctcagttctgctttgcctgtcggaccaagaagacactgttcccagatctggtggccatgccctga

SEQ ID NO: 216 - DNA, 918 bp, synthetic construct
  source 1..918: mol_type = other DNA
atggcctccgtggacctgtttatcggcatgatcgtgctgttccaggtggtggtgggcatcctgggcaacttttccctgctgtaccactatatgttcctgtactttaggggctgcaagccccgcagcacagacctgatcctgcgccacctgaccgtggccaactctctggtcatcctgagccggggcatccccgagacaatggcagcctttggcctgaagcacttcgataattactttggctgcaagttcctgctgtatgtgcacagggtggcccgcggcgtgtccatcggctctacatgtctgctgagcgtgttccaggtcatcaccatcaaccctcggaacagccggtgggccgagatgaaggtgaaggccccaaagtacatcggcctgagctccatcctgtgctgggtgctgcacatgctggtgaatgccatctttccaatctataccaccggcaagtggtccaacaagaatatcaccaagaagggcgacctgggatactgctctgccccactgcacgatgaagtgatcaagtccgtgtatgccgccctgacatcttttcacgacgtgctgtgcctgggcctgatgacctgggcctctagctccatggtgttcgtgctgtacagacacaagcagcaggtgcagcacatccaccggaacaatctgtctcccagatctagccctgagaacagggccacacagagcatcctggtgctggtgagcaccttcgtgtccttttatgccctgtcctctatcatctacgtgtatctggccctgttcgacaacagctcctggtggctggtgaataccgccgccctgatcacagcctgctttccaaccatcagccccttcgtgctgatgtgccacgatccttctatcagccggctgtgctgtatctgctgtggccggaatagatga

SEQ ID NO: 217 - DNA, 909 bp, synthetic construct
  source 1..909: mol_type = other DNA
atggctagccggtacgtggccgtgggaatgatcttcctgagccagaccgtggtgggcgtgctgggaaattttagcctgctgctgcactacctgagcctttattgcaccggctgcagactgaggtcaacagatctgatcgttaagcacctgatcgtggccaacttcctggccctgctgtgcaagggcgtgccccagaccatggccgccttcggcgtgagatacttcctgaacgccatcggctgtaaactggtgttctacctgcatcgggtgggcagaggcgtctctatcggcaccacctgtctgctatctgtgttccaggtgatcaccatcagcagcagaaaaagcagatgggctaagctgaaggaaaaggcccctaagcacgtgggcttctctgtgctgctgtgctggatcctgtgcatgctggtcaatattatctttcctatgtacgtgaccggcaagtggaactacaccaacatcacagtgaacaaagacctgggctactgcagcggcggaggaaacaacaagatcgcccagaccctgcgggccatgctcctgagcttccctgatgtgctgtgtctgggcctgatgctgtgggccagctctagcatggtgtgcattctgcacagacacaagcagagagtgcagcacatcgacagaagcaacctgagccccagagccagccctgagaacagagctacacagagcatcctgatcctggtgtccaccttcgtgtcctcttacacactgtcctgcctgttccaagtgtgcatcgccctgctggacaaccctaatagcctgctggttaacacatccgctctgatgtctgtgtgttttcccaccctgtccccattcgtgctcatgagctgcgaccctagcgtctaccggctgtgcttcgcctggaagcggtga

SEQ ID NO: 218 - DNA, 1074 bp, synthetic construct
  source 1..1074: mol_type = other DNA
atgctgaaactggtgatcatcgaaaacatggccgaaatcatgctgttcagcctggacctgctgctgttcagcacagacatcttgtgcttcaacttcccttccaagatgatcaagctgcctggctttataacaattcagatcttcttctaccctcaggcctcctttggcatcagcgctaataccatcctgctcctttttcacatcttcaccttcgtgttctctcacagaagcaagagcatcgacatgatcatcagccatctgtctctgattcacatcctgctgctgtttacccaggccatcctggtttctctggatttcttcggcagccagaacacccaggacgatctgaggtgcaaggtgatcgtgtttctgaacaaggtgatgagaggactgagcatctgcacaccttgtctgctgtccgtgctgcaggctatcatcagcccatctatcttctccctggccaagctgaagcaccccagcgcctctcatatcctcggcttctttctgttcagctgggtgctgaacatgttcatcggcgtgatcttctgctgcaccctgcggctgccccccgtgaaacggggccagagcagcgtctgtcacaccgccctgttcctgttcgcccacgagctgcaccctcaagagacagtgttccacaccaacgatttcgagggctgtcacctgtaccgggtgcacggacctctgaaaagactgcacggcgactacttcatccagaccatcagaggatatctgtctgccttcacccaacctgcctgccccagagtgagtcctgtgaagcgcgccagccagacaatcctgctgctcgtgtccttcgtgttcatctactgggtcgacttcacattcagcttctcaagaggcgtgacctggatcaacgacagcctgctggtgtggtttcaggtgattgtggccaacagctacgccaccatcagccccctgatgctgatctacgctgataaccagatctttaagaccctgcaaatgctgtggttcaagtacctgagccctccaaagctgatgctcaagttcaatagacagtgcggctctacaaaaaagtga

SEQ ID NO: 219 - DNA, 2526 bp, synthetic construct
  source 1..2526: mol_type = other DNA
atgctgctgtgtaccgctagactggtgggcctgcaactgctgttgagctgctgctgggctttcgcttgtcactctaccgagagcagccctgatttctccctgcctggcgactacctgctggccggcctgttccctctccattctggctgtctgcaggtgaggcatagacctgaagtgacactgtgcgacagatcttgcagcttcaacgagcacggctaccacctctttcaggctatgcggttcggcatcgaagaaatcaacaacagcaccgccctgctgcctaacgtgaccctgggctacgagctgtacgacgtgtgcagcgaaagcgccaacgtgtacgccaccctgagagtgctgagtttgcctggccagcaccacatcgagctgcaaggcgacctgctccactacagccctacagtggtggccgtgatcggacctgacagcacaaatagagccgccaccacagccgccctgctctctccattcctggtccctctgatctcttatgaggccagcagcgagacactgtcagtgaagagacagtaccccagcttcctgagaaccatccccagcgacaagtaccaggtggaaactatggtgctgctgctgcagaagttcggctggacctggatctcccttgtgggaagctccggagattacggccaactgggcgtgcaggccctggaaaaccaggccacaggccagggaatttgcatcgcttttaaggacatcatgcccttctccgcccaagtgggcgacgagagaatgcagtgcatgatgcggcacctggctcaggctcgggccaccgtggtcgtggtgttctcctccagacagctggccagagtgttcttcgagagcgtggttcttgccaacctgaccggaaaagtgtggatcgcctccgaagattgggctatcagccggcacatcaccggagtgcctggcatccagcggatcggaaccgtgcttggagttgccatccagcagagagcagtgcctggactgaaagagttcgaggaggcctacgccagagccgacaagggcgctcctcggccttgccataagggctcctggtgctccagcaaccagctgtgcagagaatgccaggccttcacggcccacaccatgcccaagctgaaggccttcagcatgagcagcgcctataacgtgtacagagccgtgtacgccgtggctcacggactgcaccagctgctgggctgcgccagcggagcctgcagccggggccgagtgtacccttggcagctgctggagcagatccacaaggtgaacttcctgctgcacaaggatacagtggctttcaacgacaacggcgaccctctgtctggatatgatatcatcgcctgggactggagcggccctaaatggacattcaccgtcatcggcagcagcacctggtcacctgttcagctggacatcaatgagacaaagatccagtggcatggcaaagataaccaggtgccaaagagcgtgtgtagcagcgactgcctggaaggccaccagagagtcgtggtcggcttccaccactgttgttttgaatgtgtgccctgtgaagccggcacatttctgaacaagtccgatctgtaccggtgccagccttgtggcaaggaagagtgggcccctgagggcagccagacctgttttcccagaacagtggtgttcctggcttggcacgagcctaccagctgggtgctcctagccgccaacactctgctgctgctgctgctgcttggtacagccggccttttcgcctggcacctggacacccctgtggtgagaagcgcgggcggcaggctgtgcttcctgatgctggggagcctggccgccggcagctgcagcctgtacggcttcttcggcgagcccacccggcccacctgcctactgcggcaggccctgtttgccttgggattcgctatctttctgagctgtctgaccgtgcggtccttccagctcgtgattattttcaagttcagcaccaaggtgccaacattctaccacgcctgggtgcagaaccacggcgccggcctgttcgtgatgatctcttctgccgcccagctgctgatctgcctgacatggctggtggtgtggacccctctgcccaccagagagtaccagcgcttcccccacctagtggtcctggagtgcaccgaagccaatagcctgggctttatcctggcttttctgtacaacggcctcctgtctatctcagccttcgcctgcagctacctgggcaaggacctgcctgagaactacaatgaggccaagtgcgtgacctttagcctgctgctgaatttcgtgtcttggatcgcttttttcaccaccgccagcgtgtatcaaggcaaatacctgcccgccgtcaacgtgctggctggcctgtccagcctgagcggcggcttctctggctacttcctgccaaagtgctacgtgatcctgtgcagaccagatctgaactccaccgaacacttccaagccagcatccaggactacaccagaagatgcggctctacctga

SEQ ID NO: 220 - DNA, 2547 bp, synthetic construct
  source 1..2547: mol_type = other DNA
atgctgggcccagccgttctgggcctgagcctgtggctgcaccctggaaccggcgcccctctgtgtctgtcccagcagctgcggatgaaaggcgattacgtgctgggcggactgtttccactgggcgccgaagaggccggcctgcggtccagaaccagacctagctctcctgtttgcaccagattcagcagcaacggcctgctgtgggccttagctatgaagatggccgtggaggaaatcaacaacaagagcgacctgctgcccggcctgagactgggctacgacctgtttgatacatgttctgaacccgtggtggccatgaaaccttctctgatgttcctggccaaggccggctctcgggacatcgccgcttactgtaactacacccagtaccagcccagagtgctggccgtgatcggcccccactcctctgagctggccctggtgaccggcaagttcttcagcttctttctgatgcctcaagtgagctacggcgccagcatggacagattaagcaatagagagacattcccctctttcttcagaaccgtgcctagcgatagagtgcagctcacagccgctgtggaactgctgcaggagttcggctggaactgggtcgccgctctgggtagcgatgatgagtacggcagacagggcctcagtctgttcagctccctggccgccgccaggggcatctgcatcgcccacgagggcctggtccctctgcccagagcggacgacagcagactggggaaagtgcaagatctgctgcatcaggtgaaccagagcagcgtgcaggtggtggtgctgttcgccagcgctagggcggctcatgccctgttctcctattctatcagcagccggctgagccccaaggtgtgggtggcctcagaggcctggctgaccagcgacctggttatgactctgcctggcatggctcaagtgggcaccgtgcttggcttcctgcaaagaggcgcccagttgcctgagttccctcagtacgtgaagacccacctcgccctggccgctgatccagccttttgtgccagcctaggtgctagagagcagggcctggaagagcacgtagtgggcccaagatgccctcagtgcgaccacattaccctgcagaacgtgtccgccggactgctgcatcaccagaccttcgctgcctatgccgccgtgtacagcgttgctcaagccctgcacaacaccctgcagtgcaatgccagcggctgccccgcccaggagcccgtgcggcctcagctgctggagaacatgtacaacctgagcttccacgcccggggcctgcctctgagattcgacagcagcggcaatgtggacatggaatacgacctgaagctgtgggtctggcagggaagcgtccctcggctgcacacggtgggcagattcaacggcagcctgcaactggaaagatctaagatgagatggcacacacccggaaatcaaaagcctgtgtctcagtgcagcagacagtgtcaggagggccaggtgcggcgcgtgaagggctttcacagctgctgctacgactgcgtggactgtaaagccggcagctatagacagaaccccgacgacctggcttgcaccttctgcggccaggaccagtggtcccctgagcggagcacccggtgtttccctagaagacctcggttcctggcctggggagaacctgccgtgctgctgctgctgctccttctgtcactggcattaggccttgtcctggctgccctgggcctcttcgtgcaccacagagattcccctctggtacaggccagcgggggacctctggcctgctttggcctggtctgtctgggcctggtgtgcctgtctgtgttactgttccccggacagccttctcctgcctcttgtctggcccagcagccactaagccacctgccactgacaggctgcctgtctacactgttcctgcaggccgctgagatcttcgtggaatccgagctgcctctgagctgggctgaccggctgagtggatgtctgcgcggcccctgggcttggctggtggtgctgctggccatgctggtggaagccgccctgtgcgcctggtacctggtggccttcccccccgaggtggttacagattggcacgtgctgcctaccgaagccctggtgcactgcagaacacgcagctgggtcagcttcggcctggtgcacgccaccaacgccacactggcattcctgtgcttcctgggtacatttctggtgcaatctcagcctggaagatacaaccgggcccggggcctgacattcgctatgctggcttacttcatcacctgggtcagctttgtgcccctgtttgccaatgtgcaggtggtgtaccagcctgcagtgcagatgggcgccatcctgctgtgcgccctgggaatcctggccaccttccaccttcctaagtgctacctgcttctgtggcagccaggcctgaacaccccagagttcttcctgggaggcggccctggcgacgctcagggccagaacgacggcaataccggcaaccagggaaagcacgagtga

SEQ ID NO: 221 - DNA, 930 bp, synthetic construct
  source 1..930: mol_type = other DNA
atgtttagccctgaagacaacatctttatcatcatcatcacaggcgagttcatcatcggaatcctgggcaacggctacatcggcctggtgaactggatcgactggatcaagaaaaagaagatctccagcatcgactacatcctgaccagcctggctatttctagaatctgtctgatctgcgtgatggtgctgaatggcatcatcatcgtgctgtatcctgacgtgtacaccaacaacaagctccagatcgtgatcttcaccttctggacatttgccaattacctgtctatgtggttcgccacctgcctgaacgtgttctacttcctgaagatcgctaatttcagccaccccctgttcctgtggctgaagtggcggatcgatagagtggtgcactggatcctgctcggctgcctggccatttctctgctggtcagcctgatcgccgccatcgttctgagctgcgactacagattccataagattgctaagcacaagcggaacatcacagaaatgttccacgtgtccaagatccagtacttcgagcctctgaccctgtttaacctgcttgccatcgtgccattcaccgtgtccctgatcagcttcttcctgctgattagaagcctgtggcgccacaccaagcaaatgaagctttatgtgaccggatgtagggatccttcaacagaggcccacgtcagagccatgaaaaccatgacaagcttcctgttcctgctgttcgtgtactacatcagcagcctgctgatgacctttagctacctgatgaaagagtacaagctggccgtgatgttcggcgaaatcatcgccatcctgtaccccagcggccacagcctgatcctgatcatcctgaacaacaaactgagacaggcctctgtgcggatgctgacatgcagaaagatcgcatgcatgatgtga

SEQ ID NO: 222 - DNA, 888 bp, synthetic construct
  source 1..888: mol_type = other DNA
atgatccccatccaactgacagtctttttcatgatcatctatgtgctggaatctctgaccatcatcgtgcagagctctctgatcgtggccgtgctgggcagagagtgggttcaagtgcgcagactgagccctgtggacatgatcctcatcagcttgggaatctgtagattctgcctgcagtgggcctctatgctctacaacttctgcagctacttcaaccccaattacgtgttctggtacctgacaattacctgggagttcaccaacatcctgaccttctggctgacaagcctgctcgctgttttctactgcgtgaaggtgtcctcctttacccaccctatcttcctgtggctgagatggcggatcctgagactggtcccttggctgctgctgggcagcctgatgatttcttgcgtgacaatcattcccagcgccatcggcaactacatccagatccagctgatcaccatggaacacctgcctcggaactctacagtgaccgagagactggagaacttccaccagtacttcttccaggcccacaagaccgtggctctggtgatccctttcctgctgtttctggctagcacaatcctgctgatggccagcctgacccagcacctggaacagatgcagcaccacagcacaggacactgtaatagctctatgaaagcccatttcaccgccctgcggagccttgccgtgttcctgatcttcttcaccagctactttctgaccatcctgatcagcatcatcggcaccctgtttgataagagatcctggttctgggtgtgggaggccttcatctacgccttcgtgtccatccacagcaccagcctgatgctgagcagcccaacactgaaacgggtgctgaagggcaagtgctga

SEQ ID NO: 223 - DNA, 1008 bp, synthetic construct
  source 1..1008: mol_type = other DNA
atgctgacactgacacctatcagaaccgtgtcctacgaggtgaagagcaccttcctcttcctgagcgtgctggagttcgccgtgggcatcctcacaaacgccttcatcttcctggtgaacttctgggacgtggtcaggcggcaacctctgagcaactgcgacctggtgctgctgtgcctgtctatcaccagactgttcctgcacggcctgctctttcttgatgccatccagctgacccactttcagaagatgaaagaccccctgagccacagctaccagaccatcatcatgctgtggatgatcgccaaccaggccaatctgtggctggccacctgtctgtctctgctgtactgcagcaagattgtgcggttcagccatacattcctgctctgcctggccagctgggtctccagaaagatccctcagatgctgctgggcgccatcctgttttcatgcatctgcaccgtcctgtgtctgtgggactttttcagcagaagccacttcacagtgaccacagtgctgttcatgaacaacaacaccgagctgaatctgcagatcaagaagctgaacttcttctacagcttcctgttctgctacctgggaagcatcccccccttcctcctgtttctggtgtccagcggcgtgctgatcgtgtccctgggcagacacatgcggaccatgaaagcctatacaagagacagccgggaccctagcctggaagcccacatcaaggccctgaagtccctggtttctttcctgtgcttctacgtggtgtctttttgcgccgctctgatcagcgtgcctctgctgatcctgtggcacaacaagatcggcgtgatggtgtgcgtgggcattatggccgcttgtccttctggccacgctgctatcctgatcagcggaaatgccaagctgagaagagccgtgatgaccatcctgctgtgggcccagagcagcctgaaagtgcgcgccgaccacaaggctgatccaagaacccctgatctgtgttga

SEQ ID NO: 224 - DNA, 939 bp, synthetic construct
  source 1..939: mol_type = other DNA
atggccaccggcctggataagatcttcctgattctggccatcgccgagttcatcatcggcatgctgggcaatgtgttcatcggcctggtcaactgctctgaatgggtgaagaaccagaaggtgtccagcgccgacttcatcctgacatgcctggctatcagcaggatcggacagctgctggtgatcctcttcgacagcttcctggtgggcctggctcctcacctgtacaccacctacagactgggcaagacagtgatcatgctgtggcacatgaccaaccacctgacaacatggctggccacctgtctctccatcttctacttcctgaaaatcgcccacttcagccacagcctgttcctgtggctgagatggcggatgaacagagtgatcctgatgctgctgatcctgtccctgtttctgctgatctttgatagcctgctgctggagatcttcattgatatctctctgaactacatcatcgacaagagcaacctgaccctgtatctggacgaaagcaagaccctgtacgacaaactgctgatcctgcttagcctgacatacttcatccccttcagtctgtctctgaccagcctgctgctgctgttcctgtcccttgtgcggcacacaagaaacctgcagctgaatagcctgggcagccgggacagcagcaccgaggcccataagagagccatgaaaatggtgatgagctttctgtttctgttcatagttcacttcttcagcctgcaactggctaattggatctttttcatgctttggaacaacaagtgcatcaagttcgtgatgctggccctgaacgcctttccaagcggccactctttcatcctgatcctgggaaattctaagctgcggcagaccgccctgagactgctgtggcacctgagaaactacctgaagacccctaaccccctgcctctgtga

SEQ ID NO: 225 - DNA, 930 bp, synthetic construct
  source 1..930: mol_type = other DNA
atgatcacatttctgcctatcatctttagcatcctggtcgtggtcacattcgtgatcggcaacttcgctaacggcttcatcgccctggtgaacagcaccgagtgggtcaagcggcaaaaaatctctttcgccgatcagatcctgaccgccctggctgtgtctagaatcggcctgctgtgggtcctgttgctccactggtactctattgtgctgaaccccgccttctacagcgtggaagtgcggatcacaacctacaacgtgtgggccgtgacatctcacttcagcaattggctggccaccagcctgtccatcttctacctgctgaagatcgccaatttcagcaacctgatcttcctgcacctgaaaagaagagtgaagtccgtgatcctggttatgctgctgggccctctgctgttccttccttgccacctgtttgtgatcaacatgaaccagatcgtgcaaaccaaggaatacgagggcaatatgacctggaagatcaagctgagaagaaccatgtttctgagcgacaccaccgtgacaatgctggctaatctggtgcccttcactctgacactgatttcttttttgctgctcatctgcagcctgtgcaagcacctgaagaagatgcagctgcacggaaagggaagccaggaccctaacaccaaagtgcacatcaaggccctgcagacagtgatcagcttcctgcttctgtgtgccatctacttcgtgttcgtgaccatcagcgtgtggtcctttcagaccctggacaacaacccagtgttcatgttctgccaggccatcaccttctcatatcctagcgcccatcctttcatcctgatctggggcaacaagaaactgaagcagaccttcctgagcgtgctgtggcaggtgcgctactgggtgaagggccagaagcccagcagcccatga

SEQ ID NO: 226 - DNA, 930 bp, synthetic construct
  source 1..930: mol_type = other DNA
atgatcaccttcctgcctatcatcttttccatcctgatcgttgtgaccttcgtgatcggaaacttcgccaatggcttcatcgctctggtgaacagcatcgaatgggtgaaaagacagaagatctcttttgctgatcaaatcttgacagccctggctgtgtccagagtgggcctgctgtgggtcctgctgctccattggtacgccacagagttcaacctggctttttacagcatcgaggtgcggatcaccgcctacaacgtgtgggccgtgaccaaccacttctctaattggctggccacctctctgagcatcttctatctgctgaagatcgccaattttagcaatctgatcttcctgcacctcaagagacgggtgaagagcgtgatcctggtgattctgctgggacctctgctcttcctggtctgccacctgttcgtgattaacatgaaccagatcgtgcagaccaaggaatacgagggcaacatgacctggaagatcaagctgagaagcgccatgtacctgagcaacatgaccgtgaccatgctggccaactttgtgccattcaccctgacactgatcagcttcctgctgcttatctgtagcctgtgcaagcacctgaagaagatgcagctgcacggcaagggctctcaggacccttctacaaaggtgcacatcaaggccctgcagacagtgaccagcttcctgctgctgtgcgccatctacttcctgtctattatcatgagcgtgtggagctttgagagcctggaaaacaagcctgtgttcatgttctgccaggccatcgccttcagctaccctagcacacaccccttcatcctgatctggggcaacaagaaactgaaacagaccttcctgtccgtgctgtggcacgtgcgctactgggtcaagggccaaaaaccctccagcagctga

SEQ ID NO: 227 - DNA, 1008 bp, synthetic construct
  source 1..1008: mol_type = other DNA
atgcctttctgccacaacatcattaacatctcatgcgtgaagagctcttggtccaacgatgtgcgggctagcctgtacagcctgatggtcctgatcatcctgaccaccctggtgggaaatctgatagtgatcatcagcatcagccacttcaagcagctgcacacccctacaaactggctgatccattctatggccacagtggacttcctgctgggatgtctggtgatgccatacagcatggtgcgctccgtcgagcactgttggtacttcggcgaggtgttttgcaagatccacacaagcacagatatcatgctgtcttccgccagcattttccacctgagcttcatctccatcgacagatactacgccgtgtgcgaccctctgcggtacaaggccaagatcaacatcctggttatctgtgtgatgatcttcatctcttggagcgtccctgctgtgttcgccttcggcatgatcttcctggagctgaatttcaagggcgccgaggaaatctactataagcacgtgcactgcagaggcggctgcagcgtgttctttagcaaaaccagcggcgtgctggcttttatgacctctttttacatccctggcagcatcatgctgtgcgtgtactacagaatctacctgatcgccaaagagcaggccagaagcatcagcgacgccaaccagaaactgcaaatcggcctggagatgaaaaacggcatcagccagagcaaggaaagaaaggccgctaagaccctgggcatcgtgatgggcgtgttcctcatttgctggtgtccttttttcatctgcacagtgatggaccccttcctgcactacatcatcccccccaccctgaatgatgccctgatctggttcggctacctgaacagcaccttcaaccccatggtgtacgccttcttctatccttggttccggagagccctgaagatgatcctgttcggaaagatctttcagaaggacagctctagatgcaagctgtttctggaatga

SEQ ID NO: 228 - DNA, 921 bp, synthetic construct
  source 1..921: mol_type = other DNA
atgtactccttcatggctggcgccatcttcatcacagtgttcggcaacctggccatgatcatcagcatctcatatttcaagcagctgcacacccctacaaatttcctgatcctgagcatggctgtgaccgacttcctgcttggatttacaatcatgccctacagcatgatcagaagcgtggaaaactgctggtacttcggactgaccttctgcaagatccactactcttttgacctgatgctgtctattaccagcatcttccacctgtgtagcgtggccatcgacagattctacgccatctgctaccctctgctgtacagcaccaagatgaccatccctgtgatcaagcggctgctgctgctgtgttggtccgtccccggcgcttttgccttcggcgttgtgtttagcgaggcctacgctgatggaatcgagggctacgacatcctggtggcctgcagcagcagctgtcctgtcatgttcaacaagctgtggggcaccaccctgtttatggccggctttttcaccccaggcagcgtgatggtgggcatctacggcaagatcttcgccgtgtccagaaagcacgccagagccatcaacaacctgccagaaaaccagaacaatcaaatgcggaaggacaagaaagccgccaagaccctcggaatcgtgatgggcgtgttcctgctgtgctggtttccttgcttcttcaccattctgcttgatcctttcctgaacttctctacacctgtggtgctgttcgatgccctgacatggttcggctatttcaacagcacatgcaaccccctgatctacggcttcttctacccctggttcagacgggccctgaagtacatcctgctgggcaaaatctttagctctcatttccacaacaccaatctgttcacccagaaagagacagagtga

SEQ ID NO: 229 - DNA, 1014 bp, synthetic construct
  source 1..1014: mol_type = other DNA
atgagggccgtgttcatccagggcgccgaggagcaccctgccgccttttgctaccaagtcaacggcagctgtcctagaacagtgcaccccctgggcattcagctggctatctacctggcttgtgccgctggaatgctgatcaccgtgctgggcaatctgttcgtggtgttcgccgtgtcctacttcaaggccctgcacacccctacaaacttcctgctgctgagcctggccctggctgatatgctgctcggcctgctcgtgctgcccctgtccaccatcagaagcgtggaatcctgctggtttttcggcgacttcctgtgcagactgcatacatacctggacacactgttctgcctgacaagcatcttccacctgtgcttcatttctatcgacagacactgcgccatctgcgaccccctgctgtaccctagcaagttcaccgtgcgggtcgccctgagatacatcctggccggatggggagtgcctgctgcatacaccgccttcttcctgtatacagacgtggtggaaaccggcctgagccagtggctggaagagatgccttgtgtgggaagctgccagctgctgtttaacaagttctggggctggctgaatttccccgtgttcttctttccatgtctgatcatgatcagcctgtacgtgaagatctttgtggtcgccacccggcaggcccagcagatcaccaccctgtctaagtccctggccggcgccgctaaaagagagcgcaaggccgccaagaccctgggcatcgccgtgggcatctacctgctctgctggctgccttttaccatcgatacaatggtggacagcctgctgaacttcatcacacctccactggtgttcgacatcttcatctggttcgcctacttcaacagcgcctgcaaccccatcatctatgtgttcagctaccggtggtttagaaaggccctgaagctgaccctttctcaaaaaatcttcagccctcggaccagaaccgttgatctgtaccaggagtga

SEQ ID NO: 230 - DNA, 1029 bp, synthetic construct
  source 1..1029: mol_type = other DNA
atgacaagcaatttcagccagcctgtggtccagctgtgctacgagaacgtgaacggctcctgcatcaagacaccttactcccctggctctagagtgatcctgtacaccgtgttcggatttggaagcctgctggctgtgttcggcaatctgctggtgatgaccagcgtgctgcacttcaagcagctgcattctccagccaacttcctgattgctagcctcgcctgcgccgattttctggttggcgttaccgtgatgcctttcagcatggtcagaagcgtggaaagctgctggtacttcggcgccaagttctgcactctgcacagctgttgcgacgtggctttttgctacagctctctgtttcacctgtgcttcatctccatcgataggtacatcgccgtgaccgaccccctcgtgtaccccacaaagttcaccgtgtccgtgtctggcatctgcatcagcatcagctggatcctgccactggtgtactctggcgccgtgttctacaccggcgtcagcgacgacggcatggaagagctggttagtgccctgaactgcgtgggaggatgtcagatcgtggtgaaccaggactgggtgctgattgatttcctgctgttcttcatccccaccctggtgatgatcatcctgtatagcaagatctttctggtggccaagcaacaggccatcaaaatcgaaacaacaggcagcaaagctgagtctagctctgagagctacaaggccagagtggccaagcgggaacggaaggccgccaaaaccctgggcgtgacagtggtggccttcatgatcagctggctgccttataccatcgacaccctgatcgacgcctttatgggcttcatcacccctgcctacatctacgagatctgttgttggggcgcttactacaacagcgccatgaaccccctgatctacgccctgttctatccttggttcagaaaggctatcaagctgatcttgtctggcgaggtgctgaaggcctccagcagcaccatcagcctgttcagcgagtga

SEQ ID NO: 231 - DNA, 1047 bp, synthetic construct
  source 1..1047: mol_type = other DNA
atggtcaacaacttcagccaggccgaggccgtggaactgtgctacgagaacgtgaacggcagctgcatcaagacaccatatagccccggccctagagccattctgtacgccgtgcttggatttggtgctgtgctggccgttttcggcaacctgctggtgatcatcgccatcctgcatttcaagcagctgcacacccccaccaatttcctgatcgcttctctggcctgcgccgacttcctggtgggcgtgaccgtcatgcctttctccaccgtgcggagcgtggaatcttgctggtacttcggcgagagctactgcaagttccacacatgcttcgacaccagcttctgctttgccagcctgtttcacctgtgttgtatcagcatcgacagatacatcgccgtgacagaccccctgacctaccctacaaagttcaccgtgtccgtgtctggcatctgcatcgtgctgagctggttcttcagcgtgacatacagcttttcaatcttctacaccggcgccaacgaggaaggcattgaggaactggttgtggccctgacatgtgttggaggctgccaggcccctctgaaccagaactgggtgctcctctgtttcctgctgttcttcatccctaccgtggccatggtgttcatctacggcaagatcttcctggtggccaagcaccaggctaggaagatcgagagcaccgccagccaagcccagtctagcagcgagtcttataaggaacgggtggctaaaagagagagaaaggctgccaaaaccctgggcattgccatggccgcttttctggtctcctggctgccttacatcatcgatgctgtgatcgacgcctacatgaatttcatcacacctccatacgtgtacgagatcctggtgtggtgcgtgtactacaacagcgccatgaaccccctgatctacgcctttttctatccttggttccggaaggcgatcaagctgatcgtgtctggaaaagtgctgagaaccgacagcagcaccaccaatctgttctccgaggaagccgatacagattga

SEQ ID NO: 232 - DNA, 1038 bp, synthetic construct
  source 1..1038: mol_type = other DNA
atgtcttccaattcttctcctctggccgctgtgcagctgtgctacgagaatgtgaatggcagctgcgtgaagaccccttactcgccaggcagcagagtgatcctgtacatcgtgtttggctttggcgctgtgctggccgtgttcggcaacctgctggtcatgatcagcatcctgcatttcaaacagctgcacagccctacaaacttcctgatcgccagcctggcctgcgccgatttcctggtcggcgtgaccgtgatgcccttcagcatggtgcggagcgtggaaagctgttggtacttcggcagaagcttctgcaccttccacacctgttgcgacgtggccttttgctatagctccctgtttcacctgtgcttcatctctatcgatagatacatcgccgtgaccgatcctctggtgtaccccaccaagttcaccgtgtccgtgagcggaatctgtatcagcatcagctggatcctgcctcttgtttactctggcgccgtgttctacaccggcgcctacgacgacggcctggaagagctgagctctgccctgaactgcgtgggcggatgtcaaacagttgtgaaccagaactgggtgctcatcgacttcctgtccttcttcatccccaccctggtgatgatcatcctgtacagcaacatcttcctggtggctagacagcaggccaagaaaatcgagaacaccggcagcaagacagaaagcagctccgagagctacaaggccagagtggccaagcgggaaaggaaggcagctaaaacactgggaatcaccgtggtggccttcatgattagctggctgccatactctatcgacagcctaatcgacgccttcatgggcttcattacacctgcctacatctacgagatctgctgctggtgcgcctattacaacagcgccatgaaccccctgatctacgccctgttttatccttggttccggaaggccatcaaggtgatcgtgtccggacaggtcttcaagaacagcagcgctacaatgaacctgttctctgagcagatctga

SEQ ID NO: 233 - DNA, 936 bp, synthetic construct
  source 1..936: mol_type = other DNA
atggaacctcgggaagccggccagcacgtgggcgccgccaacggcgctcaggaggacgtggccttcaacctgatcatcctgtctctgacagagggcctgggactgggcggactgctgggcaacggcgccgtcctgtggctgctgagcagcaacgtgtacagaaaccccttcagcatctacctgctggatgtggcctgcgcagatctgatcttcctgggctgccacatggtggctatcattcctgacctgctgcaaggcagactggacttccccggctttgtgcagacatctctggccaccctccgcttcttctgctacatcgtgggcctgagcctgctcgccgccgtgtccgtggaacagtgcctggccacactgttccccgcctggtactcttgtagaagacctcggcacctgaccacctgtgtgtgcgccctgacctgggccctgtgtctgctgctgcacctgctgctgagcggagcttgtacccagttcttcggcgagcctagcagacacctgtgcagaaccctgtggctggtggccgccgtgctgctggccctgctgtgctgcaccatgtgcggcgccagcctgttactgctgctgagagtggaaagaggtcctcagaggcctcaacctagaggcttccctggcctcgtgctgctggctgtgctgctttttctgttttgtggcctgccttttggcatctactggctgtccagaaatctgctgtggcacatcccccactacttctaccatttcagcttcctgatggccgctgttcactgcgctgcaaagccagtgatctatttctgcctgggcagcgcccagggcagacggcttccactgagactggtgctgcagagagccctgggcgacgaggccgagctgggagctgtgcgggagacaagccggcggggactggtcgacatcgccgcctga

SEQ ID NO: 234 - DNA, 1032 bp, synthetic construct
  source 1..1032: mol_type = other DNA
atggccggaaattgcagctgggaagcccaccccggcaatagaaacaagatgtgccccggcctgagcgaggcccctgagctgtactctagaggcttcctgaccatcgagcagatcgccatgctgcctccacctgctgttatgaactacatcttcctgctgctgtgtctgtgcggccttgtcggaaatggcctggtgctgtggttcttcggcttctctatcaagcggaaccccttcagcatttacttcctgcacctggctagcgctgatgtgggatatctgttctcaaaggccgtgttcagcattctgaacacaggcggctttctgggcaccttcgccgactacgtgagagccgtgtgcagaatcctgggactgtgtatgttcctgacaggtgtttccctgctgcccgccatcagcgccgagcggtgcctgtctgtgatcttccctgcttggtactggcggagacgccccaaaagactgagcgccgtggtctgtgccctgctgtgggtcctgagcctgctggtgacatgcatccacaactacttctgcgtgttcctgggcagaggagccagcggcgccgcctgcagacacatggacatctttctgggcatcctgctgttcctggtgttctgtcctctgatggtgctgccttgcctcgccctgatcctgcatgtggaatgcagagccagacggcggcagagatctgctaaactgaaccacgtgatcctggccatggtgtccgtgtttctcgtgtccagcatctacctgggcatcgactggtttctgttctgggtgtttcagatccctgccccattccccgagtacgtgaccgacctgtgcatctgcatcaacagcagcgccaagcctgtggtgtactttctggccggcagagataagagccagcggctgtgggagcctctgagagtggtgttccaaagggcgctgcgggacggcgctgaactgggcgaggccggaggcggcacccctaacaccgtgaccatggaaatgcagtgtccatctggcaacgccagctga

SEQ ID NO: 235 - DNA, 684 bp, Homo sapiens
  source 1..684: mol_type = genomic DNA
atgtgtaaaagcgtgaccacagatgagtggaagaaagtcttctatgagaagatggaggaggcaaagccggctgacagctgggacctcatcatagaccccaacctcaagcacaatgtgctgagccctggttggaagcagtacctggaattgcatgcttcaggcaggttccactgctcctggtgctggcacacctggcagtcgccctacgtggtcatcctcttccacatgttcctggaccgcgcccagcgggcgggctcggtgcgcatgcgcgtcttcaagcagctgtgctatgagtgcggcacggcgcggctggacgagtccagcatgctggaggagaacatcgagggcctggtggacaacctcatcaccagcctgcgcgagcagtgctacggcgagcgtggcggccagtaccgcatccacgtggccagccgccaggacaaccggcggcaccgcggagagttctgcgaggcctgccaggagggcatcgtgcactggaagcccagcgagaagctgctggaggaggaggcgaccacctacaccttctcccgggcgcccagccccaccaagtcgcaggaccagacgggctcaggctggaacttctgctctatcccctggtgcttgttttgggccacggtcctgctgctgatcatctacctgcagttctctttccgtagctccgtataa

SEQ ID NO: 236 - protein, 227 aa, Homo sapiens
MCKSVTTDEWKKVFYEKMEEAKPADSWDLIIDPNLKHNVLSPGWKQYLELHASGRFHCSWCWHTWQSPYVVILFHMFLDRAQRAGSVRMRVFKQLCYECGTARLDESSMLEENIEGLVDNLITSLREQCYGERGGQYRIHVASRQDNRRHRGEFCEACQEGIVHWKPSEKLLEEEATTYTFSRAPSPTKSQDQTGSGWNFCSIPWCLFWATVLLLIIYLQFSFRSSV

SEQ ID NO: 237 - protein, 346 aa, Homo sapiens
MDTGPDQSYFSGNHWFVFSVYLLTFLVGLPLNLLALVVFVGKLRCRPVAVDVLLLNLTASDLLLLLFLPFRMVEAANGMHWPLPFILCPLSGFIFFTTIYLTALFLAAVSIERFLSVAHPLWYKTRPRLGQAGLVSVACWLLASAHCSVVYVIEFSGDISHSQGTNGTCYLEFWKDQLAILLPVRLEMAVVLFVVPLIITSYCYSRLVWILGRGGSHRRQRRVAGLVAATLLNFLVCFGPYNVSHVVGYICGESPVWRIYVTLLSTLNSCVDPFVYYFSSSGFQADFHELLRRLCGLWGQWQQESSMELKEQKGGEEQRADRPAERKTSEHSQGCGTGGQVACAEN

SEQ ID NO: 238 - protein, 560 aa, Homo sapiens
MDLKTVLSLPRYPGEFLHPVVYACTAVMLLCLLASFVTYIVHQSAIRISRKGRHTLLNFCFHAALTFTVFAGGINRTKYPILCQAVGIVLHYSTLSTMLWIGVTARNIYKQVTKKAPLCLDTDQPPYPRQPLLRFYLVSGGVPFIICGVTAATNIRNYGTEDEDTAYCWMAWEPSLGAFYGPAAIITLVTCVYFLGTYVQLRRHPGRRYELRTQPEEQRRLATPEGGRGIRPGTPPAHDAPGASVLQNEHSFQAQLRAAAFTLFLFTATWAFGALAVSQGHFLDMVFSCLYGAFCVTLGLFVLIHHCAKREDVWQCWWACCPPRKDAHPALDANGAALGRAACLHSPGLGQPRGFAHPPGPCKMTNLQAAQGHASCLSPATPCCAKMHCEPLTADEAHVHLQEEGAFGHDPHLHGCLQGRTKPPYFSRHPAEEPEYAYHIPSSLDGSPRSSRTDSPPSSLDGPAGTHTLACCTQGDPFPMVTQPEGSDGSPALYSCPTQPGREAALGPGHLEMLRRTQSLPFGGPSQNGLPKGKLLEGLPFGTDGTGNIRTGPWKNETTV

SEQ ID NO: 239 - protein, 1338 aa, Homo sapiens
MGAGGRRMRGAPARLLLPLLPWLLLLLAPEARGAPGCPLSIRSCKCSGERPKGLSGGVPGPARRRVVCSGGDLPEPPEPGLLPNGTVTLLLSNNKITGLRNGSFLGLSLLEKLDLRNNIISTVQPGAFLGLGELKRLDLSNNRIGCLTSETFQGLPRLLRLNISGNIFSSLQPGVFDELPALKVVDLGTEFLTCDCHLRWLLPWAQNRSLQLSEHTLCAYPSALHAQALGSLQEAQLCCEGALELHTHHLIPSLRQVVFQGDRLPFQCSASYLGNDTRIRWYHNRAPVEGDEQAGILLAESLIHDCTFITSELTLSHIGVWASGEWECTVSMAQGNASKKVEIVVLETSASYCPAERVANNRGDFRWPRTLAGITAYQSCLQYPFTSVPLGGGAPGTRASRRCDRAGRWEPGDYSHCLYTNDITRVLYTFVLMPINASNALTLAHQLRVYTAEAASFSDMMDVVYVAQMIQKFLGYVDQIKELVEVMVDMASNLMLVDEHLLWLAQREDKACSRIVGALERIGGAALSPHAQHISVNARNVALEAYLIKPHSYVGLTCTAFQRREGGVPGTRPGSPGQNPPPEPEPPADQQLRFRCTTGRPNVSLSSFHIKNSVALASIQLPPSLFSSLPAALAPPVPPDCTLQLLVFRNGRLFHSHSNTSRPGAAGPGKRRGVATPVIFAGTSGCGVGNLTEPVAVSLRHWAEGAEPVAAWWSQEGPGEAGGWTSEGCQLRSSQPNVSALHCQHLGNVAVLMELSAFPREVGGAGAGLHPVVYPCTALLLLCLFATIITYILNHSSIRVSRKGWHMLLNLCFHIAMTSAVFAGGITLTNYQMVCQAVGITLHYSSLSTLLWMGVKARVLHKELTWRAPPPQEGDPALPTPSPMLRFYLIAGGIPLIICGITAAVNIHNYRDHSPYCWLVWRPSLGAFYIPVALILLITWIYFLCAGLRLRGPLAQNPKAGNSRASLEAGEELRGSTRLRGSGPLLSDSGSLLATGSARVGTPGPPEDGDSLYSPGVQLGALVTTHFLYLAMWACGALAVSQRWLPRVVCSCLYGVAASALGLFVFTHHCARRRDVRASWRACCPPASPAAPHAPPRALPAAAEDGSPVFGEGPPSLKSSPSGSSGHPLALGPCKLTNLQLAQSQVCEAGAAAGGEGEPEPAGTRGNLAHRHPNNVHHGRRAHKSRAKGHRAGEACGKNRLKALRGGAAGALELLSSESGSLHNSPTDSYLGSSRNSPGAGLQLEGEPMLTPSEGSDTSAAPLSEAGRAGQRRSASRDSLKGGGALEKESHRRSYPLNAASLNGAPKGGKYDDVTLMGAEVASGGCMKTGLWKSETTV

SEQ ID NO: 240 - protein, 833 aa, Homo sapiens
MEPPGRRRGRAQPPLLLPLSLLALLALLGGGGGGGAAALPAGCKHDGRPRGAGRAAGAAEGKVVCSSLELAQVLPPDTLPNRTVTLILSNNKISELKNGSFSGLSLLERLDLRNNLISSIDPGAFWGLSSLKRLDLTNNRIGCLNADIFRGLTNLVRLNLSGNLFSSLSQGTFDYLASLRSLEFQTEYLLCDCNILWMHRWVKEKNITVRDTRCVYPKSLQAQPVTGVKQELLTCDPPLELPSFYMTPSHRQVVFEGDSLPFQCMASYIDQDMQVLWYQDGRIVETDESQGIFVEKNMIHNCSLIASALTISNIQAGSTGNWGCHVQTKRGNNTRTVDIVVLESSAQYCPPERVVNNKGDFRWPRTLAGITAYLQCTRNTHGSGIYPGNPQDERKAWRRCDRGGFWADDDYSRCQYANDVTRVLYMFNQMPLNLTNAVATARQLLAYTVEAANFSDKMDVIFVAEMIEKFGRFTKEEKSKELGDVMVDIASNIMLADERVLWLAQREAKACSRIVQCLQRIATYRLAGGAHVYSTYSPNIALEAYVIKSTGFTGMTCTVFQKVAASDRTGLSDYGRRDPEGNLDKQLSFKCNVSNTFSSLALKNTIVEASIQLPPSLFSPKQKRELRPTDDSLYKLQLIAFRNGKLFPATGNSTNLADDGKRRTVVTPVILTKIDGVNVDTHHIPVNVTLRRIAHGADAVAARWDFDLLNGQGGWKSDGCHILYSDENITTIQCYSLSNYAVLMDLTGSELYTQAASLLHPVVYTTAIILLLCLLAVIVSYIYHHSLIRISLKSWHMLVNLCFHIFLTCVVFVGGITQTRNASICQAAVTTHL

SEQ ID NO: 241 - protein, 1584 aa, Homo sapiens
MRGQAAAPGPVWILAPLLLLLLLLGRRARAAAGADAGPGPEPCATLVQGKFFGYFSAAAVFPANASRCSWTLRNPDPRRYTLYMKVAKAPVPCSGPGRVRTYQFDSFLESTRTYLGVESFDEVLRLCDPSAPLAFLQASKQFLQMRRQQPPQHDGLRPRAGPPGPTDDFSVEYLVVGNRNPSRAACQMLCRWLDACLAGSRSSHPCGIMQTPCACLGGEAGGPAAGPLAPRGDVCLRDAVAGGPENCLTSLTQDRGGHGATGGWKLWSLWGECTRDCGGGLQTRTRTCLPAPGVEGGGCEGVLEEGRQCNREACGPAGRTSSRSQSLRSTDARRREELGDELQQFGFPAPQTGDPAAEEWSPWSVCSSTCGEGWQTRTRFCVSSSYSTQCSGPLREQRLCNNSAVCPVHGAWDEWSPWSLCSSTCGRGFRDRTRTCRPPQFGGNPCEGPEKQTKFCNIALCPGRAVDGNWNEWSSWSACSASCSQGRQQRTRECNGPSYGGAECQGHWVETRDCFLQQCPVDGKWQAWASWGSCSVTCGAGSQRRERVCSGPFFGGAACQGPQDEYRQCGTQRCPEPHEICDEDNFGAVIWKETPAGEVAAVRCPRNATGLILRRCELDEEGIAYWEPPTYIRCVSIDYRNIQMMTREHLAKAQRGLPGEGVSEVIQTLVEISQDGTSYSGDLLSTIDVLRNMTEIFRRAYYSPTPGDVQNFVQILSNLLAEENRDKWEEAQLAGPNAKELFRLVEDFVDVIGFRMKDLRDAYQVTDNLVLSIHKLPASGATDISFPMKGWRATGDWAKVPEDRVTVSKSVFSTGLTEADEASVFVVGTVLYRNLGSFLALQRNTTVLNSKVISVTVKPPPRSLRTPLEIEFAHMYNGTTNQTCILWDETDVPSSSAPPQLGPWSWRGCRTVPLDALRTRCLCDRLSTFAILAQLSADANMEKATLPSVTLIVGCGVSSLTLLMLVIIYVSVWRYIRSERSVILINFCLSIISSNALILIGQTQTRNKVVCTLVAAFLHFFFLSSFCWVLTEAWQSYMAVTGHLRNRLIRKRFLCLGWGLPALVVAISVGFTKAKGYSTMNYCWLSLEGGLLYAFVGPAAAVVLVNMVIGILVFNKLVSKDGITDKKLKERAGASLWSSCVVLPLLALTWMSAVLAVTDRRSALFQILFAVFDSLEGFVIVMVHCILRREVQDAVKCRVVDRQEEGNGDSGGSFQNGHAQLMTDFEKDVDLACRSVLNKDIAACRTATITGTLKRPSLPEEEKLKLAHAKGPPTNFNSLPANVSKLHLHGSPRYPGGPLPDFPNHSLTLKRDKAPKSSFVGDGDIFKKLDSELSRAQEKALDTSYVILPTATATLRPKPKEEPKYSIHIDQMPQTRLIHLSTAPEASLPARSPPSRQPPSGGPPEAPPAQPPPPPPPPPPPPQQPLPPPPNLEPAPPSLGDPGEPAAHPGPSTGPSTKNENVATLSVSSLERRKSRYAELDFEKIMHTRKRHQDMFQDLNRKLQHAAEKDKEVLGPDSKPEKQQTPNKRPWESLRKAHGTPTWVKKELEPLQPSPLELRSVEWERSGATIPLVGQDIIDLQTEV

SEQ ID NO: 242 - protein, 1584 aa, Homo sapiens
MENTGWMGKGHRMTPACPLLLSVILSLRLATAFDPAPSACSALASGVLYGAFSLQDLFPTIASGCSWTLENPDPTKYSLYLRFNRQEQVCAHFAPRLLPLDHYLVNFTCLRPSPEEAVAQAESEVGRPEEEEAEAAAGLELCSGSGPFTFLHFDKNFVQLCLSAEPSEAPRLLAPAALAFRFVEVLLINNNNSSQFTCGVLCRWSEECGRAAGRACGFAQPGCSCPGEAGAGSTTTTSPGPPAAHTLSNALVPGGPAPPAEADLHSGSSNDLFTTEMRYGEEPEEEPKVKTQWPRSADEPGLYMAQTGDPAAEEWSPWSVCSLTCGQGLQVRTRSCVSSPYGTLCSGPLRETRPCNNSATCPVHGVWEEWGSWSLCSRSCGRGSRSRMRTCVPPQHGGKACEGPELQTKLCSMAACPVEGQWLEWGPWGPCSTSCANGTQQRSRKCSVAGPAWATCTGALTDTRECSNLECPATDSKWGPWNAWSLCSKTCDTGWQRRFRMCQATGTQGYPCEGTGEEVKPCSEKRCPAFHEMCRDEYVMLMTWKKAAAGEIIYNKCPPNASGSASRRCLLSAQGVAYWGLPSFARCISHEYRYLYLSLREHLAKGQRMLAGEGMSQVVRSLQELLARRTYYSGDLLFSVDILRNVTDTFKRATYVPSADDVQRFFQVVSFMVDAENKEKWDDAQQVSPGSVHLLRVVEDFIHLVGDALKAFQSSLIVTDNLVISIQREPVSAVSSDITFPMRGRRGMKDWVRHSEDRLFLPKEVLSLSSPGKPATSGAAGSPGRGRGPGTVPPGPGHSHQRLLPADPDESSYFVIGAVLYRTLGLILPPPRPPLAVTSRVMTVTVRPPTQPPAEPLITVELSYIINGTTDPHCASWDYSRADASSGDWDTENCQTLETQAAHTRCQCQHLSTFAVLAQPPKDLTLELAGSPSVPLVIGCAVSCMALLTLLAIYAAFWRFIKSERSIILLNFCLSILASNILILVGQSRVLSKGVCTMTAAFLHFFFLSSFCWVLTEAWQSYLAVIGRMRTRLVRKRFLCLGWGLPALVVAVSVGFTRTKGYGTSSYCWLSLEGGLLYAFVGPAAVIVLVNMLIGIIVFNKLMARDGISDKSKKQRAGSERCPWASLLLPCSACGAVPSPLLSSASARNAMASLWSSCVVLPLLALTWMSAVLAMTDRRSVLFQALFAVFNSAQGFVITAVHCFLRREVQDVVKCQMGVCRADESEDSPDSCKNGQLQILSDFEKDVDLACQTVLFKEVNTCNPSTITGTLSRLSLDEDEEPKSCLVGPEGSLSFSPLPGNILVPMAASPGLGEPPPPQEANPVYMCGEGGLRQLDLTWLRPTEPGSEGDYMVLPRRTLSLQPGGGGGGGEDAPRARPEGTPRRAAKTVAHTEGYPSFLSVDHSGLGLGPAYGSLQNPYGMTFQPPPPTPSARQVPEPGERSRTMPRTVPGSTMKMGSLERKKLRYSDLDFEVMHTRKRHSELYHELNQKFHTFDRYRSQSTAKREKRWSVSSGGAAERSVCTDKPSPGERPSLSQHRRHQSWSTFKSMTLGSLPPKPRERLTLHRAAAWEPTEPPDGDFQTEV

SEQ ID NO: 243 - protein, 1522 aa, Homo sapiens
MKAVRNLLIYIFSTYLLVMFGFNAAQDFWCSTLVKGVIYGSYSVSEMFPKNFTNCTWTLENPDPTKYSIYLKFSKKDLSCSNFSLLAYQFDHFSHEKIKDLLRKNHSIMQLCNSKNAFVFLQYDKNFIQIRRVFPTNFPGLQKKGEEDQKSFFEFLVLNKVSPSQFGCHVLCTWLESCLKSENGRTESCGIMYTKCTCPQHLGEWGIDDQSLILLNNVVLPLNEQTEGCLTQELQTTQVCNLTREAKRPPKEEFGMMGDHTIKSQRPRSVHEKRVPQEQADAAKFMAQTGESGVEEWSQWSTCSVTCGQGSQVRTRTCVSPYGTHCSGPLRESRVCNNTALCPVHGVWEEWSPWSLCSFTCGRGQRTRTRSCTPPQYGGRPCEGPETHHKPCNIALCPVDGQWQEWSSWSQCSVTCSNGTQQRSRQCTAAAHGGSECRGPWAESRECYNPECTANGQWNQWGHWSGCSKSCDGGWERRIRTCQGAVITGQQCEGTGEEVRRCNEQRCPAPYEICPEDYLMSMVWKRTPAGDLAFNQCPLNATGTTSRRCSLSLHGVAFWEQPSFARCISNEYRHLQHSIKEHLAKGQRMLAGDGMSQVTKTLLDLTQRKNFYAGDLLMSVEILRNVTDTFKRASYIPASDGVQNFFQIVSNLLDEENKEKWEDAQQIYPGSIELMQVIEDFIHIVGMGMMDFQNSYLMTGNVVASIQKLPAASVLTDINFPMKGRKGMVDWARNSEDRVVIPKSIFTPVSSKELDESSVFVLGAVLYKNLDLILPTLRNYTVINSKIIVVTIRPEPKTTDSFLEIELAHLANGTLNPYCVLWDDSKTNESLGTWSTQGCKTVLTDASHTKCLCDRLSTFAILAQQPREIIMESSGTPSVTLIVGSGLSCLALITLAVVYAALWRYIRSERSIILINFCLSIISSNILILVGQTQTHNKSICTTTTAFLHFFFLASFCWVLTEAWQSYMAVTGKIRTRLIRKRFLCLGWGLPALVVATSVGFTRTKGYGTDHYCWLSLEGGLLYAFVGPAAAVVLVNMVIGILVFNKLVSRDGILDKKLKHRAGQMSEPHSGLTLKCAKCGVVSTTALSATTASNAMASLWSSCVVLPLLALTWMSAVLAMTDKRSILFQILFAVFDSLQGFVIVMVHCILRREVQDAFRCRLRNCQDPINADSSSSFPNGHAQIMTDFEKDVDIACRSVLHKDIGPCRAATITGTLSRISLNDDEEEKGTNPEGLSYSTLPGNVISKVIIQQPTGLHMPMSMNELSNPCLKKENSELRRTVYLCTDDNLRGADMDIVHPQERMMESDYIVMPRSSVNNQPSMKEESKMNIGMETLPHERLLHYKVNPEFNMNPPVMDQFNMNLEQHLAPQEHMQNLPFEPRTAVKNFMASELDDNAGLSRSETGSTISMSSLERRKSRYSDLDFEKVMHTRKRHMELFQELNQKFQTLDRFRDIPNTSSMENPAPNKNPWDTFKNPSEYPHYTTINVLDTEAKDALELRPAEWEKCLNLPLDVQEGDFQTEV

SEQ ID NO: 244 - protein, 3019 aa, Homo sapiens
MAPPPPPVLPVLLLLAAAAALPAMGLRAAAWEPRVPGGTRAFALRPGCTYAVGAACTPRAPRELLDVGRDGRLAGRRRVSGAGRPLPLQVRLVARSAPTALSRRLRARTHLPGCGARARLCGTGARLCGALCFPVPGGCAAAQHSALAAPTTLPACRCPPRPRPRCPGRPICLPPGGSVRLRLLCALRRAAGAVRVGLALEAATAGTPSASPSPSPPLPPNLPEARAGPARRARRGTSGRGSLKFPMPNYQVALFENEPAGTLILQLHAHYTIEGEEERVSYYMEGLFDERSRGYFRIDSATGAVSTDSVLDRETKETHVLRVKAVDYSTPPRSATTYITVLVKDTNDHSPVFEQSEYRERVRENLEVGYEVLTIRASDRDSPINANLRYRVLGGAWDVFQLNESSGVVSTRAVLDREEAAEYQLLVEANDQGRNPGPLSATATVYIEVEDENDNYPQFSEQNYVVQVPEDVGLNTAVLRVQATDRDQGQNAAIHYSILSGNVAGQFYLHSLSGILDVINPLDFEDVQKYSLSIKAQDGGRPPLINSSGVVSVQVLDVNDNEPIFVSSPFQATVLENVPLGYPVVHIQAVDADSGENARLHYRLVDTASTFLGGGSAGPKNPAPTPDFPFQIHNSSGWITVCAELDREEVEHYSFGVEAVDHGSPPMSSSTSVSITVLDVNDNDPVFTQPTYELRLNEDAAVGSSVLTLQARDRDANSVITYQLTGGNTRNRFALSSQRGGGLITLALPLDYKQEQQYVLAVTASDGTRSHTAHVLINVTDANTHRPVFQSSHYTVSVSEDRPVGTSIATLSANDEDTGENARITYVIQDPVPQFRIDPDSGTMYTMMELDYENQVAYTLTIMAQDNGIPQKSDTTTLEILILDANDNAPQFLWDFYQGSIFEDAPPSTSILQVSATDRDSGPNGRLLYTFQGGDDGDGDFYIEPTSGVIRTQRRLDRENVAVYNLWALAVDRGSPTPLSASVEIQVTILDINDNAPMFEKDELELFVEENNPVGSVVAKIRANDPDEGPNAQIMYQIVEGDMRHFFQLDLLNGDLRAMVELDFEVRREYVLVVQATSAPLVSRATVHILLVDQNDNPPVLPDFQILFNNYVTNKSNSFPTGVIGCIPAHDPDVSDSLNYTFVQGNELRLLLLDPATGELQLSRDLDNNRPLEALMEVSVSDGIHSVTAFCTLRVTIITDDMLTNSITVRLENMSQEKFLSPLLALFVEGVAAVLSTTKDDVFVFNVQNDTDVSSNILNVTFSALLPGGVRGQFFPSEDLQEQIYLNRTLLTTISTQRVLPFDDNICLREPCENYMKCVSVLRFDSSAPFLSSTTVLFRPIHPINGLRCRCPPGFTGDYCETEIDLCYSDPCGANGRCRSREGGYTCECFEDFTGEHCEVDARSGRCANGVCKNGGTCVNLLIGGFHCVCPPGEYERPYCEVTTRSFPPQSFVTFRGLRQRFHFTISLTFATQERNGLLLYNGRFNEKHDFIALEIVDEQVQLTFSAGETTTTVAPKVPSGVSDGRWHSVQVQYYNKPNIGHLGLPHGPSGEKMAVVTVDDCDTTMAVRFGKDIGNYSCAAQGTQTGSKKSLDLTGPLLLGGVPNLPEDFPVHNRQFVGCMRNLSVDGKNVDMAGFIANNGTREGCAARRNFCDGRRCQNGGTCVNRWNMYLCECPLRFGGKNCEQAMPHPQLFSGESVVSWSDLNIIISVPWYLGLMFRTRKEDSVLMEATSGGPTSFRLQILNNYLQFEVSHGPSDVESVMLSGLRVTDGEWHHLLIELKNVKEDSEMKHLVTMTLDYGMDQNKADIGGMLPGLTVRSVVVGGASEDKVSVRRGFRGCMQGVRMGGTPTNVATLNMNNALKVRVKDGCDVDDPCTSSPCPPNSRCHDAWEDYSCVCDKGYLGINCVDACHLNPCENMGACVRSPGSPQGYVCECGPSHYGPYCENKLDLPCPRGWWGNPVCGPCHCAVSKGFDPDCNKTNGQCQCKENYYKLLAQDTCLPCDCFPHGSHSRTCDMATGQCACKPGVIGRQCNRCDNPFAEVTTLGCEVIYNGCPKAFEAGIWWPQTKFGQPAAVPCPKGSVGNAVRHCSGEKGWLPPELFNCTTISFVDLRAMNEKLSRNETQVDGARALQLVRALRSATQHTGTLFGNDVRTAYQLLGHVLQHESWQQGFDLAATQDADFHEDVIHSGSALLAPATRAAWEQIQRSEGGTAQLLRRLEGYFSNVARNVRRTYLRPFVIVTANMILAVDIFDKFNFTGARVPRFDTIHEEFPRELESSVSFPADFFRPPEEKEGPLLRPAGRRTTPQTTRPGPGTEREAPISRRRRHPDDAGQFAVALVIIYRTLGQLLPERYDPDRRSLRLPHRPIINTPMVSTLVYSEGAPLPRPLERPVLVEFALLEVEERTKPVCVFWNHSLAVGGTGGWSARGCELLSRNRTHVACQCSHTASFAVLMDISRRENGEVLPLKIVTYAAVSLSLAALLVAFVLLSLVRMLRSNLHSIHKHLAVALFLSQLVFVIGINQTENPFLCTVVAILLHYIYMSTFAWTLVESLHVYRMLTEVRNIDTGPMRFYYVVGWGIPAIVTGLAVGLDPQGYGNPDFCWLSLQDTLIWSFAGPIGAVIIINTVTSVLSAKVSCQRKHHYYGKKGIVSLLRTAFLLLLLISATWLLGLLAVNRDALSFHYLFAIFSGLQGPFVLLFHCVLNQEVRKHLKGVLGGRKLHLEDSATTRATLLTRSLNCNTTFGDGPDMLRTDLGESTASLDSIVRDEGIQKLGVSSGLVRGSHGEPDASLMPRSCKDPPGHDSDSDSELSLDEQSSSYASSHSSDSEDDGVGAEEKWDPARGAVHSTPKGDAVANHVPAGWPDQSLAESDSEDPSGKPRLKVETKVSVELHREEQGSHRGEYPPDQESGGAARLASSQPPEQRKGILKNKVTYPPPLTLTEQTLKGRLREKLADCEQSPTSSRTSSLGSGGPDCAITVKSPGREPGRDHLNGVAMNVRTGSAQADGSDSEGSNETSI

SEQ ID NO: 245 - protein, 2923 aa, Homo sapiens
MRSPATGVPLPTPPPPLLLLLLLLLPPPLLGDQVGPCRSLGSRGRGSSGACAPMGWLCPSSASNLWLYTSRCRDAGTELTGHLVPHHDGLRVWCPESEAHIPLPPAPEGCPWSCRLLGIGGHLSPQGKLTLPEEHPCLKAPRLRCQSCKLAQAPGLRAGERSPEESLGGRRKRNVNTAPQFQPPSYQATVPENQPAGTPVASLRAIDPDEGEAGRLEYTMDALFDSRSNQFFSLDPVTGAVTTAEELDRETKSTHVFRVTAQDHGMPRRSALATLTILVTDTNDHDPVFEQQEYKESLRENLEVGYEVLTVRATDGDAPPNANILYRLLEGSGGSPSEVFEIDPRSGVIRTRGPVDREEVESYQLTVEASDQGRDPGPRSTTAAVFLSVEDDNDNAPQFSEKRYVVQVREDVTPGAPVLRVTASDRDKGSNAVVHYSIMSGNARGQFYLDAQTGALDVVSPLDYETTKEYTLRVRAQDGGRPPLSNVSGLVTVQVLDINDNAPIFVSTPFQATVLESVPLGYLVLHVQAIDADAGDNARLEYRLAGVGHDFPFTINNGTGWISVAAELDREEVDFYSFGVEARDHGTPALTASASVSVTVLDVNDNNPTFTQPEYTVRLNEDAAVGTSVVTVSAVDRDAHSVITYQITSGNTRNRFSITSQSGGGLVSLALPLDYKLERQYVLAVTASDGTRQDTAQIVVNVTDANTHRPVFQSSHYTVNVNEDRPAGTTVVLISATDEDTGENARITYFMEDSIPQFRIDADTGAVTTQAELDYEDQVSYTLAITARDNGIPQKSDTTYLEILVNDVNDNAPQFLRDSYQGSVYEDVPPFTSVLQISATDRDSGLNGRVFYTFQGGDDGDGDFIVESTSGIVRTLRRLDRENVAQYVLRAYAVDKGMPPARTPMEVTVTVLDVNDNPPVFEQDEFDVFVEENSPIGLAVARVTATDPDEGTNAQIMYQIVEGNIPEVFQLDIFSGELTALVDLDYEDRPEYVLVIQATSAPLVSRATVHVRLLDRNDNPPVLGNFEILFNNYVTNRSSSFPGGAIGRVPAHDPDISDSLTYSFERGNELSLVLLNASTGELKLSRALDNNRPLEAIMSVLVSDGVHSVTAQCALRVTIITDEMLTHSITLRLEDMSPERFLSPLLGLFIQAVAATLATPPDHVVVFNVQRDTDAPGGHILNVSLSVGQPPGPGGGPPFLPSEDLQERLYLNRSLLTAISAQRVLPFDDNICLREPCENYMRCVSVLRFDSSAPFIASSSVLFRPIHPVGGLRCRCPPGFTGDYCETEVDLCYSRPCGPHGRCRSREGGYTCLCRDGYTGEHCEVSARSGRCTPGVCKNGGTCVNLLVGGFKCDCPSGDFEKPYCQVTTRSFPAHSFITFRGLRQRFHFTLALSFATKERDGLLLYNGRFNEKHDFVALEVIQEQVQLTFSAGESTTTVSPFVPGGVSDGQWHTVQLKYYNKPLLGQTGLPQGPSEQKVAVVTVDGCDTGVALRFGSVLGNYSCAAQGTQGGSKKSLDLTGPLLLGGVPDLPESFPVRMRQFVGCMRNLQVDSRHIDMADFIANNGTVPGCPAKKNVCDSNTCHNGGTCVNQWDAFSCECPLGFGGKSCAQEMANPQHFLGSSLVAWHGLSLPISQPWYLSLMFRTRQADGVLLQAITRGRSTITLQLREGHVMLSVEGTGLQASSLRLEPGRANDGDWHHAQLALGASGGPGHAILSFDYGQQRAEGNLGPRLHGLHLSNITVGGIPGPAGGVARGFRGCLQGVRVSDTPEGVNSLDPSHGESINVEQGCSLPDPCDSNPCPANSYCSNDWDSYSCSCDPGYYGDNCTNVCDLNPCEHQSVCTRKPSAPHGYTCECPPNYLGPYCETRIDQPCPRGWWGHPTCGPCNCDVSKGFDPDCNKTSGECHCKENHYRPPGSPTCLLCDCYPTGSLSRVCDPEDGQCPCKPGVIGRQCDRCDNPFAEVTTNGCEVNYDSCPRAIEAGIWWPRTRFGLPAAAPCPKGSFGTAVRHCDEHRGWLPPNLFNCTSITFSELKGFAERLQRNESGLDSGRSQQLALLLRNATQHTAGYFGSDVKVAYQLATRLLAHESTQRGFGLSATQDVHFTENLLRVGSALLDTANKRHWELIQQTEGGTAWLLQHYEAYASALAQNMRHTYLSPFTIVTPNIVISVVRLDKGNFAGAKLPRYEALRGEQPPDLETTVILPESVFRETPPVVRPAGPGEAQEPEELARRQRRHPELSQGEAVASVIIYRTLAGLLPHNYDPDKRSLRVPKRPIINTPVVSISVHDDEELLPRALDKPVTVQFRLLETEERTKPICVFWNHSILVSGTGGWSARGCEVVFRNESHVSCQCNHMTSFAVLMDVSRRENGEILPLKTLTYVALGVTLAALLLTFFFLTLLRILRSNQHGIRRNLTAALGLAQLVFLLGINQADLPFACTVIAILLHFLYLCTFSWALLEALHLYRALTEVRDVNTGPMRFYYMLGWGVPAFITGLAVGLDPEGYGNPDFCWLSIYDTLIWSFAGPVAFAVSMSVFLYILAARASCAAQRQGFEKKGPVSGLQPSFAVLLLLSATWLLALLSVNSDTLLFHYLFATCNCIQGPFIFLSYVVLSKEVRKALKLACSRKPSPDPALTTKSTLTSSYNCPSPYADGRLYQPYGDSAGSLHSTSRSGKSQPSYIPFLLREESALNPGQGPPGLGDPGSLFLEGQDQQHDPDTDSDSDLSLEDDQSGSYASTHSSDSEEEEEEEEEEAAFPGEQGWDSLLGPGAERLPLHSTPKDGGPGPGKAPWPGDFGTTAKESSGNGAPEERLRENGDALSREGSLGPLPGSSAQPHKGILKKKCLPTISEKSSLLRLPLEQCTGSSRGSSASEGSRGGPPPRPPPRQSLQEQLNGVMPIAMSIKAGTVDEDSSGSEFLFFNFLH

SEQ ID NO: 246 - protein, 3312 aa, Homo sapiens
MMARRPPWRGLGGRSTPILLLLLLSLFPLSQEELGGGGHQGWDPGLAATTGPRAHIGGGALALCPESSGVREDGGPGLGVREPIFVGLRGRRQSARNSRGPPEQPNEELGIEHGVQPLGSRERETGQGPGSVLYWRPEVSSCGRTGPLQRGSLSPGALSSGVPGSGNSSPLPSDFLIRHHGPKPVSSQRNAGTGSRKRVGTARCCGELWATGSKGQGERATTSGAERTAPRRNCLPGASGSGPELDSAPRTARTAPASGSAPRESRTAPEPAPKRMRSRGLFRCRFLPQRPGPRPPGLPARPEARKVTSANRARFRRAANRHPQFPQYNYQTLVPENEAAGTAVLRVVAQDPDAGEAGRLVYSLAALMNSRSLELFSIDPQSGLIRTAAALDRESMERHYLRVTAQDHGSPRLSATTMVAVTVADRNDHSPVFEQAQYRETLRENVEEGYPILQLRATDGDAPPNANLRYRFVGPPAARAAAAAAFEIDPRSGLISTSGRVDREHMESYELVVEASDQGQEPGPRSATVRVHITVLDENDNAPQFSEKRYVAQVREDVRPHTVVLRVTATDRDKDANGLVHYNIISGNSRGHFAIDSLTGEIQVVAPLDFEAEREYALRIRAQDAGRPPLSNNTGLASIQVVDINDHIPIFVSTPFQVSVLENAPLGHSVIHIQAVDADHGENARLEYSLTGVAPDTPFVINSATGWVSVSGPLDRESVEHYFFGVEARDHGSPPLSASASVTVTVLDVNDNRPEFTMKEYHLRLNEDAAVGTSVVSVTAVDRDANSAISYQITGGNTRNRFAISTQGGVGLVTLALPLDYKQERYFKLVLTASDRALHDHCYVHINITDANTHRPVFQSAHYSVSVNEDRPMGSTIVVISASDDDVGENARITYLLEDNLPQFRIDADSGAITLQAPLDYEDQVTYTLAITARDNGIPQKADTTYVEVMVNDVNDNAPQFVASHYTGLVSEDAPPFTSVLQISATDRDAHANGRVQYTFQNGEDGDGDFTIEPTSGIVRTVRRLDREAVSVYELTAYAVDRGVPPLRTPVSIQVMVQDVNDNAPVFPAEEFEVRVKENSIVGSVVAQITAVDPDEGPNAHIMYQIVEGNIPELFQMDIFSGELTALIDLDYEARQEYVIVVQATSAPLVSRATVHVRLVDQNDNSPVLNNFQILFNNYVSNRSDTFPSGIIGRIPAYDPDVSDHLFYSFERGNELQLLVVNQTSGELRLSRKLDNNRPLVASMLVTVTDGLHSVTAQCVLRVVIITEELLANSLTVRLENMWQERFLSPLLGRFLEGVAAVLATPAEDVFIFNIQNDTDVGGTVLNVSFSALAPRGAGAGAAGPWFSSEELQEQLYVRRAALAARSLLDVLPFDDNVCLREPCENYMKCVSVLRFDSSAPFLASASTLFRPIQPIAGLRCRCPPGFTGDFCETELDLCYSNPCRNGGACARREGGYTCVCRPRFTGEDCELDTEAGRCVPGVCRNGGTCTDAPNGGFRCQCPAGGAFEGPRCEVAARSFPPSSFVMFRGLRQRFHLTLSLSFATVQQSGLLFYNGRLNEKHDFLALELVAGQVRLTYSTGESNTVVSPTVPGGLSDGQWHTVHLRYYNKPRTDALGGAQGPSKDKVAVLSVDDCDVAVALQFGAEIGNYSCAAAGVQTSSKKSLDLTGPLLLGGVPNLPENFPVSHKDFIGCMRDLHIDGRRVDMAAFVANNGTMAGCQAKLHFCDSGPCKNSGFCSERWGSFSCDCPVGFGGKDCQLTMAHPHHFRGNGTLSWNFGSDMAVSVPWYLGLAFRTRATQGVLMQVQAGPHSTLLCQLDRGLLSVTVTRGSGRASHLLLDQVTVSDGRWHDLRLELQEEPGGRRGHHVLMVSLDFSLFQDTMAVGSELQGLKVKQLHVGGLPPGSAEEAPQGLVGCIQGVWLGSTPSGSPALLPPSHRVNAEPGCVVTNACASGPCPPHADCRDLWQTFSCTCQPGYYGPGCVDACLLNPCQNQGSCRHLPGAPHGYTCDCVGGYFGHHCEHRMDQQCPRGWWGSPTCGPCNCDVHKGFDPNCNKTNGQCHCKEFHYRPRGSDSCLPCDCYPVGSTSRSCAPHSGQCPCRPGALGRQCNSCDSPFAEVTASGCRVLYDACPKSLRSGVWWPQTKFGVLATVPCPRGALGAAVRLCDEAQGWLEPDLFNCTSPAFRELSLLLDGLELNKTALDTMEAKKLAQRLREVTGHTDHYFSQDVRVTARLLAHLLAFESHQQGFGLTATQDAHFNENLLWAGSALLAPETGDLWAALGQRAPGGSPGSAGLVRHLEEYAATLARNMELTYLNPMGLVTPNIMLSIDRMEHPSSPRGARRYPRYHSNLFRGQDAWDPHTHVLLPSQSPRPSPSEVLPTSSSIENSTTSSVVPPPAPPEPEPGISIIILLVYRTLGGLLPAQFQAERRGARLPQNPVMNSPVVSVAVFHGRNFLRGILESPISLEFRLLQTANRSKAICVQWDPPGLAEQHGVWTARDCELVHRNGSHARCRCSRTGTFGVLMDASPRERLEGDLELLAVFTHVVVAVSVAALVLTAAILLSLRSLKSNVRGIHANVAAALGVAELLFLLGIHRTHNQLVCTAVAILLHYFFLSTFAWLFVQGLHLYRMQVEPRNVDRGAMRFYHALGWGVPAVLLGLAVGLDPEGYGNPDFCWISVHEPLIWSFAGPVVLVIVMNGTMFLLAARTSCSTGQREAKKTSALTLRSSFLLLLLVSASWLFGLLAVNHSILAFHYLHAGLCGLQGLAVLLLFCVLNADARAAWMPACLGRKAAPEEARPAPGLGPGAYNNTALFEESGLIRITLGASTVSSVSSARSGRTQDQDSQRGRSYLRDNVLVRHGSAADHTDHSLQAHAGPTDLDVAMFHRDAGADSDSDSDLSLEEERSLSIPSSESEDNGRTRGRFQRPLCRAAQSERLLTHPKDVDGNDLLSYWPALGECEAAPCALQTWGSERRLGLDTSKDAANNNQPDPALTSGDETSLGRAQRQRKGILKNRLQYPLVPQTRGAPELSWCRAATLGHRAVPAASYGRIYAGGGTGSLSQPASRYSSREQLDLLLRRQLSRERLEEAPAPVLRPLSRPGSQECMDAAPGRLEPKDRGSTLPRRQPPRDYPGAMAGRFGSRDALDLGAPREWLSTLPPPRRTRDLDPQPPPLPLSPQRQLSRDPLLPSRPLDSLSRSSNSREQLDQVPSRHPSREALGPLPQLLRAREDSVSGPSHGPSTEQLDILSSILASFNSSALSSVQSSSTPLGPHTTATPSATASVLGPSTPRSATSHSISELSPDSEVPRSEGHS

SEQ ID NO: 247 - protein, 906 aa, Homo sapiens
MEKLLRLCCWYSWLLLFYYNFQVRGVYSRSQDHPGFQVLASASHYWPLENVDGIHELQDTTGASRTHKLTVLPSRNATFVYSNDSAYSNLSATVDIVEGKVNKGIYLKEEKGVTLLYYGRYNSSCISKPEQCGPEGVTFSFFWKTQGEQSRPIPSAYGGQVISNGFKVCSSGGRGSVELYTRDNSMTWEASFSPPGPYWTHVLFTWKSKEGLKVYVNGTLSTSDPSGKVSRDYGESNVNLVIGSEQDQAKCYENGAFDEFIIWERALTPDEIAMYFTAAIGKHALLSSTLPSLFMTSTASPVMPTDAYHPIITNLTEERKTFQSPGVILSYLQNVSLSLPSKSLSEQTALNLTKTFLKAVGEILLLPGWIALSEDSAVVLSLIDTIDTVMGHVSSNLHGSTPQVTVEGSSAMAEFSVAKILPKTVNSSHYRFPAHGQSFIQIPHEAFHRHAWSTVVGLLYHSMHYYLNNIWPAHTKIAEAMHHQDCLLFATSHLISLEVSPPPTLSQNLSGSPLITVHLKHRLTRKQHSEATNSSNRVFVYCAFLDFSSGEGVWSNHGCALTRGNLTYSVCRCTHLTNFAILMQVVPLELARGHQVALSSISYVGCSLSVLCLVATLVTFAVLSSVSTIRNQRYHIHANLSFAVLVAQVLLLISFRLEPGTTPCQVMAVLLHYFFLSAFAWMLVEGLHLYSMVIKVFGSEDSKHRYYYGMGWGFPLLICIISLSFAMDSYGTSNNCWLSLASGAIWAFVAPALFVIVVNIGILIAVTRVISQISADNYKIHGDPSAFKLTAKAVAVLLPILGTSWVFGVLAVNGCAVVFQYMFATLNSLQGLFIFLFHCLLNSEVRAAFKHKTKVWSLTSSSARTSNAKPFHSDLMNGTRPGMASTKLSPWDKSSHSAHRVDLSAV

SEQ ID NO: 248 - protein, 982 aa, Homo sapiens
MAPWCYCFLCLLIRSLSGTPSNSPGESRNPWAPAPVAAGEVVKTAGGVCKFSGQRLSWWQAQESCEQQFGHLALQPPDGVLASRLRDPVWVGQREAPLRRPPQRRARTTAVLVFDERTADRAARLRSPLPELAALTACTHVQWDCASPDPAALFSVAAPALPNALQLRAFAEPGGVVRAALVVRGQHAPFLAAFRADGRWHHVCATWEQRGGRWALFSDGRRRAGARGLGAGHPVPSGGILVLGQDQDSLGGGFSVRHALSGNLTDFHLWARALSPAQLHRARACAPPSEGLLFRWDPGALDVTPSLLPTVWVRLLCPVPSEECPTWNPGPRSEGSELCLEPQPFLCCYRTEPYRRLQDAQSWPGQDVISRVNALANDIVLLPDPLSEVHGALSPAEASSFLGLLEHVLAMEMAPLGPAALLAVVRFLKRVVALGAGDPELLLTGPWEQLSQGVVSVASLVLEEQVADTWLSLREVIGGPMALVASVQRLAPLLSTSMTSERPRMRIQHRHAGLEVRSLRLREASTRGCLFTMPGGRPEGPGHIHIPASEVRRLLRKGLSGVTVIHSWFTSRVFQHTLEGPDLEPQAPASSEEANRVQRFLSTQVGSAIISSEVWDVTGEVNVAMTFHLQHRAQSPLFPPHPPSPYTGGAWATTGCSVAALYLDSTACFCNHSTSFAILLQIYEVQRGPEEESLLRTLSFVGCGVSFCALTTTFLLFLVAGVPKSERTTVHKNLTFSLASAEGFLMTSEWAKANEVACVAVTVAMHFLFLVAFSWMLVEGLLLWRKVVAVSMHPGPGMRLYHATGWGVPVGIVAVTLAMLPHDYVAPGHCWLNVHTNAIWAFVGPVLFVLTANTCILARVVMITVSSARRRARMLSPQPCLQQQIWTQIWATVKPVLVLLPVLGLTWLAGILVHLSPAWAYAAVGLNSIQGLYIFLVYAACNEEVRSALQRMAEKKVAEGPMALELPQHSPPLQTRRDRLWN

SEQ ID NO: 249 - protein, 867 aa, Homo sapiens
MRGFNLLLFWGCCVMHSWEGHIRPTRKPNTKGNNCRDSTLCPAYATCTNTVDSYYCACKQGFLSSNGQNHFKDPGVRCKDINECLTSSVCPEHSDCVNSMGSYSCSCQVGFISRNSTCEDVDECADPRACPEHATCNNTVGNYSCFCNPGFESSSGHLSFQGLKASCEDIDECTEMCPINSTCTNTPGSYFCTCHPGFAPSNGQLNFTDQGVECRDIDECRQDPSTCGPNSICTNALGSYSCGCIAGFHPNPEGSQKDGNFSCQRVLFKCKEDVIPDNKQIQQCQEGTAVKPAYVSFCAQINNIFSVLDKVCENKTTVVSLKNTTESFVPVLKQISTWTKFTKEETSSLATVFLESVESMTLASFWKPSANITPAVRTEYLDIESKVINKECSEENVTLDLVAKGDKMKIGCSTIEESESTETTGVAFVSFVGMESVLNERFFKDHQAPLTTSEIKLKMNSRVVGGIMTGEKKDGFSDPIIYTLENIQPKQKFERPICVSWSTDVKGGRWTSFGCVILEASETYTICSCNQMANLAVIMASGELTMDFSLYIISHVGIIISLVCLVLAIATFLLCRSIRNHNTYLHLHLCVCLLLAKTLFLAGIHKTDNKMGCAIIAGFLHYLFLACFFWMLVEAVILFLMVRNLKVVNYFSSRNIKMLHICAFGYGLPMLVVVISASVQPQGYGMHNRCWLNTETGFIWSFLGPVCTVIVVSKYYNSLAKCVLKEEQGDLRDLEFPGTCAAERINSLLLTWTLWILRQRLSSVNAEVSTLKDTRLLTFKAFAQLFILGCSWVLGIFQIGPVAGVMAYLFTIINSLQGAFIFLIHCLLNGQVREEYKRWITGKTKPSSQSQTSRILLSSMPSASKTG

SEQ ID NO: 250 - protein, 765 aa, Homo sapiens
MGGRVFLVFLAFCVWLTLPGAETQDSRGCARWCPQDSSCVNATACRCNPGFSSFSEIITTPMETCDDINECATLSKVSCGKFSDCWNTEGSYDCVCSPGYEPVSGAKTFKNESENTCQDVDECQQNPRLCKSYGTCVNTLGSYTCQCLPGFKLKPEDPKLCTDVNECTSGQNPCHSSTHCLNNVGSYQCRCRPGWQPIPGSPNGPNNTVCEDVDECSSGQHQCDSSTVCFNTVGSYSCRCRPGWKPRHGIPNNQKDTVCEDMTFSTWTPPPGVHSQTLSRFFDKVQDLGRDYKPGLANNTIQSILQALDELLEAPGDLETLPRLQQHCVASHLLDGLEDVLRGLSKNLSNGLLNFSYPAGTELSLEVQKQVDRSVTLRQNQAVMQLDWNQAQKSGDPGPSVVGLVSIPGMGKLLAEAPLVLEPEKQMLLHETHQGLLQDGSPILLSDVISAFLSNNDTQNLSSPVTFTFSHREEDPVLTVITYMGLSVSLLCLLLAALTFLLCKAIQNTSTSLHLQLSLCLFLAHLLFLVAIDQTGHKVLCSIIAGTLHYLYLATLTWMLLEALYLFLTARNLTVVNYSSINRFMKKLMFPVGYGVPAVTVAISAASRPHLYGTPSRCWLQPEKGFIWGFLGPVCAIFSVNLVLFLVTLWILKNRLSSLNSEVSTLRNTRMLAFKATAQLFILGCTWCLGILQVGPAARVMAYLFTIINSLQGVFIFLVYCLLSQQVREQYGKWSKGIRKLKTESEMHTLSSSAKADTSKPSTVN

SEQ ID NO: 251 - protein, 600 aa, Homo sapiens
MQGPLLLPGLCFLLSLFGAVTQKTKTSCAKCPPNASCVNNTHCTCNHGYTSGSGQKLFTFPLETCNDTTSSKTTEGRKELQKIVDKFESLLTNQTLWRTEGRQEISSTATTILRDVESKVLETALKDPEQKVLKIQNDSVAIETQAITDNCSEERKTFNLNVQMNSMDIRCSDIIQGDTQGPSAIAFISYSSLGNIINATFFEEMDKKDQVYLNSQVVSAAIGPKRNVSLSKSVTLTFQHVKMTPSTKKVFCVYWKSTGQGSQWSRDGCFLIHVNKSHTMCNCSHLSSFAVLMALTSQEEDPVLTVITYVGLSVSLLCLLLAALTFLLCKAIRNTSTSLHLQLSLCLFLAHLLFLVGIDRTEPKVLCSIIAGALHYLYLAAFTWMLLEGVHLFLTARNLTVVNYSSINRLMKWIMFPVGYGVPAVTVAISAASWPHLYGTADRCWLHLDQGFMWSFLGPVCAIFSANLVLFILVFWILKRKLSSLNSEVSTIQNTRMLAFKATAQLFILGCTWCLGLLQVGPAAQVMAYLFTIINSLQGFFIFLVYCLLSQQVQKQYQKWFREIVKSKSESETYTLSSKMGPDSKPSEGDVFPGQVKRKY

SEQ ID NO: 252 - protein, 786 aa, Homo sapiens
MGGRVFLAFCVWLTLPGAETQDSRGCARWCPQNSSCVNATACRCNPGFSSFSEIITTPTETCDDINECATPSKVSCGKFSDCWNTEGSYDCVCSPGYEPVSGAKTFKNESENTCQDVDECQQNPRLCKSYGTCVNTLGSYTCQCLPGFKFIPEDPKVCTDVDECSSGQHQCDSSTVCFNTVGSYSCRCRPGWKPRHGIPNNQKDTVCEDMTFSTWTPPPGVHSQTLSRFFDKVQDLGRDSKTSSAEVTIQNVIKLVDELMEAPGDVEALAPPVRHLIATQLLSNLEDIMRILAKSLPKGPFTYISPSNTELTLMIQERGDKNVTMGQSSARMKLNWAVAAGAEDPGPAVAGILSIQNMTTLLANASLNLHSKKQAELEEIYESSIRGVQLRRLSAVNSIFLSHNNTKELNSPILFAFSHLESSDGEAGRDPPAKDVMPGPRQELLCAFWKSDSDRGGHWATEGCQVLGSKNGSTTCQCSHLSSFAILMAHYDVEDWKLTLITRVGLALSLFCLLLCILTFLLVRPIQGSRTTIHLHLCICLFVGSTIFLAGIENEGGQVGLRCRLVAGLLHYCFLAAFCWMSLEGLELYFLVVRVFQGQGLSTRWLCLIGYGVPLLIVGVSAAIYSKGYGRPRYCWLDFEQGFLWSFLGPVTFIILCNAVIFVTTVWKLTQKFSEINPDMKKLKKARALTITAIAQLFLLGCTWVFGLFIFDDRSLVLTYVFTILNCLQGAFLYLLHCLLNKKVREEYRKWACLVAGGSKYSEFTSTTSGTGHNQTRALRASESGI

SEQ ID NO: 253 - protein, 910 aa, Homo sapiens
MKVGVLWLISFFTFTDGHGGFLGKNDGIKTKKELIVNKKKHLGPVEEYQLLLQVTYRDSKEKRDLRNFLKLLKPPLLWSHGLIRIIRAKATTDCNSLNGVLQCTCEDSYTWFPPSCLDPQNCYLHTAGALPSCECHLNNLSQSVNFCERTKIWGTFKINERFTNDLLNSSSAIYSKYANGIEIQLKKAYERIQGFESVQVTQFRNGSIVAGYEVVGSSSASELLSAIEHVAEKAKTALHKLFPLEDGSFRVFGKAQCNDIVFGFGSKDDEYTLPCSSGYRGNITAKCESSGWQVIRETCVLSLLEELNKNFSMIVGNATEAAVSSFVQNLSVIIRQNPSTTVGNLASVVSILSNISSLSLASHFRVSNSTMEDVISIADNILNSASVTNWTVLLREEKYASSRLLETLENISTLVPPTALPLNFSRKFIDWKGIPVNKSQLKRGYSYQIKMCPQNTSIPIRGRVLIGSDQFQRSLPETIISMASLTLGNILPVSKNGNAQVNGPVISTVIQNYSINEVFLFFSKIESNLSQPHCVFWDFSHLQWNDAGCHLVNETQDIVTCQCTHLTSFSILMSPFVPSTIFPVVKWITYVGLGISIGSLILCLIIEALFWKQIKKSQTSHTRRICMVNIALSLLIADVWFIVGATVDTTVNPSGVCTAAVFFTHFFYLSLFFWMLMLGILLAYRIILVFHHMAQHLMMAVGFCLGYGCPLIISVITIAVTQPSNTYKRKDVCWLNWSNGSKPLLAFVVPALAIVAVNFVVVLLVLTKLWRPTVGERLSRDDKATIIRVGKSLLILTPLLGLTWGFGIGTIVDSQNLAWHVIFALLNAFQGFFILCFGILLDSKLRQLLFNKLSALSSWKQTEKQNSSDLSAKPKFSKPFNPLQNKGHYAFSHTGDSSDNIMLTQFVSNE

SEQ ID NO: 254 - protein, 1079 aa, Homo sapiens
MVCSAAPLLLLATTLPLLGSPVAQASQPVSETGVRPREGLQRRQWGPLIGRDKAWNERIDRPFPACPIPLSSSFGRWPKGQTMWAQTSTLTLTEEELGQSQAGGESGSGQLLDQENGAGESALVSVYVHLDFPDKTWPPELSRTLTLPAASASSSPRPLLTGLRLTTECNVNHKGNFYCACLSGYQWNTSICLHYPPCQSLHNHQPCGCLVFSHPEPGYCQLLPPGSPVTCLPAVPGILNLNSQLQMPGDTLSLTLHLSQEATNLSWFLRHPGSPSPILLQPGTQVSVTSSHGQAALSVSNMSHHWAGEYMSCFEAQGFKWNLYEVVRVPLKATDVARLPYQLSISCATSPGFQLSCCIPSTNLAYTAAWSPGEGSKASSFNESGSQCFVLAVQRCPMADTTYACDLQSLGLAPLRVPISITIIQDGDITCPEDASVLTWNVTKAGHVAQAPCPESKRGIVRRLCGADGVWGPVHSSCTDARLLALFTRTKLLQAGQGSPAEEVPQILAQLPGQAAEASSPSDLLTLLSTMKYVAKVVAEARIQLDRRALKNLLIATDKVLDMDTRSLWTLAQARKPWAGSTLLLAVETLACSLCPQDHPFAFSLPNVLLQSQLFGPTFPADYSISFPTRPPLQAQIPRHSLAPLVRNGTEISITSLVLRKLDHLLPSNYGQGLGDSLYATPGLVLVISIMAGDRAFSQGEVIMDFGNTDGSPHCVFWDHSLFQGRGGWSKEGCQAQVASASPTAQCLCQHLTAFSVLMSPHTVPEEPALALLTQVGLGASILALLVCLGVYWLVWRVVVRNKISYFRHAALLNMVFCLLAADTCFLGAPFLSPGPRSPLCLAAAFLCHFLYLATFFWMLAQALVLAHQLLFVFHQLAKHRVLPLMVLLGYLCPLGLAGVTLGLYLPQGQYLREGECWLDGKGGALYTFVGPVLAIIGVNGLVLAMAMLKLLRPSLSEGPPAEKRQALLGVIKALLILTPIFGLTWGLGLATLLEEVSTVPHYIFTILNTLQGVFILLFGCLMDRKIQEALRKRFCRAQAPSSTISLVSCCLQILSCASKSMSEGIPWPSSEDMGTARS

SEQ ID NO: 255 - protein, 695 aa, Homo sapiens
MKMKSQATMICCLVFFLSTECSHYRSKIHLKAGDKLQSPEGKPKTGRIQEKCEGPCISSSNCSQPCAKDFHGEIGFTCNQKKWQKSAETCTSLSVEKLFKDSTGASRLSVAAPSIPLHILDFRAPETIESVAQGIRKNCPFDYACITDMVKSSETTSGNIAFIVELLKNISTDLSDNVTREKMKSYSEVANHILDTAAISNWAFIPNKNASSDLLQSVNLFARQLHIHNNSENIVNELFIQTKGFHINHNTSEKSLNFSMSMNNTTEDILGMVQIPRQELRKLWPNASQAISIAFPTLGAILREAHLQNVSLPRQVNGLVLSVVLPERLQEIILTFEKINKTRNARAQCVGWHSKKRRWDEKACQMMLDIRNEVKCRCNYTSVVMSFSILMSSKSMTDKVLDYITCIGLSVSILSLVLCLIIEATVWSRVVVTEISYMRHVCIVNIAVSLLTANVWFIIGSHFNIKAQDYNMCVAVTFFSHFFYLSLFFWMLFKALLIIYGILVIFRRMMKSRMMVIGFAIGYGCPLIIAVTTVAITEPEKGYMRPEACWLNWDNTKALLAFAIPAFVIVAVNLIVVLVVAVNTQRPSIGSSKSQDVVIIMRISKNVAILTPLLGLTWGFGIATLIEGTSLTFHIIFALLNAFQGFFILLFGTIMDHKIRDALRMRMSSLKGKSRAAENASLGPTNGSKLMNRQG

SEQ ID NO: 256 - protein, 1346 aa, Homo sapiens
MKSPRRTTLCLMFIVIYSSKAALNWNYESTIHPLSLHEHEPAGEEALRQKRAVATKSPTAEEYTVNIEISFENASFLDPIKAYLNSLSFPIHGNNTDQITDILSINVTTVCRPAGNEIWCSCETGYGWPRERCLHNLICQERDVFLPGHHCSCLKELPPNGPFCLLQEDVTLNMRVRLNVGFQEDLMNTSSALYRSYKTDLETAFRKGYGILPGFKGVTVTGFKSGSVVVTYEVKTTPPSLELIHKANEQVVQSLNQTYKMDYNSFQAVTINESNFFVTPEIIFEGDTVSLVCEKEVLSSNVSWRYEEQQLEIQNSSRFSIYTALFNNMTSVSKLTIHNITPGDAGEYVCKLILDIFEYECKKKIDVMPIQILANEEMKVMCDNNPVSLNCCSQGNVNWSKVEWKQEGKINIPGTPETDIDSSCSRYTLKADGTQCPSGSSGTTVIYTCEFISAYGARGSANIKVTFISVANLTITPDPISVSEGQNFSIKCISDVSNYDEVYWNTSAGIKIYQRFYTTRRYLDGAESVLTVKTSTREWNGTYHCIFRYKNSYSIATKDVIVHPLPLKLNIMVDPLEATVSCSGSHHIKCCIEEDGDYKVTFHTGSSSLPAAKEVNKKQVCYKHNFNASSVSWCSKTVDVCCHFTNAANNSVWSPSMKLNLVPGENITCQDPVIGVGEPGKVIQKLCRFSNVPSSPESPIGGTITYKCVGSQWEEKRNDCISAPINSLLQMAKALIKSPSQDEMLPTYLKDLSISIDKAEHEISSSPGSLGAIINILDLLSTVPTQVNSEMMTHVLSTVNVILGKPVLNTWKVLQQQWTNQSSQLLHSVERFSQALQSGDSPPLSFSQTNVQMSSMVIKSSHPETYQQRFVFPYFDLWGNVVIDKSYLENLQSDSSIVTMAFPTLQAILAQDIQENNFAESLVMTTTVSHNTTMPFRISMTFKNNSPSGGETKCVFWNFRLANNTGGWDSSGCYVEEGDGDNVTCICDHLTSFSILMSPDSPDPSSLLGILLDIISYVGVGFSILSLAACLVVEAVVWKSVTKNRTSYMRHTCIVNIAASLLVANTWFIVVAAIQDNRYILCKTACVAATFFIHFFYLSVFFWMLTLGLMLFYRLVFILHETSRSTQKAIAFCLGYGCPLAISVITLGATQPREVYTRKNVCWLNWEDTKALLAFAIPALIIVVVNITITIVVITKILRPSIGDKPCKQEKSSLFQISKSIGVLTPLLGLTWGFGLTTVFPGTNLVFHIIFAILNVFQGLFILLFGCLWDLKVQEALLNKFSLSRWSSQHSKSTSLGSSTPVFSMSSPISRRFNNLFGKTGTYNVSTPEATSSSLENSSSASSLLN

SEQ ID NO: 257 - protein, 687 aa, Homo sapiens
MTPQSLLQTTLFLLSLLFLVQGAHGRGHREDFRFCSQRNQTHRSSLHYKPTPDLRISIENSEEALTVHAPFPAAHPASRSFPDPRGLYHFCLYWNRHAGRLHLLYGKRDFLLSDKASSLLCFQHQEESLAQGPPLLATSVTSWWSPQNISLPSAASFTFSFHSPPHTAAHNASVDMCELKRDLQLLSQFLKHPQKASRRPSAAPASQQLQSLESKLTSVRFMGDMVSFEEDRINATVWKLQPTAGLQDLHIHSRQEEEQSEIMEYSVLLPRTLFQRTKGRSGEAEKRLLLVDFSSQALFQDKNSSQVLGEKVLGIVVQNTKVANLTEPVVLTFQHQLQPKNVTLQCVFWVEDPTLSSPGHWSSAGCETVRRETQTSCFCNHLTYFAVLMVSSVEVDAVHKHYLSLLSYVGCVVSALACLVTIAAYLCSRRKPRDYTIKVHMNLLLAVFLLDTSFLLSEPVALTGSEAGCRASAIFLHFSLLTCLSWMGLEGYNLYRLVVEVFGTYVPGYLLKLSAMGWGFPIFLVTLVALVDVDNYGPIILAVHRTPEGVIYPSMCWIRDSLVSYITNLGLFSLVFLFNMAMLATMVVQILRLRPHTQKWSHVLTLLGLSLVLGLPWALIFFSFASGTFQLVVLYLFSIITSFQGFLIFIWYWSMRLQARGGPSPLKSNSDSARLPISSGSTSSSRI

SEQ ID NO: 258 - protein, 1017 aa, Homo sapiens
MVFSVRQCGHVGRTEEVLLTFKIFLVIICLHVVLVTSLEEDTDNSSLSPPPAKLSVVSFAPSSNGTPEVETTSLNDVTLSLLPSNETEKTKITIVKTFNASGVKPQRNICNLSSICNDSAFFRGEIMFQYDKESTVPQNQHITNGTLTGVLSLSELKRSELNKTLQTLSETYFIMCATAEAQSTLNCTFTIKLNNTMNACAVIAALERVKIRPMEHCCCSVRIPCPSSPEELEKLQCDLQDPIVCLADHPRGPPFSSSQSIPVVPRATVLSQVPKATSFAEPPDYSPVTHNVPSPIGEIQPLSPQPSAPIASSPAIDMPPQSETISSPMPQTHVSGTPPPVKASFSSPTVSAPANVNTTSAPPVQTDIVNTSSISDLENQVLQMEKALSLGSLEPNLAGEMINQVSRLLHSPPDMLAPLAQRLLKVVDDIGLQLNFSNTTISLTSPSLALAVIRVNASSFNTTTFVAQDPANLQVSLETQAPENSIGTITLPSSLMNNLPAHDMELASRVQFNFFETPALFQDPSLENLSLISYVISSSVANLTVRNLTRNVTVTLKHINPSQDELTVRCVFWDLGRNGGRGGWSDNGCSVKDRRLNETICTCSHLTSFGVLLDLSRTSVLPAQMMALTFITYIGCGLSSIFLSVTLVTYIAFEKIRRDYPSKILIQLCAALLLLNLVFLLDSWIALYKMQGLCISVAVFLHYFLLVSFTWMGLEAFHMYLALVKVFNTYIRKYILKFCIVGWGVPAVVVTIILTISPDNYGLGSYGKFPNGSPDDFCWINNNAVFYITVVGYFCVIFLLNVSMFIVVLVQLCRIKKKKQLGAQRKTSIQDLRSIAGLTFLLGITWGFAFFAWGPVNVTFMYLFAIFNTLQGFFIFIFYCVAKENVRKQWRRYLCCGKLRLAENSDWSKTATNGLKKQTVNQGVSSSSNSLQSSSNSTNSTTLLVNNDCSVHASGNGNASTERNGVSFSVQNGDVCLHDFTGKQHMFNEKEDSCNGKGRMALRRTSKRGSLHFIEQM

SEQ ID NO: 259 - protein, 3080 aa, Homo sapiens
MKEHIIYQKLYGLILMSSFIFLSDTLSLKGKKLDFFGRGDTYVSLIDTIPELSRFTACIDLVFMDDNSRYWMAFSYITNNALLGREDIDLGLAGDHQQLILYRLGKTFSIRHHLASFQWHTICLIWDGVKGKLELFLNKERILEVTDQPHNLTPHGTLFLGHFLKNESSEVKSMMRSFPGSLYYFQLWDHILENEEFMKCLDGNIVSWEEDVWLVNKIIPTVDRTLRCFVPENMTIQEKSTTVSQQIDMTTPSQITGVKPQNTAHSSTLLSQSIPIFATDYTTISYSNTTSPPLETMTAQKILKTLVDETATFAVDVLSTSSAISLPTQSISIDNTTNSMKKTKSPSSESTKTTKMVEAMATEIFQPPTPSNFLSTSRFTKNSVVSTTSAIKSQSAVTKTTSLFSTIESTSMSTTPCLKQKSTNTGALPISTAGQEFIESTAAGTVPWFTVEKTSPASTHVGTASSFPPEPVLISTAAPVDSVFPRNQTAFPLATTDMKIAFTVHSLTLPTRLIETTPAPRTAETELTSTNFQDVSLPRVEDAMSTSMSKETSSKTFSFLTSFSFTGTESVQTVIDAEATRTALTPEITLASTVAETMLSSTITGRVYTQNTPTADGHLLTLMSTRSASTSKAPESGPTSTTDEAAHLFSSNETIWTSRPDQALLASMNTTTILTFVPNENFTSAFHENTTYTEYLSATTNITPLKASPEGKGTTANDATTARYTTAVSKLTSPWFANFSIVSGTTSITNMPEFKLTTLLLKTIPMSTKPANELPLTPRETVVPSVDIISTLACIQPNFSTEESASETTQTEINGAIVFGGTTTPVPKSATTQRLNATVTRKEATSHYLMRKSTIAAVAEVSPFSTMLEVTDESAQRVTASVTVSSFPDIEKLSTPLDNKTATTEVRESWLLTKLVKTTPRSSYNEMTEMFNFNHTYVAHWTSETSEGISAGSPTSGSTHIFGEPLGASTTRISETSFSTTPTDRTATSLSDGILPPQPTAAHSSATPVPVTHMFSLPVNGSSVVAEETEVTMSEPSTLARAFSTSVLSDVSNLSSTTMTTALVPPLDQTASTTIVIVPTHGDLIRTTSEATVISVRKTSMAVPSLTETPFHSLRLSTPVTAKAETTLFSTSVDTVTPSTHTLVCSKPPPDNIPPASSTHVISTTSTPEATQPISQVEETSTYALSFPYTFSGGGVVASLATGTTETSVVDETTPSHISANKLTTSVNSHISSSATYRVHTPVSIQLVTSTSVLSSDKDQMTISLGKTPRTMEVTEMSPSKNSFISYSRGTPSLEMTDTGFPETTKISSHQTHSPSEIPLGTPSDGNLASSPTSGSTQITPTLTSSNTVGVHIPEMSTSLGKTALPSQALTITTFLCPEKESTSALPAYTPRTVEMIVNSTYVTHSVSYGQDTSFVDTTTSSSTRISNPMDINTTFSHLHSLRTQPEVTSVASFISESTQTFPESLSLSTAGLYNDGFTVLSDRITTAFSVPNVPTMLPRESSMATSTPIYQMSSLPVNVTAFTSKKVSDTPPIVITKSSKTMHPGCLKSPCTATSGPMSEMSSIPVNNSAFTPATVSSDTSTRVGLFSTLLSSVTPRTTMTMQTSTLDVTPVIYAGATSKNKMVSSAFTTEMIEAPSRITPTTFLSPTEPTLPFVKTVPTTIMAGIVTPFVGTTAFSPLSSKSTGAISSIPKTTFSPFLSATQQSSQADEATTLGILSGITNRSLSTVNSGTGVALTDTYSRITVPENMLSPTHADSLHTSFNIQVSPSLTSFKSASGPTKNVKTTTNCFSSNTRKMTSLLEKTSLTNYATSLNTPVSYPPWTPSSATLPSLTSFVYSPHSTEAEISTPKTSPPPTSQMVEFPVLGTRMTSSNTQPLLMTSWNIPTAEGSQFPISTTINVPTSNEMETETLHLVPGPLSTFTASQTGLVSKDVMAMSSIPMSGILPNHGLSENPSLSTSLRAITSTLADVKHTFEKMTTSVTPGTTLPSILSGATSGSVISKSPILTWLLSSLPSGSPPATVSNAPHVMTSSTVEVSKSTFLTSDMISAHPFTNLTTLPSATMSTILTRTIPTPTLGGITTGFPTSLPMSINVTDDIVYISTHPEASSRTTITANPRTVSHPSSFSRKTMSPSTTDHTLSVGAMPLPSSTITSSWNRIPTASSPSTLIIPKPTLDSLLNIMTTTSTVPGASFPLISTGVTYPFTATVSSPISSFFETTWLDSTPSFLSTEASTSPTATKSTVSFYNVEMSFSVFVEEPRIPITSVINEFTENSLNSIFQNSEFSLATLETQIKSRDISEEEMVMDRAILEQREGQEMATISYVPYSCVCQVIIKASSSLASSELMRKIKSKIHGNFTHGNFTQDQLTLLVNCEHVAVKKLEPGNCKADETASKYKGTYKWLLTNPTETAQTRCIKNEDGNATRFCSISINTGKSQWEKPKFKQCKLLQELPDKIVDLANITISDENAEDVAEHILNLINESPALGKEETKIIVSKISDISQCDEISMNLTHVMLQIINVVLEKQNNSASDLHEISNEILRIIERTGHKMEFSGQIANLTVAGLALAVLRGDHTFDGMAFSIHSYEEGTDPEIFLGNVPVGGILASIYLPKSLTERIPLSNLQTILFNFFGQTSLFKTKNVTKALTTYVVSASISDDMFIQNLADPVVITLQHIGGNQNYGQVHCAFWDFENNNGLGGWNSSGCKVKETNVNYTICQCDHLTHFGVLMDLSRSTVDSVNEQILALITYTGCGISSIFLGVAVVTYIAFHKLRKDYPAKILINLCTALLMLNLVFLINSWLSSFQKVGVCITAAVALHYFLLVSFTWMGLEAVHMYLALVKVFNIYIPNYILKFCLVGWGIPAIMVAITVSVKKDLYGTLSPTTPFCWIKDDSIFYISVVAYFCLIFLMNLSMFCTVLVQLNSVKSQIQKTRRKMILHDLKGTMSLTFLLGLTWGFAFFAWGPMRNFFLYLFAIFNTLQGFFIFVFHCVMKESVREQWQIHLCCGWLRLDNSSDGSSRCQIKVGYKQEGLKKIFEHKLLTPSLKSTATSSTFKSLGSAQGTPSEISFPNDDFDKDPYCSSP

SEQ ID NO: 260 - protein, 528 aa, Homo sapiens
MDHCGALFLCLCLLTLQNATTETWEELLSYMENMQVSRGRSSVFSSRQLHQLEQMLLNTSFPGYNLTLQTPTIQSLAFKLSCDFSGLSLTSATLKRVPQAGGQHARGQHAMQFPAELTRDACKTRPRELRLICIYFSNTHFFKDENNSSLLNNYVLGAQLSHGHVNNLRDPVNISFWHNQSLEGYTLTCVFWKEGARKQPWGGWSPEGCRTEQPSHSQVLCRCNHLTYFAVLMQLSPALVPAELLAPLTYISLVGCSISIVASLITVLLHFHFRKQSDSLTRIHMNLHASVLLLNIAFLLSPAFAMSPVPGSACTALAAALHYALLSCLTWMAIEGFNLYLLLGRVYNIYIRRYVFKLGVLGWGAPALLVLLSLSVKSSVYGPCTIPVFDSWENGTGFQNMSICWVRSPVVHSVLVMGYGGLTSLFNLVVLAWALWTLRRLRERADAPSVRACHDTVTVLGLTVLLGTTWALAFFSFGVFLLPQLFLFTILNSLYGFFLFLWFCSQRCRSEAEAKAQIEAFSSSQTTQ

SEQ ID NO: 261 - protein, 1193 aa, Homo sapiens
MMFRSDRMWSCHWKWKPSPLLFLFALYIMCVPHSVWGCANCRVVLSNPSGTFTSPCYPNDYPNSQACMWTLRAPTGYIIQITFNDFDIEEAPNCIYDSLSLDNGESQTKFCGATAKGLSFNSSANEMHVSFSSDFSIQKKGFNASYIRVAVSLRNQKVILPQTSDAYQVSVAKSISIPELSAFTLCFEATKVGHEDSDWTAFSYSNASFTQLLSFGKAKSGYFLSISDSKCLLNNALPVKEKEDIFAESFEQLCLVWNNSLGSIGVNFKRNYETVPCDSTISKVIPGNGKLLLGSNQNEIVSLKGDIYNFRLWNFTMNAKILSNLSCNVKGNVVDWQNDFWNIPNLALKAESNLSCGSYLIPLPAAELASCADLGTLCQDGIIYRISVVIQNILRHPEVKVQSKVAEWLNSTFQNWNYTVYVVNISFHLSAGEDKIKVKRSLEDEPRLVLWALLVYNATNNTNLEGKIIQQKLLKNNESLDEGLRLHTVNVRQLGHCLAMEEPKGYYWPSIQPSEYVLPCPDKPGFSASRICFYNATNPLVTYWGPVDISNCLKEANEVANQILNLTADGQNLTSANITNIVEQVKRIVNKEENIDITLGSTLMNIFSNILSSSDSDLLESSSEALKTIDELAFKIDLNSTSHVNITTRNLALSVSSLLPGTNAISNFSIGLPSNNESYFQMDFESGQVDPLASVILPPNLLENLSPEDSVLVRRAQFTFFNKTGLFQDVGPQRKTLVSYVMACSIGNITIQNLKDPVQIKIKHTRTQEVHHPICAFWDLNKNKSFGGWNTSGCVAHRDSDASETVCLCNHFTHFGVLMDLPRSASQLDARNTKVLTFISYIGCGISAIFSAATLLTYVAFEKLRRDYPSKILMNLSTALLFLNLLFLLDGWITSFNVDGLCIAVAVLLHFFLLATFTWMGLEAIHMYIALVKVFNTYIRRYILKFCIIGWGLPALVVSVVLASRNNNEVYGKESYGKEKGDEFCWIQDPVIFYVTCAGYFGVMFFLNIAMFIVVMVQICGRNGKRSNRTLREEVLRNLRSVVSLTFLLGMTWGFAFFAWGPLNIPFMYLFSIFNSLQGLFIFIFHCAMKENVQKQWRQHLCCGRFRLADNSDWSKTATNIIKKSSDNLGKSLSSSSIGSNSTYLTSKSKSSSTTYFKRNSHTDNVSYEHSFNKSGSLRQCFHGQVLVKTGPC

SEQ ID NO: 262 - protein, 502 aa, Homo sapiens
MPVKMLFKELLLLLMMMPLQHYTKTCGFVVYQNDKLFQSKTFTAKSDFSQKIISSKTDENEQDQSASVDMVFSPKYNQKEFQLYSYACVYWNLSAKDWDTYGCQKDKGTDGFLRCRCNHTTNFAVLMTFKKDYQYPKSLDILSNVGCALSVTGLALTVIFQIVTRKVRKTSVTWVLVNLCISMLIFNLLFVFGIENSNKNLQTSDGDINNIDFDNNDIPRTDTINIPNPMCTAIAALLHYFLLVTFTWNALSAAQLYYLLIRTMKPLPRHFILFISLIGWGVPAIVVAITVGVIYSQNGNNPQWELDYRQEKICWLAIPEPNGVIKSPLLWSFIVPVTIILISNVVMFITISIKVLWKNNQNLTSTKKVSSMKKIVSTLSVAVVFGITWILAYLMLVNDDSIRIVFSYIFCLFNTTQGLQIFILYTVRTKVFQSEASKVLMLLSSIGRRKSLPSVTRPRLRVKMYNFLRSLPTLHERFRLLETSPSTEEITLSESDNAKESI

SEQ ID NO: 263 - protein, 1474 aa, Homo sapiens
MARLAAVLWNLCVTAVLVTSATQGLSRAGLPFGLMRRELACEGYPIELRCPGSDVIMVENANYGRTDDKICDADPFQMENVQCYLPDAFKIMSQRCNNRTQCVVVAGSDAFPDPCPGTYKYLEVQYDCVPYKVEQKVFVCPGTLQKVLEPTSTHESEHQSGAWCKDPLQAGDRIYVMPWIPYRTDTLTEYASWEDYVAARHTTTYRLPNRVDGTGFVVYDGAVFYNKERTRNIVKYDLRTRIKSGETVINTANYHDTSPYRWGGKTDIDLAVDENGLWVIYATEGNNGRLVVSQLNPYTLRFEGTWETGYDKRSASNAFMVCGVLYVLRSVYVDDDSEAAGNRVDYAFNTNANREEPVSLTFPNPYQFISSVDYNPRDNQLYVWNNYFVVRYSLEFGPPDPSAGPATSPPLSTTTTARPTPLTSTASPAATTPLRRAPLTTHPVGAINQLGPDLPPATAPVPSTRRPPAPNLHVSPELFCEPREVRRVQWPATQQGMLVERPCPKGTRGIASFQCLPALGLWNPRGPDLSNCTSPWVNQVAQKIKSGENAANIASELARHTRGSIYAGDVSSSVKLMEQLLDILDAQLQALRPIERESAGKNYNKMHKRERTCKDYIKAVVETVDNLLRPEALESWKDMNATEQVHTATMLLDVLEEGAFLLADNVREPARFLAAKENVVLEVTVLNTEGQVQELVFPQEEYPRKNSIQLSAKTIKQNSRNGVVKVVFILYNNLGLFLSTENATVKLAGEAGPGGPGGASLVVNSQVIAASINKESSRVFLMDPVIFTVAHLEDKNHFNANCSFWNYSERSMLGYWSTQGCRLVESNKTHTTCACSHLTNFAVLMAHREIYQGRINELLLSVITWVGIVISLVCLAICISTFCFLRGLQTDRNTIHKNLCINLFLAELLFLVGIDKTQYEIACPIFAGLLHYFFLAAFSWLCLEGVHLYLLLVEVFESEYSRTKYYYLGGYCFPALVVGIAAAIDYRSYGTEKACWLRVDNYFIWSFIGPVSFVIVVNLVFLMVTLHKMIRSSSVLKPDSSRLDNIKSWALGAIALLFLLGLTWAFGLLFINKESVVMAYLFTTFNAFQGVFIFVFHCALQKKVHKEYSKCLRHSYCCIRSPPGGTHGSLKTSAMRSNTRYYTGTQSRIRRMWNDTVRKQTESSFMAGDINSTPTLNRGTMGNHLLTNPVLQPRGGTSPYNTLIAESVGFNPSSPPVFNSPGSYREPKHPLGGREACGMDTLPLNGNFNNSYSLRSGDFPPGDGGPEPPRGRNLADAAAFEKMIISELVHNNLRGSSSAAKGPPPPEPPVPPVPGGGGEEEAGGPGGADRAEIELLYKALEEPLLLPRAQSVLYQSDLDESESCTAEDGATSRPLSSPPGRDSLYASGANLRDSPSYPDSSPEGPSEALPPPPPAPPGPPEIYYTSRPPALVARNPLQGYYQVRRPSHEGYLAAPGLEGPGPDGDGQMQLVTSL

SEQ ID NO: 264 - protein, 1403 aa, Homo sapiens
MVSSGCRMRSLWFIIVISFLPNTEGFSRAALPFGLVRRELSCEGYSIDLRCPGSDVIMIESANYGRTDDKICDADPFQMENTDCYLPDAFKIMTQRCNNRTQCIVVTGSDVFPDPCPGTYKYLEVQYECVPYIFVCPGTLKAIVDSPCIYEAEQKAGAWCKDPLQAADKIYFMPWTPYRTDTLIEYASLEDFQNSRQTTTYKLPNRVDGTGFVVYDGAVFFNKERTRNIVKFDLRTRIKSGEAIINYANYHDTSPYRWGGKTDIDLAVDENGLWVIYATEQNNGMIVISQLNPYTLRFEATWETVYDKRAASNAFMICGVLYVVRSVYQDNESETGKNSIDYIYNTRLNRGEYVDVPFPNQYQYIAAVDYNPRDNQLYVWNNNFILRYSLEFGPPDPAQVPTTAVTITSSAELFKTIISTTSTTSQKGPMSTTVAGSQEGSKGTKPPPAVSTTKIPPITNIFPLPERFCEALDSKGIKWPQTQRGMMVERPCPKGTRGTASYLCMISTGTWNPKGPDLSNCTSHWVNQLAQKIRSGENAASLANELAKHTKGPVFAGDVSSSVRLMEQLVDILDAQLQELKPSEKDSAGRSYNKAIVDTVDNLLRPEALESWKHMNSSEQAHTATMLLDTLEEGAFVLADNLLEPTRVSMPTENIVLEVAVLSTEGQIQDFKFPLGIKGAGSSIQLSANTVKQNSRNGLAKLVFIIYRSLGQFLSTENATIKLGADFIGRNSTIAVNSHVISVSINKESSRVYLTDPVLFTLPHIDPDNYFNANCSFWNYSERTMMGYWSTQGCKLVDTNKTRTTCACSHLTNFAILMAHREIAYKDGVHELLLTVITWVGIVISLVCLAICIFTFCFFRGLQSDRNTIHKNLCINLFIAEFIFLIGIDKTKYAIACPIFAGLLHFFFLAAFAWMCLEGVQLYLMLVEVFESEYSRKKYYYVAGYLFPATVVGVSAAIDYKSYGTEKACWLHVDNYFIWSFIGPVTFIILLNIIFLVITLCKMVKHSNTLKPDSSRLENIKSWVLGAFALLCLLGLTWSFGLLFINEETIVMAYLFTIFNAFQGVFIFIFHCALQKKVRKEYGKCFRHSYCCGGLPTESPHSSVKASTTRTSARYSSGTQSRIRRMWNDTVRKQSESSFISGDINSTSTLNQGHSLNNARDTSAMDTLPLNGNFNNSYSLHKGDYNDSVQVVDCGLSLNDTAFEKMIISELVHNNLRGSSKTHNLELTLPVKPVIGGSSSEDDAIVADASSLMHSDNPGLELHHKELEAPLIPQRTHSLLYQPQKKVKSEGTDSYVSQLTAEAEDHLQSPNRDSLYTSMPNLRDSPYPESSPDMEEDLSPSRRSENEDIYYKSMPNLGAGHQLQMCYQISRGNSDGYIIPINKEGCIPEGDVREGQMQLVTSL

SEQ ID NO: 265 - protein, 1240 aa, Homo sapiens
MWPSQLLIFMMLLAPIIHAFSRAPIPMAVVRRELSCESYPIELRCPGTDVIMIESANYGRTDDKICDSDPAQMENIRCYLPDAYKIMSQRCNNRTQCAVVAGPDVFPDPCPGTYKYLEVQYECVPYKVEQKVFLCPGLLKGVYQSEHLFESDHQSGAWCKDPLQASDKIYYMPWTPYRTDTLTEYSSKDDFIAGRPTTTYKLPHRVDGTGFVVYDGALFFNKERTRNIVKFDLRTRIKSGEAIIANANYHDTSPYRWGGKSDIDLAVDENGLWVIYATEQNNGKIVISQLNPYTLRIEGTWDTAYDKRSASNAFMICGILYVVKSVYEDDDNEATGNKIDYIYNTDQSKDSLVDVPFPNSYQYIAAVDYNPRDNLLYVWNNYHVVKYSLDFGPLDSRSGQAHHGQVSYISPPIHLDSELERPSVKDISTTGPLGMGSTTTSTTLRTTTLSPGRSTTPSVSGRRNRSTSTPSPAVEVLDDMTTHLPSASSQIPALEESCEAVEAREIMWFKTRQGQIAKQPCPAGTIGVSTYLCLAPDGIWDPQGPDLSNCSSPWVNHITQKLKSGETAANIARELAEQTRNHLNAGDITYSVRAMDQLVGLLDVQLRNLTPGGKDSAARSLNKLQKRERSCRAYVQAMVETVNNLLQPQALNAWRDLTTSDQLRAATMLLHTVEESAFVLADNLLKTDIVRENTDNIKLEVARLSTEGNLEDLKFPENMGHGSTIQLSANTLKQNGRNGEIRVAFVLYNNLGPYLSTENASMKLGTEALSTNHSVIVNSPVITAAINKEFSNKVYLADPVVFTVKHIKQSEENFNPNCSFWSYSKRTMTGYWSTQGCRLLTTNKTHTTCSCNHLTNFAVLMAHVEVKHSDAVHDLLLDVITWVGILLSLVCLLICIFTFCFFRGLQSDRNTIHKNLCISLFVAELLFLIGINRTDQPIACAVFAALLHFFFLAAFTWMFLEGVQLYIMLVEVFESEHSRRKYFYLVGYGMPALIVAVSAAVDYRSYGTDKVCWLRLDTYFIWSFIGPATLIIMLNVIFLGIALYKMFHHTAILKPESGCLDNINYEDNRPFIKSWVIGAIALLCLLGLTWAFGLMYINESTVIMAYLFTIFNSLQGMFIFIFHCVLQKKVRKEYGKCLRTHCCSGKSTESSIGSGKTSGSRTPGRYSTGSQSRIRRMWNDTVRKQSESSFITGDINSSASLNREPYRETSMGVKLNIAYQIGASEQCQGYKCHGYSTTEW

SEQ ID NO: 266 - protein, 690 aa, Homo sapiens
MKRLPLLVVFSTLLNCSYTQNCTKTPCLPNAKCEIRNGIEACYCNMGFSGNGVTICEDDNECGNLTQSCGENANCTNTEGSYYCMCVPGFRSSSNQDRFITNDGTVCIENVNANCHLDNVCIAANINKTLTKIRSIKEPVALLQEVYRNSVTDLSPTDIITYIEILAESSSLLGYKNNTISAKDTLSNSTLTEFVKTVNNFVQRDTFVVWDKLSVNHRRTHLTKLMHTVEQATLRISQSFQKTTEFDTNSTDIALKVFFFDSYNMKHIHPHMNMDGDYINIFPKRKAAYDSNGNVAVAFVYYKSIGPLLSSSDNFLLKPQNYDNSEEEERVISSVISVSMSSNPPTLYELEKITFTLSHRKVTDRYRSLCAFWNYSPDTMNGSWSSEGCELTYSNETHTSCRCNHLTHFAILMSSGPSIGIKDYNILTRITQLGIIISLICLAICIFTFWFFSEIQSTRTTIHKNLCCSLFLAELVFLVGINTNTNKLFCSIIAGLLHYFFLAAFAWMCIEGIHLYLIVVGVIYNKGFLHKNFYIFGYLSPAVVVGFSAALGYRYYGTTKVCWLSTENNFIWSFIGPACLIILVNLLAFGVIIYKVFRHTAGLKPEVSCFENIRSCARGALALLFLLGTTWIFGVLHVVHASVVTAYLFTVSNAFQGMFIFLFLCVLSRKIQEEYYRLFKNVPCCFGCLR

SEQ ID NO: 267 - protein, 479 aa, Homo sapiens
MANFTPVNGSSGNQSVRLVTSSSHNRYETVEMVFIATVTGSLSLVTVVGNILVMLSIKVNRQLQTVNNYFLFSLACADLIIGAFSMNLYTVYIIKGYWPLGAVVCDLWLALDYVVSNASVMNLLIISFDRYFCVTKPLTYPARRTTKMAGLMIAAAWVLSFVLWAPAILFWQFVVGKRTVPDNQCFIQFLSNPAVTFGTAIAAFYLPVVIMTVLYIHISLASRSRVHKHRPEGPKEKKAKTLAFLKSPLMKQSVKKPPPGEAAREELRNGKLEEAPPPALPPPPRPVADKDTSNESSSGSATQNTKERPATELSTTEATTPAMPAPPLQPRALNPASRWSKIQIVTKQTGNECVTAIEIVPATPAGMRPAANVARKFASIARNQVRKKRQMAARERKVTRTIFAILLAFILTWTPYNVMVLVNTFCQSCIPDTVWSIGYWLCYVNSTINPACYALCNATFKKTFRHLLLCQYRNIGTAR

SEQ ID NO: 268 - protein, 397 aa, Homo sapiens
MRSPSAAWLLGAAILLAASLSCSGTIQGTSRSSKGRSLIGKVDGTSHVTGKGVTVETVFSVDEFSASVLTGKLTTVFLPIVYTIVFVVGLPSNGMALWVFLFRTKKKHPAVIYMANLALADLLSVIWFPLKIAYHIHGNNWIYGEALCNVLIGFFYGNMYCSILFMTCLSVQRYWVIVNPMGHSRKKANIAIGISLAIWLLILLVTIPLYVVKQTIFIPALNITTCHDVLPEQLLVGDMFNYFLSLAIGVFLFPAFLTASAYVLMIRMLRSSAMDENSEKKRKRAIKLIVTVLAMYLICFTPSNLLLVVHYFLIKSQGQSHVYALYIVALCLSTLNSCIDPFVYYFVSHDFRDHAKNALLCRSVRTVKQMQVSLTSKKHSRKSSSYSSSSTTVKTSY

SEQ ID NO: 269 - protein, 1212 aa, Homo sapiens
MVLLLILSVLLLKEDVRGSAQSSERRVVAHMPGDIIIGALFSVHHQPTVDKVHERKCGAVREQYGIQRVEAMLHTLERINSDPTLLPNITLGCEIRDSCWHSAVALEQSIEFIRDSLISSEEEEGLVRCVDGSSSSFRSKKPIVGVIGPGSSSVAIQVQNLLQLFNIPQIAYSATSMDLSDKTLFKYFMRVVPSDAQQARAMVDIVKRYNWTYVSAVHTEGNYGESGMEAFKDMSAKEGICIAHSYKIYSNAGEQSFDKLLKKLTSHLPKARVVACFCEGMTVRGLLMAMRRLGLAGEFLLLGSDGWADRYDVTDGYQREAVGGITIKLQSPDVKWFDDYYLKLRPETNHRNPWFQEFWQHRFQCRLEGFPQENSKYNKTCNSSLTLKTHHVQDSKMGFVINAIYSMAYGLHNMQMSLCPGYAGLCDAMKPIDGRKLLESLMKTNFTGVSGDTILFDENGDSPGRYEIMNFKEMGKDYFDYINVGSWDNGELKMDDDEVWSKKSNIIRSVCSEPCEKGQIKVIRKGEVSCCWTCTPCKENEYVFDEYTCKACQLGSWPTDDLTGCDLIPVQYLRWGDPEPIAAVVFACLGLLATLFVTVVFIIYRDTPVVKSSSRELCYIILAGICLGYLCTFCLIAKPKQIYCYLQRIGIGLSPAMSYSALVTKTNRIARILAGSKKKICTKKPRFMSACAQLVIAFILICIQLGIIVALFIMEPPDIMHDYPSIREVYLICNTTNLGVVTPLGYNGLLILSCTFYAFKTRNVPANFNEAKYIAFTMYTTCIIWLAFVPIYFGSNYKIITMCFSVSLSATVALGCMFVPKVYIILAKPERNVRSAFTTSTVVRMHVGDGKSSSAASRSSSLVNLWKRRGSSGETLRYKDRRLAQHKSEIECFTPKGSMGNGGRATMSSSNGKSVTWAQNEKSSRGQHLWQRLSIHINKKENPNQTAVIKPFPKSTESRGLGAGAGAGGSAGGVGATGGAGCAGAGPGGPESPDAGPKALYDVAEAEEHFPAPARPRSPSPISTLSHRAGSASRTDDDVPSLHSEPVARSSSSQGSLMEQISSVVTRFTANISELNSMMLSTAAPSPGVGAPLCSSYLIPKEIQLPTTMTTFAEIQPLPAIEVTGGAQPAAGAQAAGDAARESPAAGPEAAAAKPDLEELVALTPPSPFRDSVDSGSTTPNSPVSESALCIPSSPKYDTLIIRDYTQSSSSL

SEQ ID NO: 270 - protein, 380 aa, Homo sapiens
MEEGGDFDNYYGADNQSECEYTDWKSSGALIPAIYMLVFLLGTTGNGLVLWTVFRSSREKRRSADIFIASLAVADLTFVVTLPLWATYTYRDYDWPFGTFFCKLSSYLIFVNMYASVFCLTGLSFDRYLAIVRPVANARLRLRVSGAVATAVLWVLAALLAMPVMVLRTTGDLENTTKVQCYMDYSMVATVSSEWAWEVGLGVSSTTVGFVVPFTIMLTCYFFIAQTIAGHFRKERIEGLRKRRRLLSIIVVLVVTFALCWMPYHLVKTLYMLGSLLHWPCDFDLFLMNIFPYCTCISYVNSCLNPFLYAFFDPRFRQACTSMLCCGQSRCAGTSHSSSGEKSASYSSGHSQGPGPNMGKGGEQMHEKSIPYSQETLVVD

SEQ ID NO: 271 - protein, 461 aa, Homo sapiens [sequence omitted]

SEQ ID NO: 272 - protein, 553 aa, Homo sapiens
MKLGSSRAGPGRGSAGLLPGVHELPMGIPAPWGTSPLSFHRKCSLWAPGRPFLTLVLLVSIKQVTGSLLEETTRKWAQYKQACLRDLLKEPSGIFCNGTFDQYVCWPHSSPGNVSVPCPSYLPWWSEESSGRAYRHCLAQGTWQTIENATDIWQDDSECSENHSFKQNVDRYALLSTLQLMYTVGYSFSLISLFLALTLLLFLRKLHCTRNYIHMNLFASFILRTLAVLVKDVVFYNSYSKRPDNENGWMSYLSEMSTSCRSVQVLLHYFVGANYLWLLVEGLYLHTLLEPTVLPERRLWPRYLLLGWAFPVLFVVPWGFARAHLENTGCWTTNGNKKIWWIIRGPMMLCVTVNFFIFLKILKLLISKLKAHQMCFRDYKYRLAKSTLVLIPLLGVHEILFSFITDDQVEGFAKLIRLFIQLTLSSFHGFLVALQYGFANGEVKAELRKYWVRFLLARHSGCRACVLGKDFRFLGKCPKKLSEGDGAEKLRKLQPSLNSGRLLHLAMRGLGELGAQPQQDHARWPRGSSLSECSEGDVTMANTMEEILEESEI

SEQ ID NO: 273 - protein, 332 aa, Homo sapiens [sequence omitted]

SEQ ID NO: 274 - protein, 374 aa, Homo sapiens
MSGESMNFSDVFDSSEDYFVSVNTSYYSVDSEMLLCSLQEVRQFSRLFVPIAYSLICVFGLLGNILVVITFAFYKKARSMTDVYLLNMAIADILFVLTLPFWAVSHATGAWVFSNATCKLLKGIYAINFNCGMLLLTCISMDRYIAIVQATKSFRLRSRTLPRSKIICLVVWGLSVIISSSTFVFNQKYNTQGSDVCEPKYQTVSEPIRWKLLMLGLELLFGFFIPLMFMIFCYTFIVKTLVQAQNSKRHKAIRVIIAVVLVFLACQIPHNMVLLVTAANLGKMNRSCQSEKLIGYTKTVTEVLAFLHCCLNPVLYAFIGQKFRNYFLKILKDLWCVRRKYKSSGFSCAGRYSENISRQTSETADNDNASSFTM

SEQ ID NO: 275 - protein, 325 aa, synthetic construct
MDTSPDQSFFPGNHWLVFSVYLFTFLVGLPLNLLALVIFVGKLRRRPVAVDVLLLNLTLSDLLLLLFLPFRMVEAASGMRWPLPFILCPLSGFLFFTTIYLTSLFLAAVSIERFLSVAYPLWYKTRPRLGQAGLVSGACWLLASAHCSVVYVIEFSGNSSHSQGTNGTCYLEFREDQLAILLPVRLEMAVVLFGVPLLITSYCYSRLVWILSRGASHRRRRRVAGLVAATLLNFLVCFGPYNVSHVVGYIQGESPVWRSYVLLLSTLNSCVDPLVYYFSSSGFQADFHELLRRLCGLWGPWQQESSMELKEKKGGEEQRAERPAE

SEQ ID NO: 276 - protein, 572 aa, synthetic construct
MDLKTVLSLPQYPGEFLHPVVYACTAVMLLCLLASVITYIVHQSAIRISRKGRHTLLNFCFHAALTFTVFAGGINRTKYPILCQAVGIVLHYSTLSTMLWIGVTARNIYKQVTKKAPPCPDADQPPYPKQPLLRFYLISGGVPFIICGVTAATNIRNYGTEDEDTAYCWMAWEPSLGAFYGPAAFIALVTCVYFLGTYVQLRRHPERRYELRERTEEQQRLATPEGGHSRGIRPGTPPACDALGASLLQNEHSFKAQLRAAAFTLFLFTATWTFGALAVSQGHFLDMIFSCLYGAFCVTLGLFVLIHHCAKRDDVWHCWWSCCPSRKDAYSTKLNAHPALDANGDALGHAACLQDSPCPGKPRGFAHPPAGHCKMTNLQAAQGHVSCLSPATPCCAKMHCEQLTAEEAHVHLHEEDAFGHDPHLHRCLQGRTKPPYFSRHRAAAEPEYAYHIPSSLDGSPHSSRTDSPPSSLEGPAGTHTLACCAQGDPFPMVSQPEGSDGSPALYGCPTQPGREAALGPAHFEMLRRTQSLPFGGPSQNGLLKGDLLEGLPFGTDGTGNIRTGPWKNETTV

SEQ ID NO: 277 - protein, 1337 aa, synthetic construct
MGAGGRRMRGAPARLLLPLLPWLLLLAPETRGAPGCPVPIRSCKCSGERPKGLSGGAPNPARRRVVCGGGDLPEPPEPGLLPNGTVTLLLSNNKITGLRNGSFLGLSLLEKLDLRNNVISTVQPGAFLGLGELKRLDLSNNRIGCLTSETFQGLPRLLRLNISGNIFSSLQPGVFDELPALKVVDLGTEFLTCDCRLRWLLPWARNRSLQLSERTLCAYPSALHAQALGSLQEAQLRCEGALELHTHHLIPSLRQVVFQGDRLPFQCSASYLGNDTRIRWYHNRAPVEGDEQAGILLAESLIHDCTFITSELTLSHIGVWASGEWECSVSTAQGNASKKVEIVVLETSASYCPAERVANNRGDFRWPRTLAGITAYQSCLQYPFTSVPLSGGAPGTRASRRCDRAGRWEPGDYSHCLYTNDITRVLYTFVLMPINASNALTLAHQLRVYTAEAASFSDMMDVVYVAQMIQKFLGYVDQIKELVEVMVDMASNLMLVDEHLLWLAQREDKACSGIVGALERIGGAALSPHAQHISVNSRNVALEAYLIKPHSYVGLTCTAFQRREAGVPGTRPGGPGQNPPPEPEPLADQQLRFRCTTGRPNISLSSFHIKNSVALASIQLPPSLFSSLPAALAPPVPPDCTLQLLVFRNGRLFRSHGNTSRPGAAGPGKRRGVATPVIFAGTSGCGVGNLTEPVAVSLRHWAEGAEPVAAWWSQEGPGGPGGWSSEGCQLRSSQPNVSSLHCQHLGNVAVLMELSAFPREVGGSGAGLHPVVYPCTALLLLCLFSTIITYILNHSSIHVSRKGWHMLLNLCFHMAMTSAVFAGGITLTNYQMVCQAVGITLHYSSLSTLLWMGVKARVLHKELTWRAPPPQEGDPAPPAPRPMLRFYLIAGGIPLIICGITAAVNIHNYRDHSPYCWLVWRPSLGAFYIPVALILLITWIYFLCAGLRLRGPLAQSPKGGNSRASLEPGEELRGSTRLRSSGPLLSDSGSLLATGSAGVGTPGPPEDGDGLYSPGVQLGALVTTHFLYLAMWACGALAVSQRWLPRVVCSCLYGVAASALGLFVFTHHCARRRDVRASWRACCPPASASHASPRALPAAAEDGSPVFGEGPPSLKSSPSGSSGGHPPPLGPCKLTNLQLAQSQVCEAGVAARGEGEPEPAGSRGSLAPRHPNNLHHGRRAHKSRAKGHRAGEAGGKNRLKALRGGAAGGAPELLSSESGSLHNSPSDSYPGSSRNSPGAGLQLEGEPMLTPSEGSDTSAAPLPEAGRPGQRRSASRDNLKGGGALEKESKRRSYPLNAASLNGAPKGGKYDDVTLMGAEAAGGGCMKTGLWKSETTV

SEQ ID NO: 278 - protein, 1314 aa, synthetic construct
MEPPGRRRGRAPPPLPLLLLALLALLGGAAALPPGCKHDGRPRGAGRAAGAAEGKVVCSSLELAQVLPPDTLPNRTVTLILSNNKISELKNGSFSGLSLLERLDLRNNLISSIDPGAFWGLSSLKRLDLTNNRIGCLNADIFRGLTNLVRLNLSGNLFSSLSQGTFDYLGSLRSLEFQTEYLLCDCNILWMHRWVKERNITVRDTRCVYPKSLQAQPVTGVKQELLTCDPPLELPSFYMTPSHRQVVFEGDSLPFQCMASYIDQDMQVLWYQDGRIVETDESQGIFVEKNMIHNCSLIASALTISNIQAGSTGNWGCHVQTKRGNNTRTVDIVVLESSAQYCPPERVVNNKGDFRWPRTLAGITAYLQCTRNTHGSGIYPGNPQDERKAWRRCDRGGFWADDDYSRCQYANDVTRVLYMFNQMPLNLTNAVATARQLLAYTVEAANFSDKMDVIFVAEMIEKFGRFTKEEKSKELGDVMVDIASNIMLADERVLWLAQREAKACSRIVQCLQRIATYRLANGAHVYSTYSPNIALEAYVIKAAGFTGMTCTVFQKVAASDRTGLSDYGRRDPDGNLDKQLSFKCNVSNTFSSLALKNTIVEASIQLPPSLFSPKQKREVRPTDDSLYKLQLIAFRNGKLFPATGNSTNLADDGKRRTVVTPVILTKIDGVNVDTHHIPVNVTLRRIAHGADAVAAQWDFDLLNGQGGWKSDGCHILYSDENITTIQCYSLSNYAVLMDLTGSELYTQAASLLHPVVYTTAVILLLCLLAVIVSYIYHHSLIRISLKSWHMLVNLCFHIFLTCVVFVGGITQTRNASVCQAVGIILHYSTLATVLWVGVTARNIYKQVTKKAKRCQDPDELPPPPRPMLRFYLIGGGIPIIVCGITAAANIKNYGSRPNAPYCWMAWEPSLGAFYGPASFITFVNCMYFLSIFIQLKRHPERKYELKEPTEEQQRLAANENGEVNHQDSMSLSLISTSALENEHTFHSQLLGASLTLLLYVALWMFGALAVSLYYPLDLVFSFFFGATCLSLSAFIVVHHCVNREDVRLAWIMTCCPGRSSYSVQVNVQPPSSSGTNGEAPKCTNSSAESSCTNKSASSFKNSSQGCKLTNLQAAAAQCHTNSLPLNATPQLDNSLTEHSMDNDIKMHVAPLEVQFRTNVHPSRHHKNRSKGHRASRLTVLREYAYDVPTSVEGSVQNGLPKSRPGNNEGHSRSRRAYLAYRERQYNPPQQDSSDACSTLPKSSRNFEKPVSTSSKKDALRKPTVVELESQQKSYGLNLAIQNGPIKSSGQDGPLLGTDSTGNVRTGLWKHETTV

SEQ ID NO: 279 - protein, 1584 aa, synthetic construct
MRGQAAAPGPVWILAPLLLLLLLLGRRARAAAGADAGPGAEPCATLVQGKFFGYFSAAAVFPANASRCSWTLRNPDPRRYTLYMKVAKAPAPCSGPGRVRTYQFDSFLESTRTYLGVESFDEVLRLCDPSAPLAFLQASKQFLQMQRQQPPQDDGLGPRAGPPGPTDDFSVEYLVVGNRNPSRAACQMLCRWLDACLAGSRSSHPCGIMQTPCACLGGDAGDPASGPLAPRGDVCLRDGVAGGPENCLTSLTQDRGGHGATGGWKLWSLWGECTRDCGGGLQTRTRTCLPAPGVEGGGCEGVLEEGRLCNRKACGPAGRTSSRSQSLRSTDARRREELGDELQQFGFPSPQTGDPAAEEWSPWSVCSSTCGEGWQTRTRFCVSSSYSTQCSGPLREQRLCNNSAVCPVHGAWDEWSPWSLCSSTCGRGFRDRTRTCRPPQFGGNPCEGPEKQTKFCNIALCPGRAVDGNWNEWSSWSTCSASCSQGRQQRTRECNGPSYGGAECQGHWVETRDCFLQQCPVDGKWQAWASWGSCSVTCGGGSQRRERVCSGPFFGGAACQGPQDEYRQCGAQRCPEPHEICDEDNFGAVVWKETPAGEVAAVRCPRNATGLILRRCELDEEGIAYWEPPTYIRCVSIDYRNIQMMTREHLAKAQRGLPGEGVSEVIQTLVEISQDGTSYSGDLLSTIDVLRNMTEIFRRAYYSPTPGDVQNFVQIISNLLAEENRDKWEEAQLMGPNAKELFRLVEDFVDVIGFRMKDLRDAYQVTDNLVLSIHKLPASGATDISFPMKGWRATGDWAKVPEDRVTVSKSVFSTGLAEADDSSVFVVGTVLYRNLGSFLALQRNTTVLNSKVISVTVKPPPRSLLTPLEIEFAHMYNGTTNQTCILWDETDVPSSSAPPQLGPWSWRGCRTVPLDALRTRCLCDRLSTFAILAQLSADANMEKATVPSVTLIVGCGVSSLTLLMLVIIYVSVWRYIRSERSVILINFCLSIISSNALILIGQTQTRNKVVCTLVAAFLHFFFLSSFCWVLTEAWQSYMAVTGRLRNRLIRKRFLCLGWGLPALVVAISVGFTKAKGYSTMNYCWLSLEGGLLYAFVGPAAAVVLVNMVIGILVFNKLVSKDGITDKKLKERAGASLWSSCVVLPLLALTWMSAVLAVTDRRSALFQILFAVFDSLEGFVIVMVHCILRREVQDAVKCRVVDRQEEGNGDSGGSFQNGHAQLMTDFEKDVDLACRSVLNKDIAACRTATITGTLKRPSLPEEEKLKLAHAKGPPTNFNSLPANVSKLHLHGSPRYPGGPLPDFPNHSLTLKKDKAPKSSFVGDGDIFKKLDSELSRAQEKALDTSYVILPTATATLRPKPKEEPKYSIHIDQMPQTRLIHLSMAPDASLPARSPPSRQPPGGGPPEAPPAQPPPPPPPPPPPPQQPLPPPPNLEPAPPSLGEPGEPAAHPGPSSGPGTKNENVATLSVSSLERRKSRYAELDFEKIMHTRKRHQDMFQDLNRKLQHAAEKDKEVLGPDSKPEKQQTPNKRPWESLRKAHGTPAWVKKELEPLPPSPLELRSVEWEKSGATIPLVGQDIIDLQTEV

SEQ ID NO: 280 - protein, 1570 aa, synthetic construct
MTPACPLLLSVILSLRLAAAFDPAPSACSALASGVLYGAFSLQDLFPTIASGCSWTLENPDPTKYSLYLRFNRQEQVCAHFAPRLLPLDHYLVNFTCLRPSPEEAVAQAESEVGRPEEEEAAAGLELCGGSGPFTFLHFDKNFVQLCLSAEPSEAPRLLAPAALAFRFVEVLLINNNNSSQFTCGVLCRWSEECGRAAGRACGFAQPGCSCPGEAGAGSATTTPPGPPAAHTLSNALVPGGPAPPAEADLHSGSSNDLFTTEMRYGEEPEEEPKVKTQWPRSADEPGLYMAQTGDPAAEEWSPWSVCSLTCGQGLQVRTRSCVSSPYGTLCSGPLRETRPCNNSATCPVHGVWEEWGSWSLCSRSCGRGSRSRMRTCVPPQHGGKACEGPELQTKLCSMAACPVEGQWLEWGPWGPCSTSCANGTQQRSRKCSVAGPAWATCTGALTDTRECSNLECPATDGKWGPWNAWSLCSKTCDTGWQRRFRMCQATGTQGYPCEGTGEEVKPCSEKRCPAFHEMCRDEYVMLMTWKKAAAGEIIYNKCPPNASGSASRRCLLSAQGVAYWGLPSFARCISHEYRYLYLSLREHLAKGQRMLAGEGMSQVVRSLQELLARRTYYSGDLLFSVDILRNVTDTFKRATYVPSADDVQRFFQVVSFMVDAENKEKWDDAQQVSPGSVHLLRVVEDFIHLVGDALKAFQSSLIVTDNLVISIQREPVSAVSSDITFPMRGRRGMKDWVRHSEDRLFLPKEVLSLSSPGKPATSGAAGSPGRGRGPGTVPPGPGHSHQRLLPADPDESSYFVIGAVLYRTLGLILPPPRPPLAVTSRVMTVTVRPPTQPPAEPLITVELSYIINGTTDPHCASWDYSRADASSGDWDTENCQTLETQAAHTRCQCQHLSTFAVLAQPPKDLTLELAGSPSVPLVIGCAVSCMALLTLLAIYAAFWRFIKSERSIILLNFCLSILASNILILVGQSRVLSKGVCTMTAAFLHFFFLSSFCWVLTEAWQSYLAVIGRMRTRLVRKRFLCLGWGLPALVVAVSVGFTRTKGYGTSSYCWLSLEGGLLYAFVGPAAVIVLVNMLIGIIVFNKLMARDGISDKSKKQRAGSERCPWASLLLPCSACGAVPSPLLSSASARNAMASLWSSCVVLPLLALTWMSAVLAMTDRRSVLFQALFAVFNSAQGFVITAVHCFLRREVQDVVKCQMGVCRADESEDSPDSCKNGQLQILSDFEKDVDLACQTVLFKEVNTCNPSTITGTLSRLSLDEDEEPKSCLVGPEGSLSFSPLPGNILVPMAASPGLGEPPPPQEANPVYMCGEGGLRQLDLTWLRPTEPGSEGDYMVLPRRTLSLQPGGGGGGGEDAPRARPEGTPRRAAKTVAHTEGYPSFLSVDHSGLGLGPAYGSLQNPYGMTFQPPPPTPSARQVPEPGERSRTMPRTVPGSTMKLGSLERKKLRYSDLDFEVMHTRKRHSELYHELNQKFHTFDRYRSQSTAKREKRWSVSSGGAAERSVCTDKPSPGERPSLSQHRRHQSWSTFKSMTLGSLPPKPRERLTLHRAAAWEPTEPPDGDFQTEV

SEQ ID NO: 281 - protein, 1522 aa, synthetic construct
MKAVRNLLIYIFSTYLLVMFGFNAAQDFWCSTLVKGVIYGSYSVSEMFPKNFTNCTWTLENPDPTKYSIYLKFSKKDLSCSNFSLLAYQFDHFSHEKIKDLLRKNHSIMQLCNSKNAFVFLQYDKNFIQIRRVFPTDFPGLQKKGEEDQKSFFEFLVLNKVSPSQFGCHVLCTWLESCLKSENGRTESCGIMYTKCTCPQHLGEWGIDDQSLVLLNNVVLPLNEQTEGCLTQELQTTQVCNLTREAKRPPKEEFGMMGDHTIKSQRPRSVHEKRVPQEQADAAKFMAQTGESGVEEWSQWSTCSVTCGQGSQVRTRTCVSPYGTHCSGPLRESRVCNNTALCPVHGVWEEWSPWSLCSFTCGRGQRTRTRSCTPPQYGGRPCEGPETHHKPCNIALCPVDGQWQEWSSWSQCSVTCSNGTQQRSRQCTAAAHGGSECRGPWAESRECYNPECTANGQWNQWGHWSGCSKSCDGGWERRIRTCQGAAITGQQCEGTGEEVRRCSEQRCPAPYEICPEDYLMSMVWKRTPAGDLAFNQCPLNATGTTSRRCSLSLHGVAFWEQPSFARCISNEYRHLQHSIKEHLAKGQRMLAGDGMSQVTKTLLDLTQRKNFYAGDLLMSVEILRNVTDTFKRASYIPASDGVQNFFQIVSNLLDEENKEKWEDAQQIYPGSIELMQVIEDFIHIVGMGMMDFQNSYLMTGNVVASIQKLPAASVLTDINFPMKGRKGMVDWARNSEDRVVIPKSIFTPVSSKELDESSVFVLGAVLYKNLDLILPTLRNYTVVNSKIIVVTIRPEPKTTDSFLEIELAHLANGTLNPYCVLWDDSKTNESLGTWSTQGCKTVLTDASHTKCLCDRLSTFAILAQQPREIIMESSGTPSVTLIVGSGLSCLALITLAVVYAALWRYIRSERSIILINFCLSIISSNILILVGQTQTHNKSICTTTTAFLHFFFLASFCWVLTEAWQSYMAVTGKIRTRLIRKRFLCLGWGLPALVVATSVGFTRTKGYGTDHYCWLSLEGGLLYAFVGPAAAVVLVNMVIGILVFNKLVSRDGILDKKLKHRAGQMSEPHSGLTLKCAKCGVVSTTALSATTASNAMASLWSSCVVLPLLALTWMSAVLAMTDKRSILFQILFAVFDSLQGFVIVMVHCILRREVQDAFRCRLRNCQDPINADSSSSFPNGHAQIMTDFEKDVDIACRSVLHKDIGPCRAATITGTLSRISLNDDEEEKGTNPEGLSYSTLPGNVISKVIIQQPTGLHMPMSMNELSNQCLKKENSELRRTVYLCTDDNLRGADMDIVHPQERMMESDYIVMPRSSVNTQPSMKEESKMNIGMETLPHERLLHYKVNPEFNMNPPVMDQFNMNLDQHLAPQEHMQNLPFEPRTAVKNFMASELDDNAGLSRSETGSTISMSSLERRKSRYSDLDFEKVMHTRKRHMELFQELNQKFQTLDRFRDIPNTSSMENPAPNKNPWDTFKNPSEYQHYTTINVLDTEAKDALELRPAEWEKCLNLPLDVQEGDFQTEV

SEQ ID NO: 282 - protein, 3041 aa, synthetic construct
MAPPPPPVLPALLLAAAAALPALGLRAAAWELRVPGGARAFALGPGWTYALDAARTPRALRELLDVSRDGRLAGRRRGPGAGPRGCARLGGRPLPLQVRLAARGAPTALSLRLRARAHGPGCGARARRRRAPGAELRARAVLTVPGLGGALCFPAPGGGAAALHSALAALTTFPACSCPPRPGPRCPRRPICLPPGGSARLRLLCALRRAAGAVRVELALEAATGTPSASPSPSPSPPNLPQARAGPARRARRGAGGSTSPQFPLPSYQVSVPENEPAGTAVIELRAHDPDEGEAGRLSYQMEALFDERSNGYFLIDSATGAVSTARALDRETKDTHVLKVSAVDHGSPRRSAATYLTVTVSDTNDHSPVFEQSEYRERVRENLEVGYEVLTIRATDGDAPSNANMRYRLLEGAGGVFEIDARSGVVRTRAVVDREEAAEYQLLVEANDQGRNPGPLSATATVHIVVEDENDNYPQFSEKRYVVQVPEDVAVNTAVLRVQATDRDQGQNAAIHYSIVSGNLKGQFYLHSLSGSLDVINPLDFEAIREYTLRIKAQDGGRPPLINSSGLVSVQVLDVNDNAPIFVSSPFQAAVLENVPLGHSVLHIQAVDADAGENARLRYRLVDTASAFLGGGSAGPKNPASAPDFPFQIHNSSGWITVCAELDREEVEHYSFGVEAVDHGSPPMSSSASVSITVLDVNDNDPVFTQPVYELRLNEDAAVGSSVLTLRARDRDANSVITYQLTGGNTRNRFALSSQSGGGLITLALPLDYKQERQYVLAVTASDGTRSHTAQVFINVTDANTHRPVFQSSHYTVSVSEDRPVGTSIATISATDEDTGENARITYVLEDPVPQFRIDPDTGTIYTMTELDYEDQAAYTLAITAQDNGIPQKSDTTSLEILILDANDNAPRFLRDFYQGSVFEDAPPSTSVLQVSATDRDSGPNGRLLYTFQGGDDGDGDFYIEPTSGVIRTQRRLDRENVAVYNLRALAVDRGSPTPLSASVEIQVTVLDINDNPPVFERDELELFVEENSPVGSVVARIRANDPDEGPNAQIMYQIVEGNVPEVFQLDLLSGDLRALVELDFEVRREYVLVVQATSAPLVSRATVHIRLLDQNDNPPVLPDFQILFNNYVTNKSNSFPTGVIGRIPAHDPDLSDSLNYTFLQGNELRLLLLDPATGELQLSRDLDNNRPLEALMEVSVSDGIHSVTALCTLRVTIITDDMLTNSITVRLENMSQEKFLSPLLSLFVEGVATVLSTTKDDVFVFNIQNDTDVSSNILNVTFSALLPGGVRGQFFPSEDLQEQIYLNRTLLTTISTQRVLPFDDNICLREPCENYMKCVSVLRFDSSAPFISSTTVLFRPIHPINGLRCRCPPGFTGDYCETEIDLCYSSPCGANGRCRSREGGYTCECFEDFTGEHCEVNARSGRCANGVCKNGGTCVNLLIGGFHCVCPPGEYERPYCEVTTRSFPPQSFVTFRGLRQRFHFTVSLTFATQERNALLLYNGRFNEKHDFIALEIVDEQVQLTFSAGETTTTVAPQVPGGVSDGRWHSVQVQYYNKPNIGRLGLPHGPSGEKVAVVTVDDCDTAVAVRFGSDVGNYSCAAQGTQSGSKKSLDLTGPLLLGGVPNLPEDFPVHNRQFVGCMRNLSVDGRNVDMAGFIANNGTRAGCAAQRNFCDGTWCQNGGTCVNRWNTYLCECPLRFGGKNCEQVMPHPQRFSGESVVSWSDLDITISVPWYLGLMFRTRKEDGVLMEATAGGSSRLHLQILNNYLQFEVSHGPSDVASMMLSRSRVTDGEWHHLLIELKSAKEGKDIKYLAVMTLDYGMDQNTVQIGNQLPGLKMRSVVVGGVSEDKVSVRRGFRGCMQGVRMGETSTNIATLNMNDALKVRVKDGCDVEDPCTSSPCPPHSRCHDTWDDYSCVCDKGYFGRKCVDACHLNPCEHVAACVRSPGSPRGYVCECGPSHYGQYCENKLDLPCPKGWWGNPVCGPCHCAVSKGFDPDCNKTNGQCQCKENYYKPPAQDACLPCDCFPHGSHSRACDMDTGQCACKPGVIGRQCNRCDNPFAEVTTLGCEVIYNGCPRAFEAGIWWPQTKFGQPAAVPCPKGSVGNAVRHCSGEKGWLPPELFNCTTISFVDLKAMNEKLSRNETRMDGARSLRLARALRNATQHTGTLFGNDVRTAYQLLGRVLQHESWQQGFDLAATRDADFHEDVVHTGSALLAPATRAAWEQIQRSEGGAAQLLRRFEAYFSNVARNVRRTYLRPFVIVTANMILAVDIFDKFNFTGARVPRFEDIREEFPRELESSVSFPADFFKPPEEKEGPLVRPAGRRATPQTARPGPGAEREAPFSRRRRHPDEPGQFAVALVIIYRTLGQLLPEHYDPDRRSLRLPNRPVINTPVVSALVYSEGAPLPSPLERPVLVEFALLETEERTKPVCVFWNHSLAVGGTGGWSAKGCELLSRNRTHVACQCSHTASFAVLMDISRREHGEVLPLKIVTYAAVSLSLAALLVAFVLLSLVRTLRSNLHSIHKNLIVALFFSQLVFVIGINQTENPFLCTVVAILLHYVYMSTFAWTLVESLHVYRMLTEVRNIDAGPMRFYYVVGWGIPAIVTGLAVGLDPQGYGNPDFCWLSLQDTLIWSFAGPIGAVIIINTVIFVLSAKVSCQRKHHYYERKGVVSLLRTAFLLLLLISATWLLGLLAVNSDALSFHYLFAIFSCLQGLFVLLFHCVLNREVRKHLKGVLAGKKLHLDDSATTRATLLTRSLNCNNTYSEGPDMLRTALGESTASLDSTVRDEGIQKLSVSSGPARGGHGEPDASFVPRSSKKPHGHDSDSDSELSLDEQSSSYASSHSSDSEDDGVEAEDKWDPARGPVHSTPKGDAVANHVPAGWPDESLAGSDSEEPGGKPRLKVETKVSVELHLEEQGNHCGERPPDQESGGAARPAAVLSSQPPEQRKGILKNKVTYPPPLTEQTLKGRLREKLADCEQSPASSRTSSLGSGDGRAPDCAITVKTPRREPGREHLNGVAMNVRTGSAQADGSDSEGSNETSI

SEQ ID NO: 283 - protein, 2923 aa, synthetic construct
MRSRAARAPLPTPLPPPLLLLLLLLLLLPPLLGDQVGPCRSLGPGGRGSSGACAPVGWLCPASASNLWLYTSRCRDAGTELTGHLVPHHDGLRVWCPESGAHIPLPPAPEGCPWSCRLLGIGGHLSPQGKLTLPQEHPCLKAPRLRCQSCKLVQTPGLRAGERSPEESMGGRRKRNVNTAPQFQPPSYQATVPENQPAGTPVASLRAIDPDEGEAGRLEYTMDALFDSRSNHFFSLDPITGAVTTAEELDRETKSTHVFRVTAQDHGMPRRSALATLTILVTDTNDHDPVFEQQEYKESLRENLEVGYEVLTVRATDGDAPPNANILYRLLEGPGGSPSEVFEIDPRSGVIRTRGPVDREEVESYQLTVEASDQGRDPGPRSATAAVFLSVEDDNDNAPQFSEKRYVVQVREDVTPGAPVLRVTASDRDKGSNALVHYSIMSGNARGQFYLDAQTGALDVVSPLDYETTKEYTLRVRAQDGGRPPLSNVSGLVTVQVLDINDNAPIFVSTPFQATVLESVPLGYLVLHVQAIDADAGDNARLEYRLAGVGHDFPFTINNGTGWISVAAELDREEVDFYSFGVEARDHGTPALTASASVSVTILDVNDNNPTFTQPEYTVRLNEDAAVGTSVVTVSAVDRDAHSVITYQITSGNTRNRFSITSQSGGGLVSLALPLDYKLERQYVLAVTASDGTRQDTAQVVVNVTDANTHRPVFQSSHYTVNVNEDRPAGTTVVLISATDEDTGENARITYFMEDSIPQFRIDADTGAVTTQAELDYEDQVSYTLAITARDNGIPQKSDTTYLEILVNDVNDNAPQFLRDSYQGSVYEDVPPFTSVLQISATDRDSGLNGRVFYTFQGGDDGDGDFIVESTSGIVRTLRRLDRENVAQYVLRAYAVDKGMPPARTPMEVTVTVLDVNDNPPVFEQDEFDVFVEENSPIGLAVARVTATDPDEGTNAQIMYQIVEGNIPEVFQLDIFSGELTALVDLDYEDRPEYILVIQATSAPLVSRATVHVRLLDRNDNPPVLGNFEILFNNYVTNRSSSFPGGAIGRVPAHDPDISDSLTYSFERGNELSLVLLNASTGELRLSRALDNNRPLEAIMSVLVSDGVHSVTAQCALRVTIITDEMLTHSITLRLEDMSPERFLSPLLGLFIQAVAATLATPPDHVVVFNVQRDTDAPGGHILNVSLSVGQPPGPGGGPPFLPSEDLQERLYLNRSLLTAISAQRVLPFDDNICLREPCENYMRCVSVLRFDSSAPFIASSSVLFRPIHPVGGLRCRCPPGFTGDYCETEVDLCYSRPCGPHGRCRSREGGYTCLCRDGYTGEHCEVSARSGRCTPGVCKNGGTCVNLLVGGFKCDCPSGDFEKPYCQVTTRSFPARSFITFRGLRQRFHFTLALSFATKERDGLLLYNGRFNEKHDFVALEVIQEQVQLTFSAGESTTTVSPFVPGGVSDGQWHTVQLKYYNKPLLGQTGLPQGPSEQKVAVVTVDGCDTGVALRFGAVLGNYSCAAQGTQGGSKKSLDLTGPLLLGGVPDLPESFPVRTRHFVGCMRNLQVDSRHVDMADFIANNGTVPGCPAKKNVCDSNTCHNGGTCVNQWDAFSCECPLGFGGKSCAQEMANPQRFLGSSLVAWHGLSLPISQPWHLSLMFRTRQADGVLLQAVTRGRSTITLQLREGHVVLSVEGTGLQASSLRLEPGRANDGDWHHAQLALGASGGPGHAILSFDYGQQRAEGNLGPRLHGLHLSNITVGGVPGPASGVARGFRGCLQGVRVSETPEGVSSLDPSRGESINVEPGCSLPDPCDSNPCPANSYCSDDWDSYSCSCDPGYYGDNCTNVCDLNPCEHQSVCTRKPSAPHGYTCECPPNYLGPYCETRIDQPCPRGWWGHPTCGPCNCDVSKGFDPDCNKTSGECHCKENHYRPPGSPTCLLCDCYPTGSLSRVCDPEDGQCPCKPGVIGRQCDRCDNPFAEVTTNGCEVNYDSCPRAIEAGIWWPRTRFGLPAAAPCPKGSFGTAVRHCDEHRGWLPPNLFNCTSVTFSELKGFAERLQRNESGLDSGRSQRLALLLRNATQHTAGYFGSDVKVAYQLATRLLAHESAQRGFGLSATQDVHFTENLLRVGSALLDAANKRHWELIQQTEGGTAWLLQHYEAYASALAQNMRHTYLSPFTIVTPNIVISVVRLDKGNFAGAKLPRYEALRGERPPDLETTVILPESVFRETPPVVRPAGPGEAQEPEELARRQRRHPELSQGEAVASVIIYRTLAGLLPHNYDPDKRSLRVPKRPVINTPVVSISVHDDEELLPRALDKPVTVQFRLLETEERTKPICVFWNHSILVSGTGGWSARGCEVVFRNESHVSCQCNHMTSFAVLMDVSRRENGEILPLKTLTYVALGVTLAALLLTFLFLTLLRALRSNQHGIRRNLTAALGLAQLVFLLGINQADLPFACTVIAILLHFLYLCTFSWALLEALHLYRALTEVRDVNAGPMRFYYMLGWGVPAFITGLAVGLDPEGYGNPDFCWLSIYDTLIWSFAGPVAFAVSMSVFLYILAARASCAAQRQGFEKKGPVSGLRPSFAVLLLLSATWLLALLSVNSDTLLFHYLFAACNCIQGPFIFLSYVVLSKEVRKALKFACSRKPSPDPALTTKSTLTSSYNCPSPYADGRLYQPYGDSAGSLHSASRSGKSQPSYIPFLLREESTLNPGQGPPGLGDPGSLFLEGQDQQHDPDTDSDSDLSLEDDQSGSYASTHSSDSEEEEEEEEEEAAFPGEPGWDSLLGPGAERLPLHSTPKDGGPGPGKAPWPGDFGTTAKESSGNGASEERPRENGDALPREGSLGPLPGPSAQPHKGILKKKCLPTISEKSSLLRLPLEQGTGSSRGSSASEGSRGGPPPRPPPRQSLQEQLNGVMPIAMSIKAGTVDEDSSGSEFLFFNF

SEQ ID NO: 284 - protein, 3314 aa, synthetic construct
MARRPPWWGLGGPSTPPLLLLLLLSLFPLSREELGGGGHQGWDPGVAAATGPRAHIGGGALALCPESPGVREDGGPGLGVREPVFVGLRGGRQSARNGRGPPEQPNEELGIEHGVQALGSREQETGQGPGSLLCWRPEVSSCGRTGPLRRGSLSPEALSPGVPGLGNSSPLPSDLLVRPHGPKPVSSQRNAGRGSRKRVGTARCCGELWAPGRKGQGERATTSGAERTAPRRDCLPGASGSGPGLDSAPRTARTAPASGSAPRESRTAPEPAPERMRSRGLFRRRFLPQRPGPRPPGLPARPEARRITSANRARPRRAANRHPQFPQYNYQTLVPENEAAGTAVLRVVAQDPDAGEAGRLVYSLAALMNSRSLELFSIDPQSGLIRTAAALDRESMERHYLRVTAQDHGSPRLSATTMVAVTVADRNDHAPVFEQAQYRETLRENVEEGYPILQLRATDGDAPPNANLRYRFVGPPAARAAAAAAFEIDPRSGLISTSGRVDREHMESYELVVEASDQGQEPGPRSATVRVHITVLDENDNAPQFSEKRYVAQVREDVRPHTVVLRVTATDRDKDANGLVHYNIISGNSRGHFAIDSLTGEIQVVAPLDFEAEREYALRIRAQDAGRPPLSNNTGLASIQVVDINDHTPIFVSTPFQVSVLENAPLGHSVIHIQAVDADHGENARLEYSLTGVAPDTPFVINSATGWVSVSGPLDRESVEHYFFGVEARDHGSPPLSASASVTVTVLDVNDNRPEFTMKEYHLRLNEDAAVGTSVVSVTAVDRDANSAISYQITGGNTRNRFAISTQGGVGLVTLALPLDYKQERYFKLVLTASDRALHDHCYVHINITDANTHRPVFQSAHYSVSVNEDRPVGSTVVVISASDDDVGENARITYLLEDNLPQFRIDADSGAITLQAPLDYEDQVTYTLAITARDNGIPQKADTTYVEVMVNDVNDNAPQFVASHYTGLVSEDAPPFTSVLQISATDRDAHANGRVQYTFQNGEDGDGDFTIEPTSGIVRTVRRLDREAVPVYELTAYAVDRGVPPLRTPVSIQVTVQDVNDNAPVFPAEEFEVRVKENSIVGSVVAQITAVDPDEGPNAHIMYQIVEGNIPELFQMDIFSGELTALIDLDYEARQEYVIVVQATSAPLVSRATVHVRLVDQNDNSPVLNNFQILFNNYVSNRSDTFPSGIIGRIPAYDPDVSDHLFYSFERGNELQLLVVNQTSGELRLSRKLDNNRPLVASMLVTVTDGLHSVTAQCVLRVVIITEELLANSLTVRLENMWQERFLSPLLGHFLEGVAAVLATPAEDVFIFNIQNDTDVGGTVLNVSFSALAPRGAGAGAAGPWFSSEELQEQLYVRRAALAARSLLDVLPFDDNVCLREPCENYMKCVSVLRFDSSAPFLASASTLFRPIQPIAGLRCRCPPGFTGDFCETELDLCYSNPCRNGGACARREGGYTCVCRPRFTGEDCELDTEAGRCVPGVCRNGGTCTDAPNGGFRCQCPAGGAFEGPRCEVAARSFPPSSFVMFRGLRQRFHLTLSLSFATVQPSGLLFYNGRLNEKHDFLALELVAGQVRLTYSTGESNTVVSPTVPGGLSDGQWHTVHLRYYNKPRTDALGGAQGPSKDKVAVLSVDDCDVAVALQFGAEIGNYSCAAAGVQTSSKKSLDLTGPLLLGGVPNLPENFPVSHKDFIGCMRDLHIDGRRMDMAAFVANNGTMAGCQAKLHFCDSGPCKNSGFCSERWGGFSCDCPVGFGGKDCRLTMAHPHHFRGNGTLSWDFGNDMAVSVPWYLGLAFRTRATQGVLMQVQAGPHSTLLCQLDRGLLSVTVTRGSGRAAHLLLDQVTVSDGRWHDLRLELQEEPGGRRGHHVLMVSLDFSLFQDTMAVGSELQGLKVKQLHVGGLPPSSAEEAPQGLVGCIQGVWLGSTPSGSPALLPPSHRVNVEPGCVVTNACASGPCPPHADCRDLWQTFSCTCWPGYYGPGCVDACLLNPCQNQGSCRHLPGAPHGYTCDCVGGYFGHHCEHRMDQQCPRGWWGSPTCGPCNCDVHKGFDPNCNKTNGQCHCKEFHYRPRGSDSCLPCDCYPVGSTSRSCAPHSGQCPCRPGALGRQCNSCDSPFAEVTASGCRVLYDACPKSLRSGVWWPQTKFGVLATVPCPRGALGAAVRLCDEDQGWLEPDLFNCTSPAFRELSLLLDGLELNKTALDTVEAKKLAQRLREVTGHTDHYFSQDVRVTARLLAHLLAFESHQQGFGLTATQDAHFNENLLWAGSALLAPETGDLWAALGQRAPGGSPGSAGLVRHLEEYAATLARNMELTYLNPVGLVTPNIMLSIDRMEHPSSPRGARRYPRYHSNLFRGQDAWDPHTHVLLPSQSPRPSPSEVLPTSSSIENSTTSSVVPPPAPPEPEPEPGISIVILLVYRTLGGLLPAQFQAERRGARLPQNPVMNSPVVSVAVFHGRNFLRGVLESPISLEFRLLQTANRSKAICVQWDPPGPADQHGMWTARDCELVHRNGSHARCRCSRTGTFGVLMDASPRERLEGDLELLAVFTHVVVAVSVAALVLTAAVLLSLRSLKSNVRGIHANVAAALGVAELLFLLGIHRTHNQLVCTAVAILLHYFFLSTFAWLLVQGLHLYRMQVEPRNVDRGAMRFYHALGWGVPAVLLGLAVGLDPEGYGNPDFCWISVHEPLIWSFAGPVVLVIVMNGTMFLLAARTSCSTGQREAKKTSVLTLRSSFLLLLLVSASWLFGLLAVNHSILAFHYLHAGLCGLQGLAVLLLFCVLNADARAAWTPACLGRKAAPEEARPAPGTGPGAYNNTALFEESGLIRITLGASTVSSVSSARSGRTQDQDSQRGRSYLRDNVLVRHGSAADHTDHSLQAHAGPTDLDVAMFHRDAGADSDSDSDLSLEEERSLSIPSSESEDNGRTRGRFQRPLRRAAQSERLLTHPKDVDGNDLLSYWPALGECEAAPCALQTWGSERRLGLDTSKDAANNNQPDLALTSGDETSLGRAQRQRKGILKNRLQYPLVPQTRGAPELSWCRAATLGHRAVPAASYGRIYAGGGTGSLSQPASRYSSREQLDLLLRRQLSRERLEEAPAPVLHPLSRPGSQECLDAAPGRLEPRDRGSTLPRRQPPRDYPGAMAGRFGSRDALDLGAPREWLSTLPPPRRTRDLDPQPPPLPLSPQRQLSRDPLLPSRPLDSLSRSSNSREQLDQVPSRHPSREALGPPPQLLRAREDPASGPSHGPSTEQLDILSSILASFNSSALSSVQSSSTPSGPHTTATPSATASALGPSTPRSATSHSISELSPDSEVPRSEGHS

SEQ ID NO: 285 - protein, 874 aa, synthetic construct
MRKLLRLCCWYSWLLLFYCNFQVRGVYSRSQDHPGFQVLASASHYWPLENVDGIHELQDTTGDIVEGKVNKGIYLKEEKGVTLLYYGRYNSSCISNPAQCGPEGVTFSFFWKTQGEQSRPIPSAYGGQVISNGFKVCSSGGKGSVELYTRDNSMTWEATFSPPGPYWTHVLFTWKSKEGLKVYVNGTLSTSDPSGKVSHAYGEPNVNLVIGSEQDQTKRYENGAFDEFIIWERALTPDEIAMYFTAAIGKHALLSSTPPSLFMTPTANTMMPTDAYHPIITNLTEERKNFQSPGVVLSYLQNVSLSLPNKSLSEETALNLTKTFLKTVGEVLLLPSWTAVSEDSAVVLGLIDTIDTVMGHISSNLHASTPQVTIEGSSSMAEFSVAKILPKTVNSSHYRFPAHGQSYIEIPHEAFHSQAWTTIVGLLYHSMHYYLNNIWPAHTKIAEAANYQDCLLSATSHLISLEVSPPPTLSQNLSGSPLITVHLRHRLTRKQHSEATNSSNRVFLYCAFLDFSSGEGVWSNQGCALTEGNLSYSVCRCTHLTNFAILMQVVPLELTRGHQVALSSISYIGCSLSVLCLVATLVTFAVLSSVSTIRNQRYHIHANLSFAVLVAQVLLLISFRLEPGTTPCQVLAVLLHYFFLSAFAWMLVEGLHLYSMVIKVFGSEDSKHRYYYGIGWGFPLLICIISLSFAMDSYGTSNNCWLSLGSGAIWAFVAPALFVIVVNIGILIAVTRVISQISADNYKIHGDPSAFKLTAKAVAVLLPILGTSWVFGVLAVNGQAVVFQYMFATLNSLQGLFIFLFHCLLNSEVRAAFKHKTKVWSLTSSSARTANAKPFSSDIMNGTRPGTASTKLSPWDKSSHSAHRVDLSAV

SEQ ID NO: 286 - protein, 1017 aa, synthetic construct
MAPWCFLCLLIRSLSPSNSPGESRNPWAPAPGEVVETAGGVCKFSGQRLSWWQAQESCEQRFGHLALQPPDGVLASRLRDPVWVGQREAPLRRPPQRRTAVLVFGEKTADRAARLRSPLPELAALTACAHVQWDCASPDPAALFSVAVPALPNALQLRAFAEPGGVVRAALVVRGHHAPFLAAFRADGRWHHVCATWEQRGGRWALFADGRRRAGARGLGAGHPVPSGGILVLGQDQDSLGGGFSARDAFSGNLTDFHLWARALSPAQLHRARACAPSEGLLFRWDPGALDVTPSLPTVWVRLLCPVPSEECPTWNGSEGSELCLQPLPFLCCYRTETYRRLQDAQSWPGQDVISRVNALANDIVLLPDPLSEVHGALSLAEASSFLGLLEHVLAEMAPLGPAALLAVVRFLKRVVALGAGEPELLGPWEQLGQGVVSVASLVLEEQVADTWLSISEVVGGPMALVASVQRLAPLLSTSLTSERPRMRIQHRHAGLEVRSLRLREASTRGCLFTMPGGRPEGPGHIHIPASEVRRLLRKGLSGVTVIHSWFTSSVFQHTLEGPGLEPQAPASSEEANRVQRFLSTQVGSAIISSEVWDVTGEVSTAVTFHLQHQAQDLLVEPSCAFWNFSSPDTGGAWATTGCSVAALYLDSTACFCNHSTNFAVLLQVYEVQRGPEEESLLRTLSFVGCGVSFCALTTTFLLFLAAGVPKSERTTVHKNLTFSLASAEGFLMTSEWAKANEVACVAVTAAMHLLFLAAFSWMLVEGLLLWSKVVAVSMHPGPRMRLYYATGWGVPVGIVAVTLAMSPHDYVAPGHCWLNVHTDAIWAFVGPVLFVLTANTCILARVVMVTVSSARRRARMLSPQPCLQQQIWIQIWATVKPVLVLLPVLGLTWLVGILVHLSPAWAYAAVGLNSIQGLYIFLVYAAYNEEVRNALQRMAEKKVAEGFTACSHPPPLLSSPRNTTSWERLWNSPSALASARSHPAQKDNFGPKIPISSIMSPERPAVELTAFKSSGF

SEQ ID NO: 287 - protein, 888 aa, synthetic construct
MWGFNLLLFWGCCGMHSWEGHIRPTRKPNDGNNCRDTTLCPAYATCTNTVDSYYCTCKRGFLSSNGLNHFKGPGVECKDIDECSQSPQPCGPNSVCRNLPGRYKCSCLPGFSSPTGNNWIPGKPGHFSCTDIDECLTSSVCPEHSDCVNSMGSYSCSCQVGFISRNSTCEDVDECADPRACPEHATCHNSVGSYSCFCNPGFESSSGHLSFQGPGATCEDIDECDECTEMCPINSTCTNTPGSYFCTCHPGFAPSNGQLNFTDQEVECRDIDECRQDPSPCGPNSVCTNALGSYSCGCIAGFHPNPEGSQKDGNFSCKRIPFKCKEDVIPNNEQVQLCQEGTAVEPEYVSFCALMNATFSVLDNVCENKTTVVSLKSTAESFVSVLEQTSTWSNFTKEETSSLATVLLESVESTTLAAFLKPSANVSQTVQTEHLDIESKVINKECSEENVTFDLKAKGDEMKIGCSTIEESESTGTTGVAFVSFVGMESVLDERFFQDHQAPLANSEIKLKMNSRVVGGIMTGEKKDGFSDPVIYTLENIQPKQKFERPICVSWSTDVEGGRWTPSGCVILEASETHTVCSCNRMANLAVIMASGELTMEFSLYIISHVGIIISLVCLVLAIATFLLCRSIRNHNTYLHLHLCVCLFLAKTLFLTGVDKTDNQMGCAIIAGFLHYLFLACFFWMLVEAVMLFLMVRNLKVVNYFSSRNIKMLYLCAFGYGLPGLVVAVSASVQPQGYGMHNRCWLNTETGFIWSFLGPVCTIIVINSILLTWTLCILRQKLSSVNAEVSTLKDTRLLTFKAFAQLFILGCSWVLGIFQIGPMAGIMAYLFTIINSLQGAFIFLIHCLLNRQVREEYRRWITRKTKPSSESQTSGILLSSVPSTSKTG

SEQ ID NO: 288 - protein, 819 aa, synthetic construct
MGGRVFLVFLAFCVWLTLPGAETQDSRGCARWCPQNSSCVNATACRCNPGFSSFSEIFTSPMETCDDINECATPSKVSCGKFSDCWNTEGSYDCVCSPGYELVSGAKTFKNESENTCQDVDECQQNPRLCKSYGTCVNTLGSYTCQCLPGFKLKPEDPKLCTDVNECTSGQNPCHSSTHCLNNVGSYQCRCRPGWQPIPGSPNGPNNTVCEDVDECSSGQHQCDSSTVCFNTVGSYTCRCRPGWEPKHGIPNNQKDTVCEDMTFSTWTPPPGVHSQTLSRFFDKVQDLGRDFKPGSANNTIQSILQALDELLEAPGDLETLPRLQQHCVATHLLDGLEDVLRGLSKNLSNGLLNFSYPAGTELSLEVQKQVDRNVTLRQNQAVMQLDWNLAQKSGDPGPSVVGLVSIPGMGKLLAEAPLVLEPEKQVVLHETHQGLLPILLSDVISAFLSNNDTQNLSSPVTFTFSHRSVIPRRKVLCVFWEHGQNGCGHWATTGCSTMGTRDTSTICRCTHLSSFAVLMAHYDVQEEDPVLTVITYMGLSVSLLCLLLAALTFLLCKAIQNTSTSLHLQLSLCLFLAHLLFLVAIDQTGHKVLCAIIAGALHYLYLAAFTWMLLEALYLFLTARNLTVVNYSSINRFMKKLMFPVGYGVPAVIVAISAASRPHLYGTPSRCWLQPEKGFIWGFLGPVCAIFSVNLALFLVTLWILKNRLSSLNSEVSTLQNTRMLAFKATAQLFILGCTWCLGILQVGPAARVMAYLFTIINSLQGVFIFLVYCLLSQQVREQYRKWSKGIRKLRTESEMHTLSSSAKADTSKPSTVN

SEQ ID NO: 289 - protein, 638 aa, synthetic construct
MQGPSLLPGLCFLLSLSGVVTQKTKSCCKQCPPNASCVNNTHCTCNHGYTSGSGQKLFTFPLETCNDIDECKPPISIYCGLNAACQNVEGSFYCHCNPGYKLLSGDTQFKNSNENTCQDTTSSKTTEGRKELQKVVEKFESLLTNQTLWRTEEKQEVASTATTILQDVESKVLETALKDPEQKIQKIQNSTVAIETRVVTDNCSEERKIFNLNVQMNSMDIHCNDIIQGNTQGPSAVAFISYSSLGNIINATFFEEMNEKDRVYLNSQVVSAAIGPKRNVSLSKSVILSFQHVKMKPSTKKVFCVYWKSTGEGGQWSRDGCFLIQVNKSHTICNSTHLSSFAVLMALTSQEEDPVLTVITYVGLSLSLLCLLLAALTFLLCKAIQNTSTSLHLQLSLCLFLAHLLFLTAIDRTEPKVLCAIIAGALHYLYLASFTWMLLEGLHLFLTARNLTVVNYSSVNRFMKWLMFPVGYGVPAVIVAISAASRPHLYGTPDRCWLHLDQGFIWSFLGPVCAIICVNLVFFLLVLWILKRKLSSLNSEVSTIQNTRMLTLKATAQLFILGCTWCLGLLQVGPAAQVMAYLFTIINSLQGFFIFLVYCLLSQQVRKWFGEIVKSKSESETYTLSSRFGPDSKPSEGD

SEQ ID NO: 290 - protein, 773 aa, synthetic construct
MGGRVFLALCVWLTLPEQDSTRGCARWCPQNSSCVNATACRCNPGFSSSSFEIFTTPTETCDDINECAPPSKVSCGKFADCQNTEGSYDCVCSPGYELVSGAKTFKNESENTCQDVDECQQNPRLCKSYGTCVNTLGSYTCQCLPGFKFIPEDPKVCTVCEDVDECSSGQHQCHNSTVCFNTVGSYSCRCRPGWEPKPGIPNNQKDTCEEMTFPTWTPPPGVHSQTLSRFFDKVQDLGRDFKTSSAEVTIQNLIKLVDELLEAPGDLEALAPPVRHLIATQLLSNLEDILRILAKSLPKGPFTYISPSNTELSLMIQEQGDGNVTMGQSSARMLLNWAVAAGAEDSGPTVAGILSSQNMTTLLANASLNLHSEKQAELEEIYESSVRGAQLRRLSAVNSVFLSNTNTKKLNSPVTFAFSHLESKDVMPGPRQELICAFWKSDSNRGGHWATEGCQVLGSKNGSTTCQCSHLSSFAILMAHYDVEDWKLTLITKVGLALSLFCLLLCILTFLLVRPIQGSRTTVHLHLCICLFVGSTIFLAGIENEGQVGLRCRLVAGLLHYCFLAAFCWMSLEGLELYFLVVRVFQGQGLSTRWLCLIGYGVPLLIVGVSAAVYSKGYGRPRYCWLDFEQGFLWSFLGPVTFIILCNAVIFVTTVWKLTQKFSEINPDMKKLKKARVLTITAIAQLFVLGCTWVFGLFLFDDRSWVLTYVFTILNCLQGAFLFVLHCLLNKKVEEYRKWACLVAGNKYSEFTSSTSGTGHNQTRALRPSESGM

SEQ ID NO: 291 - protein, 906 aa, synthetic construct
MRVGVLWLISFFTFTEGHGGFLGNDGIKTKRELIVNKKKHPGVQEYELLLQVAYRDSKEKRDLKNFLKLLKPPSLWLHGPMKIIRAKATTYCGSQNGVLQCACEDGYTWFPPSCLDPQKCYLHTAGSLQSCECHLNNLTQSVNFCERTKVWGTFKINERFTKDLLNSSSAIYSKYTTGIEIQLKEAYKRIQGFESVQVTQFRNGSIIAGYEVVGSSSTSELLSAIEQVAEKAKAGLHKLFPLEDGSFRVFGKAQCNSIVFGFGSKNDEYTLPCSSGYTGNITARCQPSGWQVIRETCVLSQLEELKKNFSVIAGNATEAAVSSLVQNLSVIIQQNPSTTAGNLASVVSILGNVSSLSLASHFRVSNSTMEDVISIADHILNSASVTNWTVLLQEEKHASSRLLETLENISTLVPPTALPLNFSREFINWKGIPVSKSQLKRGYNYQTEMFPQNTSIPIRGHVLIGSDQFQRSLPETIISMASLTLGNILPITKNGNAQVNGPVISTVIQNYSINEIFLFFSKIESNLSQPHCVFWDFSHLQWNNAGCHLVNETPDTVTCRCTHLTSFSMLMSPFVPPAIIPVVKWITFVGLGISIGSLILCLIIEALFWKQVKKNQTSHTRHICMVNIALCLLIADVWFIVAATVDTTVNPSGVCIAAVFFTHFFYLSLFFWMLMLGILLAYRIILVFHHMAQPLMMAVGFCLGYGCPLIISVITIAVTQPSNTYKRKDVCWLNWSDGSKPLLAFAVPALTIVAVNLVVVLLVLTKLWRPAVGERLSQDDKATIVRMGKSLLILTPLLGLTWGFGIGTMVDSQNLAWHVIFALLNAFQGFFILCFGMLLDSKLRQLLFNKLSPLSSWKQTSKQNSSDLSAKPKFSKPFNPLQHKGYAFSHGESSNDIMLTQFLSTE

SEQ ID NO: 292 - protein, 986 aa, synthetic construct
MVCSAAPLLLLATTLPSPVAQASQPGQSQAGGESGQLLDQENGAGESALVSVYVHLDFSDKTWPPELSRTLTLPAASASSSPPLLTGLRLTTECNVNHKGNFYCACLSGYQWNTSICLHYPPCQSPHNHQPCGCLVFSHPEPGYCQLLPPVPGILSLNSQLQMPGDTLSLTLHLSQEATNLSWFLRHPGSPSPILLQPGTQVSVTSSHGQAALSISNMSHHWAGEYMSCFEAQGFKWNLYEVVRVPLKATDVARLPDQLSISCATSPGFQLSCCIPSTNLAYTAAWSPGEGSKASSFNESGSQCFVLAVQRCPMADTTYTCDLQSPGLAPLRVPISITIIQDGDITCPEDASVLTWNVTKAGHVAQAPCPESKRGIVRRLCGADGVWGPVHSSCTDARLLALFTRAKLLQAGQGSPAEEVPQILAQLPGQAAEASSPSDLLTLLSTMKYLAKVVAKARIQLDRSALKNLLITTDKVLDMDTRSLWTLAQARKPWAGSTLLLAVETLACSLCPQDHPFAFSLPNVLLQSQLFGPTFPADYSISFPTRPPLQAQIPRHSLAPLVRNGTEISITSLVLRKLDHLLPSNYGQGLGDSLYATPGLVLVISIMAGDQAFSQGEVIMDFGNTDGSPHCVFWDHSLFQGRGGWSKEGCQAQAASASPTAQCLCQHLTAFSVLMSPHTVPEEPALALLTQVGLGASILALLVCLGVYRLVWRVVVRNKVSYFRHAALLNMVLCLLAADTCFLGAPFLPPGPRSPLCLAAAFLCHFLYLATFFWMLAQALVLAHQLLFVFHQLAKHRVLPLMVLLGYLCPLGLAGVTLGLYLPQGQYLREGECWLDGKGGALYTFVGPVLAIVGVNGLVLAMAMLKLLRPSLSEGPPAEKRQALLGVIKALLILTPIFGLTWGLGLATLLEEVSTVPHYIFTILNTLQGVFILLFGCLMDKKVQEALRKRFCRAQAPNSTISLVTCELQILECSKGMSEGARWPSS

SEQ ID NO: 293 - protein, 691 aa, synthetic construct
MKSQATMICCLMLFLATECSHYRSKIHIKDGDKLQSPEGKPKTGRIQEKCEGPCISSSNCSQPCAQHFRGEIGFTCNQNKWQKSTETCTSLSVETLFKDSNSASRLSVAAPSIPLHILDFRAPEPIESVAQGIRKNCPFDYACIIDVVKSSEATSGNIAFIVELLKNISTDLSDNVTREKMKSYSEVANHILDTAAISNWAFIPDKNASSDLLQSVNLFARQLHIHNESENIVDELFIQTKGFHINHNTSEKSFNFSMSMNNTTEGILGMIEIPRQELWKLPPNASQAISIAFPTLGAILKEAHLQNVSLPRPVNGLVLSVILPERLKQILLTFEKINKSRNARAQCVGWHSRKRRWDENACETTLDIRNKVKCRCNYTNVVMSFSILMSPKSMDDKVLDYITCIGLSISILSLILCLIIEATVWSRVVVTEISYMRHVCIVNIAVSLLTANVWFIIGSNFNKKAQDYNWCVAVTFFSHFFYLSLFFWMLFKALLIIYGILVVFRRMMKSRMMAIGFAIGYGCPLVIAVTTVAITVPEKGYMRPDACWLNWDNTKALLAFAIPALVIVAVNLIVVLVVAVNTQRPSIGSSKSQDVAIIMRISKNVAILTPLLGLTWGFGIATLIEGTSLIFHIIFALLNAFQGFFILLFGTIMDHKIRDALRMRMSSLKGKSRAAENASLSPTNGSKLMNR

SEQ ID NO: 294 - protein, 1346 aa, synthetic construct
MKSPRRTTLCLMFIVIYSSQATLNLNLESIVHPLILHEHEPAGEEALRQKRAVATSSPAAEEYTVDIEISFENASFLEPIKAYLNSLSFPIQGNSTDQITDILSIEVTTVCRPAGNEIWCSCETGYGWPRERCLHNLTCQEHDVFLPGHHCSCLKGLPPKGPFCQLQGDVTLRMSVRLNVGFQEDLMNTSSALYRSYKTDLETAFRKGYSILPGFKGVTVTGFRPGSVVVTYEVKTTTPSPELMHKANEQVVQNLNQTYKMDYNSFQAVTSNETKFFVTPEIIFEGDTVSLVCENEVLSSNVSWHHVERQLDIQNSSRFSIYTAVLNNMTSVSKLTIYNITPGDAGEYICKLILDIFEYESRKKIDVMPIRILANEEMKVMCDNNPVSLNCCSEGNVNWSKVEWKQEGKINIPGNPETDIDSSCSRYTLKADGTQCPSGSSGTTVVYTCEFISAHGARGSKNIKVTFTSVANLTITPDPISVSEGQNFSIKCISDVSNYDEVYWNTSAGIKIYQRFYTTRRYLDGAESVLTVKTSTREWNGTYHCIFRYKNSYSIATKDVTVHPLPLELNIMVDPLEATVSCSGSHHFKCCIEEDEDYKVTFQMDSLSFPAEKEVNGKQVCYKHNFNASSVSWCSKTVDVFCHFTNAANNSVWSPSMKLNLVPGENITCQDPVIGVGEPGKVIQKLCQFSNVPSSPGSPIGGIITYKCVGSQWEVKRNDCISAPINSLLQLAKALIKSPSQDEKLPTYLKDLSISTDKVKHEISSSPGSLGAIINILDLLSTVPTQVNSEMMTHVLSTVNVILGKPVLSTWKVLQQQQTNQSSQLLHSVERFSQALQSGDSPPLSFSQTNVQMSSMVIKSGHPKTYQQRFVFSDSDLWGNVVIDKCYLENLQSDSSIVTVAFPTLQAILAQDIQEKNFANSLVMTTTVSHNITMPFRISMTFKNNSPSGGEPKCVFWNFRLANNTGGWDSSGCYVEEVDGDSVTCICDHLTSFSILMSPDSPDPGSLLGILLDIISYIGLGFSILSLAACLVVEAVVWKSVTKNRTSYMRHTCIVNIAASLLVADTWFIVAAAIQDNRYILCKTACVAATFFIHFFYLSVFFWMLTLGLMLFYRLVFILHDTSKSIQKAIAFSLGYGCPLAISVITVGATQPQEVYTRKNACWLNWEDTKALLAFVIPALIIVVVNITITVVVITKILRPSIGDKPCKQEKSSLFQISKSIGVLTPLLGLTWGFGLATVFQGSNAVFHIIFTLLNAFQGLFILLFGCLWDQKVQEALLNKFSLSRWSSQHSKSTSLGSSTPVFSMSSPISRRFNNLFGKTGTYNVSTPETTSSSLENSSSAYSLLN

SEQ ID NO: 295 - protein, 687 aa, synthetic construct
MAAQVLLQTTLFLLGLLFLVQGAHGRGHREDFRFCGQRNQTHRSSLHYKPTPDLHISIENSEEALTVHAPFPAAHPASRSFPDPRGLYHFCLYWNRHAGRLHLRYGKRDFLLSDQASSLLCFRHQEESLAQGPPLFATSVSSWWSPQNTSLPSAAGFTFSFHSPPHKASHNASVDMCELKRDLQLLSQFLKHPQKASRRPSATPASQQLQSLESKLTSVRFMGDTVSFEEDRVNATVWKLQPTASLQDLHIHSRQEEEQSEILEYSVLLPRTLFQKTKGRRGEAEKRLLLVDFSSQALFQDKNSSQVLGEKVLGIVVQNTKVANLSEPVVLTFQHQPQPKNVTLQCVFWVEDPTLSSPGSWSDAGCETIRRETQTSCLCNHLTYFAVLMVSSVEVDAVHKHYLTLLSYVGCVISALACVLTIAAYLCSRRKPRDYTIKVHMNLLLAVFLLDVSFLLSEPVALTGSEAGCRASAIFLHFSLLACLSWMGLEGYNLYRLVVEVFGTYVPGYLLKLSIVGWGFPIFLVTLVALVDVNNYGPIILAVHRTPESVIYPSMCWIRDSLVSHVTNLGLFSLVFLFNMAMLGTMVVQILRLRPHTQKWPHVLTLLGLSLVLGLPWALVFFSFASGTFQLVVLYFFSIITSFQGFLIFLWYWSMRLQARGGPSPLKSSSDSARLPISSGSTSSSRI

SEQ ID NO: 296 - protein, 1014 aa, synthetic construct
MVFSGRQCGHVGRTEEVLLTFKIFLVIICLHVVLVTSLEEDTDNSSLSPPPAKLSVVSFAPSSNEVETTSLNDVTLSLLTLNKTEKTKITIVKTFNASGVKPQRNICNLSSICNDSAFFRGEIMFQYDKESTIPQNQHITNGTLTGVLSLSELKRSELNKTLQTLSETYFIMCATAEAQSTLNCTFTIKLNNTMNACAVIAALERVKIRPMEHCCCSVRTPCPSSPEELEKLQCDLQDPIVCLADHPRGPPFSSSQSIPVVPRATVLSQVPKATSFAEPPDYSPVTHNVPSPIGEIHPLSPQPSAPIASSPAIDMPPQSETISSPMPQTHVSGTPPPVKASFSSPTVSAPANVITTSAPPVQTDIVNTSSISDLENQVSQMEKALSLGSLEPNLAGEMINQVSKLLHSPPDMLAPLAQRLLKVVDDIGLQLNFSNKTISLTSPSLALAVIRVNASSFNTTTFVAQDPANLQVSLETQAPENSIGTITLPSSLMNNLPANDMELASRVQFNFFETPALFQDPSLENLSLISYVISSSVANLTVRNLTRNVTVTLKHINPSQDELTVRCVFWDLGRNGGRGGWSDDGCSVKDRRLNETICTCSHLTSFGVLLDLSRTSVLPAQTMALTFITYIGCGLSSIFLSVTLVTYIAFEKIRRDYPSKILIQLCAALLLLNLVFLLDSWIALYKMQGLCISVAVFLHYFLLVSFTWMGLEAFHMYLALVKVFNTYIRKYILKFCIVGWGVPAVVVTIILTISPDNYGLGSYGKFPNGSPDDFCWINNNAVFYITVVGYFCVIFLLNVSMFIVVLVQLCRIKKKKQLGAQRKTSIQDLRSIAGLTFLLGITWGFAFFAWGPVNVTFMYLFAIFNTLQGFFIFIFYCVAKENVRKQWRRYLCCGKLRLAENSDWSKTATNGLKKQTVNQGVSSSSNSLQSNSNSTNSTTLLVNNDCSVHASGNGNASTERNGVSFSVQNGDVCLHDFTGKQHMFNEKEDSCNGKGRMALRRTSKRGSLHFIEQM

SEQ ID NO: 297 - protein, 3018 aa, synthetic construct
MSSFIFLSTLSLKGKKLDFFGRGDTYVSLINTIPELSRFTACIDLVFMDDNSRYWMAFSYITNNALLGREDIDLGLAGDHQQLILYRLGKTFSIRYHLAPFQWHTICLIWDGVKGRLELFLNKERILEVMDQPHNLTPNGTLVLGHFLKNESSEVKSMMPSFPGSLYYFQLWDHILENEEFMKCLDGNVVSWEEDVWLVNKIIPTVDRTLRCFVSENMTIQEKSTTVSQQILTTPSQITGLKPQKTAHSSTLLSQSIPIFATDYTTISYSNTTSPPLETMTAQKILKTLVDETATFAVDVLSTSSAISLPTQSTSIDNTTNSMKKTKSPSSESTKTTKMVEAMATEIFQPPTATNFLSTSRFTKNSVVSTTSAIKSQSAVTKTTSLFSTIESTSMSTTSCLKQKSTNTGALPISTAGQEFLESTAAGTVPWFTVEKTSPASTHVGTASSFPPESVLISTAAPVDSVFPRNQTASTLATTDMKIAFTVHSLTLIETTPAPRTAETELTSTNFQDVSSPRVEDAMSTSMPKETSSKTLSFLTSSSFTGTQSVQTVIDAEATHTALTPEITLAPTVAETMLSSTITGRVYTQNTPTADGHMLTLMSTRSASTSKAPESGPTSTTDEAAHLFSTNETIWTSRPDQTLLTSAFHESTTNTEHSTTTNIITPLEASPEGKGTTANDATTARYTTALSKLTSPWFANFSIVSGTTSITNMPEFKLTTLLLKTIPMSTKPANELPSTPRETVVPSVDIISTLACIQPNFSTEESASETTQTEINGAIVFGGTTTPVPKSATTQRLNATVTRKETTSHLMGKSTIAAVAEVSPFSTMLEVTDESAQMVTASVTVSPFPDIEKLTTPLDNKTATTEVRESWLSTKLVKTTPRSSYNETTEMFNSTHTYVAHWTSETSEGNSAGSPTSGSTHIFGEPLGASTTRISETSFSTTPTDRTATSLSDGILPPQPTAAHSSATPVPVTHMFSGSEPSTRAFTSVLSNLSSTTMTTALVPPLDQTASTTSVIVPTHGDSIRTTSEATVISVRKTSMAVPSLTETPFPSLRLSTPVTAKAETTLFSTSVDTVTPSTHTLVCSKPPPDIPPASSTHVISTTSTPEATQPISQVEETSTYALSFPYTFSGGGDVASLATGTTETSVVDETTPSHISANKLTTSVNSHISSSATYRVHTPSTQLVTSTSVLSSDKDQMTISLGKTPRTMEVTEMSPSKNSFISYSRGTPSLEMTDTGFPETTKISSHQTHSPSEIPLGTPSDGNLASSPTSGSTQITPTLTSSNTVGVHIPEMSTSLGKTALPSQALTITTFLSPEKESTSALPAYTPRTVEMIVNSTYVTHSVSYGQDTSFVDTTTSSTTRISNPMDINTTFSHLHSRTQPEVTSVASFISESTQTFPESLSLSTAGLYNDGFTVLSDRITTAFSVPNVPTMLPRETSMATSTPIYQMSSLPVNVTAFTSKKVSDTPTILITKSSKTMHPGCLKSPSTATSGPMSEMSSMPVNNSAFTPATVSSDTSTRVGLFSTLLSSVTPRTTMTMQTSTLDVTPVIYAGATSKNKMVSSAFTTEMIEVPSRITPTTFSSPTEPTFPSVKTIPTTIMAGIVTPFVGTTAFSLLSSKNTEAISSIPKTTFSPFLSTTQQSSQADEATTLGILSGITNRSLSTVNSGTGTALTNTYSRTTVPENMLSPTHSDSLHTSFNIQVSPSLTSFKSTSGPTKNVKTTTYLSSNTRKMTSLSEKTLTNYATSLNTPVSYPPWTPSSATPPSLTSFLYSPHSTEAEFSTPKTSPPPTSQMVEFPVLGTRMTSSNTQPLLMTSWNIPTAEGSQFPISTTIHVPTSNEMETETLHLVPGPLSTFTASQTGLVSKDVMAMSSIPMSGILPTHGLSENPSLSTSLRAITSTLADVKHTFEKMTTSVTPGTTLPSILSSVISKATTSPILTWLLSSLPSGSPLATVSNAPHVMTSSTVEVSKSTFLTSDMISAHPFTNLTTLPSATMSTILTRTIPTPTLGGITTGFPTSLPMSIKVTDDIVYISTHPEASSRTTVTANPRTVSHPSSFSRKTMSPSTTDHTLSVGSMPLPSSTITSSWSRIPAASSPSTLIIPKPTLDSLLNIMTTTSTVPGASFPLISTGVTHPSTATVSSLISSSFETTWLDSTPSFLSTEASTSPTATKSTVSFYNVEMSFSVFDEEPRIPITSVINEFTENWLNSIFQNSEFSLANLETQIKSRDISEEEMVMDRAIQREGQEMATISYVPYSCVCQVIIKASSSLASSELISKIKSKIHGNFTHGNFTQDQLTLLVKSEHVAVKKLEPGNCKADETASKYKGTYKWLLTNPTETAQTRCIKNEDGNATRICSISINTGKSQWEKPKFKQCKLLQELPDKIVDLANITISDENAEDVAEHILNLINESPALDEEETKIIVSKVSDISQCDEISMNLTQVILQIINVVLEKQNNSASDLHEVSNEILRIIERTGHKMEFSGRIANLTVAGLALAVLRVDHTFEGMAFSIHSYEEGTDPEIFLGNVPVGGILASIYLPKSLTERIPLSNLQTILFNFFGQTSLFKTKNVTKALTTYVVSASISDMSIQNLADPVVITLQHIGGNQNYDQVHCAFWDFENNNGLGGWNSSGCKVKETNVNYTICQCDHLTHFGVLMDLSRSTVDAVNERILVLITYTGCGISSIFLGVAVVTYIAFHKLRKDYPSKILINLCTALLMLNLVFLVNSWLSSFQKVGLCITAAVALHYFLLVSLTWMGLEAVHMYFALVKVFNIYIPNYILKFCLVGWGIPAIMVAITLSVKKDLYGTLSPTTPFCWIKDDSIFYISVVAYFCLIFLMNLSMFCTVLVQLNSVKSQSQKTRRKMILHDLKGTMSLTFLLGLTWGFAFFAWGPVRIFFLYLFAIFNTLQGFLIFVFHCVMKESVREQWQIHLCCGWLRLDNSSDGSSRCGIKVGYKQEGLKKTFEHKLLTPSLKSTATSSTFKSLGSAQGTPSEISFPNDDFDKDPYCSSPLSCEVVPNC

SEQ ID NO: 298 - protein, 520 aa, synthetic construct
MDHCGALFLCLCLLTLQSATTETSQELLSWMENMEMAGRSSVFSSDQIHQLEQMLLNASFPGYNLTLQTPTIQSLAFKLGCDFSGLSLSSATLKRVPQAGQHAMQFPAELTRDACRTTRPRELRLICIYFSTTHFFQDENNSSLLNNYVLGAQLSHGHVNNLREPVNISFWHNQSLEGYTVTCVFWKEGASKQPWGGWSPEGCRTEQPSPSQVLCRCNHLTYFAVLMQLSPAPVPAELLAPLTYISLVGCSISIVASLLTVLLHFHARKQSDSLTRIHMNLHASVLLLNVAFLLSPAFAMPPVPGSACTALAAALHYALLSCLTWMAIEGFNLYLLLGRVYNIYIRRYVLKLCALGWGVPALLVLLLLSVKSSVYGPCTIPVSDSQENGTGFQNMSICWVRSPVVHSVLVMGYGGLTSLFNLVVLAWALRTLRRLRARAKAPSVRACRDTVTVLGLTVLLGTTWALAFFSFGVFLLPQLFLFTIFNSLYGFFLFLWFCSQRCRSEAEAEMEAFSSSQTTQ

SEQ ID NO: 299 - protein, 1193 aa, synthetic construct
MMFRSDRMWSCHWKWKPSPLLFLFALYIMCVPHSVWGCANCRVVLSNPSGTFTSPCYPNDYPNSQACMWTLRAPTGYIIQITFNDFDIEEAPNCIYDSLSLDNGESQTKFCGATAKGLSFNSSANEMHVSFSSDFSIQKKGFNASYIRVAVSLRNQKVILPQTSDAYQVSVAKSVSIPELSAFTLCFEATKVGHEDNDWTAFSYSNASFTQLLSFGKAKSGYFLSISDSKCLLNNALPVKEKEDIFAESFEQLCLVWNNSLGSIGVNFKRNYETVPCDSTISKVIPGNGKLLLGSNQNEIVSLKGDIYNFRLWNFTMNAKILSNLSCNVKGNVVDWQNDFWNIPNLALKAESNLSCGSYLIPLPAAELASCADLGTLCQDGIIYRISVVIQNILRHPEVKVQSKVAEWLNSTFQNWNYTVYVVNISFHLSAGEDKIKVKRSIENEPRLVLWALLVYNATNNTNLEGKIIQQKLLKNNESLDEGLRLHTVNVRQLGHCLAMEEPKGYYWPSIQPSEYVLPCPDKPGFSASRICYYNATNPSVAYWGPPDISNCSKEANEVANQILNLTADGQNLTSANITNIVEQVKRIVNKEENIDITLGSTLMNIFSNILSSSDSDLLESSSEALKTIDELAFKIDLNSTSHVNITTRNLALGVSSLLPGTNAISNFSIGLPSNNESYFQMDFESGQVDPLASVILPPNLLENLSQEDSVLVRRAQFTFFNKTGLFQDVGPQRKTLVSYVMACSIGNITIQNLKDPVQIKIKHTRTQEVHHPICAFWDLNKNKSFGGWNTSGCVAHRDSDASETVCLCNHFTHFGVLMDLPRSASQLDARNTKVLTFISYIGCGISAIFSAATLLTYVAFEKLRRDYPSKILMNLSTALLFLNLLFLLDGWITSFNVDGLCIAVAVLLHFFLLATFTWMGLEAIHMYIALVKVFNTYIRRYILKFCIIGWGLPALVVSIVLASRNNNEVYGKESYGKEKGDEFCWIQDPVIFYVTCAGYFGVMFFLNIAMFIVVMVQICGRNGKRSNRTLREEVLRNLRSVVSLTFLLGMTWGFAFFAWGPLNIPFMYLFSIFNSLQGLFIFIFHCAMKENVQKQWRRHLCCGRFRLADNSDWSKTATNIIKKSSDNLGKSLSSSSIGSNSTYLTSKSKSSSTTYFKRNSHTDNASMDKSFSKLGHADGCQTSIIPVHQGYC

SEQ ID NO: 300 - protein, 794 aa, synthetic construct
MASCRACNLRVLVAIVCGLLTAIVLGLGIWRIVIRIQRTSTSSSSTPIEFCRNGGTWENGRCICPEEWKGLRCTIANFCENSTYMGFTFARIPVGRYGPSLQTCDKNTLNAGNPIATRLCNLSEYGEIELQNVTIGNCNENLETLEKQIVNISTQNNISSEAQILTSDASKLTPENITSATMVVGQIFNTSRNASPEAKELAVTTVSQLLDASEDVFQRAAAADNDDTFTTLIEQMETYSLSLGNESVVEPNIAIQSVNFSSEGTVGSTSVLFSVQKGTSDSLVSGSTSVDTNVDGLNPDGQTELQILLNTSKSTKACGFVVYQNDKLFQSKTFTAKSDFSQKIISSKTDENEQQSASVDMVFSPKYNQKEFQLHSYACVYWNFSAKDWDTYGCQKDKGTDGFLRCRCNHTTNFAVLMSFKKDYKYPESLDILSNVGCALSITGLALTIIFQIVTRKVRKTSVTWVLVSLCTSMLIFNLLFVFGIENSNKNLKTSDGDINNIDFDNNEIPRTDTVVIPNPMCTAIAALLHYFLLVTFTWNGLSAAQLYFLLIRTMKPLPQHFILFISLIGWGVPAIVVAITVGIIYSQNGNNSQWELDYRQEEICWLAIPEPNGVIKSPLLWSFIVPVTIILISNIVIFIIISVKVLWKNNQNLTSTKKVSSLKKILSTLSIAVVFGITWILAYLMLINNDSIRIIFSYIFCLFNTTQGLQIFILYTVRTKIFQSEASKVLKSLSSSIGRVKSLPSTRPLRLRVRMYNMLRSLPALHERFRLLEPSPSTEEITLSESDQAKESI

SEQ ID NO: 301 - protein, 1472 aa, synthetic construct
MARLAAVLWSLCVTAVLVTSATQGLSRAGLPFGLMRRELACEGYPIELRCPGSDVIMVENANYGRTDDKICDADPFQMENVQCYLPDAFKIMSQRCNNRTQCVVVAGSDAFPDPCPGTYKYLEVQYDCVPYVEQKVFVCPGTLQKVLEPTSTHESEHQSGAWCKDPLQAGDRIYVMPWIPYRTDTLTEYASWEDYVAARHTTTYRLPNRVDGTGFVVYDGAVFYNKERTRNIVKYDLRTRIKSGETVINTANYHDTSPYRWGGKTDIDLAVDENGLWVIYATEGNNGRLVVSQLNPYTLRFEGTWETGYDKRSASNAFMVCGVLYVLRSVYVDDDSEAAGNRVDYAFNTNANREEPVSLAFPNPYQFVSSVDYNPRDNQLYVWNNYFVVRYSLEFGPPDPSAGPATSPPLSTTTTARPTPLTSTASPAATTPLRRAPLTTHPVGAINQLGPDLPPATAPAPSTRRPPAPNLHVSPELFCEPREVRRVQWPATQQGMLVERPCPKGTRGIASFQCLPALGLWNPRGPDLSNCTSPWVNQVAQKIKSGENAANIASELARHTRGSIYAGDVSSSVKLMEQLLDILDAQLQALRPIERESAGKNYNKMHKRERTCKDYIKAVVETVDNLLRPEALESWKDMNATEQVHTATMLLDVLEEGAFLLADNVREPARFLAAKQNVVLEVTVLNTEGQVQELVFPQEYPSENSIQLSANTIKQNSRNGVVKVVFILYNNLGLFLSTENATVKLAGEAGPGGPGGASLVVNSQVIAASINKESSRVFLMDPVIFTVAHLEAKNHFNANCSFWNYSERSMLGYWSTQGCRLVESNKTHTTCACSHLTNFAVLMAHREIYQGRINELLLSVITWVGIVISLVCLAICISTFCFLRGLQTDRNTIHKNLCINLFLAELLFLVGIDKTQYEIACPIFAGLLHYFFLAAFSWLCLEGVHLYLLLVEVFESEYSRTKYYYLGGYCFPALVVGIAAAIDYRSYGTEKACWLRVDNYFIWSFIGPVSFVIVVNLVFLMVTLHKMIRSSSVLKPDSSRLDNIKSWALGAIALLFLLGLTWAFGLLFINKESVVMAYLFTTFNAFQGVFIFVFHCALQKKVHKEYSKCLRHSYCCIRSPPGGAHGSLKTSAMRSNTRYYTGTQSRIRRMWNDTVRKQTESSFMAGDINSTPTLNRGTMGNHLLTNPVLQPRGGTSPYNTLIAESVGFNPSSPPVFNSPGSYREPKHPLGGREACGMDTLPLNGNFNNSYSLRSGDFPPGDGAPEPPRGRNLADAAAFEKMIISELVHNNLRGSSSGAKGPPPPEPPVPPVPGGGGEEEAGGPGGADRAEIELLYKALEEPLLLPRAQSVLYQSDLDESESCTAEDGATSRPLSSPPGRDSLYASGANLRDSPSYPDSSPEGPSEALPPPPPAPPGPPEIYYTSRPPALVARNPLQGYYQVRRPSHEGYLAAPGLEGPGPDGDGQMQLVTSL

SEQ ID NO: 302 - protein, 1403 aa, synthetic construct
MVSSGCRMRSLWFIIVISFLPNTEGFSRAALPFGLVRRELSCEGYSIDLRCPGSDVIMIESANYGRTDDKICDADPFQMENTDCYLPDAFKIMTQRCNNRTQCIVVTGSDVFPDPCPGTYKYLEVQYECVPYIFVCPGTLKAIVDSPCIYEAEQKAGAWCKDPLQAADKIYFMPWTPYRTDTLIEYASLEDFQNSRQTTTYKLPNRVDGTGFVVYDGAVFFNKERTRNIVKFDLRTRIKSGEAIINYANYHDTSPYRWGGKTDIDLAVDENGLWVIYATEQNNGMIVISQLNPYTLRFEATWETVYDKRAASNAFMICGVLYVVRSVYQDNESETGKNAIDYIYNTRLNRGEYVDVPFPNQYQYIAAVDYNPRDNQLYVWNNNFILRYSLEFGPPDPAQVPTTAVTITSSAELFKTTVSTTSTTSQKGPMSTTVAGSQEGSKGTKPPPAVSTTKIPPVTNIFPLPERFCEALDSRGIKWPQTQRGMMVERPCPKGTRGTASYLCMVSTGTWNPKGPDLSNCTSHWVNQLAQKIRSGENAASLANELAKHTKGPVFAGDVSSSVRLMEQLVDILDAQLQELKPSEKDSAGRSYNKAIVDTVDNLLRPEALESWKHMNSSEQAHTATMLLDTLEEGAFVLADNLLEPTRVSMPTENIVLEVAVLSTEGQIQDFKFPLGIKGAGSSIQLSANTVKQNSRNGLAKLVFIIYRSLGQFLSTENATIKLGADFIGRNSTIAVNSHVISVSINKESSRVYLTDPVLFTLPHIDPDNYFNANCSFWNYSERTMMGYWSTQGCKLVDTNKTRTTCACSHLTNFAILMAHREIAYKDGVHELLLTVITWVGIVISLVCLAICIFTFCFFRGLQSDRNTIHKNLCINLFIAEFIFLIGIDKTKYAIACPIFAGLLHFFFLAAFAWMCLEGVQLYLMLVEVFESEYSRKKYYYVAGYLFPATVVGVSAAIDYKSYGTEKACWLHVDNYFIWSFIGPVTFIILLNIIFLVITLCKMVKHSNTLKPDSSRLENIKSWVLGAFALLCLLGLTWSFGLLFINEETIVMAYLFTIFNAFQGVFIFIFHCALQKKVRKEYGKCFRHSYCCGGLPTESPHSSVKASTTRTSARYSSGTQSRIRRMWNDTVRKQSESSFISGDINSTSTLNQGHSLNNARDTSAMDTLPLNGNFNNSYSLRKGDYNDSVQVVDCGLSLNDTAFEKMIISELVHNNLRGSSKTHNLELTLPVKPVIGGSSSEDDAIVADASSLMHSDNPGLELHHKELEAPLIPQRTHSLLYQPQKKVKSEGTDSYVSQLTAEAEDHLQSPNRDSLYTSMPNLRDSPYPESSPDMEEDLSPSRRSENEDIYYKSMPNLGAGHQLQMCYQISRGNSDGYIIPINKEGCIPEGDVREGQMQLVTSL

SEQ ID NO: 303 - protein, 1240 aa, synthetic construct
MWPSQLLIFMMLLAPIIHAFSRAPIPMAVVRRELSCESYPIELRCPGTDVIMIESANYGRTDDKICDSDPAQMENIRCYLPDAYKIMSQRCNNRTQCAVVAGPDVFPDPCPGTYKYLEVQYECVPYKVEQKVFLCPGLLKGVYQSEHLFESDHQSGAWCKDPLQASDKIYYMPWTPYRTDTLTEYSSKDDFIAGRPTTTYKLPHRVDGTGFVVYDGALFFNKERTRNIVKFDLRTRIKSGEAIIANANYHDTSPYRWGGKSDIDLAVDENGLWVIYATEQNNGKIVISQLNPYTLRIEGTWDTAYDKRSASNAFMICGILYVVKSVYEDDDNEATGNKIDYIYNTDQSKDSLVDVPFPNSYQYIAAVDYNPRDNLLYVWNNYHVVKYSLDFGPLDSRSGQAHHGQVSYISPPIHLDSELERPPVRDISTTGPLGMGSTTTSTTLRTTTWSPGRSTTPSVSGRRNRSTSTPSPAVEVLDDMTTHLPSASSQIPALEESCEAVEAREIMWFKTRQGQIAKQPCPAGTIGVSTYLCLAPDGIWDPQGPDLSNCSSPWVNHITQKLKSGETAANIARELAEQTRNHLNAGDITYSVRAMDQLVGLLDVQLRNLTPGGKDSAARSLNKLQKRERSCRAYVQAMVETVNNLLQPQALNAWRDLTTSDQLRAATMLLDTVEESAFVLADNLLKTDIVRENTDNIQLEVARLSTEGNLEDLKFPENMGHGSTIQLSANTLKQNGRNGEIRVAFVLYNNLGPYLSTENASMKLGTEAMSTNHSVIVNSPVITAAINKEFSNKVYLADPVVFTVKHIKQSEENFNPNCSFWSYSKRTMTGYWSTQGCRLLTTNKTHTTCSCNHLTNFAVLMAHVEVKHSDAVHDLLLDVITWVGILLSLVCLLICIFTFCFFRGLQSDRNTIHKNLCISLFVAELLFLIGINRTDQPIACAVFAALLHFFFLAAFTWMFLEGVQLYIMLVEVFESEHSRRKYFYLVGYGMPALIVAVSAAVDYRSYGTDKVCWLRLDTYFIWSFIGPATLIIMLNVIFLGIALYKMFHHTAILKPESGCLDNINYEDNRPFIKSWVIGAIALLCLLGLTWAFGLMYINESTVIMAYLFTIFNSLQGMFIFIFHCVLQKKVRKEYGKCLRTHCCSGKSTESSIGSGKTSGSRTPGRYSTGSQSRIRRMWNDTVRKQSESSFITGDINSSASLNREPYRETSMGVKLNIAYQIGASEQCQGYKCHGYSTTEW

SEQ ID NO: 304 - protein, 739 aa, synthetic construct
MKLLPLLVGFSTLLNCSYTQNCTKTPCLPNAKCEIRNGIEACYCNMGFSGNGVTICEDDNECGNLTQSCGENANCTNTEGSYYCMCVPGFRSSSNQDRFITNDGTVCIIDECSESAACGDHAVCENVDGGYNCSCKEGYQTSTGKSQFTPNDGTYCQENVNANCHLDNACIAANINKTLTKIRSIKEPVALLQEVYRNSVKDLSPMDIITYIEILAESSPLLGYMNSTNSAKDTLSNSTLTEFVKTVNNFVQKDTFIVWDKLSTNHRRTHLTKLMHTAEQATLRISQNFQKTTQFDTNSSDIALKVFFFDSYHMKHIHPHMNVDGDYIKIFPKRKAAYDSNGNVAVAFLYYKSIGPLFSSSDNFLLEPQSYDNSEEEERVISSVISVSISSNPPTLYELEKITFTLSHRKTTDKYRSQCAFWNYSPDTMNGSWSSEGCELTYSNETHTSCRCNHLTHFAILMSSGPSIGIKDYNILTRITQLGIIISLICLAICIFTFWFFSEIQSTRTTIHKNLCCSLFLAELVFLVGINTNTNKLFCSIIAGLLHYFFLAAFAWMCIEGIHLYLIVVGVIYNKGFLHKNFYIFGYLSPAVVVGFSASLGYRYYGTTKVCWLSTENNFIWSFIGPACLIILVNLLAFGVIIYKVFRHTAGLKPEVSCYENIRSCARGALALLFLLGTTWIFGVLHVVHASVVTAYLFTVSNAFQGMFIFLFLCVLSRKIQEEYYRLFKNVPCCFGCLR

SEQ ID NO: 305 - protein, 482 aa, synthetic construct
MANFTPVNGSSGNQSVRLVTSSHNRYKTVEMVFIATVTGSLSLVTVVGNILVMLSIKVNRQLQTVNNYFLFSLACADLIIGVFSMNLYTVYIIKGYWPLGAVVCDLWLALDYVVSNASVMNLLIISFDRYFCVTKPLTYPARRTTKMAGLMIAAAWILSFILWAPAILFWQFIVGKRTVPDNECYIQFLSNPAVTFGTAIAAFYLPVVIMTVLYIHISLASRSRVHKHKPEGPKEKKAKTLAFLKSPLMKQNNNKPPKRSLEAAREEVRNGKVEEAPPPALPPPPRPQEEKETSNESSTGSATQNTKERPASTEATPPAMPAPPLQPRALNPASKWSKIKIVTKQTGNECVTAIEIVPATPASERNSLGMRRPANVARKFASIARSQVRKKRQMAAREKKVTRTIFAILLAFILTWTPYNVMVLINTFCQSCVPDTVWSIGYWLCYVNSTINPACYALCNATFKKTFKHLLMCQYRNIGTAR

SEQ ID NO: 306 - protein, 396 aa, synthetic construct
MRSPSAAWLLGGAILLAASLSCSGTIQGTNRSSKGRSLIGKVDGTSHVTGKGVTVEPGFSVDEFSASVLTGKLTTVFLPIVYTIVFVIGLPSNGMALWVFLFRTKKKHPAVIYMANLALADLLSVIWFPLKIAYHIHGNNWIYGEALCKVLIGFFYGNMYCSILFMTCLSVQRYWVIVNPMVHPRKKANIAIGVSLGIWLLILLVTIPLYVVKQTIYIPALNITTCHDVLPEEVLVGDMFNYFLSLAIGVFLFPAFLTASAYVLMIRTLRSSAMDENSEKKRKRAIKLIVTVLAMYLICFTPSNLLLVVHYFLIKSQGQSHVYALYIVALCLSTLNSCIDPFVYYFVSQDFRDHAKNALLCRSVRTVKRMQVSLTSKFSRKSSSYSSSSTSVKTSY

SEQ ID NO: 307 - protein, 1207 aa, synthetic construct
MVLLLILSVLLLKEDVRGSAQSSERRVVAHMPGDIIIGALFSVHHQPTVDKVHERKCGAVREQYGIQRVEAMLHTLERINSDPTLLPNITLGCEIRDSCWHSAVALEQSIEFIRDSLISSEEEEGLVRCVDGSSSSFRSKKPIVGVIGPGSSSVAIQVQNLLQLFNIPQIAYSATSMDLSDKTLFKYFMRVVPSDAQQARAMVDIVKRYNWTYVSAVHTEGNYGESGMEAFKDMSAKEGICIAHSYKIYSNAGEQSFDKLLKKLRSHLPKARVVACFCEGMTVRGLLMAMRRLGLAGEFLLLGSDGWADRYDVTDGYQREAVGGITIKLQSPDVKWFDDYYLKLRPETNLRNPWFQEFWQHRFQCRLEGFAQENSKYNKTCNSSLTLRTHHVQDSKMGFVINAIYSMAYGLHNMQMSLCPGYAGLCDAMKPIDGRKLLDSLMKTNFTGVSGDMILFDENGDSPGRYEIMNFKEMGKDYFDYINVGSWDNGELKMDDDEVWSKKNNIIRSVCSEPCEKGQIKVIRKGEVSCCWTCTPCKENEYVFDEYTCKACQLGSWPTDDLTGCDLIPVQYLRWGDPEPIAAVVFACLGLLATLFVTAVFIIYRDTPVVKSSSRELCYIILAGICLGYLCTFCLIAKPKQIYCYLQRIGIGLSPAMSYSALVTKTNRIARILAGSKKKICTKKPRFMSACAQLVIAFILICIQLGIIVALFIMEPPDIMHDYPSIREVYLICNTTNLGVVTPLGYNGLLILSCTFYAFKTRNVPANFNEAKYIAFTMYTTCIIWLAFVPIYFGSNYKIITMCFSVSLSATVALGCMFVPKVYIILAKPERNVRSAFTTSTVVRMHVGDGKSSSAASRSSSLVNLWKRRGSSGETLRYKDRRLAQHKSEIECFTPKGSMGNGGRATMSSSNGKSVTWAQNEKSSRGQHLWQRLSIHINKKENPNQTAVIKPFPKSTESRGLGAGAGGAGGVGATGGAGCAGAGGPEPPDAGPKALYDVAEAEEHFPAPARPRSPSPISTLSHRAGSASRTDDDVPSLHSEPAARSSSSQGSLMEQISSVVTRFTANISELNSMMLSTAAPGPGVGAPLCSSYLIPKEIQLPTTMTTFAEIQPLPAIEVTGGAQPAAGAPPAGGAARESPAAGPEAAAGKPDLEELVALTPPSPFRDSVDSGSTTPNSPVSESALCIPSSPKYDTLIIRDYTQSSSSL

SEQ ID NO: 308 - protein, 380 aa, synthetic construct
MEEGGDFDNYYGADNQSECEYTDWKSSGALIPAIYMLVFLLGTTGNGLVLWTVFRSSREKRRSADIFIASLAVADLTFVVTLPLWATYTYRDYDWPFGTFACKLSSYLIFVNMYASVFCLTGLSFDRYLAIVRPVANARLRLRVSGAVATAVLWVLAALLAMPVMVFRTTGDLENTTKVQCYMDYSMVATVSSEWAWEVGLGVSSTAVGFVVPFTVMLTCYFFIAQTIAGHFRKERIEGLRKRRRLLSIIVVLVVTFALCWMPYHLVKTLYMLGSLLHWPCDFDLFLMNVFPYCTCISYVNSCLNPFLYAFFDPRFRQACTSMLCCGQSRCAGTSHSSSGEKSASYSSGHSQGPGPNMGKGGEQMHEKSIPYSQETLVVD

SEQ ID NO: 309 - protein, 462 aa, synthetic construct
MEKKCILYFLVLLPFFMILVTAELEEHSPEDSIQLGVTRNKIMTAQYECYQKIMQDPIQQAEGVYCNRTWDGWLCWNDVAAGTESMQLCPDYFQDFDPSEKVTKICDQDGNWFRHPESNRTWTNYTQCNVNTHEKVKTALNLFYLTIIGHGLSIASLLISLGIFFYFKSLSCQRITLHKNLFFSFVCNSVVTIIHLTAVANNQALVATNPVSCKVSQFIHLYLMGCNYFWMLCEGIYLHTLIVVAVFAEKQHLMWYYFLGWGFPLIPACIHAVARSLYYNDNCWISSDTHLLYIIHGPICAALLVNLFFLLNIVRVLITKLKVTHQAESNLYMKAVRATLILVPLLGIEFVLIPWRPEGRIAEEVYDYIMHILMHYQGLLVSTIFCFFNGEVQAILRRNWNQYKIQFGNSFSHSDALRSASYTVSTISDVPGYSHDCPSEHLNGKSIHDIENVVLKPEKLYD

SEQ ID NO: 310 - protein, 527 aa, synthetic construct
MGIPAPWGTSPLSFHRKCSLWAPGRPFLTLLLLVSIKQVTGSLLEETTRKWAQYKEKCLRDLLKEPSGIFCNGTFDQYVCWPHSSPGNVSVPCPSYLPWWSEESSGRAYRHCLAQGTWQTLENSTDIWQDDSECSENHSFKQNVDRYALLSTLQLLYTVGYSLSLISLFLALTLLLFLRKLHCTRNYIHMNLFASFILRALAVLVKDVIFYNSYSKRPDNENGWMSYLSEMSTSCRSAQVLLHYFVGANYSWLLVEGLYLHTLLEPTVLSERRLWPRYLLVGWAFPVLFVVPWGIARAHLENTGCWGTNGNKKIWWIIRGPMLLCVTVNFFIFLKILKLLISKLKAHQMCFRDYKYRLAKSTLVLIPLLGVHEILFSFITDDQVEGFSKLIRLFIQLTLSSFHGLLVALQYCFANGEVKAELRKYWVRFLLARHSGCRAWVLGKNFRFLGKCPKKLSEGDGAEKLRKLQPSLNSGRLLHLAMRGLGELGARPQQGHAAWPRSSLSESSEGDFTLANTMEEILEESEI

SEQ ID NO: 311 - protein, 332 aa, synthetic construct
MNSTTHHGMHTSLHFWNRSSYGLHSNASESLGKGYSDGGCYEQLFVSPEVFVTLGVISLLENILVIVAIAKNKNLHSPMYFFICSLAVADMLVSVSNGSETIVITLLNSTDTDAQSFTVNIDNVIDSVICSSLLASICSLLSIAVDRYFTIFYALQYHNIMTVKRVGIIISCIWAACTVSGILFIIYSDSSAVIICLITMFFTMLALMASLYVHMFLMARLHIKRIAVLPGTGTIRQGANMKGAITLTILIGVFVVCWAPFFLHLIFYISCPQNPYCVCFMSHFNLYLILIMCNSIIDPLIYALRSQELRKTFKEIICCYPLGGLCDLSSRY

SEQ ID NO: 312 - protein, 376 aa, synthetic construct
MSGESMNFSDVFDSSEDYFVSVNTSYYYVLDSEMLLCSLQEVRQFSRLFVPIAYSLICVFGLLGNILVVITFAFYKKAKSMTDVYLLNMAIADILFVLTLPFWAVSHATGAWVFSNATCKLMKGIYAVNFNCGMLLLACISMDRYIAIVQATKSFRLRSRTLAHSKIICLVVWGLSVLISSSTFVFNQKYNTQGSDVCEPRYQTVSEPIRWKLLMLGLQLLFGFFIPLVFMIFCYTFIVKTLVQAQNSKRHKAIRVIIAVVLVFLACQIPHNMVLLVTAANLGRMNRSCQSEKLLGYTKNVTEVLAFLHCCLNPVLYAFIGQKFRSYFLKIMKDLWCVRRKYKSSGFSCSRRYSENFISRQTSETADNDNASSFTM

SEQ ID NO: 313 - DNA, 942 bp, synthetic construct
  source 1..942: mol_type = other DNA
atgcctttccccaactgcagcgcccctagcaccgtggtggagacagccgtggccgtgctgctgctgctggaatgtggcctgggactgctgggcaacgccgttgccctgtggaccttcttctttcggctgaaagtgtggaagccttacgccgtctacctgcttaatctggtgctggctgatctgctgctggctgcttgcctgccattcctggccgctttttacctgcggagcaagacctggcatctgggcagagtgggttgtcaggctctgctgttcctgctggacctgtcaagaggagtcggcgtggcctttctgaccgccgtcgccctcgacagatacctgcgcgtggtgcacccccggctgaaagtgaatctgctgtcccctagggccgcttggggaatcagcggcctggtgtggctgctgatggtggctctgacacacctgtccctgatcagcgagagcgccgagtgtccttctttctaccctagagacggctcttttagcatcatctggcaggaggccctctttttcctgcaattcgtgctgccattcggcctgatcctgttctgcaacgccggcattatccggaccctgcagaagcggctgagagatcctgacaagcagcctaagctgcaaagagcccaggccctggttacagtggtggtggtgctgttcgccctgtgcttcctgccttctttcctggccagagtcctgatggccatcttccggcagctgggcagctgcagagccttgtgcgccgtggtgcacaccagcgacgtgaccggcagcctgacctacctgcagagcgtgctcaaccccgtggtgtactgcttcagcaaccctgccttcagatcctcttatagaaaggtgttccacacactgcggggcagaggccaggccgccgaacctcccggcttcgaccccagagatagctacagctga

SEQ ID NO: 314 - DNA, 1005 bp, synthetic construct
  source 1..1005: mol_type = other DNA
atgaacagcacatgtatcgaggaacaacacgacctggaccactacctctttccaatcgtgtacatcttcgtgatcatcgtgtccatccccgctaatatcggctctctgtgtgtgtccttcctgcaggctaagaaagagaacgagctgggcatctacctgtttagcctgagcctttctgatctgctgtacgccctgaccctgcctctgtggatcgactacacctggaacaaagacaactggaccttcagccccgccctgtgcaagggcagcgccttcctgatgtacatgaacttctacagcagcaccgccttcctgacctgcatcgccgtggacagatacctggccgtcgtgtatcctctgaaattcttcttcctgcggaccagaagattcgcctttatggtcagcctgagcatctggatcctggaaaccattttcaacgccgttatcctgtgggaggacgagacagtggtggaatactgcgacgccgagaagtccaacttcaccctgtgctacgataagtaccccctggagaagtggcagatcaacctgaatctgttcagaacatgcaccggctacgccatccctctggtgatcatcctgatctgcaacagaaaggtgtaccaggctgttagacacaaccaggccacagagaacaaggaaaaaaagcggatcattaagctgctcgtgtctatcaccctgacattcgtgctgtgcttcaccccttttcatgtgatgctgctgattagaagcatcctggagcacgccgtgaaccacagcaagagcggcaagcagacctacaagatgtaccggatcaccgtggccctgacatctctgaactgcgtggctgatcctatcctgtattgttttgtgaccgagactggacggtacgacatgtggaatatcctgaagttctgcacaggaaggtgtaataccagccagagacagcggaagagaatcctgagcgtgtctacaaaggataccatggaactggaagtgctggagtga

SEQ ID NO: 315 - DNA, 1008 bp, synthetic construct
  source 1..1008: mol_type = other DNA
atgaacaacaatagcacctgtatccaaccatctatgatcagctctatggccctgcctattatctacatctttctgtgcatcgtgggactgttcggcaacagcctgagccagtgggtctttctgaccaagatcggaaagaagaccagcacccacatctatctggctcatctggtgaccgccaacctgcttgtgtgcagcgccatgcccttcatgagcatctacttcctgaaaggctttcaatgggaataccagtctgctcagtgcagagtggtgaacttcctgggcacactgtccatgcacgtgtccatgttcgtgtccctgctgattctcagctggatcgccatcagcagatacgccaccctgatgaaaaaagacagctctcaggagacaacaagctgctacgagaagatcttctacggccacctgctgaagaagttcagacagcccaacttcgcccgcaagctgtgtatctacatctggggcgtggtgctgggaatcatcatccctgtgattatctactacagcgtggtcgaggccacagagggcgaggaaagcctgtgctacaaccggcagatggaactgggcgccatgatctcccagatcgccggcctgatcggcaccacattcatcggcttcagcttcctggttgtgctgaccagctactactctttcgtgtcccacctgagaaagatccggacatgtacctctatcatggaaaaggacctgacatacagcagcgtgaagcggcacctgctggtgatccagattctgctgatcgtgtgcttcctgccttactcaatcttcaagcctatcttttacgtgctgcaccagagagatgactgccagcagctgaactacctgatcgagatcaagaacatcctgacctgcctggccagcgctagaagctctactgatcctatcatcttcctgctgctcgacaagacctttaagaaaaccctttataatctgttcaccaagagcaatagccacatgcagagctacggctga

SEQ ID NO: 316 - DNA, 1002 bp, synthetic construct
  source 1..1002: mol_type = other DNA
atgaccaacagcacctctggcggcagcctgctgctgctgtgtgaaagctgggccggcaggaggatccccgtgagcctgctgtacagcggcctggccatcggcggaacactggctaatggcatggtgatctacctggtgtccagctttagaaagctgcagaccaccagcaacgccttcatcgtgaacggctgcgccgctgatctgagcgtgtgcgccctgtggatgcctcaggaggccgtgctgggcctgctccccaccggctccgccgagcctcctggcggaagctacagactgctcagaggcggcctgctgggcctgggactgaccgtgtctctgctgtcccactgcctggtcgccctcaacagatacctgctgattacaagagctcctgcttatcaagctctgtaccagcggcggcacaccgccggaatgctggctctgtcttgggccctggccctgggcctggtgctgctcctgcctccatgggcccctagacctggcgccgccccacctagagtgcactaccccgccctgctggccgccgccgctttactggcccaaacagcccttcttctgcattgctacctgggtatcgtgcggagagtgagagtgtccgttaagcgggtcagcgtgctgaacttccacctgctgcaccagctgcctggatgtgccgccgctgccaaccccagaagagcccagagacgcctgagcggactgagcgtgctgctgctttgttgcgtgttcctgctggctacacagcctctggtgtgggtgtctctggccagcggcttcagcctgcccgtgccttggggcgtgcaggccgcttcttggctgctgtgctgcgccctgagcgccctgaatcctctgctgtacacctggcggaacgaggagttcagaagaagcgtgcggagcgtgctgccaggcgtgggcgacgccgccgcagccgccgccgccgccacagccgttcccgctgtgggcaccagagccgccggccagcactga

SEQ ID NO: 317 - DNA, 960 bp, synthetic construct
  source 1..960: mol_type = other DNA
atgaccaacagcagcttcttctgccctgtgtacaaggacctggaaccctttacctacttcttctacctggtgttcctggtgggcatcatcggctcttgttttgccacctgggccttcatccagaaaaacaccaaccacagatgtgtgtccatctatcttatcaacctgctgaccgccgatttcctgctgacactggctctgcctgtgaagatcgtggtggacctgggcgtggccccttggaagctgagaatcttccactgccaggtgaccgcctgcctgatctacatcaacatgtacctgagcattatctttctggccttcgtgtccatcgacagatgcctgcagctgacacactcttgcaagatctacagaatccaagagcctggatttgccaagatgatcagcaccgtggtgtggctgatggtcctgctgatcatggtgcctaatatgatgatccccatcaaggacatcaaggagaaacctaacgtgggatgtatggagttcaagaaggagttcggcagaaactggcacctgctcaccaatttcatctgcgtggccatcttcctgaacttcagcgccatcatcctgattagcaactgcctggttatccggcagctgtaccggaacaaggataacgagaactaccccaatgtgaaaaaagctctgattaacatcctgctggtcacagccggctacatcatttgcttcgttccttatcatatcgtgcggatcccatacaccctgagccagaccgaggtgatctctgattgcagcacaagaatcagcctgttcaaggctaaagaggccacactgctgctggccgtgagcaatctgtgcttcgaccccatcctctactaccacctgagcaaggcttttagactgaaggtgaccgaaaccttcgcctctcctaaggaaacaaaggcccagaaggagaagctgaggtgtgaaaacaacgcctga